European Patent Application EP 4 644 548 A1, published November 5, 2025. Title: 会合が制御されたポリペプチド. Applicant: CHUGAI SEIYAKU KABUSHIKI KAISHA. The sequence listing filed with the application follows.

SEQUENCE LISTING (620 sequences)

SEQ ID NO: 1 - protein, 447 aa, Homo sapiens
QVQLQESGPGLVRPSQTLSLTCTVSGYSITSDHAWSWVRQPPGRGLEWIGYISYSGITTYNPSLKSRVTMLRDTSKNQFSLRLSSVTAADTAVYYCARSLARTTAMDYWGQGSLVTVSSASTKGPSVFPLAPSSKSTSGGTAALGCLVKDYFPEPVTVSWNSGALTSGVHTFPAVLQSSGLYSLSSVVTVPSSSLGTQTYICNVNHKPSNTKVDKRVEPKSCDKTHTCPPCPAPELLGGPSVFLFPPKPKDTLMISRTPEVTCVVVDVSHEDPEVKFNWYVDGVEVHNAKTKPREEQYNSTYRVVSVLTVLHQDWLNGKEYKCKVSNKALPAPIEKTISKAKGQPREPQVYTLPPSREEMTKNQVSLTCLVKGFYPSDIAVEWESNGQPENNYKTTPPVLDSDGSFFLYSKLTVDKSRWQQGNVFSCSVMHEALHNHYTQKSLSLSP

SEQ ID NO: 2 - protein, 447 aa, Homo sapiens
QVQLQESGPGLVRPSQTLSLTCTVSGYSITSDHAWSWVRQPPGRGLEWIGYISYSGITTYNPSLKSRVTMLRDTSKNQFSLRLSSVTAADTAVYYCARSLARTTAMDYWGQGSLVTVSSASTKGPSVFPLAPSSKSTSGGTAALGCLVKDYFPEPVTVSWNSGALTSGVHTFPAVLQSSGLYSLSSVVTVPSSSLGTQTYICNVNHKPSNTKVDKRVEPKSCDKTHTCPPCPAPELLGGPSVFLFPPKPKDTLMISRTPEVTCVVVDVSHEDPEVKFNWYVDGVEVHNAKTKPREEQYNSTYRVVSVLTVLHQDWLNGKEYKCKVSNKALPAPIEKTISKAKGQPRKPQVYTLPPSREEMTENQVSLTCLVKGFYPSDIAVEWESNGQPENNYKTTPPVLDSDGSFFLYSKLTVDKSRWQQGNVFSCSVMHEALHNHYTQKSLSLSP

SEQ ID NO: 3 - protein, 447 aa, Homo sapiens
QVQLQESGPGLVRPSQTLSLTCTVSGYSITSDHAWSWVRQPPGRGLEWIGYISYSGITTYNPSLKSRVTMLRDTSKNQFSLRLSSVTAADTAVYYCARSLARTTAMDYWGQGSLVTVSSASTKGPSVFPLAPSSKSTSGGTAALGCLVKDYFPEPVTVSWNSGALTSGVHTFPAVLQSSGLYSLSSVVTVPSSSLGTQTYICNVNHKPSNTKVDKRVEPKSCDKTHTCPPCPAPELLGGPSVFLFPPKPKDTLMISRTPEVTCVVVDVSHEDPEVKFNWYVDGVEVHNAKTKPREEQYNSTYRVVSVLTVLHQDWLNGKEYKCKVSNKALPAPIEKTISKAKGQPRRPQVYTLPPSREEMTENQVSLTCLVKGFYPSDIAVEWESNGQPENNYKTTPPVLDSDGSFFLYSKLTVDKSRWQQGNVFSCSVMHEALHNHYTQKSLSLSP

SEQ ID NO: 4 - protein, 447 aa, Homo sapiens
QVQLQESGPGLVRPSQTLSLTCTVSGYSITSDHAWSWVRQPPGRGLEWIGYISYSGITTYNPSLKSRVTMLRDTSKNQFSLRLSSVTAADTAVYYCARSLARTTAMDYWGQGSLVTVSSASTKGPSVFPLAPSSKSTSGGTAALGCLVKDYFPEPVTVSWNSGALTSGVHTFPAVLQSSGLYSLSSVVTVPSSSLGTQTYICNVNHKPSNTKVDKRVEPKSCDKTHTCPPCPAPELLGGPSVFLFPPKPKDTLMISRTPEVTCVVVDVSHEDPEVKFNWYVDGVEVHNAKTKPREEQYNSTYRVVSVLTVLHQDWLNGKEYKCKVSNKALPAPIEKTISKAKGQPREPQVYTLPPSREKMTKNQVSLTCLVEGFYPSDIAVEWESNGQPENNYKTTPPVLDSDGSFFLYSKLTVDKSRWQQGNVFSCSVMHEALHNHYTQKSLSLSP

SEQ ID NO: 5 - protein, 447 aa, Homo sapiens
QVQLQESGPGLVRPSQTLSLTCTVSGYSITSDHAWSWVRQPPGRGLEWIGYISYSGITTYNPSLKSRVTMLRDTSKNQFSLRLSSVTAADTAVYYCARSLARTTAMDYWGQGSLVTVSSASTKGPSVFPLAPSSKSTSGGTAALGCLVKDYFPEPVTVSWNSGALTSGVHTFPAVLQSSGLYSLSSVVTVPSSSLGTQTYICNVNHKPSNTKVDKRVEPKSCDKTHTCPPCPAPELLGGPSVFLFPPKPKDTLMISRTPEVTCVVVDVSHEDPEVKFNWYVDGVEVHNAKTKPREEQYNSTYRVVSVLTVLHQDWLNGKEYKCKVSNKALPAPIEKTISKAKGQPREPQVYTLPPSREEMTKNQVSLTCLVKGFYPSDIAVEWESNGQPENNYKTTPPVLKSDGSFFLYSELTVDKSRWQQGNVFSCSVMHEALHNHYTQKSLSLSP

SEQ ID NO: 6 - protein, 447 aa, Homo sapiens
QVQLQESGPGLVRPSQTLSLTCTVSGYSITSDHAWSWVRQPPGRGLEWIGYISYSGITTYNPSLKSRVTMLRDTSKNQFSLRLSSVTAADTAVYYCARSLARTTAMDYWGQGSLVTVSSASTKGPSVFPLAPSSKSTSGGTAALGCLVKDYFPEPVTVSWNSGALTSGVHTFPAVLQSSGLYSLSSVVTVPSSSLGTQTYICNVNHKPSNTKVDKRVEPKSCDKTHTCPPCPAPELLGGPSVFLFPPKPKDTLMISRTPEVTCVVVDVSHEDPEVKFNWYVDGVEVHNAKTKPREEQYNSTYRVVSVLTVLHQDWLNGKEYKCKVSNKALPAPIEKTISKAKGQPREPQVYTLPPSREEMTKNQVSLTCLVKGFYPSDIAVEWESNGQPENNYKTTPPVLKSDGSFFLYSDLTVDKSRWQQGNVFSCSVMHEALHNHYTQKSLSLSP

SEQ ID NO: 7 - protein, 447 aa, Homo sapiens
QVQLQESGPGLVRPSQTLSLTCTVSGYSITSDHAWSWVRQPPGRGLEWIGYISYSGITTYNPSLKSRVTMLRDTSKNQFSLRLSSVTAADTAVYYCARSLARTTAMDYWGQGSLVTVSSASTKGPSVFPLAPSSKSTSGGTAALGCLVKDYFPEPVTVSWNSGALTSGVHTFPAVLQSSGLYSLSSVVTVPSSSLGTQTYICNVNHKPSNTKVDKRVEPKSCDKTHTCPPCPAPELLGGPSVFLFPPKPKDTLMISRTPEVTCVVVDVSHEDPEVKFNWYVDGVEVHNAKTKPREEQYNSTYRVVSVLTVLHQDWLNGKEYKCKVSNKALPAPIEKTISKAKGQPREPQVYTLPPSREEMTKNQVSLTCLVKGFYPSDIAVEWESNGQPENNYKTTPPVLRSDGSFFLYSELTVDKSRWQQGNVFSCSVMHEALHNHYTQKSLSLSP

SEQ ID NO: 8 - protein, 447 aa, Homo sapiens
QVQLQESGPGLVRPSQTLSLTCTVSGYSITSDHAWSWVRQPPGRGLEWIGYISYSGITTYNPSLKSRVTMLRDTSKNQFSLRLSSVTAADTAVYYCARSLARTTAMDYWGQGSLVTVSSASTKGPSVFPLAPSSKSTSGGTAALGCLVKDYFPEPVTVSWNSGALTSGVHTFPAVLQSSGLYSLSSVVTVPSSSLGTQTYICNVNHKPSNTKVDKRVEPKSCDKTHTCPPCPAPELLGGPSVFLFPPKPKDTLMISRTPEVTCVVVDVSHEDPEVKFNWYVDGVEVHNAKTKPREEQYNSTYRVVSVLTVLHQDWLNGKEYKCKVSNKALPAPIEKTISKAKGQPREPQVYTLPPSREEMTKNQVSLTCLVKGFYPSDIAVEWESNGQPENNYKTTPPVLRSDGSFFLYSDLTVDKSRWQQGNVFSCSVMHEALHNHYTQKSLSLSP

SEQ ID NO: 9 - protein, 447 aa, Homo sapiens
QVQLQESGPGLVRPSQTLSLTCTVSGYSITSDHAWSWVRQPPGRGLEWIGYISYSGITTYNPSLKSRVTMLRDTSKNQFSLRLSSVTAADTAVYYCARSLARTTAMDYWGQGSLVTVSSASTKGPSVFPLAPSSKSTSGGTAALGCLVKDYFPEPVTVSWNSGALTSGVHTFPAVLQSSGLYSLSSVVTVPSSSLGTQTYICNVNHKPSNTKVDKRVEPKSCDKTHTCPPCPAPELLGGPSVFLFPPKPKDTLMISRTPEVTCVVVDVSHEDPEVKFNWYVDGVEVHNAKTKPREEQYNSTYRVVSVLTVLHQDWLNGKEYKCKVSNKALPAPIEKTISKAKGQPREPQVYTLPPSREEMTKNQVSLTCLVKGFYPSDIAVEWESNGQPENNYETTPPVLKSDGSFFLYSKLTVDKSRWQQGNVFSCSVMHEALHNHYTQKSLSLSP

SEQ ID NO: 10 - protein, 447 aa, Homo sapiens
QVQLQESGPGLVRPSQTLSLTCTVSGYSITSDHAWSWVRQPPGRGLEWIGYISYSGITTYNPSLKSRVTMLRDTSKNQFSLRLSSVTAADTAVYYCARSLARTTAMDYWGQGSLVTVSSASTKGPSVFPLAPSSKSTSGGTAALGCLVKDYFPEPVTVSWNSGALTSGVHTFPAVLQSSGLYSLSSVVTVPSSSLGTQTYICNVNHKPSNTKVDKRVEPKSCDKTHTCPPCPAPELLGGPSVFLFPPKPKDTLMISRTPEVTCVVVDVSHEDPEVKFNWYVDGVEVHNAKTKPREEQYNSTYRVVSVLTVLHQDWLNGKEYKCKVSNKALPAPIEKTISKAKGQPREPQVYTLPPSREEMTKNQVSLTCLVKGFYPSDIAVEWESNGQPENNYDTTPPVLKSDGSFFLYSKLTVDKSRWQQGNVFSCSVMHEALHNHYTQKSLSLSP

SEQ ID NO: 11 - protein, 447 aa, Homo sapiens
QVQLQESGPGLVRPSQTLSLTCTVSGYSITSDHAWSWVRQPPGRGLEWIGYISYSGITTYNPSLKSRVTMLRDTSKNQFSLRLSSVTAADTAVYYCARSLARTTAMDYWGQGSLVTVSSASTKGPSVFPLAPSSKSTSGGTAALGCLVKDYFPEPVTVSWNSGALTSGVHTFPAVLQSSGLYSLSSVVTVPSSSLGTQTYICNVNHKPSNTKVDKRVEPKSCDKTHTCPPCPAPELLGGPSVFLFPPKPKDTLMISRTPEVTCVVVDVSHEDPEVKFNWYVDGVEVHNAKTKPREEQYNSTYRVVSVLTVLHQDWLNGKEYKCKVSNKALPAPIEKTISKAKGQPREPQVYTLPPSREEMTKNQVSLTCLVKGFYPSDIAVEWESNGQPENNYETTPPVLRSDGSFFLYSKLTVDKSRWQQGNVFSCSVMHEALHNHYTQKSLSLSP

SEQ ID NO: 12 - protein, 447 aa, Homo sapiens
QVQLQESGPGLVRPSQTLSLTCTVSGYSITSDHAWSWVRQPPGRGLEWIGYISYSGITTYNPSLKSRVTMLRDTSKNQFSLRLSSVTAADTAVYYCARSLARTTAMDYWGQGSLVTVSSASTKGPSVFPLAPSSKSTSGGTAALGCLVKDYFPEPVTVSWNSGALTSGVHTFPAVLQSSGLYSLSSVVTVPSSSLGTQTYICNVNHKPSNTKVDKRVEPKSCDKTHTCPPCPAPELLGGPSVFLFPPKPKDTLMISRTPEVTCVVVDVSHEDPEVKFNWYVDGVEVHNAKTKPREEQYNSTYRVVSVLTVLHQDWLNGKEYKCKVSNKALPAPIEKTISKAKGQPREPQVYTLPPSREEMTKNQVSLTCLVKGFYPSDIAVEWESNGQPENNYDTTPPVLRSDGSFFLYSKLTVDKSRWQQGNVFSCSVMHEALHNHYTQKSLSLSP

SEQ ID NO: 13 - protein, 447 aa, Homo sapiens
QVQLQESGPGLVRPSQTLSLTCTVSGYSITSDHAWSWVRQPPGRGLEWIGYISYSGITTYNPSLKSRVTMLRDTSKNQFSLRLSSVTAADTAVYYCARSLARTTAMDYWGQGSLVTVSSASTKGPSVFPLAPSSKSTSGGTAALGCLVKDYFPEPVTVSWNSGALTSGVHTFPAVLQSSGLYSLSSVVTVPSSSLGTQTYICNVNHKPSNTKVDKRVEPKSCDKTHTCPPCPAPELLGGPSVFLFPPKPKDTLMISRTPEVTCVVVDVSHEDPEVKFNWYVDGVEVHNAKTKPREEQYNSTYRVVSVLTVLHQDWLNGKEYKCKVSNKALPAPIEKTISKAKGQPREPQVYTLPPSREEMTKNQVSLTCLVKGFYPSDIAVEWESNGQPENNYCTTPPVLCSDGSFFLYSKLTVDKSRWQQGNVFSCSVMHEALHNHYTQKSLSLSP

SEQ ID NO: 14 - protein, 447 aa, Homo sapiens
QVQLQESGPGLVRPSQTLSLTCTVSGYSITSDHAWSWVRQPPGRGLEWIGYISYSGITTYNPSLKSRVTMLRDTSKNQFSLRLSSVTAADTAVYYCARSLARTTAMDYWGQGSLVTVSSASTKGPSVFPLAPSSKSTSGGTAALGCLVKDYFPEPVTVSWNSGALTSGVHTFPAVLQSSGLYSLSSVVTVPSSSLGTQTYICNVNHKPSNTKVDKRVEPKSCDKTHTCPPCPAPELLGGPSVFLFPPKPKDTLMISRTPEVTCVVVDVSHEDPEVKFNWYVDGVEVHNAKTKPREEQYNSTYRVVSVLTVLHQDWLNGKEYKCKVSNKALPAPIEKTISKAKGQPREPQVCTLPPCREEMTKNQVSLTCLVKGFYPSDIAVEWESNGQPENNYKTTPPVLDSDGSFFLYSKLTVDKSRWQQGNVFSCSVMHEALHNHYTQKSLSLSP

SEQ ID NO: 15 - protein, 447 aa, Homo sapiens
QVQLQESGPGLVRPSQTLSLTCTVSGYSITSDHAWSWVRQPPGRGLEWIGYISYSGITTYNPSLKSRVTMLRDTSKNQFSLRLSSVTAADTAVYYCARSLARTTAMDYWGQGSLVTVSSASTKGPSVFPLAPSSKSTSGGTAALGCLVKDYFPEPVTVSWNSGALTSGVHTFPAVLQSSGLYSLSSVVTVPSSSLGTQTYICNVNHKPSNTKVDKRVEPKSCDKTHTCPPCPAPELLGGPSVFLFPPKPKDTLMISRTPEVTCVVVDVSHEDPEVKFNWYVDGVEVHNAKTKPREEQYNSTYRVVSVLTVLHQDWLNGKEYKCKVSNKALPAPIEKTISKAKGQPREPQVCTLPPSRCEMTKNQVSLTCLVKGFYPSDIAVEWESNGQPENNYKTTPPVLDSDGSFFLYSKLTVDKSRWQQGNVFSCSVMHEALHNHYTQKSLSLSP

SEQ ID NO: 16 - protein, 447 aa, Homo sapiens
QVQLQESGPGLVRPSQTLSLTCTVSGYSITSDHAWSWVRQPPGRGLEWIGYISYSGITTYNPSLKSRVTMLRDTSKNQFSLRLSSVTAADTAVYYCARSLARTTAMDYWGQGSLVTVSSASTKGPSVFPLAPSSKSTSGGTAALGCLVKDYFPEPVTVSWNSGALTSGVHTFPAVLQSSGLYSLSSVVTVPSSSLGTQTYICNVNHKPSNTKVDKRVEPKSCDKTHTCPPCPAPELLGGPSVFLFPPKPKDTLMISRTPEVTCVVVDVSHEDPEVKFNWYVDGVEVHNAKTKPREEQYNSTYRVVSVLTVLHQDWLNGKEYKCKVSNKALPAPIEKTISKAKGQPREPQVCTLPPSRECMTKNQVSLTCLVKGFYPSDIAVEWESNGQPENNYKTTPPVLDSDGSFFLYSKLTVDKSRWQQGNVFSCSVMHEALHNHYTQKSLSLSP

SEQ ID NO: 17 - protein, 447 aa, Homo sapiens
QVQLQESGPGLVRPSQTLSLTCTVSGYSITSDHAWSWVRQPPGRGLEWIGYISYSGITTYNPSLKSRVTMLRDTSKNQFSLRLSSVTAADTAVYYCARSLARTTAMDYWGQGSLVTVSSASTKGPSVFPLAPSSKSTSGGTAALGCLVKDYFPEPVTVSWNSGALTSGVHTFPAVLQSSGLYSLSSVVTVPSSSLGTQTYICNVNHKPSNTKVDKRVEPKSCDKTHTCPPCPAPELLGGPSVFLFPPKPKDTLMISRTPEVTCVVVDVSHEDPEVKFNWYVDGVEVHNAKTKPREEQYNSTYRVVSVLTVLHQDWLNGKEYKCKVSNKALPAPIEKTISKAKGQPREPQVYTCPPCREEMTKNQVSLTCLVKGFYPSDIAVEWESNGQPENNYKTTPPVLDSDGSFFLYSKLTVDKSRWQQGNVFSCSVMHEALHNHYTQKSLSLSP

SEQ ID NO: 18 - protein, 447 aa, Homo sapiens
QVQLQESGPGLVRPSQTLSLTCTVSGYSITSDHAWSWVRQPPGRGLEWIGYISYSGITTYNPSLKSRVTMLRDTSKNQFSLRLSSVTAADTAVYYCARSLARTTAMDYWGQGSLVTVSSASTKGPSVFPLAPSSKSTSGGTAALGCLVKDYFPEPVTVSWNSGALTSGVHTFPAVLQSSGLYSLSSVVTVPSSSLGTQTYICNVNHKPSNTKVDKRVEPKSCDKTHTCPPCPAPELLGGPSVFLFPPKPKDTLMISRTPEVTCVVVDVSHEDPEVKFNWYVDGVEVHNAKTKPREEQYNSTYRVVSVLTVLHQDWLNGKEYKCKVSNKALPAPIEKTISKAKGQPREPQVYTLPPSREEMTKNQVSLTCLVKGFYPSDIAVEWESNGQPENNYKTCPPCLDSDGSFFLYSKLTVDKSRWQQGNVFSCSVMHEALHNHYTQKSLSLSP

SEQ ID NO: 19 - protein, 447 aa, Homo sapiens
QVQLQESGPGLVRPSQTLSLTCTVSGYSITSDHAWSWVRQPPGRGLEWIGYISYSGITTYNPSLKSRVTMLRDTSKNQFSLRLSSVTAADTAVYYCARSLARTTAMDYWGQGSLVTVSSASTKGPSVFPLAPSSKSTSGGTAALGCLVKDYFPEPVTVSWNSGALTSGVHTFPAVLQSSGLYSLSSVVTVPSSSLGTQTYICNVNHKPSNTKVDKRVEPKSCDKTHTCPPCPAPELLGGPSVFLFPPKPKDTLMISRTPEVTCVVVDVSHEDPEVKFNWYVDGVEVHNAKTKPREEQYNSTYRVVSVLTVLHQDWLNGKEYKCKVSNKALPAPIEKTISKAKGQPREPQVYTLPPSREEMTKNQVSLTCLVKGFYPSDIAVEWESNGQPENNYKTWPPVLDSDGSFALYSKLTVDKSRWQQGNVFSCSVMHEALHNHYTQKSLSLSP

SEQ ID NO: 20 - protein, 447 aa, Homo sapiens
QVQLQESGPGLVRPSQTLSLTCTVSGYSITSDHAWSWVRQPPGRGLEWIGYISYSGITTYNPSLKSRVTMLRDTSKNQFSLRLSSVTAADTAVYYCARSLARTTAMDYWGQGSLVTVSSASTKGPSVFPLAPSSKSTSGGTAALGCLVKDYFPEPVTVSWNSGALTSGVHTFPAVLQSSGLYSLSSVVTVPSSSLGTQTYICNVNHKPSNTKVDKRVEPKSCDKTHTCPPCPAPELLGGPSVFLFPPKPKDTLMISRTPEVTCVVVDVSHEDPEVKFNWYVDGVEVHNAKTKPREEQYNSTYRVVSVLTVLHQDWLNGKEYKCKVSNKALPAPIEKTISKAKGQPREPQVYTDPPSREEMTKNQVSLKCLVKGFYPSDIAVEWESNGQPENNYKTTPPVLDSDGSFFLYSKLTVDKSRWQQGNVFSCSVMHEALHNHYTQKSLSLSP

SEQ ID NO: 21 - protein, 447 aa, Homo sapiens
QVQLQESGPGLVRPSQTLSLTCTVSGYSITSDHAWSWVRQPPGRGLEWIGYISYSGITTYNPSLKSRVTMLRDTSKNQFSLRLSSVTAADTAVYYCARSLARTTAMDYWGQGSLVTVSSASTKGPSVFPLAPSSKSTSGGTAALGCLVKDYFPEPVTVSWNSGALTSGVHTFPAVLQSSGLYSLSSVVTVPSSSLGTQTYICNVNHKPSNTKVDKRVEPKSCDKTHTCPPCPAPELLGGPSVFLFPPKPKDTLMISRTPEVTCVVVDVSHEDPEVKFNWYVDGVEVHNAKTKPREEQYNSTYRVVSVLTVLHQDWLNGKEYKCKVSNKALPAPIEKTISKAKGQPREPQVYTEPPSREEMTKNQVSLKCLVKGFYPSDIAVEWESNGQPENNYKTTPPVLDSDGSFFLYSKLTVDKSRWQQGNVFSCSVMHEALHNHYTQKSLSLSP

SEQ ID NO: 22 - protein, 447 aa, Homo sapiens
QVQLQESGPGLVRPSQTLSLTCTVSGYSITSDHAWSWVRQPPGRGLEWIGYISYSGITTYNPSLKSRVTMLRDTSKNQFSLRLSSVTAADTAVYYCARSLARTTAMDYWGQGSLVTVSSASTKGPSVFPLAPSSKSTSGGTAALGCLVKDYFPEPVTVSWNSGALTSGVHTFPAVLQSSGLYSLSSVVTVPSSSLGTQTYICNVNHKPSNTKVDKRVEPKSCDKTHTCPPCPAPELLGGPSVFLFPPKPKDTLMISRTPEVTCVVVDVSHEDPEVKFNWYVDGVEVHNAKTKPREEQYNSTYRVVSVLTVLHQDWLNGKEYKCKVSNKALPAPIEKTISKAKGQPREPQVYTKPPSREEMTKNQVSLDCLVKGFYPSDIAVEWESNGQPENNYKTTPPVLDSDGSFFLYSKLTVDKSRWQQGNVFSCSVMHEALHNHYTQKSLSLSP

SEQ ID NO: 23 - protein, 447 aa, Homo sapiens
QVQLQESGPGLVRPSQTLSLTCTVSGYSITSDHAWSWVRQPPGRGLEWIGYISYSGITTYNPSLKSRVTMLRDTSKNQFSLRLSSVTAADTAVYYCARSLARTTAMDYWGQGSLVTVSSASTKGPSVFPLAPSSKSTSGGTAALGCLVKDYFPEPVTVSWNSGALTSGVHTFPAVLQSSGLYSLSSVVTVPSSSLGTQTYICNVNHKPSNTKVDKRVEPKSCDKTHTCPPCPAPELLGGPSVFLFPPKPKDTLMISRTPEVTCVVVDVSHEDPEVKFNWYVDGVEVHNAKTKPREEQYNSTYRVVSVLTVLHQDWLNGKEYKCKVSNKALPAPIEKTISKAKGQPREPQVYTKPPSREEMTKNQVSLECLVKGFYPSDIAVEWESNGQPENNYKTTPPVLDSDGSFFLYSKLTVDKSRWQQGNVFSCSVMHEALHNHYTQKSLSLSP

SEQ ID NO: 24 - protein, 447 aa, Homo sapiens
QVQLQESGPGLVRPSQTLSLTCTVSGYSITSDHAWSWVRQPPGRGLEWIGYISYSGITTYNPSLKSRVTMLRDTSKNQFSLRLSSVTAADTAVYYCARSLARTTAMDYWGQGSLVTVSSASTKGPSVFPLAPSSKSTSGGTAALGCLVKDYFPEPVTVSWNSGALTSGVHTFPAVLQSSGLYSLSSVVTVPSSSLGTQTYICNVNHKPSNTKVDKRVEPKSCDKTHTCPPCPAPELLGGPSVFLFPPKPKDTLMISRTPEVTCVVVDVSHEDPEVKFNWYVDGVEVHNAKTKPREEQYNSTYRVVSVLTVLHQDWLNGKEYKCKVSNKALPAPIEKTISKAKGQPREPQVYTLPPSREEMTKNQVSLTCLVKGFYPSDIAVEWESNGQPENNYKTTPPVLDSDGSFLLYSRLTVDKSRWQQGNVFSCSVMHEALHNHYTQKSLSLSP

SEQ ID NO: 25 - protein, 447 aa, Homo sapiens
QVQLQESGPGLVRPSQTLSLTCTVSGYSITSDHAWSWVRQPPGRGLEWIGYISYSGITTYNPSLKSRVTMLRDTSKNQFSLRLSSVTAADTAVYYCARSLARTTAMDYWGQGSLVTVSSASTKGPSVFPLAPSSKSTSGGTAALGCLVKDYFPEPVTVSWNSGALTSGVHTFPAVLQSSGLYSLSSVVTVPSSSLGTQTYICNVNHKPSNTKVDKRVEPKSCDKTHTCPPCPAPELLGGPSVFLFPPKPKDTLMISRTPEVTCVVVDVSHEDPEVKFNWYVDGVEVHNAKTKPREEQYNSTYRVVSVLTVLHQDWLNGKEYKCKVSNKALPAPIEKTISKAKGQPREPQVYTLPPSRKEMTKNQVSLTCLVKGFYPSDIAVEWESNGQPENNYKTTPPVLDSDGSFFLYSKLTVDKSRWQQGNVFSCSVMHEALHNHYTQESLSLSP

SEQ ID NO: 26 - protein, 447 aa, Homo sapiens
QVQLQESGPGLVRPSQTLSLTCTVSGYSITSDHAWSWVRQPPGRGLEWIGYISYSGITTYNPSLKSRVTMLRDTSKNQFSLRLSSVTAADTAVYYCARSLARTTAMDYWGQGSLVTVSSASTKGPSVFPLAPSSKSTSGGTAALGCLVKDYFPEPVTVSWNSGALTSGVHTFPAVLQSSGLYSLSSVVTVPSSSLGTQTYICNVNHKPSNTKVDKRVEPKSCDKTHTCPPCPAPELLGGPSVFLFPPKPKDTLMISRTPEVTCVVVDVSHEDPEVKFNWYVDGVEVHNAKTKPREEQYNSTYRVVSVLTVLHQDWLNGKEYKCKVSNKALPAPIEKTISKAKGQPREPQVYTLPPSREEMTKNQVSLWCAVKGFYPSDIAVEWESNGQPENNYKTTPPVLDSDGSFFLVSKLTVDKSRWQQGNVFSCSVMHEALHNHYTQKSLSLSP

SEQ ID NO: 27 - protein, 447 aa, Homo sapiens
QVQLQESGPGLVRPSQTLSLTCTVSGYSITSDHAWSWVRQPPGRGLEWIGYISYSGITTYNPSLKSRVTMLRDTSKNQFSLRLSSVTAADTAVYYCARSLARTTAMDYWGQGSLVTVSSASTKGPSVFPLAPSSKSTSGGTAALGCLVKDYFPEPVTVSWNSGALTSGVHTFPAVLQSSGLYSLSSVVTVPSSSLGTQTYICNVNHKPSNTKVDKRVEPKSCDKTHTCPPCPAPELLGGPSVFLFPPKPKDTLMISRTPEVTCVVVDVSHEDPEVKFNWYVDGVEVHNAKTKPREEQYNSTYRVVSVLTVLHQDWLNGKEYKCKVSNKALPAPIEKTISKAKGQPREPQVYTLPPSREEMTKNQVSLYCLVKGFYPSDIAVEWESNGQPENNYKTTPPVLDSDGSFFLTSKLTVDKSRWQQGNVFSCSVMHEALHNHYTQKSLSLSP

SEQ ID NO: 28 - protein, 447 aa, Homo sapiens
QVQLQESGPGLVRPSQTLSLTCTVSGYSITSDHAWSWVRQPPGRGLEWIGYISYSGITTYNPSLKSRVTMLRDTSKNQFSLRLSSVTAADTAVYYCARSLARTTAMDYWGQGSLVTVSSASTKGPSVFPLAPSSKSTSGGTAALGCLVKDYFPEPVTVSWNSGALTSGVHTFPAVLQSSGLYSLSSVVTVPSSSLGTQTYICNVNHKPSNTKVDKRVEPKSCDKTHTCPPCPAPELLGGPSVFLFPPKPKDTLMISRTPEVTCVVVDVSHEDPEVKFNWYVDGVEVHNAKTKPREEQYNSTYRVVSVLTVLHQDWLNGKEYKCKVSNKALPAPIEKTISKAKGQPREPQVYTLPPSREEMTKNQVSLWCLVKGFYPSDIAVEWESNGQPENNYKTTPPVLDSDGSFFLASKLTVDKSRWQQGNVFSCSVMHEALHNHYTQKSLSLSP

SEQ ID NO: 29 - protein, 447 aa, Homo sapiens
QVQLQESGPGLVRPSQTLSLTCTVSGYSITSDHAWSWVRQPPGRGLEWIGYISYSGITTYNPSLKSRVTMLRDTSKNQFSLRLSSVTAADTAVYYCARSLARTTAMDYWGQGSLVTVSSASTKGPSVFPLAPSSKSTSGGTAALGCLVKDYFPEPVTVSWNSGALTSGVHTFPAVLQSSGLYSLSSVVTVPSSSLGTQTYICNVNHKPSNTKVDKRVEPKSCDKTHTCPPCPAPELLGGPSVFLFPPKPKDTLMISRTPEVTCVVVDVSHEDPEVKFNWYVDGVEVHNAKTKPREEQYNSTYRVVSVLTVLHQDWLNGKEYKCKVSNKALPAPIEKTISKAKGQPREPQVYTLPPSREEMTKNQVSLYCLVKGFYPSDIAVEWESNGQPENNYKTWPPVLDSDGSFALTSKLTVDKSRWQQGNVFSCSVMHEALHNHYTQKSLSLSP

SEQ ID NO: 30 - protein, 447 aa, Homo sapiens
QVQLQESGPGLVRPSQTLSLTCTVSGYSITSDHAWSWVRQPPGRGLEWIGYISYSGITTYNPSLKSRVTMLRDTSKNQFSLRLSSVTAADTAVYYCARSLARTTAMDYWGQGSLVTVSSASTKGPSVFPLAPSSKSTSGGTAALGCLVKDYFPEPVTVSWNSGALTSGVHTFPAVLQSSGLYSLSSVVTVPSSSLGTQTYICNVNHKPSNTKVDKRVEPKSCDKTHTCPPCPAPELLGGPSVFLFPPKPKDTLMISRTPEVTCVVVDVSHEDPEVKFNWYVDGVEVHNAKTKPREEQYNSTYRVVSVLTVLHQDWLNGKEYKCKVSNKALPAPIEKTISKAKGQPREPQVYTLPPSRENMTKNQVSLTCLVEGFYPSDIAVEWESNGQPENNYKTTPPVLVSDGSFTLYSWLTVDKSRWQQGNVFSCSVMHEALHNHYTQKSLSLSP

SEQ ID NO: 31 - protein, 447 aa, Homo sapiens
QVQLQESGPGLVRPSQTLSLTCTVSGYSITSDHAWSWVRQPPGRGLEWIGYISYSGITTYNPSLKSRVTMLRDTSKNQFSLRLSSVTAADTAVYYCARSLARTTAMDYWGQGSLVTVSSASTKGPSVFPLAPSSKSTSGGTAALGCLVKDYFPEPVTVSWNSGALTSGVHTFPAVLQSSGLYSLSSVVTVPSSSLGTQTYICNVNHKPSNTKVDKRVEPKSCDKTHTCPPCPAPELLGGPSVFLFPPKPKDTLMISRTPEVTCVVVDVSHEDPEVKFNWYVDGVEVHNAKTKPREEQYNSTYRVVSVLTVLHQDWLNGKEYKCKVSNKALPAPIEKTISKAKGQPREPRVYTLPPSREEMTENQVSLTCLVKGFYPSDIAVEWESNGQPENNYKTTPPVLVSDGSFTLYSWLTVDKSRWQQGNVFSCSVMHEALHNHYTQKSLSLSP

SEQ ID NO: 32 - protein, 447 aa, Homo sapiens
QVQLQESGPGLVRPSQTLSLTCTVSGYSITSDHAWSWVRQPPGRGLEWIGYISYSGITTYNPSLKSRVTMLRDTSKNQFSLRLSSVTAADTAVYYCARSLARTTAMDYWGQGSLVTVSSASTKGPSVFPLAPSSKSTSGGTAALGCLVKDYFPEPVTVSWNSGALTSGVHTFPAVLQSSGLYSLSSVVTVPSSSLGTQTYICNVNHKPSNTKVDKRVEPKSCDKTHTCPPCPAPELLGGPSVFLFPPKPKDTLMISRTPEVTCVVVDVSHEDPEVKFNWYVDGVEVHNAKTKPREEQYNSTYRVVSVLTVLHQDWLNGKEYKCKVSNKALPAPIEKTISKAKGQPREPQVTTLPPSREEMTKNQVHLTCLVKGFYPSDIAVEWESNGQPENNYKTFPPVLDSDGSFALYSKLTVDKSRWQQGNVFSCSVMHEALHNHYTQKSLSLSP

SEQ ID NO: 33 - protein, 447 aa, Homo sapiens
QVQLQESGPGLVRPSQTLSLTCTVSGYSITSDHAWSWVRQPPGRGLEWIGYISYSGITTYNPSLKSRVTMLRDTSKNQFSLRLSSVTAADTAVYYCARSLARTTAMDYWGQGSLVTVSSASTKGPSVFPLAPSSKSTSGGTAALGCLVKDYFPEPVTVSWNSGALTSGVHTFPAVLQSSGLYSLSSVVTVPSSSLGTQTYICNVNHKPSNTKVDKRVEPKSCDKTHTCPPCPAPELLGGPSVFLFPPKPKDTLMISRTPEVTCVVVDVSHEDPEVKFNWYVDGVEVHNAKTKPREEQYNSTYRVVSVLTVLHQDWLNGKEYKCKVSNKALPAPIEKTISKAKGQPREPQVTTLPPSREEMTKNQVHLTCLVKGFYPSDIAVEWESNGQPENNYKTTPPVLDSDGSFFLYSKLTVDKSRWQQGNVFSCSVMHEALHNHYTQKSLSLSP

SEQ ID NO: 34 - protein, 447 aa, Homo sapiens
QVQLQESGPGLVRPSQTLSLTCTVSGYSITSDHAWSWVRQPPGRGLEWIGYISYSGITTYNPSLKSRVTMLRDTSKNQFSLRLSSVTAADTAVYYCARSLARTTAMDYWGQGSLVTVSSASTKGPSVFPLAPSSKSTSGGTAALGCLVKDYFPEPVTVSWNSGALTSGVHTFPAVLQSSGLYSLSSVVTVPSSSLGTQTYICNVNHKPSNTKVDKRVEPKSCDKTHTCPPCPAPELLGGPSVFLFPPKPKDTLMISRTPEVTCVVVDVSHEDPEVKFNWYVDGVEVHNAKTKPREEQYNSTYRVVSVLTVLHQDWLNGKEYKCKVSNKALPAPIEKTISKAKGQPREPQVYTLPPSREEMTKNQVSLTCLVKGFYPSDIAVEWESNGQPENNYKTFPPVLDSDGSFALYSKLTVDKSRWQQGNVFSCSVMHEALHNHYTQKSLSLSP

SEQ ID NO: 35 - protein, 447 aa, Homo sapiens
QVQLQESGPGLVRPSQTLSLTCTVSGYSITSDHAWSWVRQPPGRGLEWIGYISYSGITTYNPSLKSRVTMLRDTSKNQFSLRLSSVTAADTAVYYCARSLARTTAMDYWGQGSLVTVSSASTKGPSVFPLAPSSKSTSGGTAALGCLVKDYFPEPVTVSWNSGALTSGVHTFPAVLQSSGLYSLSSVVTVPSSSLGTQTYICNVNHKPSNTKVDKRVEPKSCDKTHTCPPCPAPELLGGPSVFLFPPKPKDTLMISRTPEVTCVVVDVSHEDPEVKFNWYVDGVEVHNAKTKPREEQYNSTYRVVSVLTVLHQDWLNGKEYKCKVSNKALPAPIEKTISKAKGQPREPQVYTLPPSREKMTKNQVSLTCLVEGFYPSDIAVEWESNGQPENNYKTTPPVLKSDGSFFLYSELTVDKSRWQQGNVFSCSVMHEALHNHYTQKSLSLSP

SEQ ID NO: 36 - protein, 447 aa, Homo sapiens
QVQLQESGPGLVRPSQTLSLTCTVSGYSITSDHAWSWVRQPPGRGLEWIGYISYSGITTYNPSLKSRVTMLRDTSKNQFSLRLSSVTAADTAVYYCARSLARTTAMDYWGQGSLVTVSSASTKGPSVFPLAPSSKSTSGGTAALGCLVKDYFPEPVTVSWNSGALTSGVHTFPAVLQSSGLYSLSSVVTVPSSSLGTQTYICNVNHKPSNTKVDKRVEPKSCDKTHTCPPCPAPELLGGPSVFLFPPKPKDTLMISRTPEVTCVVVDVSHEDPEVKFNWYVDGVEVHNAKTKPREEQYNSTYRVVSVLTVLHQDWLNGKEYKCKVSNKALPAPIEKTISKAKGQPREPQVYTLPPSRKEMTKNQVSLTCLVKGFYPSDIAVEWESNGQPENNYKTTPPVLKSDGSFFLYSELTVDKSRWQQGNVFSCSVMHEALHNHYTQESLSLSP

SEQ ID NO: 37 - protein, 447 aa, Homo sapiens
QVQLQESGPGLVRPSQTLSLTCTVSGYSITSDHAWSWVRQPPGRGLEWIGYISYSGITTYNPSLKSRVTMLRDTSKNQFSLRLSSVTAADTAVYYCARSLARTTAMDYWGQGSLVTVSSASTKGPSVFPLAPSSKSTSGGTAALGCLVKDYFPEPVTVSWNSGALTSGVHTFPAVLQSSGLYSLSSVVTVPSSSLGTQTYICNVNHKPSNTKVDKRVEPKSCDKTHTCPPCPAPELLGGPSVFLFPPKPKDTLMISRTPEVTCVVVDVSHEDPEVKFNWYVDGVEVHNAKTKPREEQYNSTYRVVSVLTVLHQDWLNGKEYKCKVSNKALPAPIEKTISKAKGQPREPQVYTLPPSRKKMTKNQVSLTCLVEGFYPSDIAVEWESNGQPENNYKTTPPVLDSDGSFFLYSKLTVDKSRWQQGNVFSCSVMHEALHNHYTQESLSLSP

SEQ ID NO: 38 - protein, 447 aa, Homo sapiens
QVQLQESGPGLVRPSQTLSLTCTVSGYSITSDHAWSWVRQPPGRGLEWIGYISYSGITTYNPSLKSRVTMLRDTSKNQFSLRLSSVTAADTAVYYCARSLARTTAMDYWGQGSLVTVSSASTKGPSVFPLAPSSKSTSGGTAALGCLVKDYFPEPVTVSWNSGALTSGVHTFPAVLQSSGLYSLSSVVTVPSSSLGTQTYICNVNHKPSNTKVDKRVEPKSCDKTHTCPPCPAPELLGGPSVFLFPPKPKDTLMISRTPEVTCVVVDVSHEDPEVKFNWYVDGVEVHNAKTKPREEQYNSTYRVVSVLTVLHQDWLNGKEYKCKVSNKALPAPIEKTISKAKGQPREPQVYTLPPSRKKMTKNQVSLTCLVEGFYPSDIAVEWESNGQPENNYKTTPPVLKSDGSFFLYSELTVDKSRWQQGNVFSCSVMHEALHNHYTQESLSLSP

SEQ ID NO: 39 - protein, 447 aa, Homo sapiens
QVQLQESGPGLVRPSQTLSLTCTVSGYSITSDHAWSWVRQPPGRGLEWIGYISYSGITTYNPSLKSRVTMLRDTSKNQFSLRLSSVTAADTAVYYCARSLARTTAMDYWGQGSLVTVSSASTKGPSVFPLAPSSKSTSGGTAALGCLVKDYFPEPVTVSWNSGALTSGVHTFPAVLQSSGLYSLSSVVTVPSSSLGTQTYICNVNHKPSNTKVDKRVEPKSCDKTHTCPPCPAPELLGGPSVFLFPPKPKDTLMISRTPEVTCVVVDVSHEDPEVKFNWYVDGVEVHNAKTKPREEQYNSTYRVVSVLTVLHQDWLNGKEYKCKVSNKALPAPIEKTISKAKGQPREPEVYTLPPYREEMTKNQVSLYCLVKGFYPSDIAVEWESNGQPENNYKTTPPVLDSDGSFFLTSKLTVDKSRWQQGNVFSCSVMHEALHNHYTQKSLSLSP

SEQ ID NO: 40 - protein, 447 aa, Homo sapiens
QVQLQESGPGLVRPSQTLSLTCTVSGYSITSDHAWSWVRQPPGRGLEWIGYISYSGITTYNPSLKSRVTMLRDTSKNQFSLRLSSVTAADTAVYYCARSLARTTAMDYWGQGSLVTVSSASTKGPSVFPLAPSSKSTSGGTAALGCLVKDYFPEPVTVSWNSGALTSGVHTFPAVLQSSGLYSLSSVVTVPSSSLGTQTYICNVNHKPSNTKVDKRVEPKSCDKTHTCPPCPAPELLGGPSVFLFPPKPKDTLMISRTPEVTCVVVDVSHEDPEVKFNWYVDGVEVHNAKTKPREEQYNSTYRVVSVLTVLHQDWLNGKEYKCKVSNKALPAPIEKTISKAKGQPREPQVYVYPPSREEMTKNQVSLLCLVKGFYPSDIAVEWESNGQPENNYKTWPPVLDSDGSFALYSKLTVDKSRWQQGNVFSCSVMHEALHNHYTQKSLSLSP

SEQ ID NO: 41 - protein, 447 aa, Homo sapiens
QVQLQESGPGLVRPSQTLSLTCTVSGYSITSDHAWSWVRQPPGRGLEWIGYISYSGITTYNPSLKSRVTMLRDTSKNQFSLRLSSVTAADTAVYYCARSLARTTAMDYWGQGSLVTVSSASTKGPSVFPLAPSSKSTSGGTAALGCLVKDYFPEPVTVSWNSGALTSGVHTFPAVLQSSGLYSLSSVVTVPSSSLGTQTYICNVNHKPSNTKVDKRVEPKSCDKTHTCPPCPAPELLGGPSVFLFPPKPKDTLMISRTPEVTCVVVDVSHEDPEVKFNWYVDGVEVHNAKTKPREEQYNSTYRVVSVLTVLHQDWLNGKEYKCKVSNKALPAPIEKTISKAKGQPREPQVYTLPPSREEMTKNQVSLTCLVKGFYPSDIAVEWESNGQPENNYLTWPPVLDSDGSFALVSKLTVDKSRWQQGNVFSCSVMHEALHNHYTQKSLSLSP

SEQ ID NO: 42 - protein, 447 aa, Homo sapiens
QVQLQESGPGLVRPSQTLSLTCTVSGYSITSDHAWSWVRQPPGRGLEWIGYISYSGITTYNPSLKSRVTMLRDTSKNQFSLRLSSVTAADTAVYYCARSLARTTAMDYWGQGSLVTVSSASTKGPSVFPLAPSSKSTSGGTAALGCLVKDYFPEPVTVSWNSGALTSGVHTFPAVLQSSGLYSLSSVVTVPSSSLGTQTYICNVNHKPSNTKVDKRVEPKSCDKTHTCPPCPAPELLGGPSVFLFPPKPKDTLMISRTPEVTCVVVDVSHEDPEVKFNWYVDGVEVHNAKTKPREEQYNSTYRVVSVLTVLHQDWLNGKEYKCKVSNKALPAPIEKTISKAKGQPREPQVCTLPPSRECMTKNQVSLTCLVKGFYPSDIAVEWESNGQPENNYCTTPPVLCSDGSFFLYSKLTVDKSRWQQGNVFSCSVMHEALHNHYTQKSLSLSP

SEQ ID NO: 43 - protein, 447 aa, Homo sapiens
QVQLQESGPGLVRPSQTLSLTCTVSGYSITSDHAWSWVRQPPGRGLEWIGYISYSGITTYNPSLKSRVTMLRDTSKNQFSLRLSSVTAADTAVYYCARSLARTTAMDYWGQGSLVTVSSASTKGPSVFPLAPSSKSTSGGTAALGCLVKDYFPEPVTVSWNSGALTSGVHTFPAVLQSSGLYSLSSVVTVPSSSLGTQTYICNVNHKPSNTKVDKRVEPKSCDKTHTCPPCPAPELLGGPSVFLFPPKPKDTLMISRTPEVTCVVVDVSHEDPEVKFNWYVDGVEVHNAKTKPREEQYNSTYRVVSVLTVLHQDWLNGKEYKCKVSNKALPAPIEKTISKAKGQPREPQVCTCPPCRECMTKNQVSLTCLVKGFYPSDIAVEWESNGQPENNYKTTPPVLDSDGSFFLYSKLTVDKSRWQQGNVFSCSVMHEALHNHYTQKSLSLSP

SEQ ID NO: 44 - protein, 447 aa, Homo sapiens
QVQLQESGPGLVRPSQTLSLTCTVSGYSITSDHAWSWVRQPPGRGLEWIGYISYSGITTYNPSLKSRVTMLRDTSKNQFSLRLSSVTAADTAVYYCARSLARTTAMDYWGQGSLVTVSSASTKGPSVFPLAPSSKSTSGGTAALGCLVKDYFPEPVTVSWNSGALTSGVHTFPAVLQSSGLYSLSSVVTVPSSSLGTQTYICNVNHKPSNTKVDKRVEPKSCDKTHTCPPCPAPELLGGPSVFLFPPKPKDTLMISRTPEVTCVVVDVSHEDPEVKFNWYVDGVEVHNAKTKPREEQYNSTYRVVSVLTVLHQDWLNGKEYKCKVSNKALPAPIEKTISKAKGQPREPQVCTLPPSRECMTKNQVSLTCLVKGFYPSDIAVEWESNGQPENNYKTCPPCLDSDGSFFLYSKLTVDKSRWQQGNVFSCSVMHEALHNHYTQKSLSLSP

SEQ ID NO: 45 - protein, 447 aa, Homo sapiens
QVQLQESGPGLVRPSQTLSLTCTVSGYSITSDHAWSWVRQPPGRGLEWIGYISYSGITTYNPSLKSRVTMLRDTSKNQFSLRLSSVTAADTAVYYCARSLARTTAMDYWGQGSLVTVSSASTKGPSVFPLAPSSKSTSGGTAALGCLVKDYFPEPVTVSWNSGALTSGVHTFPAVLQSSGLYSLSSVVTVPSSSLGTQTYICNVNHKPSNTKVDKRVEPKSCDKTHTCPPCPAPELLGGPSVFLFPPKPKDTLMISRTPEVTCVVVDVSHEDPEVKFNWYVDGVEVHNAKTKPREEQYNSTYRVVSVLTVLHQDWLNGKEYKCKVSNKALPAPIEKTISKAKGQPREPQVCTLPPSRECMTKNQVSLTCLVKGFYPSDIAVEWESNGQPENNYCTCPPCLCSDGSFFLYSKLTVDKSRWQQGNVFSCSVMHEALHNHYTQKSLSLSP

SEQ ID NO: 46 - protein, 447 aa, Homo sapiens
QVQLQESGPGLVRPSQTLSLTCTVSGYSITSDHAWSWVRQPPGRGLEWIGYISYSGITTYNPSLKSRVTMLRDTSKNQFSLRLSSVTAADTAVYYCARSLARTTAMDYWGQGSLVTVSSASTKGPSVFPLAPSSKSTSGGTAALGCLVKDYFPEPVTVSWNSGALTSGVHTFPAVLQSSGLYSLSSVVTVPSSSLGTQTYICNVNHKPSNTKVDKRVEPKSCDKTHTCPPCPAPELLGGPSVFLFPPKPKDTLMISRTPEVTCVVVDVSHEDPEVKFNWYVDGVEVHNAKTKPREEQYNSTYRVVSVLTVLHQDWLNGKEYKCKVSNKALPAPIEKTISKAKGQPREPQVYTLPPSREEMTKNQVSLTCLVKGFYPSDIAVEWESNGQPENNYCTCPPCLCSDGSFFLYSKLTVDKSRWQQGNVFSCSVMHEALHNHYTQKSLSLSP

SEQ ID NO: 47 - protein, 447 aa, Homo sapiens
QVQLQESGPGLVRPSQTLSLTCTVSGYSITSDHAWSWVRQPPGRGLEWIGYISYSGITTYNPSLKSRVTMLRDTSKNQFSLRLSSVTAADTAVYYCARSLARTTAMDYWGQGSLVTVSSASTKGPSVFPLAPSSKSTSGGTAALGCLVKDYFPEPVTVSWNSGALTSGVHTFPAVLQSSGLYSLSSVVTVPSSSLGTQTYICNVNHKPSNTKVDKRVEPKSCDKTHTCPPCPAPELLGGPSVFLFPPKPKDTLMISRTPEVTCVVVDVSHEDPEVKFNWYVDGVEVHNAKTKPREEQYNSTYRVVSVLTVLHQDWLNGKEYKCKVSNKALPAPIEKTISKAKGQPREPQVYTCPPCREEMTKNQVSLTCLVKGFYPSDIAVEWESNGQPENNYCTTPPVLCSDGSFFLYSKLTVDKSRWQQGNVFSCSVMHEALHNHYTQKSLSLSP

SEQ ID NO: 48 - protein, 447 aa, Homo sapiens
QVQLQESGPGLVRPSQTLSLTCTVSGYSITSDHAWSWVRQPPGRGLEWIGYISYSGITTYNPSLKSRVTMLRDTSKNQFSLRLSSVTAADTAVYYCARSLARTTAMDYWGQGSLVTVSSASTKGPSVFPLAPSSKSTSGGTAALGCLVKDYFPEPVTVSWNSGALTSGVHTFPAVLQSSGLYSLSSVVTVPSSSLGTQTYICNVNHKPSNTKVDKRVEPKSCDKTHTCPPCPAPELLGGPSVFLFPPKPKDTLMISRTPEVTCVVVDVSHEDPEVKFNWYVDGVEVHNAKTKPREEQYNSTYRVVSVLTVLHQDWLNGKEYKCKVSNKALPAPIEKTISKAKGQPREPQVYTLPPSRKEMTKNQVSLTCLVKGFYPSDIAVEWESNGQPENNYDTTPPVLKSDGSFFLYSKLTVDKSRWQQGNVFSCSVMHEALHNHYTQESLSLSP

SEQ ID NO: 49 - protein, 447 aa, Homo sapiens
QVQLQESGPGLVRPSQTLSLTCTVSGYSITSDHAWSWVRQPPGRGLEWIGYISYSGITTYNPSLKSRVTMLRDTSKNQFSLRLSSVTAADTAVYYCARSLARTTAMDYWGQGSLVTVSSASTKGPSVFPLAPSSKSTSGGTAALGCLVKDYFPEPVTVSWNSGALTSGVHTFPAVLQSSGLYSLSSVVTVPSSSLGTQTYICNVNHKPSNTKVDKRVEPKSCDKTHTCPPCPAPELLGGPSVFLFPPKPKDTLMISRTPEVTCVVVDVSHEDPEVKFNWYVDGVEVHNAKTKPREEQYNSTYRVVSVLTVLHQDWLNGKEYKCKVSNKALPAPIEKTISKAKGQPREPQVYTLPPSREKMTKNQVSLTCLVEGFYPSDIAVEWESNGQPENNYDTTPPVLKSDGSFFLYSKLTVDKSRWQQGNVFSCSVMHEALHNHYTQKSLSLSP

SEQ ID NO: 50 - protein, 447 aa, Homo sapiens
QVQLQESGPGLVRPSQTLSLTCTVSGYSITSDHAWSWVRQPPGRGLEWIGYISYSGITTYNPSLKSRVTMLRDTSKNQFSLRLSSVTAADTAVYYCARSLARTTAMDYWGQGSLVTVSSASTKGPSVFPLAPSSKSTSGGTAALGCLVKDYFPEPVTVSWNSGALTSGVHTFPAVLQSSGLYSLSSVVTVPSSSLGTQTYICNVNHKPSNTKVDKRVEPKSCDKTHTCPPCPAPELLGGPSVFLFPPKPKDTLMISRTPEVTCVVVDVSHEDPEVKFNWYVDGVEVHNAKTKPREEQYNSTYRVVSVLTVLHQDWLNGKEYKCKVSNKALPAPIEKTISKAKGQPREPQVYTLPPSREEMTKNQVSLTCLVKGFYPSDIAVEWESNGQPENNYDTTPPVLKSDGSFFLYSDLTVDKSRWQQGNVFSCSVMHEALHNHYTQKSLSLSP

SEQ ID NO: 51 - protein, 447 aa, Homo sapiens
QVQLQESGPGLVRPSQTLSLTCTVSGYSITSDHAWSWVRQPPGRGLEWIGYISYSGITTYNPSLKSRVTMLRDTSKNQFSLRLSSVTAADTAVYYCARSLARTTAMDYWGQGSLVTVSSASTKGPSVFPLAPSSKSTSGGTAALGCLVKDYFPEPVTVSWNSGALTSGVHTFPAVLQSSGLYSLSSVVTVPSSSLGTQTYICNVNHKPSNTKVDKRVEPKSCDKTHTCPPCPAPELLGGPSVFLFPPKPKDTLMISRTPEVTCVVVDVSHEDPEVKFNWYVDGVEVHNAKTKPREEQYNSTYRVVSVLTVLHQDWLNGKEYKCKVSNKALPAPIEKTISKAKGQPREPQVCTLPPSRECMTKNQVSLTCLVKGFYPSDIAVEWESNGQPENNYDTTPPVLKSDGSFFLYSKLTVDKSRWQQGNVFSCSVMHEALHNHYTQKSLSLSP

SEQ ID NO: 52 - protein, 447 aa, Homo sapiens
QVQLQESGPGLVRPSQTLSLTCTVSGYSITSDHAWSWVRQPPGRGLEWIGYISYSGITTYNPSLKSRVTMLRDTSKNQFSLRLSSVTAADTAVYYCARSLARTTAMDYWGQGSLVTVSSASTKGPSVFPLAPSSKSTSGGTAALGCLVKDYFPEPVTVSWNSGALTSGVHTFPAVLQSSGLYSLSSVVTVPSSSLGTQTYICNVNHKPSNTKVDKRVEPKSCDKTHTCPPCPAPELLGGPSVFLFPPKPKDTLMISRTPEVTCVVVDVSHEDPEVKFNWYVDGVEVHNAKTKPREEQYNSTYRVVSVLTVLHQDWLNGKEYKCKVSNKALPAPIEKTISKAKGQPREPQVYTLPPSREKMTKNQVSLTCLVEGFYPSDIAVEWESNGQPENNYKTCPPCLDSDGSFFLYSKLTVDKSRWQQGNVFSCSVMHEALHNHYTQKSLSLSP

SEQ ID NO: 53 - protein, 447 aa, Homo sapiens
QVQLQESGPGLVRPSQTLSLTCTVSGYSITSDHAWSWVRQPPGRGLEWIGYISYSGITTYNPSLKSRVTMLRDTSKNQFSLRLSSVTAADTAVYYCARSLARTTAMDYWGQGSLVTVSSASTKGPSVFPLAPSSKSTSGGTAALGCLVKDYFPEPVTVSWNSGALTSGVHTFPAVLQSSGLYSLSSVVTVPSSSLGTQTYICNVNHKPSNTKVDKRVEPKSCDKTHTCPPCPAPELLGGPSVFLFPPKPKDTLMISRTPEVTCVVVDVSHEDPEVKFNWYVDGVEVHNAKTKPREEQYNSTYRVVSVLTVLHQDWLNGKEYKCKVSNKALPAPIEKTISKAKGQPREPQVCTLPPSRECMTKNQVSLTCLVEGFYPSDIAVEWESNGQPENNYKTTPPVLDSDGSFFLYSKLTVDKSRWQQGNVFSCSVMHEALHNHYTQKSLSLSP

SEQ ID NO: 54 - protein, 447 aa, Homo sapiens
QVQLQESGPGLVRPSQTLSLTCTVSGYSITSDHAWSWVRQPPGRGLEWIGYISYSGITTYNPSLKSRVTMLRDTSKNQFSLRLSSVTAADTAVYYCARSLARTTAMDYWGQGSLVTVSSASTKGPSVFPLAPSSKSTSGGTAALGCLVKDYFPEPVTVSWNSGALTSGVHTFPAVLQSSGLYSLSSVVTVPSSSLGTQTYICNVNHKPSNTKVDKRVEPKSCDKTHTCPPCPAPELLGGPSVFLFPPKPKDTLMISRTPEVTCVVVDVSHEDPEVKFNWYVDGVEVHNAKTKPREEQYNSTYRVVSVLTVLHQDWLNGKEYKCKVSNKALPAPIEKTISKAKGQPREPQVYTLPPSREKMTKNQVSLTCLVEGFYPSDIAVEWESNGQPENNYCTTPPVLCSDGSFFLYSKLTVDKSRWQQGNVFSCSVMHEALHNHYTQKSLSLSP

SEQ ID NO: 55 - protein, 447 aa, Homo sapiens
QVQLQESGPGLVRPSQTLSLTCTVSGYSITSDHAWSWVRQPPGRGLEWIGYISYSGITTYNPSLKSRVTMLRDTSKNQFSLRLSSVTAADTAVYYCARSLARTTAMDYWGQGSLVTVSSASTKGPSVFPLAPSSKSTSGGTAALGCLVKDYFPEPVTVSWNSGALTSGVHTFPAVLQSSGLYSLSSVVTVPSSSLGTQTYICNVNHKPSNTKVDKRVEPKSCDKTHTCPPCPAPELLGGPSVFLFPPKPKDTLMISRTPEVTCVVVDVSHEDPEVKFNWYVDGVEVHNAKTKPREEQYNSTYRVVSVLTVLHQDWLNGKEYKCKVSNKALPAPIEKTISKAKGQPRRPRVYTLPPSREEMTDNQVSLVCLVKGFYPSDIAVEWESNGQPENNYKTTPPVLMSDGSFFLASVLTVDKSRWQQGNVFSCSVMHEALHNHYTQKSLSLSP

SEQ ID NO: 56 - protein, 447 aa, Homo sapiens
QVQLQESGPGLVRPSQTLSLTCTVSGYSITSDHAWSWVRQPPGRGLEWIGYISYSGITTYNPSLKSRVTMLRDTSKNQFSLRLSSVTAADTAVYYCARSLARTTAMDYWGQGSLVTVSSASTKGPSVFPLAPSSKSTSGGTAALGCLVKDYFPEPVTVSWNSGALTSGVHTFPAVLQSSGLYSLSSVVTVPSSSLGTQTYICNVNHKPSNTKVDKRVEPKSCDKTHTCPPCPAPELLGGPSVFLFPPKPKDTLMISRTPEVTCVVVDVSHEDPEVKFNWYVDGVEVHNAKTKPREEQYNSTYRVVSVLTVLHQDWLNGKEYKCKVSNKALPAPIEKTISKAKGQPREPQVYTLPPSRKEMTKNQVSLTCLVKGFYPSDIAVEWESNGQPENNYDTTPPVLKSDGSFFLYSDLTVDKSRWQQGNVFSCSVMHEALHNHYTQKSLSLSP

SEQ ID NO: 57 - protein, 447 aa, Homo sapiens
QVQLQESGPGLVRPSQTLSLTCTVSGYSITSDHAWSWVRQPPGRGLEWIGYISYSGITTYNPSLKSRVTMLRDTSKNQFSLRLSSVTAADTAVYYCARSLARTTAMDYWGQGSLVTVSSASTKGPSVFPLAPSSKSTSGGTAALGCLVKDYFPEPVTVSWNSGALTSGVHTFPAVLQSSGLYSLSSVVTVPSSSLGTQTYICNVNHKPSNTKVDKRVEPKSCDKTHTCPPCPAPELLGGPSVFLFPPKPKDTLMISRTPEVTCVVVDVSHEDPEVKFNWYVDGVEVHNAKTKPREEQYNSTYRVVSVLTVLHQDWLNGKEYKCKVSNKALPAPIEKTISKAKGQPRRPRVYTLPPSREEMTDNQVSLVCLVKGFYPSDIAVEWESNGQPENNYKTTPPVLDSDGSFFLYSKLTVDKSRWQQGNVFSCSVMHEALHNHYTQKSLSLSP

SEQ ID NO: 58 - protein, 447 aa, Homo sapiens
QVQLQESGPGLVRPSQTLSLTCTVSGYSITSDHAWSWVRQPPGRGLEWIGYISYSGITTYNPSLKSRVTMLRDTSKNQFSLRLSSVTAADTAVYYCARSLARTTAMDYWGQGSLVTVSSASTKGPSVFPLAPSSKSTSGGTAALGCLVKDYFPEPVTVSWNSGALTSGVHTFPAVLQSSGLYSLSSVVTVPSSSLGTQTYICNVNHKPSNTKVDKRVEPKSCDKTHTCPPCPAPELLGGPSVFLFPPKPKDTLMISRTPEVTCVVVDVSHEDPEVKFNWYVDGVEVHNAKTKPREEQYNSTYRVVSVLTVLHQDWLNGKEYKCKVSNKALPAPIEKTISKAKGQPRRPQVYTLPPSREEMTENQVSLTCLVKGFYPSDIAVEWESNGQPENNYKTTPPVLMSDGSFFLASVLTVDKSRWQQGNVFSCSVMHEALHNHYTQKSLSLSP

SEQ ID NO: 59 - protein, 447 aa, Homo sapiens
QVQLQESGPGLVRPSQTLSLTCTVSGYSITSDHAWSWVRQPPGRGLEWIGYISYSGITTYNPSLKSRVTMLRDTSKNQFSLRLSSVTAADTAVYYCARSLARTTAMDYWGQGSLVTVSSASTKGPSVFPLAPSSKSTSGGTAALGCLVKDYFPEPVTVSWNSGALTSGVHTFPAVLQSSGLYSLSSVVTVPSSSLGTQTYICNVNHKPSNTKVDKRVEPKSCDKTHTCPPCPAPELLGGPSVFLFPPKPKDTLMISRTPEVTCVVVDVSHEDPEVKFNWYVDGVEVHNAKTKPREEQYNSTYRVVSVLTVLHQDWLNGKEYKCKVSNKALPAPIEKTISKAKGQPREPQVYTLPPSREEMTKNQVSLTCLVKGFYPSDIAVEWESNGQPENNYDTCPPCLKSDGSFFLYSKLTVDKSRWQQGNVFSCSVMHEALHNHYTQKSLSLSP

SEQ ID NO: 60 - protein, 447 aa, Homo sapiens
QVQLQESGPGLVRPSQTLSLTCTVSGYSITSDHAWSWVRQPPGRGLEWIGYISYSGITTYNPSLKSRVTMLRDTSKNQFSLRLSSVTAADTAVYYCARSLARTTAMDYWGQGSLVTVSSASTKGPSVFPLAPSSKSTSGGTAALGCLVKDYFPEPVTVSWNSGALTSGVHTFPAVLQSSGLYSLSSVVTVPSSSLGTQTYICNVNHKPSNTKVDKRVEPKSCDKTHTCPPCPAPELLGGPSVFLFPPKPKDTLMISRTPEVTCVVVDVSHEDPEVKFNWYVDGVEVHNAKTKPREEQYNSTYRVVSVLTVLHQDWLNGKEYKCKVSNKALPAPIEKTISKAKGQPREPQVYVYPPSREEMTKNQVSLLCLVKGFYPSDIAVEWESNGQPENNYLTWPPVLDSDGSFALVSKLTVDKSRWQQGNVFSCSVMHEALHNHYTQKSLSLSP

SEQ ID NO: 61 - protein, 214 aa, Homo sapiens [sequence omitted]

SEQ ID NO: 62 - protein, 225 aa, Homo sapiens
DKTHTCPPCPAPELLGGPSVFLFPPKPKDTLMISRTPEVTCVVVDVSHEDPEVKFNWYVDGVEVHNAKTKPREEQYNSTYRVVSVLTVLHQDWLNGKEYKCKVSNKALPAPIEKTISKAKGQPREPQVYTLPPSREEMTKNQVSLTCLVKGFYPSDIAVEWESNGQPENNYKTTPPVLDSDGSFFLYSKLTVDKSRWQQGNVFSCSVMHEALHNHYTQKSLSLSP

SEQ ID NO: 63 - protein, 225 aa, Homo sapiens; identical to SEQ ID NO: 62

SEQ ID NO: 64 - protein, 225 aa, Homo sapiens
DKTHTCPPCPAPELLGGPSVFLFPPKPKDTLMISRTPEVTCVVVDVSHEDPEVKFNWYVDGVEVHNAKTKPREEQYNSTYRVVSVLTVLHQDWLNGKEYKCKVSNKALPAPIEKTISKAKGQPREPQVYTLPPSREEMTKNQVSLTCLVKGFYPSDIAVEWESNGQPENNYKTWPPVLDSDGSFALYSKLTVDKSRWQQGNVFSCSVMHEALHNHYTQKSLSLSP

SEQ ID NO: 65 - protein, 225 aa, Homo sapiens
DKTHTCPPCPAPELLGGPSVFLFPPKPKDTLMISRTPEVTCVVVDVSHEDPEVKFNWYVDGVEVHNAKTKPREEQYNSTYRVVSVLTVLHQDWLNGKEYKCKVSNKALPAPIEKTISKAKGQPREPQVYTLPPSREEMTKNQVSLWCAVKGFYPSDIAVEWESNGQPENNYKTTPPVLDSDGSFFLVSKLTVDKSRWQQGNVFSCSVMHEALHNHYTQKSLSLSP

SEQ ID NO: 66 - protein, 225 aa, Homo sapiens
DKTHTCPPCPAPELLGGPSVFLFPPKPKDTLMISRTPEVTCVVVDVSHEDPEVKFNWYVDGVEVHNAKTKPREEQYNSTYRVVSVLTVLHQDWLNGKEYKCKVSNKALPAPIEKTISKAKGQPREPRVYTLPPSREEMTENQVSLTCLVKGFYPSDIAVEWESNGQPENNYKTTPPVLVSDGSFTLYSWLTVDKSRWQQGNVFSCSVMHEALHNHYTQKSLSLSP

SEQ ID NO: 67 - protein, 225 aa, Homo sapiens
DKTHTCPPCPAPELLGGPSVFLFPPKPKDTLMISRTPEVTCVVVDVSHEDPEVKFNWYVDGVEVHNAKTKPREEQYNSTYRVVSVLTVLHQDWLNGKEYKCKVSNKALPAPIEKTISKAKGQPREPQVYTLPPSREEMTKNQVSLTCLVKGFYPSDIAVEWESNGQPENNYKTFPPVLDSDGSFALYSKLTVDKSRWQQGNVFSCSVMHEALHNHYTQKSLSLSP

SEQ ID NO: 68 - protein, 225 aa, Homo sapiens
DKTHTCPPCPAPELLGGPSVFLFPPKPKDTLMISRTPEVTCVVVDVSHEDPEVKFNWYVDGVEVHNAKTKPREEQYNSTYRVVSVLTVLHQDWLNGKEYKCKVSNKALPAPIEKTISKAKGQPREPQVYTLPPSRKEMTKNQVSLTCLVKGFYPSDIAVEWESNGQPENNYKTTPPVLKSDGSFFLYSELTVDKSRWQQGNVFSCSVMHEALHNHYTQESLSLSP

SEQ ID NO: 69 - protein, 225 aa, Homo sapiens
DKTHTCPPCPAPELLGGPSVFLFPPKPKDTLMISRTPEVTCVVVDVSHEDPEVKFNWYVDGVEVHNAKTKPREEQYNSTYRVVSVLTVLHQDWLNGKEYKCKVSNKALPAPIEKTISKAKGQPREPEVYTLPPYREEMTKNQVSLYCLVKGFYPSDIAVEWESNGQPENNYKTTPPVLDSDGSFFLTSKLTVDKSRWQQGNVFSCSVMHEALHNHYTQKSLSLSP

SEQ ID NO: 70 - protein, 225 aa, Homo sapiens
DKTHTCPPCPAPELLGGPSVFLFPPKPKDTLMISRTPEVTCVVVDVSHEDPEVKFNWYVDGVEVHNAKTKPREEQYNSTYRVVSVLTVLHQDWLNGKEYKCKVSNKALPAPIEKTISKAKGQPREPQVYTLPPSREEMTKNQVSLTCLVKGFYPSDIAVEWESNGQPENNYLTWPPVLDSDGSFALVSKLTVDKSRWQQGNVFSCSVMHEALHNHYTQKSLSLSP

SEQ ID NO: 71 - protein, 225 aa, Homo sapiens
DKTHTCPPCPAPELLGGPSVFLFPPKPKDTLMISRTPEVTCVVVDVSHEDPEVKFNWYVDGVEVHNAKTKPREEQYNSTYRVVSVLTVLHQDWLNGKEYKCKVSNKALPAPIEKTISKAKGQPREPQVYTLPPSRKEMTKNQVSLTCLVKGFYPSDIAVEWESNGQPENNYDTTPPVLKSDGSFFLYSKLTVDKSRWQQGNVFSCSVMHEALHNHYTQESLSLSP

SEQ ID NO: 72 - protein, 225 aa, Homo sapiens
DKTHTCPPCPAPELLGGPSVFLFPPKPKDTLMISRTPEVTCVVVDVSHEDPEVKFNWYVDGVEVHNAKTKPREEQYNSTYRVVSVLTVLHQDWLNGKEYKCKVSNKALPAPIEKTISKAKGQPREPQVYTLPPSREEMTKNQVSLTCLVKGFYPSDIAVEWESNGQPENNYDTTPPVLKSDGSFFLYSDLTVDKSRWQQGNVFSCSVMHEALHNHYTQKSLSLSP

SEQ ID NO: 73 - protein, 225 aa, Homo sapiens
DKTHTCPPCPAPELLGGPSVFLFPPKPKDTLMISRTPEVTCVVVDVSHEDPEVKFNWYVDGVEVHNAKTKPREEQYNSTYRVVSVLTVLHQDWLNGKEYKCKVSNKALPAPIEKTISKAKGQPREPQVCTLPPSRECMTKNQVSLTCLVKGFYPSDIAVEWESNGQPENNYDTTPPVLKSDGSFFLYSKLTVDKSRWQQGNVFSCSVMHEALHNHYTQKSLSLSP

SEQ ID NO: 74 - protein, 225 aa, Homo sapiens
DKTHTCPPCPAPELLGGPSVFLFPPKPKDTLMISRTPEVTCVVVDVSHEDPEVKFNWYVDGVEVHNAKTKPREEQYNSTYRVVSVLTVLHQDWLNGKEYKCKVSNKALPAPIEKTISKAKGQPRRPRVYTLPPSREEMTDNQVSLVCLVKGFYPSDIAVEWESNGQPENNYKTTPPVLMSDGSFFLASVLTVDKSRWQQGNVFSCSVMHEALHNHYTQKSLSLSP

SEQ ID NO: 75 - protein, 225 aa, Homo sapiens
DKTHTCPPCPAPELLGGPSVFLFPPKPKDTLMISRTPEVTCVVVDVSHEDPEVKFNWYVDGVEVHNAKTKPREEQYNSTYRVVSVLTVLHQDWLNGKEYKCKVSNKALPAPIEKTISKAKGQPREPQVYTLPPSRKEMTKNQVSLTCLVKGFYPSDIAVEWESNGQPENNYDTTPPVLKSDGSFFLYSDLTVDKSRWQQGNVFSCSVMHEALHNHYTQKSLSLSP

SEQ ID NO: 76 - protein, 225 aa, Homo sapiens
DKTHTCPPCPAPELLGGPSVFLFPPKPKDTLMISRTPEVTCVVVDVSHEDPEVKFNWYVDGVEVHNAKTKPREEQYNSTYRVVSVLTVLHQDWLNGKEYKCKVSNKALPAPIEKTISKAKGQPRRPQVYTLPPSREEMTENQVSLTCLVKGFYPSDIAVEWESNGQPENNYKTTPPVLMSDGSFFLASVLTVDKSRWQQGNVFSCSVMHEALHNHYTQKSLSLSP

SEQ ID NO: 77 - protein, 225 aa, Homo sapiens
DKTHTCPPCPAPELLGGPSVFLFPPKPKDTLMISRTPEVTCVVVDVSHEDPEVKFNWYVDGVEVHNAKTKPREEQYNSTYRVVSVLTVLHQDWLNGKEYKCKVSNKALPAPIEKTISKAKGQPREPQVYVYPPSREEMTKNQVSLLCLVKGFYPSDIAVEWESNGQPENNYLTWPPVLDSDGSFALVSKLTVDKSRWQQGNVFSCSVMHEALHNHYTQKSLSLSP

SEQ ID NO: 78 - protein, 447 aa, Homo sapiens
QVQLQESGPGLVKPSETLSLTCAVSGHSISHDHAWSWVRQPPGEGLEWIGFISYSGITNYNPSLQGRVTISRDNSKNTLYLQMNSLRAEDTAVYYCARSLARTTAMDYWGEGTLVTVSSASTKGPSVFPLAPSSKSTSGGTAALGCLVKDYFPEPVTVSWNSGALTSGVHTFPAVLQSSGLYSLSSVVTVPSSSLGTQTYICNVNHKPSNTKVDKRVEPKSCDKTHTCPPCPAPELLGGPSVFLFPPKPKDTLMISRTPEVTCVVVDVSHEDPEVKFNWYVDGVEVHNAKTKPREEQYNSTYRVVSVLTVLHQDWLNGKEYKCKVSNKALPAPIEKTISKAKGQPREPQVYTLPPSREEMTKNQVSLTCLVKGFYPSDIAVEWESNGQPENNYKTTPPVLDSDGSFFLYSKLTVDKSRWQQGNVFSCSVMHEALHNHYTQKSLSLSP

SEQ ID NO: 79 - protein, 447 aa, Homo sapiens
QVQLVQSGSELKKPGASVKVSCKASGYTFTDNNMDWVRQAPGQGLEWMGDINTRSGGSIYNEEFQDRVIMTVDKSTDTAYMELSSLRSEDTATYHCARRKSYGYYLDEWGEGTLVTVSSASTKGPSVFPLAPSSKSTSGGTAALGCLVKDYFPEPVTVSWNSGALTSGVHTFPAVLQSSGLYSLSSVVTVPSSSLGTQTYICNVNHKPSNTKVDKRVEPKSCDKTHTCPPCPAPELLGGPSVFLFPPKPKDTLMISRTPEVTCVVVDVSHEDPEVKFNWYVDGVEVHNAKTKPREEQYNSTYRVVSVLTVLHQDWLNGKEYKCKVSNKALPAPIEKTISKAKGQPREPQVYTLPPSREEMTKNQVSLTCLVKGFYPSDIAVEWESNGQPENNYKTTPPVLDSDGSFFLYSKLTVDKSRWQQGNVFSCSVMHEALHNHYTQKSLSLSP

SEQ ID NO: 80 - protein, 447 aa, Homo sapiens
QVQLVQSGSELKKPGASVKVSCKASGYTFTDNNMDWVRQAPGQGLEWMGDINTRSGGSIYNEEFQDRVIMTVDKSTDTAYMELSSLRSEDTATYHCARRESEGYYLDEWGEGTLVTVSSASTKGPSVFPLAPSSKSTSGGTAALGCLVKDYFPEPVTVSWNSGALTSGVHTFPAVLQSSGLYSLSSVVTVPSSSLGTQTYICNVNHKPSNTKVDKRVEPKSCDKTHTCPPCPAPELLGGPSVFLFPPKPKDTLMISRTPEVTCVVVDVSHEDPEVKFNWYVDGVEVHNAKTKPREEQYNSTYRVVSVLTVLHQDWLNGKEYKCKVSNKALPAPIEKTISKAKGQPREPQVYTLPPSREEMTKNQVSLTCLVKGFYPSDIAVEWESNGQPENNYKTTPPVLDSDGSFFLYSKLTVDKSRWQQGNVFSCSVMHEALHNHYTQKSLSLSP

SEQ ID NO: 81 - protein, 447 aa, Homo sapiens
QVQLQESGPGLVKPSETLSLTCAVSGHSISHDHAWSWVRQPPGEGLEWIGFISYSGITNYNPSLQGRVTISRDNSKNTLYLQMNSLRAEDTAVYYCARSLARTTAMDYWGEGTLVTVSSASTKGPSVFPLAPSSKSTSGGTAALGCLVKDYFPEPVTVSWNSGALTSGVHTFPAVLQSSGLYSLSSVVTVPSSSLGTQTYICNVNHKPSNTKVDKRVEPKSCDKTHTCPPCPAPELLGGPSVFLFPPKPKDTLMISRTPEVTCVVVDVSHEDPEVKFNWYVDGVEVHNAKTKPREEQYNSTYRVVSVLTVLHQDWLNGKEYKCKVSNKALPAPIEKTISKAKGQPREPQVYTLPPSREEMTKNQVSLWCAVKGFYPSDIAVEWESNGQPENNYKTTPPVLDSDGSFFLVSKLTVDKSRWQQGNVFSCSVMHEALHNHYTQKSLSLSP

SEQ ID NO: 82 - protein, 447 aa, Homo sapiens
QVQLVQSGSELKKPGASVKVSCKASGYTFTDNNMDWVRQAPGQGLEWMGDINTRSGGSIYNEEFQDRVIMTVDKSTDTAYMELSSLRSEDTATYHCARRKSYGYYLDEWGEGTLVTVSSASTKGPSVFPLAPSSKSTSGGTAALGCLVKDYFPEPVTVSWNSGALTSGVHTFPAVLQSSGLYSLSSVVTVPSSSLGTQTYICNVNHKPSNTKVDKRVEPKSCDKTHTCPPCPAPELLGGPSVFLFPPKPKDTLMISRTPEVTCVVVDVSHEDPEVKFNWYVDGVEVHNAKTKPREEQYNSTYRVVSVLTVLHQDWLNGKEYKCKVSNKALPAPIEKTISKAKGQPREPRVYTLPPSREEMTENQVSLTCLVKGFYPSDIAVEWESNGQPENNYKTTPPVLVSDGSFTLYSWLTVDKSRWQQGNVFSCSVMHEALHNHYTQKSLSLSP

SEQ ID NO: 83 - protein, 447 aa, Homo sapiens
QVQLVQSGSELKKPGASVKVSCKASGYTFTDNNMDWVRQAPGQGLEWMGDINTRSGGSIYNEEFQDRVIMTVDKSTDTAYMELSSLRSEDTATYHCARRESEGYYLDEWGEGTLVTVSSASTKGPSVFPLAPSSKSTSGGTAALGCLVKDYFPEPVTVSWNSGALTSGVHTFPAVLQSSGLYSLSSVVTVPSSSLGTQTYICNVNHKPSNTKVDKRVEPKSCDKTHTCPPCPAPELLGGPSVFLFPPKPKDTLMISRTPEVTCVVVDVSHEDPEVKFNWYVDGVEVHNAKTKPREEQYNSTYRVVSVLTVLHQDWLNGKEYKCKVSNKALPAPIEKTISKAKGQPREPQVYTLPPSRKEMTKNQVSLTCLVKGFYPSDIAVEWESNGQPENNYKTTPPVLKSDGSFFLYSELTVDKSRWQQGNVFSCSVMHEALHNHYTQESLSLSP

SEQ ID NO: 84 - protein, 447 aa, Homo sapiens
QVQLVQSGSELKKPGASVKVSCKASGYTFTDNNMDWVRQAPGQGLEWMGDINTRSGGSIYNEEFQDRVIMTVDKSTDTAYMELSSLRSEDTATYHCARRESEGYYLDEWGEGTLVTVSSASTKGPSVFPLAPSSKSTSGGTAALGCLVKDYFPEPVTVSWNSGALTSGVHTFPAVLQSSGLYSLSSVVTVPSSSLGTQTYICNVNHKPSNTKVDKRVEPKSCDKTHTCPPCPAPELLGGPSVFLFPPKPKDTLMISRTPEVTCVVVDVSHEDPEVKFNWYVDGVEVHNAKTKPREEQYNSTYRVVSVLTVLHQDWLNGKEYKCKVSNKALPAPIEKTISKAKGQPREPQVYTLPPSRKEMTKNQVSLTCLVKGFYPSDIAVEWESNGQPENNYDTTPPVLKSDGSFFLYSKLTVDKSRWQQGNVFSCSVMHEALHNHYTQESLSLSP

SEQ ID NO: 85 - protein, 447 aa, Homo sapiens
QVQLVQSGSELKKPGASVKVSCKASGYTFTDNNMDWVRQAPGQGLEWMGDINTRSGGSIYNEEFQDRVIMTVDKSTDTAYMELSSLRSEDTATYHCARRKSYGYYLDEWGEGTLVTVSSASTKGPSVFPLAPSSKSTSGGTAALGCLVKDYFPEPVTVSWNSGALTSGVHTFPAVLQSSGLYSLSSVVTVPSSSLGTQTYICNVNHKPSNTKVDKRVEPKSCDKTHTCPPCPAPELLGGPSVFLFPPKPKDTLMISRTPEVTCVVVDVSHEDPEVKFNWYVDGVEVHNAKTKPREEQYNSTYRVVSVLTVLHQDWLNGKEYKCKVSNKALPAPIEKTISKAKGQPRRPQVYTLPPSREEMTENQVSLTCLVKGFYPSDIAVEWESNGQPENNYKTTPPVLMSDGSFFLASVLTVDKSRWQQGNVFSCSVMHEALHNHYTQKSLSLSP

SEQ ID NO: 86 - protein, 443 aa, Homo sapiens
QVQLQESGPGLVRPSQTLSLTCTVSGYSITSDHAWSWVRQPPGRGLEWIGYISYSGITTYNPSLKSRVTMLRDTSKNQFSLRLSSVTAADTAVYYCARSLARTTAMDYWGQGSLVTVSSASTKGPSVFPLAPCSRSTSESTAALGCLVKDYFPEPVTVSWNSGALTSGVHTFPAVLQSSGLYSLSSVVTVPSSNFGTQTYTCNVDHKPSNTKVDKTVERKCCVECPPCPAPPVAGPSVFLFPPKPKDTLMISRTPEVTCVVVDVSHEDPEVQFNWYVDGVEVHNAKTKPREEQFNSTFRVVSVLTVVHQDWLNGKEYKCKVSNKGLPAPIEKTISKTKGQPREPQVYTLPPSREEMTKNQVSLTCLVKGFYPSDIAVEWESNGQPENNYKTTPPMLDSDGSFFLYSKLTVDKSRWQQGNVFSCSVMHEALHNHYTQKSLSLSP

SEQ ID NO: 87 - protein, 443 aa, Homo sapiens
QVQLQESGPGLVRPSQTLSLTCTVSGYSITSDHAWSWVRQPPGRGLEWIGYISYSGITTYNPSLKSRVTMLRDTSKNQFSLRLSSVTAADTAVYYCARSLARTTAMDYWGQGSLVTVSSASTKGPSVFPLAPCSRSTSESTAALGCLVKDYFPEPVTVSWNSGALTSGVHTFPAVLQSSGLYSLSSVVTVPSSNFGTQTYTCNVDHKPSNTKVDKTVERKCCVECPPCPAPPVAGPSVFLFPPKPKDTLMISRTPEVTCVVVDVSHEDPEVQFNWYVDGVEVHNAKTKPREEQFNSTFRVVSVLTVVHQDWLNGKEYKCKVSNKGLPAPIEKTISKTKGQPREPQVYTLPPSREEMTKNQVSLTCLVKGFYPSDIAVEWESNGQPENNYKTWPPMLDSDGSFALYSKLTVDKSRWQQGNVFSCSVMHEALHNHYTQKSLSLSP

SEQ ID NO: 88 - protein, 443 aa, Homo sapiens
QVQLQESGPGLVRPSQTLSLTCTVSGYSITSDHAWSWVRQPPGRGLEWIGYISYSGITTYNPSLKSRVTMLRDTSKNQFSLRLSSVTAADTAVYYCARSLARTTAMDYWGQGSLVTVSSASTKGPSVFPLAPCSRSTSESTAALGCLVKDYFPEPVTVSWNSGALTSGVHTFPAVLQSSGLYSLSSVVTVPSSNFGTQTYTCNVDHKPSNTKVDKTVERKCCVECPPCPAPPVAGPSVFLFPPKPKDTLMISRTPEVTCVVVDVSHEDPEVQFNWYVDGVEVHNAKTKPREEQFNSTFRVVSVLTVVHQDWLNGKEYKCKVSNKGLPAPIEKTISKTKGQPREPQVYTLPPSREEMTKNQVSLWCAVKGFYPSDIAVEWESNGQPENNYKTTPPMLDSDGSFFLVSKLTVDKSRWQQGNVFSCSVMHEALHNHYTQKSLSLSP

SEQ ID NO: 89 - protein, 443 aa, Homo sapiens
QVQLQESGPGLVRPSQTLSLTCTVSGYSITSDHAWSWVRQPPGRGLEWIGYISYSGITTYNPSLKSRVTMLRDTSKNQFSLRLSSVTAADTAVYYCARSLARTTAMDYWGQGSLVTVSSASTKGPSVFPLAPCSRSTSESTAALGCLVKDYFPEPVTVSWNSGALTSGVHTFPAVLQSSGLYSLSSVVTVPSSNFGTQTYTCNVDHKPSNTKVDKTVERKCCVECPPCPAPPVAGPSVFLFPPKPKDTLMISRTPEVTCVVVDVSHEDPEVQFNWYVDGVEVHNAKTKPREEQFNSTFRVVSVLTVVHQDWLNGKEYKCKVSNKGLPAPIEKTISKTKGQPREPRVYTLPPSREEMTENQVSLTCLVKGFYPSDIAVEWESNGQPENNYKTTPPMLVSDGSFTLYSWLTVDKSRWQQGNVFSCSVMHEALHNHYTQKSLSLSP

SEQ ID NO: 90 - protein, 443 aa, Homo sapiens
QVQLQESGPGLVRPSQTLSLTCTVSGYSITSDHAWSWVRQPPGRGLEWIGYISYSGITTYNPSLKSRVTMLRDTSKNQFSLRLSSVTAADTAVYYCARSLARTTAMDYWGQGSLVTVSSASTKGPSVFPLAPCSRSTSESTAALGCLVKDYFPEPVTVSWNSGALTSGVHTFPAVLQSSGLYSLSSVVTVPSSNFGTQTYTCNVDHKPSNTKVDKTVERKCCVECPPCPAPPVAGPSVFLFPPKPKDTLMISRTPEVTCVVVDVSHEDPEVQFNWYVDGVEVHNAKTKPREEQFNSTFRVVSVLTVVHQDWLNGKEYKCKVSNKGLPAPIEKTISKTKGQPREPQVYTLPPSREEMTKNQVSLTCLVKGFYPSDIAVEWESNGQPENNYLTWPPMLDSDGSFALVSKLTVDKSRWQQGNVFSCSVMHEALHNHYTQKSLSLSP

SEQ ID NO: 91 - protein, 443 aa, Homo sapiens
QVQLQESGPGLVRPSQTLSLTCTVSGYSITSDHAWSWVRQPPGRGLEWIGYISYSGITTYNPSLKSRVTMLRDTSKNQFSLRLSSVTAADTAVYYCARSLARTTAMDYWGQGSLVTVSSASTKGPSVFPLAPCSRSTSESTAALGCLVKDYFPEPVTVSWNSGALTSGVHTFPAVLQSSGLYSLSSVVTVPSSNFGTQTYTCNVDHKPSNTKVDKTVERKCCVECPPCPAPPVAGPSVFLFPPKPKDTLMISRTPEVTCVVVDVSHEDPEVQFNWYVDGVEVHNAKTKPREEQFNSTFRVVSVLTVVHQDWLNGKEYKCKVSNKGLPAPIEKTISKTKGQPREPQVYTLPPSREEMTKNQVSLTCLVKGFYPSDIAVEWESNGQPENNYDTTPPMLKSDGSFFLYSDLTVDKSRWQQGNVFSCSVMHEALHNHYTQKSLSLSP

SEQ ID NO: 92 - protein, 444 aa, Homo sapiens
QVQLQESGPGLVRPSQTLSLTCTVSGYSITSDHAWSWVRQPPGRGLEWIGYISYSGITTYNPSLKSRVTMLRDTSKNQFSLRLSSVTAADTAVYYCARSLARTTAMDYWGQGSLVTVSSASTKGPSVFPLAPCSRSTSESTAALGCLVKDYFPEPVTVSWNSGALTSGVHTFPAVLQSSGLYSLSSVVTVPSSSLGTKTYTCNVDHKPSNTKVDKRVESKYGPPCPPCPAPEFLGGPSVFLFPPKPKDTLMISRTPEVTCVVVDVSQEDPEVQFNWYVDGVEVHNAKTKPREEQFNSTYRVVSVLTVLHQDWLNGKEYKCKVSNKGLPSSIEKTISKAKGQPREPQVYTLPPSQEEMTKNQVSLTCLVKGFYPSDIAVEWESNGQPENNYKTTPPVLDSDGSFFLYSRLTVDKSRWQEGNVFSCSVMHEALHNHYTQKSLSLSL

SEQ ID NO: 93 - protein, 444 aa, Homo sapiens
QVQLQESGPGLVRPSQTLSLTCTVSGYSITSDHAWSWVRQPPGRGLEWIGYISYSGITTYNPSLKSRVTMLRDTSKNQFSLRLSSVTAADTAVYYCARSLARTTAMDYWGQGSLVTVSSASTKGPSVFPLAPCSRSTSESTAALGCLVKDYFPEPVTVSWNSGALTSGVHTFPAVLQSSGLYSLSSVVTVPSSSLGTKTYTCNVDHKPSNTKVDKRVESKYGPPCPPCPAPEFLGGPSVFLFPPKPKDTLMISRTPEVTCVVVDVSQEDPEVQFNWYVDGVEVHNAKTKPREEQFNSTYRVVSVLTVLHQDWLNGKEYKCKVSNKGLPSSIEKTISKAKGQPREPQVYTLPPSQEEMTKNQVSLTCLVKGFYPSDIAVEWESNGQPENNYKTWPPVLDSDGSFALYSRLTVDKSRWQEGNVFSCSVMHEALHNHYTQKSLSLSL

SEQ ID NO: 94 - protein, 444 aa, Homo sapiens
QVQLQESGPGLVRPSQTLSLTCTVSGYSITSDHAWSWVRQPPGRGLEWIGYISYSGITTYNPSLKSRVTMLRDTSKNQFSLRLSSVTAADTAVYYCARSLARTTAMDYWGQGSLVTVSSASTKGPSVFPLAPCSRSTSESTAALGCLVKDYFPEPVTVSWNSGALTSGVHTFPAVLQSSGLYSLSSVVTVPSSSLGTKTYTCNVDHKPSNTKVDKRVESKYGPPCPPCPAPEFLGGPSVFLFPPKPKDTLMISRTPEVTCVVVDVSQEDPEVQFNWYVDGVEVHNAKTKPREEQFNSTYRVVSVLTVLHQDWLNGKEYKCKVSNKGLPSSIEKTISKAKGQPREPQVYTLPPSQEEMTKNQVSLWCAVKGFYPSDIAVEWESNGQPENNYKTTPPVLDSDGSFFLVSRLTVDKSRWQEGNVFSCSVMHEALHNHYTQKSLSLSL

SEQ ID NO: 95 - protein, 444 aa, Homo sapiens
QVQLQESGPGLVRPSQTLSLTCTVSGYSITSDHAWSWVRQPPGRGLEWIGYISYSGITTYNPSLKSRVTMLRDTSKNQFSLRLSSVTAADTAVYYCARSLARTTAMDYWGQGSLVTVSSASTKGPSVFPLAPCSRSTSESTAALGCLVKDYFPEPVTVSWNSGALTSGVHTFPAVLQSSGLYSLSSVVTVPSSSLGTKTYTCNVDHKPSNTKVDKRVESKYGPPCPPCPAPEFLGGPSVFLFPPKPKDTLMISRTPEVTCVVVDVSQEDPEVQFNWYVDGVEVHNAKTKPREEQFNSTYRVVSVLTVLHQDWLNGKEYKCKVSNKGLPSSIEKTISKAKGQPREPRVYTLPPSQEEMTENQVSLTCLVKGFYPSDIAVEWESNGQPENNYKTTPPVLVSDGSFTLYSWLTVDKSRWQEGNVFSCSVMHEALHNHYTQKSLSLSL

SEQ ID NO: 96 - protein, 444 aa, Homo sapiens
QVQLQESGPGLVRPSQTLSLTCTVSGYSITSDHAWSWVRQPPGRGLEWIGYISYSGITTYNPSLKSRVTMLRDTSKNQFSLRLSSVTAADTAVYYCARSLARTTAMDYWGQGSLVTVSSASTKGPSVFPLAPCSRSTSESTAALGCLVKDYFPEPVTVSWNSGALTSGVHTFPAVLQSSGLYSLSSVVTVPSSSLGTKTYTCNVDHKPSNTKVDKRVESKYGPPCPPCPAPEFLGGPSVFLFPPKPKDTLMISRTPEVTCVVVDVSQEDPEVQFNWYVDGVEVHNAKTKPREEQFNSTYRVVSVLTVLHQDWLNGKEYKCKVSNKGLPSSIEKTISKAKGQPREPQVYTLPPSQEEMTKNQVSLTCLVKGFYPSDIAVEWESNGQPENNYLTWPPVLDSDGSFALVSRLTVDKSRWQEGNVFSCSVMHEALHNHYTQKSLSLSL

SEQ ID NO: 97 - protein, 444 aa, Homo sapiens
QVQLQESGPGLVRPSQTLSLTCTVSGYSITSDHAWSWVRQPPGRGLEWIGYISYSGITTYNPSLKSRVTMLRDTSKNQFSLRLSSVTAADTAVYYCARSLARTTAMDYWGQGSLVTVSSASTKGPSVFPLAPCSRSTSESTAALGCLVKDYFPEPVTVSWNSGALTSGVHTFPAVLQSSGLYSLSSVVTVPSSSLGTKTYTCNVDHKPSNTKVDKRVESKYGPPCPPCPAPEFLGGPSVFLFPPKPKDTLMISRTPEVTCVVVDVSQEDPEVQFNWYVDGVEVHNAKTKPREEQFNSTYRVVSVLTVLHQDWLNGKEYKCKVSNKGLPSSIEKTISKAKGQPREPQVYTLPPSQEEMTKNQVSLTCLVKGFYPSDIAVEWESNGQPENNYDTTPPVLKSDGSFFLYSDLTVDKSRWQEGNVFSCSVMHEALHNHYTQKSLSLSL

SEQ ID NO: 98 - protein, 443 aa, Homo sapiens
QVQLQESGPGLVRPSQTLSLTCTVSGYSITSDHAWSWVRQPPGRGLEWIGYISYSGITTYNPSLKSRVTMLRDTSKNQFSLRLSSVTAADTAVYYCARSLARTTAMDYWGQGSLVTVSSASTKGPSVFPLAPCSRSTSESTAALGCLVKDYFPEPVTVSWNSGALTSGVHTFPAVLQSSGLYSLSSVVTVPSSNFGTQTYTCNVDHKPSNTKVDKTVERKCCVECPPCPAPPVAGPSVFLFPPKPKDTLMISRTPEVTCVVVDVSHEDPEVQFNWYVDGVEVHNAKTKPREEQFNSTFRVVSVLTVVHQDWLNGKEYKCKVSNKGLPAPIEKTISKTKGQPREPQVYTLPPSRKEMTKNQVSLTCLVKGFYPSDIAVEWESNGQPENNYKTTPPMLKSDGSFFLYSELTVDKSRWQQGNVFSCSVMHEALHNHYTQKSLSLSP

SEQ ID NO: 99 - protein, 443 aa, Homo sapiens
QVQLQESGPGLVRPSQTLSLTCTVSGYSITSDHAWSWVRQPPGRGLEWIGYISYSGITTYNPSLKSRVTMLRDTSKNQFSLRLSSVTAADTAVYYCARSLARTTAMDYWGQGSLVTVSSASTKGPSVFPLAPCSRSTSESTAALGCLVKDYFPEPVTVSWNSGALTSGVHTFPAVLQSSGLYSLSSVVTVPSSNFGTQTYTCNVDHKPSNTKVDKTVERKCCVECPPCPAPPVAGPSVFLFPPKPKDTLMISRTPEVTCVVVDVSHEDPEVQFNWYVDGVEVHNAKTKPREEQFNSTFRVVSVLTVVHQDWLNGKEYKCKVSNKGLPAPIEKTISKTKGQPREPEVYTLPPYREEMTKNQVSLYCLVKGFYPSDIAVEWESNGQPENNYKTTPPMLDSDGSFFLTSKLTVDKSRWQQGNVFSCSVMHEALHNHYTQKSLSLSP

SEQ ID NO: 100 - protein, 443 aa, Homo sapiens
QVQLQESGPGLVRPSQTLSLTCTVSGYSITSDHAWSWVRQPPGRGLEWIGYISYSGITTYNPSLKSRVTMLRDTSKNQFSLRLSSVTAADTAVYYCARSLARTTAMDYWGQGSLVTVSSASTKGPSVFPLAPCSRSTSESTAALGCLVKDYFPEPVTVSWNSGALTSGVHTFPAVLQSSGLYSLSSVVTVPSSNFGTQTYTCNVDHKPSNTKVDKTVERKCCVECPPCPAPPVAGPSVFLFPPKPKDTLMISRTPEVTCVVVDVSHEDPEVQFNWYVDGVEVHNAKTKPREEQFNSTFRVVSVLTVVHQDWLNGKEYKCKVSNKGLPAPIEKTISKTKGQPRRPRVYTLPPSREEMTDNQVSLVCLVKGFYPSDIAVEWESNGQPENNYKTTPPMLMSDGSFFLASVLTVDKSRWQQGNVFSCSVMHEALHNHYTQKSLSLSP

SEQ ID NO: 101 - protein, 494 aa, Homo sapiens
QVQLQESGPGLVRPSQTLSLTCTVSGYSITSDHAWSWVRQPPGRGLEWIGYISYSGITTYNPSLKSRVTMLRDTSKNQFSLRLSSVTAADTAVYYCARSLARTTAMDYWGQGSLVTVSSASTKGPSVFPLAPCSRSTSGGTAALGCLVKDYFPEPVTVSWNSGALTSGVHTFPAVLQSSGLYSLSSVVTVPSSSLGTQTYTCNVNHKPSNTKVDKRVELKTPLGDTTHTCPRCPEPKSCDTPPPCPRCPEPKSCDTPPPCPRCPEPKSCDTPPPCPRCPAPELLGGPSVFLFPPKPKDTLMISRTPEVTCVVVDVSHEDPEVQFKWYVDGVEVHNAKTKPREEQYNSTFRVVSVLTVLHQDWLNGKEYKCKVSNKALPAPIEKTISKTKGQPREPQVYTLPPSREEMTKNQVSLTCLVKGFYPSDIAVEWESSGQPENNYNTTPPMLDSDGSFFLYSKLTVDKSRWQQGNIFSCSVMHEALHNRFTQKSLSLSP

SEQ ID NO: 102 - protein, 227 aa, Homo sapiens
ESKYGPPCPPCPAPEFLGGPSVFLFPPKPKDTLMISRTPEVTCVVVDVSQEDPEVQFNWYVDGVEVHNAKTKPREEQFNSTYRVVSVLTVLHQDWLNGKEYKCKVSNKGLPSSIEKTISKAKGQPREPQVYTLPPSQEEMTKNQVSLTCLVKGFYPSDIAVEWESNGQPENNYKTTPPVLDSDGSFFLYSRLTVDKSRWQEGNVFSCSVMHEALHNHYTQKSLSLSL

SEQ ID NO: 103 - protein, 226 aa, Homo sapiens
ERKCCVECPPCPAPPVAGPSVFLFPPKPKDTLMISRTPEVTCVVVDVSHEDPEVQFNWYVDGVEVHNAKTKPREEQFNSTFRVVSVLTVVHQDWLNGKEYKCKVSNKGLPAPIEKTISKTKGQPREPQVYTLPPSREEMTKNQVSLTCLVKGFYPSDIAVEWESNGQPENNYKTTPPMLDSDGSFFLYSKLTVDKSRWQQGNVFSCSVMHEALHNHYTQKSLSLSP

SEQ ID NO: 104 - protein, 443 aa, Homo sapiens
QVQLQESGPGLVRPSQTLSLTCTVSGYSITSDHAWSWVRQPPGRGLEWIGYISYSGITTYNPSLKSRVTMLRDTSKNQFSLRLSSVTAADTAVYYCARSLARTTAMDYWGQGSLVTVSSASTKGPSVFPLAPCSRSTSESTAALGCLVKDYFPEPVTVSWNSGALTSGVHTFPAVLQSSGLYSLSSVVTVPSSNFGTQTYTCNVDHKPSNTKVDKTVERKCCVECPPCPAPPVAGPSVFLFPPKPKDTLMISRTPEVTCVVVDVSHEDPEVQFNWYVDGVEVHNAKTKPREEQFNSTFRVVSVLTVVHQDWLNGKEYKCKVSNKGLPAPIEKTISKTKGQPREPQVYTLPPSRKEMTKNQVSLTCLVKGFYPSDIAVEWESNGQPENNYDTTPPMLKSDGSFFLYSKLTVDKSRWQQGNVFSCSVMHEALHNHYTQESLSLSP

SEQ ID NO: 105 - protein, 443 aa, Homo sapiens
QVQLQESGPGLVRPSQTLSLTCTVSGYSITSDHAWSWVRQPPGRGLEWIGYISYSGITTYNPSLKSRVTMLRDTSKNQFSLRLSSVTAADTAVYYCARSLARTTAMDYWGQGSLVTVSSASTKGPSVFPLAPCSRSTSESTAALGCLVKDYFPEPVTVSWNSGALTSGVHTFPAVLQSSGLYSLSSVVTVPSSNFGTQTYTCNVDHKPSNTKVDKTVERKCCVECPPCPAPPVAGPSVFLFPPKPKDTLMISRTPEVTCVVVDVSHEDPEVQFNWYVDGVEVHNAKTKPREEQFNSTFRVVSVLTVVHQDWLNGKEYKCKVSNKGLPAPIEKTISKTKGQPREPQVYTLPPSRKEMTKNQVSLTCLVKGFYPSDIAVEWESNGQPENNYDTTPPMLKSDGSFFLYSDLTVDKSRWQQGNVFSCSVMHEALHNHYTQKSLSLSP

SEQ ID NO: 106 - protein, 443 aa, Homo sapiens
QVQLQESGPGLVRPSQTLSLTCTVSGYSITSDHAWSWVRQPPGRGLEWIGYISYSGITTYNPSLKSRVTMLRDTSKNQFSLRLSSVTAADTAVYYCARSLARTTAMDYWGQGSLVTVSSASTKGPSVFPLAPCSRSTSESTAALGCLVKDYFPEPVTVSWNSGALTSGVHTFPAVLQSSGLYSLSSVVTVPSSNFGTQTYTCNVDHKPSNTKVDKTVERKCCVECPPCPAPPVAGPSVFLFPPKPKDTLMISRTPEVTCVVVDVSHEDPEVQFNWYVDGVEVHNAKTKPREEQFNSTFRVVSVLTVVHQDWLNGKEYKCKVSNKGLPAPIEKTISKTKGQPRRPQVYTLPPSREEMTENQVSLTCLVKGFYPSDIAVEWESNGQPENNYKTTPPMLMSDGSFFLASVLTVDKSRWQQGNVFSCSVMHEALHNHYTQKSLSLSP

SEQ ID NO: 107 - protein, 443 aa, Homo sapiens
QVQLQESGPGLVRPSQTLSLTCTVSGYSITSDHAWSWVRQPPGRGLEWIGYISYSGITTYNPSLKSRVTMLRDTSKNQFSLRLSSVTAADTAVYYCARSLARTTAMDYWGQGSLVTVSSASTKGPSVFPLAPCSRSTSESTAALGCLVKDYFPEPVTVSWNSGALTSGVHTFPAVLQSSGLYSLSSVVTVPSSNFGTQTYTCNVDHKPSNTKVDKTVERKCCVECPPCPAPPVAGPSVFLFPPKPKDTLMISRTPEVTCVVVDVSHEDPEVQFNWYVDGVEVHNAKTKPREEQFNSTFRVVSVLTVVHQDWLNGKEYKCKVSNKGLPAPIEKTISKTKGQPREPQVYVYPPSREEMTKNQVSLLCLVKGFYPSDIAVEWESNGQPENNYLTWPPMLDSDGSFALVSKLTVDKSRWQQGNVFSCSVMHEALHNHYTQKSLSLSP

SEQ ID NO: 108 - protein, 444 aa, Homo sapiens
QVQLQESGPGLVRPSQTLSLTCTVSGYSITSDHAWSWVRQPPGRGLEWIGYISYSGITTYNPSLKSRVTMLRDTSKNQFSLRLSSVTAADTAVYYCARSLARTTAMDYWGQGSLVTVSSASTKGPSVFPLAPCSRSTSESTAALGCLVKDYFPEPVTVSWNSGALTSGVHTFPAVLQSSGLYSLSSVVTVPSSSLGTKTYTCNVDHKPSNTKVDKRVESKYGPPCPPCPAPEFLGGPSVFLFPPKPKDTLMISRTPEVTCVVVDVSQEDPEVQFNWYVDGVEVHNAKTKPREEQFNSTYRVVSVLTVLHQDWLNGKEYKCKVSNKGLPSSIEKTISKAKGQPREPQVYTLPPSQKEMTKNQVSLTCLVKGFYPSDIAVEWESNGQPENNYDTTPPVLKSDGSFFLYSRLTVDKSRWQEGNVFSCSVMHEALHNHYTQESLSLSL

SEQ ID NO: 109 - protein, 444 aa, Homo sapiens
QVQLQESGPGLVRPSQTLSLTCTVSGYSITSDHAWSWVRQPPGRGLEWIGYISYSGITTYNPSLKSRVTMLRDTSKNQFSLRLSSVTAADTAVYYCARSLARTTAMDYWGQGSLVTVSSASTKGPSVFPLAPCSRSTSESTAALGCLVKDYFPEPVTVSWNSGALTSGVHTFPAVLQSSGLYSLSSVVTVPSSSLGTKTYTCNVDHKPSNTKVDKRVESKYGPPCPPCPAPEFLGGPSVFLFPPKPKDTLMISRTPEVTCVVVDVSQEDPEVQFNWYVDGVEVHNAKTKPREEQFNSTYRVVSVLTVLHQDWLNGKEYKCKVSNKGLPSSIEKTISKAKGQPREPQVYTLPPSQKEMTKNQVSLTCLVKGFYPSDIAVEWESNGQPENNYKTTPPVLKSDGSFFLYSELTVDKSRWQEGNVFSCSVMHEALHNHYTQESLSLSL

SEQ ID NO: 110 - protein, 444 aa, Homo sapiens
QVQLQESGPGLVRPSQTLSLTCTVSGYSITSDHAWSWVRQPPGRGLEWIGYISYSGITTYNPSLKSRVTMLRDTSKNQFSLRLSSVTAADTAVYYCARSLARTTAMDYWGQGSLVTVSSASTKGPSVFPLAPCSRSTSESTAALGCLVKDYFPEPVTVSWNSGALTSGVHTFPAVLQSSGLYSLSSVVTVPSSSLGTKTYTCNVDHKPSNTKVDKRVESKYGPPCPPCPAPEFLGGPSVFLFPPKPKDTLMISRTPEVTCVVVDVSQEDPEVQFNWYVDGVEVHNAKTKPREEQFNSTYRVVSVLTVLHQDWLNGKEYKCKVSNKGLPSSIEKTISKAKGQPREPEVYTLPPYQEEMTKNQVSLYCLVKGFYPSDIAVEWESNGQPENNYKTTPPVLDSDGSFFLTSRLTVDKSRWQEGNVFSCSVMHEALHNHYTQKSLSLSL

SEQ ID NO: 111 - protein, 444 aa, Homo sapiens
QVQLQESGPGLVRPSQTLSLTCTVSGYSITSDHAWSWVRQPPGRGLEWIGYISYSGITTYNPSLKSRVTMLRDTSKNQFSLRLSSVTAADTAVYYCARSLARTTAMDYWGQGSLVTVSSASTKGPSVFPLAPCSRSTSESTAALGCLVKDYFPEPVTVSWNSGALTSGVHTFPAVLQSSGLYSLSSVVTVPSSSLGTKTYTCNVDHKPSNTKVDKRVESKYGPPCPPCPAPEFLGGPSVFLFPPKPKDTLMISRTPEVTCVVVDVSQEDPEVQFNWYVDGVEVHNAKTKPREEQFNSTYRVVSVLTVLHQDWLNGKEYKCKVSNKGLPSSIEKTISKAKGQPRRPRVYTLPPSQEEMTDNQVSLVCLVKGFYPSDIAVEWESNGQPENNYKTTPPVLMSDGSFFLASVLTVDKSRWQEGNVFSCSVMHEALHNHYTQKSLSLSL

SEQ ID NO: 112 - protein, 444 aa, Homo sapiens
QVQLQESGPGLVRPSQTLSLTCTVSGYSITSDHAWSWVRQPPGRGLEWIGYISYSGITTYNPSLKSRVTMLRDTSKNQFSLRLSSVTAADTAVYYCARSLARTTAMDYWGQGSLVTVSSASTKGPSVFPLAPCSRSTSESTAALGCLVKDYFPEPVTVSWNSGALTSGVHTFPAVLQSSGLYSLSSVVTVPSSSLGTKTYTCNVDHKPSNTKVDKRVESKYGPPCPPCPAPEFLGGPSVFLFPPKPKDTLMISRTPEVTCVVVDVSQEDPEVQFNWYVDGVEVHNAKTKPREEQFNSTYRVVSVLTVLHQDWLNGKEYKCKVSNKGLPSSIEKTISKAKGQPREPQVYTLPPSQKEMTKNQVSLTCLVKGFYPSDIAVEWESNGQPENNYDTTPPVLKSDGSFFLYSDLTVDKSRWQEGNVFSCSVMHEALHNHYTQKSLSLSL

SEQ ID NO: 113 - protein, 444 aa, Homo sapiens
QVQLQESGPGLVRPSQTLSLTCTVSGYSITSDHAWSWVRQPPGRGLEWIGYISYSGITTYNPSLKSRVTMLRDTSKNQFSLRLSSVTAADTAVYYCARSLARTTAMDYWGQGSLVTVSSASTKGPSVFPLAPCSRSTSESTAALGCLVKDYFPEPVTVSWNSGALTSGVHTFPAVLQSSGLYSLSSVVTVPSSSLGTKTYTCNVDHKPSNTKVDKRVESKYGPPCPPCPAPEFLGGPSVFLFPPKPKDTLMISRTPEVTCVVVDVSQEDPEVQFNWYVDGVEVHNAKTKPREEQFNSTYRVVSVLTVLHQDWLNGKEYKCKVSNKGLPSSIEKTISKAKGQPRRPQVYTLPPSQEEMTENQVSLTCLVKGFYPSDIAVEWESNGQPENNYKTTPPVLMSDGSFFLASVLTVDKSRWQEGNVFSCSVMHEALHNHYTQKSLSLSL

SEQ ID NO: 114 - protein, 444 aa, Homo sapiens
QVQLQESGPGLVRPSQTLSLTCTVSGYSITSDHAWSWVRQPPGRGLEWIGYISYSGITTYNPSLKSRVTMLRDTSKNQFSLRLSSVTAADTAVYYCARSLARTTAMDYWGQGSLVTVSSASTKGPSVFPLAPCSRSTSESTAALGCLVKDYFPEPVTVSWNSGALTSGVHTFPAVLQSSGLYSLSSVVTVPSSSLGTKTYTCNVDHKPSNTKVDKRVESKYGPPCPPCPAPEFLGGPSVFLFPPKPKDTLMISRTPEVTCVVVDVSQEDPEVQFNWYVDGVEVHNAKTKPREEQFNSTYRVVSVLTVLHQDWLNGKEYKCKVSNKGLPSSIEKTISKAKGQPREPQVYVYPPSQEEMTKNQVSLLCLVKGFYPSDIAVEWESNGQPENNYLTWPPVLDSDGSFALVSRLTVDKSRWQEGNVFSCSVMHEALHNHYTQKSLSLSL

SEQ ID NO: 115 - protein, 447 aa, Homo sapiens
QVQLQESGPGLVRPSQTLSLTCTVSGYSITSDHAWSWVRQPPGRGLEWIGYISYSGITTYNPSLKSRVTMLRDTSKNQFSLRLSSVTAADTAVYYCARSLARTTAMDYWGQGSLVTVSSASTKGPSVFPLAPSSKSTSGGTAALGCLVKDYFPEPVTVSWNSGALTSGVHTFPAVLQSSGLYSLSSVVTVPSSSLGTQTYICNVNHKPSNTKVDKRVEPKSCDKTHTCPPCPAPELLGGPSVFLFPPKPKDTLMISRTPEVTCVVVDVSHEDPEVKFNWYVDGVEVHNAKTKPREEQYASTYRVVSVLTVLHQDWLNGKEYKCKVSNKALPAPIEKTISKAKGQPREPQVYTLPPSREEMTKNQVSLTCLVKGFYPSDIAVEWESNGQPENNYKTTPPVLDSDGSFFLYSKLTVDKSRWQQGNVFSCSVMHEALHNHYTQKSLSLSP

SEQ ID NO: 116 - protein, 447 aa, Homo sapiens
QVQLQESGPGLVRPSQTLSLTCTVSGYSITSDHAWSWVRQPPGRGLEWIGYISYSGITTYNPSLKSRVTMLRDTSKNQFSLRLSSVTAADTAVYYCARSLARTTAMDYWGQGSLVTVSSASTKGPSVFPLAPSSKSTSGGTAALGCLVKDYFPEPVTVSWNSGALTSGVHTFPAVLQSSGLYSLSSVVTVPSSSLGTQTYICNVNHKPSNTKVDKRVEPKSCDKTHTCPPCPAPELLGGPSVFLFPPKPKDTLMISRTPEVTCVVVDVSHEDPEVKFNWYVDGVEVHNAKTKPREEQYASTYRVVSVLTVLHQDWLNGKEYKCKVSNKALPAPIEKTISKAKGQPREPQVYTLPPSREEMTKNQVSLTCLVKGFYPSDIAVEWESNGQPENNYKTWPPVLDSDGSFALYSKLTVDKSRWQQGNVFSCSVMHEALHNHYTQKSLSLSP

SEQ ID NO: 117 - protein, 447 aa, Homo sapiens
QVQLQESGPGLVRPSQTLSLTCTVSGYSITSDHAWSWVRQPPGRGLEWIGYISYSGITTYNPSLKSRVTMLRDTSKNQFSLRLSSVTAADTAVYYCARSLARTTAMDYWGQGSLVTVSSASTKGPSVFPLAPSSKSTSGGTAALGCLVKDYFPEPVTVSWNSGALTSGVHTFPAVLQSSGLYSLSSVVTVPSSSLGTQTYICNVNHKPSNTKVDKRVEPKSCDKTHTCPPCPAPELLGGPSVFLFPPKPKDTLMISRTPEVTCVVVDVSHEDPEVKFNWYVDGVEVHNAKTKPREEQYASTYRVVSVLTVLHQDWLNGKEYKCKVSNKALPAPIEKTISKAKGQPREPQVYTLPPSREEMTKNQVSLWCAVKGFYPSDIAVEWESNGQPENNYKTTPPVLDSDGSFFLVSKLTVDKSRWQQGNVFSCSVMHEALHNHYTQKSLSLSP

SEQ ID NO: 118 - protein, 447 aa, Homo sapiens
QVQLQESGPGLVRPSQTLSLTCTVSGYSITSDHAWSWVRQPPGRGLEWIGYISYSGITTYNPSLKSRVTMLRDTSKNQFSLRLSSVTAADTAVYYCARSLARTTAMDYWGQGSLVTVSSASTKGPSVFPLAPSSKSTSGGTAALGCLVKDYFPEPVTVSWNSGALTSGVHTFPAVLQSSGLYSLSSVVTVPSSSLGTQTYICNVNHKPSNTKVDKRVEPKSCDKTHTCPPCPAPELLGGPSVFLFPPKPKDTLMISRTPEVTCVVVDVSHEDPEVKFNWYVDGVEVHNAKTKPREEQYASTYRVVSVLTVLHQDWLNGKEYKCKVSNKALPAPIEKTISKAKGQPREPRVYTLPPSREEMTENQVSLTCLVKGFYPSDIAVEWESNGQPENNYKTTPPVLVSDGSFTLYSWLTVDKSRWQQGNVFSCSVMHEALHNHYTQKSLSLSP

SEQ ID NO: 119 - protein, 447 aa, Homo sapiens
QVQLQESGPGLVRPSQTLSLTCTVSGYSITSDHAWSWVRQPPGRGLEWIGYISYSGITTYNPSLKSRVTMLRDTSKNQFSLRLSSVTAADTAVYYCARSLARTTAMDYWGQGSLVTVSSASTKGPSVFPLAPSSKSTSGGTAALGCLVKDYFPEPVTVSWNSGALTSGVHTFPAVLQSSGLYSLSSVVTVPSSSLGTQTYICNVNHKPSNTKVDKRVEPKSCDKTHTCPPCPAPELLGGPSVFLFPPKPKDTLMISRTPEVTCVVVDVSHEDPEVKFNWYVDGVEVHNAKTKPREEQYASTYRVVSVLTVLHQDWLNGKEYKCKVSNKALPAPIEKTISKAKGQPREPQVYTLPPSRKEMTKNQVSLTCLVKGFYPSDIAVEWESNGQPENNYKTTPPVLKSDGSFFLYSELTVDKSRWQQGNVFSCSVMHEALHNHYTQESLSLSP

SEQ ID NO: 120 - protein, 447 aa, Homo sapiens
QVQLQESGPGLVRPSQTLSLTCTVSGYSITSDHAWSWVRQPPGRGLEWIGYISYSGITTYNPSLKSRVTMLRDTSKNQFSLRLSSVTAADTAVYYCARSLARTTAMDYWGQGSLVTVSSASTKGPSVFPLAPSSKSTSGGTAALGCLVKDYFPEPVTVSWNSGALTSGVHTFPAVLQSSGLYSLSSVVTVPSSSLGTQTYICNVNHKPSNTKVDKRVEPKSCDKTHTCPPCPAPELLGGPSVFLFPPKPKDTLMISRTPEVTCVVVDVSHEDPEVKFNWYVDGVEVHNAKTKPREEQYASTYRVVSVLTVLHQDWLNGKEYKCKVSNKALPAPIEKTISKAKGQPREPQVYTLPPSRKEMTKNQVSLTCLVKGFYPSDIAVEWESNGQPENNYDTTPPVLKSDGSFFLYSKLTVDKSRWQQGNVFSCSVMHEALHNHYTQESLSLSP

SEQ ID NO: 121 - protein, 447 aa, Homo sapiens
QVQLQESGPGLVRPSQTLSLTCTVSGYSITSDHAWSWVRQPPGRGLEWIGYISYSGITTYNPSLKSRVTMLRDTSKNQFSLRLSSVTAADTAVYYCARSLARTTAMDYWGQGSLVTVSSASTKGPSVFPLAPSSKSTSGGTAALGCLVKDYFPEPVTVSWNSGALTSGVHTFPAVLQSSGLYSLSSVVTVPSSSLGTQTYICNVNHKPSNTKVDKRVEPKSCDKTHTCPPCPAPELLGGPSVFLFPPKPKDTLMISRTPEVTCVVVDVSHEDPEVKFNWYVDGVEVHNAKTKPREEQYASTYRVVSVLTVLHQDWLNGKEYKCKVSNKALPAPIEKTISKAKGQPREPQVYTLPPSREEMTKNQVSLTCLVKGFYPSDIAVEWESNGQPENNYDTTPPVLKSDGSFFLYSDLTVDKSRWQQGNVFSCSVMHEALHNHYTQKSLSLSP

SEQ ID NO: 122 - protein, 447 aa, Homo sapiens
QVQLQESGPGLVRPSQTLSLTCTVSGYSITSDHAWSWVRQPPGRGLEWIGYISYSGITTYNPSLKSRVTMLRDTSKNQFSLRLSSVTAADTAVYYCARSLARTTAMDYWGQGSLVTVSSASTKGPSVFPLAPSSKSTSGGTAALGCLVKDYFPEPVTVSWNSGALTSGVHTFPAVLQSSGLYSLSSVVTVPSSSLGTQTYICNVNHKPSNTKVDKRVEPKSCDKTHTCPPCPAPELLGGPSVFLFPPKPKDTLMISRTPEVTCVVVDVSHEDPEVKFNWYVDGVEVHNAKTKPREEQYASTYRVVSVLTVLHQDWLNGKEYKCKVSNKALPAPIEKTISKAKGQPRRPQVYTLPPSREEMTENQVSLTCLVKGFYPSDIAVEWESNGQPENNYKTTPPVLMSDGSFFLASVLTVDKSRWQQGNVFSCSVMHEALHNHYTQKSLSLSP

SEQ ID NO: 123 - protein, 447 aa, Homo sapiens
QVQLQESGPGLVRPSQTLSLTCTVSGYSITSDHAWSWVRQPPGRGLEWIGYISYSGITTYNPSLKSRVTMLRDTSKNQFSLRLSSVTAADTAVYYCARSLARTTAMDYWGQGSLVTVSSASTKGPSVFPLAPSSKSTSGGTAALGCLVKDYFPEPVTVSWNSGALTSGVHTFPAVLQSSGLYSLSSVVTVPSSSLGTQTYICNVNHKPSNTKVDKRVEPKSCDKTHTCPPCPAPELLGGPSVFLFPPKPKDTLMISRTPEVTCVVVDVSHEDPEVKFNWYVDGVEVHNAKTKPREEQYASTYRVVSVLTVLHQDWLNGKEYKCKVSNKALPAPIEKTISKAKGQPREPQVYVYPPSREEMTKNQVSLLCLVKGFYPSDIAVEWESNGQPENNYLTWPPVLDSDGSFALVSKLTVDKSRWQQGNVFSCSVMHEALHNHYTQKSLSLSP

SEQ ID NO: 124 - protein, 447 aa, Homo sapiens
QVQLQESGPGLVRPSQTLSLTCTVSGYSITSDHAWSWVRQPPGRGLEWIGYISYSGITTYNPSLKSRVTMLRDTSKNQFSLRLSSVTAADTAVYYCARSLARTTAMDYWGQGSLVTVSSASTKGPSVFPLAPSSKSTSGGTAALGCLVKDYFPEPVTVSWNSGALTSGVHTFPAVLQSSGLYSLSSVVTVPSSSLGTQTYICNVNHKPSNTKVDKRVEPKSCDKTHTCPPCPAPELLGGPSVFLFPPKPKDTLMISRTPEVTCVVVDVSHEDPEVKFNWYVDGVEVHNAKTKPREEQYNSTYRVVSVLTVLHQDWLNGKEYKCKVSNKALPAPIEKTISKAKGQPREPQVYTLPPSREEMTKNQVSLTCLVKGFYPSDIAVEWESNGQPENNYKTTPPVLDSDGSFFLYSKLTVDKSRWQQGNVFSCSVLHEALHAHTTRKELSLSP

SEQ ID NO: 125 - protein, 447 aa, Homo sapiens
QVQLQESGPGLVRPSQTLSLTCTVSGYSITSDHAWSWVRQPPGRGLEWIGYISYSGITTYNPSLKSRVTMLRDTSKNQFSLRLSSVTAADTAVYYCARSLARTTAMDYWGQGSLVTVSSASTKGPSVFPLAPSSKSTSGGTAALGCLVKDYFPEPVTVSWNSGALTSGVHTFPAVLQSSGLYSLSSVVTVPSSSLGTQTYICNVNHKPSNTKVDKRVEPKSCDKTHTCPPCPAPELLGGPSVFLFPPKPKDTLMISRTPEVTCVVVDVSHEDPEVKFNWYVDGVEVHNAKTKPREEQYNSTYRVVSVLTVLHQDWLNGKEYKCKVSNKALPAPIEKTISKAKGQPREPQVYTLPPSREEMTKNQVSLTCLVKGFYPSDIAVEWESNGQPENNYKTWPPVLDSDGSFALYSKLTVDKSRWQQGNVFSCSVLHEALHAHTTRKELSLSP

SEQ ID NO: 126 - protein, 447 aa, Homo sapiens
QVQLQESGPGLVRPSQTLSLTCTVSGYSITSDHAWSWVRQPPGRGLEWIGYISYSGITTYNPSLKSRVTMLRDTSKNQFSLRLSSVTAADTAVYYCARSLARTTAMDYWGQGSLVTVSSASTKGPSVFPLAPSSKSTSGGTAALGCLVKDYFPEPVTVSWNSGALTSGVHTFPAVLQSSGLYSLSSVVTVPSSSLGTQTYICNVNHKPSNTKVDKRVEPKSCDKTHTCPPCPAPELLGGPSVFLFPPKPKDTLMISRTPEVTCVVVDVSHEDPEVKFNWYVDGVEVHNAKTKPREEQYNSTYRVVSVLTVLHQDWLNGKEYKCKVSNKALPAPIEKTISKAKGQPREPQVYTLPPSREEMTKNQVSLWCAVKGFYPSDIAVEWESNGQPENNYKTTPPVLDSDGSFFLVSKLTVDKSRWQQGNVFSCSVLHEALHAHTTRKELSLSP

SEQ ID NO: 127 - protein, 447 aa, Homo sapiens
QVQLQESGPGLVRPSQTLSLTCTVSGYSITSDHAWSWVRQPPGRGLEWIGYISYSGITTYNPSLKSRVTMLRDTSKNQFSLRLSSVTAADTAVYYCARSLARTTAMDYWGQGSLVTVSSASTKGPSVFPLAPSSKSTSGGTAALGCLVKDYFPEPVTVSWNSGALTSGVHTFPAVLQSSGLYSLSSVVTVPSSSLGTQTYICNVNHKPSNTKVDKRVEPKSCDKTHTCPPCPAPELLGGPSVFLFPPKPKDTLMISRTPEVTCVVVDVSHEDPEVKFNWYVDGVEVHNAKTKPREEQYNSTYRVVSVLTVLHQDWLNGKEYKCKVSNKALPAPIEKTISKAKGQPREPRVYTLPPSREEMTENQVSLTCLVKGFYPSDIAVEWESNGQPENNYKTTPPVLVSDGSFTLYSWLTVDKSRWQQGNVFSCSVLHEALHAHTTRKELSLSP

SEQ ID NO: 128 - protein, 447 aa, Homo sapiens
QVQLQESGPGLVRPSQTLSLTCTVSGYSITSDHAWSWVRQPPGRGLEWIGYISYSGITTYNPSLKSRVTMLRDTSKNQFSLRLSSVTAADTAVYYCARSLARTTAMDYWGQGSLVTVSSASTKGPSVFPLAPSSKSTSGGTAALGCLVKDYFPEPVTVSWNSGALTSGVHTFPAVLQSSGLYSLSSVVTVPSSSLGTQTYICNVNHKPSNTKVDKRVEPKSCDKTHTCPPCPAPELLGGPSVFLFPPKPKDTLMISRTPEVTCVVVDVSHEDPEVKFNWYVDGVEVHNAKTKPREEQYNSTYRVVSVLTVLHQDWLNGKEYKCKVSNKALPAPIEKTISKAKGQPREPQVYTLPPSRKEMTKNQVSLTCLVKGFYPSDIAVEWESNGQPENNYKTTPPVLKSDGSFFLYSELTVDKSRWQQGNVFSCSVLHEALHAHTTREELSLSP

SEQ ID NO: 129 - protein, 447 aa, Homo sapiens
QVQLQESGPGLVRPSQTLSLTCTVSGYSITSDHAWSWVRQPPGRGLEWIGYISYSGITTYNPSLKSRVTMLRDTSKNQFSLRLSSVTAADTAVYYCARSLARTTAMDYWGQGSLVTVSSASTKGPSVFPLAPSSKSTSGGTAALGCLVKDYFPEPVTVSWNSGALTSGVHTFPAVLQSSGLYSLSSVVTVPSSSLGTQTYICNVNHKPSNTKVDKRVEPKSCDKTHTCPPCPAPELLGGPSVFLFPPKPKDTLMISRTPEVTCVVVDVSHEDPEVKFNWYVDGVEVHNAKTKPREEQYNSTYRVVSVLTVLHQDWLNGKEYKCKVSNKALPAPIEKTISKAKGQPREPQVYTLPPSRKEMTKNQVSLTCLVKGFYPSDIAVEWESNGQPENNYDTTPPVLKSDGSFFLYSKLTVDKSRWQQGNVFSCSVLHEALHAHTTREELSLSP

SEQ ID NO: 130 - protein, 447 aa, Homo sapiens
QVQLQESGPGLVRPSQTLSLTCTVSGYSITSDHAWSWVRQPPGRGLEWIGYISYSGITTYNPSLKSRVTMLRDTSKNQFSLRLSSVTAADTAVYYCARSLARTTAMDYWGQGSLVTVSSASTKGPSVFPLAPSSKSTSGGTAALGCLVKDYFPEPVTVSWNSGALTSGVHTFPAVLQSSGLYSLSSVVTVPSSSLGTQTYICNVNHKPSNTKVDKRVEPKSCDKTHTCPPCPAPELLGGPSVFLFPPKPKDTLMISRTPEVTCVVVDVSHEDPEVKFNWYVDGVEVHNAKTKPREEQYNSTYRVVSVLTVLHQDWLNGKEYKCKVSNKALPAPIEKTISKAKGQPREPQVYTLPPSREEMTKNQVSLTCLVKGFYPSDIAVEWESNGQPENNYDTTPPVLKSDGSFFLYSDLTVDKSRWQQGNVFSCSVLHEALHAHTTRKELSLSP

SEQ ID NO: 131 - protein, 447 aa, Homo sapiens
QVQLQESGPGLVRPSQTLSLTCTVSGYSITSDHAWSWVRQPPGRGLEWIGYISYSGITTYNPSLKSRVTMLRDTSKNQFSLRLSSVTAADTAVYYCARSLARTTAMDYWGQGSLVTVSSASTKGPSVFPLAPSSKSTSGGTAALGCLVKDYFPEPVTVSWNSGALTSGVHTFPAVLQSSGLYSLSSVVTVPSSSLGTQTYICNVNHKPSNTKVDKRVEPKSCDKTHTCPPCPAPELLGGPSVFLFPPKPKDTLMISRTPEVTCVVVDVSHEDPEVKFNWYVDGVEVHNAKTKPREEQYNSTYRVVSVLTVLHQDWLNGKEYKCKVSNKALPAPIEKTISKAKGQPRRPQVYTLPPSREEMTENQVSLTCLVKGFYPSDIAVEWESNGQPENNYKTTPPVLMSDGSFFLASVLTVDKSRWQQGNVFSCSVLHEALHAHTTRKELSLSP

SEQ ID NO: 132 - protein, 447 aa, Homo sapiens
QVQLQESGPGLVRPSQTLSLTCTVSGYSITSDHAWSWVRQPPGRGLEWIGYISYSGITTYNPSLKSRVTMLRDTSKNQFSLRLSSVTAADTAVYYCARSLARTTAMDYWGQGSLVTVSSASTKGPSVFPLAPSSKSTSGGTAALGCLVKDYFPEPVTVSWNSGALTSGVHTFPAVLQSSGLYSLSSVVTVPSSSLGTQTYICNVNHKPSNTKVDKRVEPKSCDKTHTCPPCPAPELLGGPSVFLFPPKPKDTLMISRTPEVTCVVVDVSHEDPEVKFNWYVDGVEVHNAKTKPREEQYNSTYRVVSVLTVLHQDWLNGKEYKCKVSNKALPAPIEKTISKAKGQPREPQVYVYPPSREEMTKNQVSLLCLVKGFYPSDIAVEWESNGQPENNYLTWPPVLDSDGSFALVSKLTVDKSRWQQGNVFSCSVLHEALHAHTTRKELSLSP

SEQ ID NO: 133 - protein, 447 aa, Homo sapiens
QVQLQESGPGLVRPSQTLSLTCTVSGYSITSDHAWSWVRQPPGRGLEWIGYISYSGITTYNPSLKSRVTMLRDTSKNQFSLRLSSVTAADTAVYYCARSLARTTAMDYWGQGSLVTVSSASTKGPSVFPLAPSSKSTSGGTAALGCLVKDYFPEPVTVSWNSGALTSGVHTFPAVLQSSGLYSLSSVVTVPSSSLGTQTYICNVNHKPSNTKVDKRVEPKSCDKTHTCPPCPAPELRRGPSVFLFPPKPKDTLMISRTPEVTCVVVDVSHEDPEVKFNWYVDGVEVHNAKTKPREEQYNSTYRVVSVLTVLHQDWLNGKEYKCKVSNKALPAPIEKTISKAKGQPREPQVYTLPPSREEMTKNQVSLTCLVKGFYPSDIAVEWESNGQPENNYKTTPPVLDSDGSFFLYSKLTVDKSRWQQGNVFSCSVMHEALHNHYTQKSLSLSP

SEQ ID NO: 134 - protein, 447 aa, Homo sapiens
QVQLQESGPGLVRPSQTLSLTCTVSGYSITSDHAWSWVRQPPGRGLEWIGYISYSGITTYNPSLKSRVTMLRDTSKNQFSLRLSSVTAADTAVYYCARSLARTTAMDYWGQGSLVTVSSASTKGPSVFPLAPSSKSTSGGTAALGCLVKDYFPEPVTVSWNSGALTSGVHTFPAVLQSSGLYSLSSVVTVPSSSLGTQTYICNVNHKPSNTKVDKRVEPKSCDKTHTCPPCPAPELRRGPSVFLFPPKPKDTLMISRTPEVTCVVVDVSHEDPEVKFNWYVDGVEVHNAKTKPREEQYNSTYRVVSVLTVLHQDWLNGKEYKCKVSNKALPAPIEKTISKAKGQPREPQVYTLPPSREEMTKNQVSLTCLVKGFYPSDIAVEWESNGQPENNYKTWPPVLDSDGSFALYSKLTVDKSRWQQGNVFSCSVMHEALHNHYTQKSLSLSP

SEQ ID NO: 135 - protein, 447 aa, Homo sapiens
QVQLQESGPGLVRPSQTLSLTCTVSGYSITSDHAWSWVRQPPGRGLEWIGYISYSGITTYNPSLKSRVTMLRDTSKNQFSLRLSSVTAADTAVYYCARSLARTTAMDYWGQGSLVTVSSASTKGPSVFPLAPSSKSTSGGTAALGCLVKDYFPEPVTVSWNSGALTSGVHTFPAVLQSSGLYSLSSVVTVPSSSLGTQTYICNVNHKPSNTKVDKRVEPKSCDKTHTCPPCPAPELRRGPSVFLFPPKPKDTLMISRTPEVTCVVVDVSHEDPEVKFNWYVDGVEVHNAKTKPREEQYNSTYRVVSVLTVLHQDWLNGKEYKCKVSNKALPAPIEKTISKAKGQPREPQVYTLPPSREEMTKNQVSLWCAVKGFYPSDIAVEWESNGQPENNYKTTPPVLDSDGSFFLVSKLTVDKSRWQQGNVFSCSVMHEALHNHYTQKSLSLSP

SEQ ID NO: 136 - protein, 447 aa, Homo sapiens
QVQLQESGPGLVRPSQTLSLTCTVSGYSITSDHAWSWVRQPPGRGLEWIGYISYSGITTYNPSLKSRVTMLRDTSKNQFSLRLSSVTAADTAVYYCARSLARTTAMDYWGQGSLVTVSSASTKGPSVFPLAPSSKSTSGGTAALGCLVKDYFPEPVTVSWNSGALTSGVHTFPAVLQSSGLYSLSSVVTVPSSSLGTQTYICNVNHKPSNTKVDKRVEPKSCDKTHTCPPCPAPELRRGPSVFLFPPKPKDTLMISRTPEVTCVVVDVSHEDPEVKFNWYVDGVEVHNAKTKPREEQYNSTYRVVSVLTVLHQDWLNGKEYKCKVSNKALPAPIEKTISKAKGQPREPRVYTLPPSREEMTENQVSLTCLVKGFYPSDIAVEWESNGQPENNYKTTPPVLVSDGSFTLYSWLTVDKSRWQQGNVFSCSVMHEALHNHYTQKSLSLSP

SEQ ID NO: 137 - protein, 447 aa, Homo sapiens
QVQLQESGPGLVRPSQTLSLTCTVSGYSITSDHAWSWVRQPPGRGLEWIGYISYSGITTYNPSLKSRVTMLRDTSKNQFSLRLSSVTAADTAVYYCARSLARTTAMDYWGQGSLVTVSSASTKGPSVFPLAPSSKSTSGGTAALGCLVKDYFPEPVTVSWNSGALTSGVHTFPAVLQSSGLYSLSSVVTVPSSSLGTQTYICNVNHKPSNTKVDKRVEPKSCDKTHTCPPCPAPELRRGPSVFLFPPKPKDTLMISRTPEVTCVVVDVSHEDPEVKFNWYVDGVEVHNAKTKPREEQYNSTYRVVSVLTVLHQDWLNGKEYKCKVSNKALPAPIEKTISKAKGQPREPQVYTLPPSRKEMTKNQVSLTCLVKGFYPSDIAVEWESNGQPENNYDTTPPVLKSDGSFFLYSKLTVDKSRWQQGNVFSCSVMHEALHNHYTQESLSLSP

SEQ ID NO: 138 - protein, 447 aa, Homo sapiens
QVQLQESGPGLVRPSQTLSLTCTVSGYSITSDHAWSWVRQPPGRGLEWIGYISYSGITTYNPSLKSRVTMLRDTSKNQFSLRLSSVTAADTAVYYCARSLARTTAMDYWGQGSLVTVSSASTKGPSVFPLAPSSKSTSGGTAALGCLVKDYFPEPVTVSWNSGALTSGVHTFPAVLQSSGLYSLSSVVTVPSSSLGTQTYICNVNHKPSNTKVDKRVEPKSCDKTHTCPPCPAPEAAGGPSVFLFPPKPKDTLMISRTPEVTCVVVDVSHEDPEVKFNWYVDGVEVHNAKTKPREEQYNSTYRVVSVLTVLHQDWLNGKEYKCKVSNKALPAPIEKTISKAKGQPREPQVYTLPPSREEMTKNQVSLTCLVKGFYPSDIAVEWESNGQPENNYKTTPPVLDSDGSFFLYSKLTVDKSRWQQGNVFSCSVMHEALHNHYTQKSLSLSP

SEQ ID NO: 139 - protein, 447 aa, Homo sapiens
QVQLQESGPGLVRPSQTLSLTCTVSGYSITSDHAWSWVRQPPGRGLEWIGYISYSGITTYNPSLKSRVTMLRDTSKNQFSLRLSSVTAADTAVYYCARSLARTTAMDYWGQGSLVTVSSASTKGPSVFPLAPSSKSTSGGTAALGCLVKDYFPEPVTVSWNSGALTSGVHTFPAVLQSSGLYSLSSVVTVPSSSLGTQTYICNVNHKPSNTKVDKRVEPKSCDKTHTCPPCPAPEAAGGPSVFLFPPKPKDTLMISRTPEVTCVVVDVSHEDPEVKFNWYVDGVEVHNAKTKPREEQYNSTYRVVSVLTVLHQDWLNGKEYKCKVSNKALPAPIEKTISKAKGQPREPQVYTLPPSREEMTKNQVSLTCLVKGFYPSDIAVEWESNGQPENNYKTWPPVLDSDGSFALYSKLTVDKSRWQQGNVFSCSVMHEALHNHYTQKSLSLSP

SEQ ID NO: 140 - protein, 447 aa, Homo sapiens
QVQLQESGPGLVRPSQTLSLTCTVSGYSITSDHAWSWVRQPPGRGLEWIGYISYSGITTYNPSLKSRVTMLRDTSKNQFSLRLSSVTAADTAVYYCARSLARTTAMDYWGQGSLVTVSSASTKGPSVFPLAPSSKSTSGGTAALGCLVKDYFPEPVTVSWNSGALTSGVHTFPAVLQSSGLYSLSSVVTVPSSSLGTQTYICNVNHKPSNTKVDKRVEPKSCDKTHTCPPCPAPEAAGGPSVFLFPPKPKDTLMISRTPEVTCVVVDVSHEDPEVKFNWYVDGVEVHNAKTKPREEQYNSTYRVVSVLTVLHQDWLNGKEYKCKVSNKALPAPIEKTISKAKGQPREPQVYTLPPSREEMTKNQVSLWCAVKGFYPSDIAVEWESNGQPENNYKTTPPVLDSDGSFFLVSKLTVDKSRWQQGNVFSCSVMHEALHNHYTQKSLSLSP

SEQ ID NO: 141 - protein, 447 aa, Homo sapiens
QVQLQESGPGLVRPSQTLSLTCTVSGYSITSDHAWSWVRQPPGRGLEWIGYISYSGITTYNPSLKSRVTMLRDTSKNQFSLRLSSVTAADTAVYYCARSLARTTAMDYWGQGSLVTVSSASTKGPSVFPLAPSSKSTSGGTAALGCLVKDYFPEPVTVSWNSGALTSGVHTFPAVLQSSGLYSLSSVVTVPSSSLGTQTYICNVNHKPSNTKVDKRVEPKSCDKTHTCPPCPAPEAAGGPSVFLFPPKPKDTLMISRTPEVTCVVVDVSHEDPEVKFNWYVDGVEVHNAKTKPREEQYNSTYRVVSVLTVLHQDWLNGKEYKCKVSNKALPAPIEKTISKAKGQPREPRVYTLPPSREEMTENQVSLTCLVKGFYPSDIAVEWESNGQPENNYKTTPPVLVSDGSFTLYSWLTVDKSRWQQGNVFSCSVMHEALHNHYTQKSLSLSP

SEQ ID NO: 142 - protein, 447 aa, Homo sapiens
QVQLQESGPGLVRPSQTLSLTCTVSGYSITSDHAWSWVRQPPGRGLEWIGYISYSGITTYNPSLKSRVTMLRDTSKNQFSLRLSSVTAADTAVYYCARSLARTTAMDYWGQGSLVTVSSASTKGPSVFPLAPSSKSTSGGTAALGCLVKDYFPEPVTVSWNSGALTSGVHTFPAVLQSSGLYSLSSVVTVPSSSLGTQTYICNVNHKPSNTKVDKRVEPKSCDKTHTCPPCPAPEAAGGPSVFLFPPKPKDTLMISRTPEVTCVVVDVSHEDPEVKFNWYVDGVEVHNAKTKPREEQYNSTYRVVSVLTVLHQDWLNGKEYKCKVSNKALPAPIEKTISKAKGQPREPQVYTLPPSRKEMTKNQVSLTCLVKGFYPSDIAVEWESNGQPENNYDTTPPVLKSDGSFFLYSKLTVDKSRWQQGNVFSCSVMHEALHNHYTQESLSLSP

SEQ ID NO: 143 - protein, 447 aa, Homo sapiens
QVQLQESGPGLVRPSQTLSLTCTVSGYSITSDHAWSWVRQPPGRGLEWIGYISYSGITTYNPSLKSRVTMLRDTSKNQFSLRLSSVTAADTAVYYCARSLARTTAMDYWGQGSLVTVSSASTKGPSVFPLAPSSKSTSGGTAALGCLVKDYFPEPVTVSWNSGALTSGVHTFPAVLQSSGLYSLSSVVTVPSSSLGTQTYICNVNHKPSNTKVDKRVEPKSCDKTHTCPPCPAPELLGGPSVFLFPPKPKDTLYITREPEVTCVVVDVSHEDPEVKFNWYVDGVEVHNAKTKPREEQYNSTYRVVSVLTVLHQDWLNGKEYKCKVSNKALPAPIEKTISKAKGQPREPQVYTLPPSREEMTKNQVSLTCLVKGFYPSDIAVEWESNGQPENNYKTTPPVLDSDGSFFLYSKLTVDKSRWQQGNVFSCSVMHEALHNHYTQKSLSLSP

SEQ ID NO: 144 - protein, 447 aa, Homo sapiens
QVQLQESGPGLVRPSQTLSLTCTVSGYSITSDHAWSWVRQPPGRGLEWIGYISYSGITTYNPSLKSRVTMLRDTSKNQFSLRLSSVTAADTAVYYCARSLARTTAMDYWGQGSLVTVSSASTKGPSVFPLAPSSKSTSGGTAALGCLVKDYFPEPVTVSWNSGALTSGVHTFPAVLQSSGLYSLSSVVTVPSSSLGTQTYICNVNHKPSNTKVDKRVEPKSCDKTHTCPPCPAPELLGGPSVFLFPPKPKDTLYITREPEVTCVVVDVSHEDPEVKFNWYVDGVEVHNAKTKPREEQYNSTYRVVSVLTVLHQDWLNGKEYKCKVSNKALPAPIEKTISKAKGQPREPQVYTLPPSREEMTKNQVSLTCLVKGFYPSDIAVEWESNGQPENNYKTWPPVLDSDGSFALYSKLTVDKSRWQQGNVFSCSVMHEALHNHYTQKSLSLSP

SEQ ID NO: 145 - protein, 447 aa, Homo sapiens
QVQLQESGPGLVRPSQTLSLTCTVSGYSITSDHAWSWVRQPPGRGLEWIGYISYSGITTYNPSLKSRVTMLRDTSKNQFSLRLSSVTAADTAVYYCARSLARTTAMDYWGQGSLVTVSSASTKGPSVFPLAPSSKSTSGGTAALGCLVKDYFPEPVTVSWNSGALTSGVHTFPAVLQSSGLYSLSSVVTVPSSSLGTQTYICNVNHKPSNTKVDKRVEPKSCDKTHTCPPCPAPELLGGPSVFLFPPKPKDTLYITREPEVTCVVVDVSHEDPEVKFNWYVDGVEVHNAKTKPREEQYNSTYRVVSVLTVLHQDWLNGKEYKCKVSNKALPAPIEKTISKAKGQPREPQVYTLPPSREEMTKNQVSLWCAVKGFYPSDIAVEWESNGQPENNYKTTPPVLDSDGSFFLVSKLTVDKSRWQQGNVFSCSVMHEALHNHYTQKSLSLSP

SEQ ID NO: 146 - protein, 447 aa, Homo sapiens
QVQLQESGPGLVRPSQTLSLTCTVSGYSITSDHAWSWVRQPPGRGLEWIGYISYSGITTYNPSLKSRVTMLRDTSKNQFSLRLSSVTAADTAVYYCARSLARTTAMDYWGQGSLVTVSSASTKGPSVFPLAPSSKSTSGGTAALGCLVKDYFPEPVTVSWNSGALTSGVHTFPAVLQSSGLYSLSSVVTVPSSSLGTQTYICNVNHKPSNTKVDKRVEPKSCDKTHTCPPCPAPELLGGPSVFLFPPKPKDTLYITREPEVTCVVVDVSHEDPEVKFNWYVDGVEVHNAKTKPREEQYNSTYRVVSVLTVLHQDWLNGKEYKCKVSNKALPAPIEKTISKAKGQPREPRVYTLPPSREEMTENQVSLTCLVKGFYPSDIAVEWESNGQPENNYKTTPPVLVSDGSFTLYSWLTVDKSRWQQGNVFSCSVMHEALHNHYTQKSLSLSP

SEQ ID NO: 147 - protein, 447 aa, Homo sapiens
QVQLQESGPGLVRPSQTLSLTCTVSGYSITSDHAWSWVRQPPGRGLEWIGYISYSGITTYNPSLKSRVTMLRDTSKNQFSLRLSSVTAADTAVYYCARSLARTTAMDYWGQGSLVTVSSASTKGPSVFPLAPSSKSTSGGTAALGCLVKDYFPEPVTVSWNSGALTSGVHTFPAVLQSSGLYSLSSVVTVPSSSLGTQTYICNVNHKPSNTKVDKRVEPKSCDKTHTCPPCPAPELLGGPSVFLFPPKPKDTLYITREPEVTCVVVDVSHEDPEVKFNWYVDGVEVHNAKTKPREEQYNSTYRVVSVLTVLHQDWLNGKEYKCKVSNKALPAPIEKTISKAKGQPREPQVYTLPPSRKEMTKNQVSLTCLVKGFYPSDIAVEWESNGQPENNYDTTPPVLKSDGSFFLYSKLTVDKSRWQQGNVFSCSVMHEALHNHYTQESLSLSP

SEQ ID NO: 148 - protein, 447 aa, Homo sapiens
QVQLQESGPGLVRPSQTLSLTCTVSGYSITSDHAWSWVRQPPGRGLEWIGYISYSGITTYNPSLKSRVTMLRDTSKNQFSLRLSSVTAADTAVYYCARSLARTTAMDYWGQGSLVTVSSASTKGPSVFPLAPSSKSTSGGTAALGCLVKDYFPEPVTVSWNSGALTSGVHTFPAVLQSSGLYSLSSVVTVPSSSLGTQTYICNVNHKPSNTKVDKRVEPKSCDKTHTCPPCPAPELLGGPSVFLFPPKPKDTLMISRTPEVTCVVVDVSHEDPEVKFNWYVDGVEVHNAKTKPREEQYNSTYRVVSVLTVLHQDWLNGKEYKCKVSNKALPAPIEKTISKAKGQPREPQVYTLPPSREEMTKNQVSLTCLVKGFYPSDIAVEWESNGQPENNYKTTPPVLDSDGSFFLYSKLTVDKSRWQQGNVFSCSVLHEALHSHYTQKSLSLSP

SEQ ID NO: 149 - protein, 447 aa, Homo sapiens
QVQLQESGPGLVRPSQTLSLTCTVSGYSITSDHAWSWVRQPPGRGLEWIGYISYSGITTYNPSLKSRVTMLRDTSKNQFSLRLSSVTAADTAVYYCARSLARTTAMDYWGQGSLVTVSSASTKGPSVFPLAPSSKSTSGGTAALGCLVKDYFPEPVTVSWNSGALTSGVHTFPAVLQSSGLYSLSSVVTVPSSSLGTQTYICNVNHKPSNTKVDKRVEPKSCDKTHTCPPCPAPELLGGPSVFLFPPKPKDTLMISRTPEVTCVVVDVSHEDPEVKFNWYVDGVEVHNAKTKPREEQYNSTYRVVSVLTVLHQDWLNGKEYKCKVSNKALPAPIEKTISKAKGQPREPQVYTLPPSREEMTKNQVSLTCLVKGFYPSDIAVEWESNGQPENNYKTWPPVLDSDGSFALYSKLTVDKSRWQQGNVFSCSVLHEALHSHYTQKSLSLSP

SEQ ID NO: 150 - protein, 447 aa, Homo sapiens
QVQLQESGPGLVRPSQTLSLTCTVSGYSITSDHAWSWVRQPPGRGLEWIGYISYSGITTYNPSLKSRVTMLRDTSKNQFSLRLSSVTAADTAVYYCARSLARTTAMDYWGQGSLVTVSSASTKGPSVFPLAPSSKSTSGGTAALGCLVKDYFPEPVTVSWNSGALTSGVHTFPAVLQSSGLYSLSSVVTVPSSSLGTQTYICNVNHKPSNTKVDKRVEPKSCDKTHTCPPCPAPELLGGPSVFLFPPKPKDTLMISRTPEVTCVVVDVSHEDPEVKFNWYVDGVEVHNAKTKPREEQYNSTYRVVSVLTVLHQDWLNGKEYKCKVSNKALPAPIEKTISKAKGQPREPQVYTLPPSREEMTKNQVSLWCAVKGFYPSDIAVEWESNGQPENNYKTTPPVLDSDGSFFLVSKLTVDKSRWQQGNVFSCSVLHEALHSHYTQKSLSLSP

SEQ ID NO: 151 - protein, 447 aa, Homo sapiens
QVQLQESGPGLVRPSQTLSLTCTVSGYSITSDHAWSWVRQPPGRGLEWIGYISYSGITTYNPSLKSRVTMLRDTSKNQFSLRLSSVTAADTAVYYCARSLARTTAMDYWGQGSLVTVSSASTKGPSVFPLAPSSKSTSGGTAALGCLVKDYFPEPVTVSWNSGALTSGVHTFPAVLQSSGLYSLSSVVTVPSSSLGTQTYICNVNHKPSNTKVDKRVEPKSCDKTHTCPPCPAPELLGGPSVFLFPPKPKDTLMISRTPEVTCVVVDVSHEDPEVKFNWYVDGVEVHNAKTKPREEQYNSTYRVVSVLTVLHQDWLNGKEYKCKVSNKALPAPIEKTISKAKGQPREPRVYTLPPSREEMTENQVSLTCLVKGFYPSDIAVEWESNGQPENNYKTTPPVLVSDGSFTLYSWLTVDKSRWQQGNVFSCSVLHEALHSHYTQKSLSLSP

SEQ ID NO: 152 - protein, 447 aa, Homo sapiens
QVQLQESGPGLVRPSQTLSLTCTVSGYSITSDHAWSWVRQPPGRGLEWIGYISYSGITTYNPSLKSRVTMLRDTSKNQFSLRLSSVTAADTAVYYCARSLARTTAMDYWGQGSLVTVSSASTKGPSVFPLAPSSKSTSGGTAALGCLVKDYFPEPVTVSWNSGALTSGVHTFPAVLQSSGLYSLSSVVTVPSSSLGTQTYICNVNHKPSNTKVDKRVEPKSCDKTHTCPPCPAPELLGGPSVFLFPPKPKDTLMISRTPEVTCVVVDVSHEDPEVKFNWYVDGVEVHNAKTKPREEQYNSTYRVVSVLTVLHQDWLNGKEYKCKVSNKALPAPIEKTISKAKGQPREPQVYTLPPSRKEMTKNQVSLTCLVKGFYPSDIAVEWESNGQPENNYDTTPPVLKSDGSFFLYSKLTVDKSRWQQGNVFSCSVLHEALHSHYTQESLSLSP

SEQ ID NO: 153 - protein, 447 aa, Homo sapiens
QVQLQESGPGLVRPSQTLSLTCTVSGYSITSDHAWSWVRQPPGRGLEWIGYISYSGITTYNPSLKSRVTMLRDTSKNQFSLRLSSVTAADTAVYYCARSLARTTAMDYWGQGSLVTVSSASTKGPSVFPLAPSSKSTSGGTAALGCLVKDYFPEPVTVSWNSGALTSGVHTFPAVLQSSGLYSLSSVVTVPSSSLGTQTYICNVNHKPSNTKVDKRVEPKSCDKTHTCPPCPAPEAAGGPSVFLFPPKPKDTLMISRTPEVTCVVVDVSHEDPEVKFNWYVDGVEVHNAKTKPREEQYNSTYRVVSVLTVLHQDWLNGKEYKCKVSNKALGAPIEKTISKAKGQPREPQVYTLPPSREEMTKNQVSLTCLVKGFYPSDIAVEWESNGQPENNYKTTPPVLDSDGSFFLYSKLTVDKSRWQQGNVFSCSVMHEALHNHYTQKSLSLSP

SEQ ID NO: 154 - protein, 447 aa, Homo sapiens
QVQLQESGPGLVRPSQTLSLTCTVSGYSITSDHAWSWVRQPPGRGLEWIGYISYSGITTYNPSLKSRVTMLRDTSKNQFSLRLSSVTAADTAVYYCARSLARTTAMDYWGQGSLVTVSSASTKGPSVFPLAPSSKSTSGGTAALGCLVKDYFPEPVTVSWNSGALTSGVHTFPAVLQSSGLYSLSSVVTVPSSSLGTQTYICNVNHKPSNTKVDKRVEPKSCDKTHTCPPCPAPEAAGGPSVFLFPPKPKDTLMISRTPEVTCVVVDVSHEDPEVKFNWYVDGVEVHNAKTKPREEQYNSTYRVVSVLTVLHQDWLNGKEYKCKVSNKALGAPIEKTISKAKGQPREPQVYTLPPSREEMTKNQVSLTCLVKGFYPSDIAVEWESNGQPENNYKTWPPVLDSDGSFALYSKLTVDKSRWQQGNVFSCSVMHEALHNHYTQKSLSLSP

SEQ ID NO: 155 - protein, 447 aa, Homo sapiens
QVQLQESGPGLVRPSQTLSLTCTVSGYSITSDHAWSWVRQPPGRGLEWIGYISYSGITTYNPSLKSRVTMLRDTSKNQFSLRLSSVTAADTAVYYCARSLARTTAMDYWGQGSLVTVSSASTKGPSVFPLAPSSKSTSGGTAALGCLVKDYFPEPVTVSWNSGALTSGVHTFPAVLQSSGLYSLSSVVTVPSSSLGTQTYICNVNHKPSNTKVDKRVEPKSCDKTHTCPPCPAPEAAGGPSVFLFPPKPKDTLMISRTPEVTCVVVDVSHEDPEVKFNWYVDGVEVHNAKTKPREEQYNSTYRVVSVLTVLHQDWLNGKEYKCKVSNKALGAPIEKTISKAKGQPREPQVYTLPPSREEMTKNQVSLWCAVKGFYPSDIAVEWESNGQPENNYKTTPPVLDSDGSFFLVSKLTVDKSRWQQGNVFSCSVMHEALHNHYTQKSLSLSP

SEQ ID NO: 156 - protein, 447 aa, Homo sapiens
QVQLQESGPGLVRPSQTLSLTCTVSGYSITSDHAWSWVRQPPGRGLEWIGYISYSGITTYNPSLKSRVTMLRDTSKNQFSLRLSSVTAADTAVYYCARSLARTTAMDYWGQGSLVTVSSASTKGPSVFPLAPSSKSTSGGTAALGCLVKDYFPEPVTVSWNSGALTSGVHTFPAVLQSSGLYSLSSVVTVPSSSLGTQTYICNVNHKPSNTKVDKRVEPKSCDKTHTCPPCPAPEAAGGPSVFLFPPKPKDTLMISRTPEVTCVVVDVSHEDPEVKFNWYVDGVEVHNAKTKPREEQYNSTYRVVSVLTVLHQDWLNGKEYKCKVSNKALGAPIEKTISKAKGQPREPRVYTLPPSREEMTENQVSLTCLVKGFYPSDIAVEWESNGQPENNYKTTPPVLVSDGSFTLYSWLTVDKSRWQQGNVFSCSVMHEALHNHYTQKSLSLSP

SEQ ID NO: 157 - protein, 447 aa, Homo sapiens
QVQLQESGPGLVRPSQTLSLTCTVSGYSITSDHAWSWVRQPPGRGLEWIGYISYSGITTYNPSLKSRVTMLRDTSKNQFSLRLSSVTAADTAVYYCARSLARTTAMDYWGQGSLVTVSSASTKGPSVFPLAPSSKSTSGGTAALGCLVKDYFPEPVTVSWNSGALTSGVHTFPAVLQSSGLYSLSSVVTVPSSSLGTQTYICNVNHKPSNTKVDKRVEPKSCDKTHTCPPCPAPEAAGGPSVFLFPPKPKDTLMISRTPEVTCVVVDVSHEDPEVKFNWYVDGVEVHNAKTKPREEQYNSTYRVVSVLTVLHQDWLNGKEYKCKVSNKALGAPIEKTISKAKGQPREPQVYTLPPSRKEMTKNQVSLTCLVKGFYPSDIAVEWESNGQPENNYDTTPPVLKSDGSFFLYSKLTVDKSRWQQGNVFSCSVMHEALHNHYTQESLSLSP

SEQ ID NO: 158 - protein, 447 aa, Homo sapiens
QVQLQESGPGLVRPSQTLSLTCTVSGYSITSDHAWSWVRQPPGRGLEWIGYISYSGITTYNPSLKSRVTMLRDTSKNQFSLRLSSVTAADTAVYYCARSLARTTAMDYWGQGSLVTVSSASTKGPSVFPLAPSSKSTSGGTAALGCLVKDYFPEPVTVSWNSGALTSGVHTFPAVLQSSGLYSLSSVVTVPSSSLGTQTYICNVNHKPSNTKVDKRVEPKSCDKTHTCPPCPAPEFEGGPSVFLFPPKPKDTLMISRTPEVTCVVVDVSHEDPEVKFNWYVDGVEVHNAKTKPREEQYNSTYRVVSVLTVLHQDWLNGKEYKCKVSNKALPASIEKTISKAKGQPREPQVYTLPPSREEMTKNQVSLTCLVKGFYPSDIAVEWESNGQPENNYKTWPPVLDSDGSFALYSKLTVDKSRWQQGNVFSCSVMHEALHNHYTQKSLSLSP

SEQ ID NO: 159 - protein, 447 aa, Homo sapiens
QVQLQESGPGLVRPSQTLSLTCTVSGYSITSDHAWSWVRQPPGRGLEWIGYISYSGITTYNPSLKSRVTMLRDTSKNQFSLRLSSVTAADTAVYYCARSLARTTAMDYWGQGSLVTVSSASTKGPSVFPLAPSSKSTSGGTAALGCLVKDYFPEPVTVSWNSGALTSGVHTFPAVLQSSGLYSLSSVVTVPSSSLGTQTYICNVNHKPSNTKVDKRVEPKSCDKTHTCPPCPAPEFEGGPSVFLFPPKPKDTLMISRTPEVTCVVVDVSHEDPEVKFNWYVDGVEVHNAKTKPREEQYNSTYRVVSVLTVLHQDWLNGKEYKCKVSNKALPASIEKTISKAKGQPREPRVYTLPPSREEMTENQVSLTCLVKGFYPSDIAVEWESNGQPENNYKTTPPVLVSDGSFTLYSWLTVDKSRWQQGNVFSCSVMHEALHNHYTQKSLSLSP

SEQ ID NO: 160 - protein, 447 aa, Homo sapiens
QVQLQESGPGLVRPSQTLSLTCTVSGYSITSDHAWSWVRQPPGRGLEWIGYISYSGITTYNPSLKSRVTMLRDTSKNQFSLRLSSVTAADTAVYYCARSLARTTAMDYWGQGSLVTVSSASTKGPSVFPLAPSSKSTSGGTAALGCLVKDYFPEPVTVSWNSGALTSGVHTFPAVLQSSGLYSLSSVVTVPSSSLGTQTYICNVNHKPSNTKVDKRVEPKSCDKTHTCPPCPAPEFEGGPSVFLFPPKPKDTLMISRTPEVTCVVVDVSHEDPEVKFNWYVDGVEVHNAKTKPREEQYNSTYRVVSVLTVLHQDWLNGKEYKCKVSNKALPASIEKTISKAKGQPREPQVYTLPPSRKEMTKNQVSLTCLVKGFYPSDIAVEWESNGQPENNYDTTPPVLKSDGSFFLYSKLTVDKSRWQQGNVFSCSVMHEALHNHYTQESLSLSP

SEQ ID NO: 161 - protein, 447 aa, Homo sapiens
QVQLQESGPGLVRPSQTLSLTCTVSGYSITSDHAWSWVRQPPGRGLEWIGYISYSGITTYNPSLKSRVTMLRDTSKNQFSLRLSSVTAADTAVYYCARSLARTTAMDYWGQGSLVTVSSASTKGPSVFPLAPSSKSTSGGTAALGCLVKDYFPEPVTVSWNSGALTSGVHTFPAVLQSSGLYSLSSVVTVPSSSLGTQTYICNVNHKPSNTKVDKRVEPKSCDKTHTCPPCPAPELLGGPSVFLFPPKPKDTLMISRTPEVTCVVVDVSHEDPEVKFNWYVDGVEVHNAKTKPREEQYNSTYRVVSVLTVLHQDWLNGKEYKCKVSNKALPAPIEKTISKAKGQPRRPQVYTLPPSREEMTKNQVSLTCLVKGFYPSDIAVEWESNGQPENNYKTTPPVLDSDGSFFLYSKLTVDKSRWQQGNVFSCSVMHGALHNHYTQKYLSLSP

SEQ ID NO: 162 - protein, 447 aa, Homo sapiens
QVQLQESGPGLVRPSQTLSLTCTVSGYSITSDHAWSWVRQPPGRGLEWIGYISYSGITTYNPSLKSRVTMLRDTSKNQFSLRLSSVTAADTAVYYCARSLARTTAMDYWGQGSLVTVSSASTKGPSVFPLAPSSKSTSGGTAALGCLVKDYFPEPVTVSWNSGALTSGVHTFPAVLQSSGLYSLSSVVTVPSSSLGTQTYICNVNHKPSNTKVDKRVEPKSCDKTHTCPPCPAPELLGGPSVFLFPPKPKDTLMISRTPEVTCVVVDVSHEDPEVKFNWYVDGVEVHNAKTKPREEQYNSTYRVVSVLTVLHQDWLNGKEYKCKVSNKALPAPIEKTISKAKGQPRRPQVYTLPPSREEMTKNQVSLTCLVKGFYPSDIAVEWESNGQPENNYKTWPPVLDSDGSFALYSKLTVDKSRWQQGNVFSCSVMHGALHNHYTQKYLSLSP

SEQ ID NO: 163 - protein, 447 aa, Homo sapiens
QVQLQESGPGLVRPSQTLSLTCTVSGYSITSDHAWSWVRQPPGRGLEWIGYISYSGITTYNPSLKSRVTMLRDTSKNQFSLRLSSVTAADTAVYYCARSLARTTAMDYWGQGSLVTVSSASTKGPSVFPLAPSSKSTSGGTAALGCLVKDYFPEPVTVSWNSGALTSGVHTFPAVLQSSGLYSLSSVVTVPSSSLGTQTYICNVNHKPSNTKVDKRVEPKSCDKTHTCPPCPAPELLGGPSVFLFPPKPKDTLMISRTPEVTCVVVDVSHEDPEVKFNWYVDGVEVHNAKTKPREEQYNSTYRVVSVLTVLHQDWLNGKEYKCKVSNKALPAPIEKTISKAKGQPRRPQVYTLPPSREEMTKNQVSLWCAVKGFYPSDIAVEWESNGQPENNYKTTPPVLDSDGSFFLVSKLTVDKSRWQQGNVFSCSVMHGALHNHYTQKYLSLSP

SEQ ID NO: 164 - protein, 447 aa, Homo sapiens
QVQLQESGPGLVRPSQTLSLTCTVSGYSITSDHAWSWVRQPPGRGLEWIGYISYSGITTYNPSLKSRVTMLRDTSKNQFSLRLSSVTAADTAVYYCARSLARTTAMDYWGQGSLVTVSSASTKGPSVFPLAPSSKSTSGGTAALGCLVKDYFPEPVTVSWNSGALTSGVHTFPAVLQSSGLYSLSSVVTVPSSSLGTQTYICNVNHKPSNTKVDKRVEPKSCDKTHTCPPCPAPELLGGPSVFLFPPKPKDTLMISRTPEVTCVVVDVSHEDPEVKFNWYVDGVEVHNAKTKPREEQYNSTYRVVSVLTVLHQDWLNGKEYKCKVSNKALPAPIEKTISKAKGQPRRPRVYTLPPSREEMTENQVSLTCLVKGFYPSDIAVEWESNGQPENNYKTTPPVLVSDGSFTLYSWLTVDKSRWQQGNVFSCSVMHGALHNHYTQKYLSLSP

SEQ ID NO: 165 - protein, 225 aa, Homo sapiens
DKTHTCPPCPAPELLGGPSVFLFPPKPKDTLMISRTPEVTCVVVDVSHEDPEVKFNWYVDGVEVHNAKTKPREEQYNSTYRVVSVLTVLHQDWLNGKEYKCKVSNKALPAPIEKTISKAKGQPRRPQVYTLPPSREEMTKNQVSLTCLVKGFYPSDIAVEWESNGQPENNYKTTPPVLDSDGSFFLYSKLTVDKSRWQQGNVFSCSVMHGALHNHYTQKYLSLSP

SEQ ID NO: 166 - protein, 466 aa, Homo sapiens
DIQMTQSPSSLSASVGDRVTITCRASQDISSYLNWYQQKPGKAPKLLIYYTSRLHSGVPSRFSGSGSGTDFTFTISSLQPEDIATYYCQQGNTLPYTFGQGTKVEIKGGGGSGGGGSGGGGSQVQLQESGPGLVRPSQTLSLTCTVSGYSITSDHAWSWVRQPPGRGLEWIGYISYSGITTYNPSLKSRVTMLRDTSKNQFSLRLSSVTAADTAVYYCARSLARTTAMDYWGQGSLVTVSSDKTHTCPPCPAPELLGGPSVFLFPPKPKDTLMISRTPEVTCVVVDVSHEDPEVKFNWYVDGVEVHNAKTKPREEQYNSTYRVVSVLTVLHQDWLNGKEYKCKVSNKALPAPIEKTISKAKGQPREPQVYTLPPSREEMTKNQVSLTCLVKGFYPSDIAVEWESNGQPENNYKTTPPVLDSDGSFFLYSKLTVDKSRWQQGNVFSCSVMHEALHNHYTQKSLSLSP

SEQ ID NO: 167 - protein, 466 aa, Homo sapiens
DIQMTQSPSSLSASVGDRVTITCRASQDISSYLNWYQQKPGKAPKLLIYYTSRLHSGVPSRFSGSGSGTDFTFTISSLQPEDIATYYCQQGNTLPYTFGQGTKVEIKGGGGSGGGGSGGGGSQVQLQESGPGLVRPSQTLSLTCTVSGYSITSDHAWSWVRQPPGRGLEWIGYISYSGITTYNPSLKSRVTMLRDTSKNQFSLRLSSVTAADTAVYYCARSLARTTAMDYWGQGSLVTVSSDKTHTCPPCPAPELLGGPSVFLFPPKPKDTLMISRTPEVTCVVVDVSHEDPEVKFNWYVDGVEVHNAKTKPREEQYNSTYRVVSVLTVLHQDWLNGKEYKCKVSNKALPAPIEKTISKAKGQPREPRVYTLPPSREEMTENQVSLTCLVKGFYPSDIAVEWESNGQPENNYKTTPPVLVSDGSFTLYSWLTVDKSRWQQGNVFSCSVMHEALHNHYTQKSLSLSP

SEQ ID NO: 168 - protein, 466 aa, Homo sapiens
DIQMTQSPSSLSASVGDRVTITCRASQDISSYLNWYQQKPGKAPKLLIYYTSRLHSGVPSRFSGSGSGTDFTFTISSLQPEDIATYYCQQGNTLPYTFGQGTKVEIKGGGGSGGGGSGGGGSQVQLQESGPGLVRPSQTLSLTCTVSGYSITSDHAWSWVRQPPGRGLEWIGYISYSGITTYNPSLKSRVTMLRDTSKNQFSLRLSSVTAADTAVYYCARSLARTTAMDYWGQGSLVTVSSDKTHTCPPCPAPELLGGPSVFLFPPKPKDTLMISRTPEVTCVVVDVSHEDPEVKFNWYVDGVEVHNAKTKPREEQYNSTYRVVSVLTVLHQDWLNGKEYKCKVSNKALPAPIEKTISKAKGQPREPQVYTLPPSRKEMTKNQVSLTCLVKGFYPSDIAVEWESNGQPENNYDTTPPVLKSDGSFFLYSKLTVDKSRWQQGNVFSCSVMHEALHNHYTQESLSLSP

SEQ ID NO: 169 - protein, 466 aa, Homo sapiens
DIQMTQSPSSLSASVGDRVTITCRASQDISSYLNWYQQKPGKAPKLLIYYTSRLHSGVPSRFSGSGSGTDFTFTISSLQPEDIATYYCQQGNTLPYTFGQGTKVEIKGGGGSGGGGSGGGGSQVQLQESGPGLVRPSQTLSLTCTVSGYSITSDHAWSWVRQPPGRGLEWIGYISYSGITTYNPSLKSRVTMLRDTSKNQFSLRLSSVTAADTAVYYCARSLARTTAMDYWGQGSLVTVSSDKTHTCPPCPAPELLGGPSVFLFPPKPKDTLMISRTPEVTCVVVDVSHEDPEVKFNWYVDGVEVHNAKTKPREEQYNSTYRVVSVLTVLHQDWLNGKEYKCKVSNKALPAPIEKTISKAKGQPREPQVYTLPPSREEMTKNQVSLTCLVKGFYPSDIAVEWESNGQPENNYKTWPPVLDSDGSFALYSKLTVDKSRWQQGNVFSCSVMHEALHNHYTQKSLSLSP

SEQ ID NO: 170 - protein, 466 aa, Homo sapiens
DIQMTQSPSSLSASVGDRVTITCRASQDISSYLNWYQQKPGKAPKLLIYYTSRLHSGVPSRFSGSGSGTDFTFTISSLQPEDIATYYCQQGNTLPYTFGQGTKVEIKGGGGSGGGGSGGGGSQVQLQESGPGLVRPSQTLSLTCTVSGYSITSDHAWSWVRQPPGRGLEWIGYISYSGITTYNPSLKSRVTMLRDTSKNQFSLRLSSVTAADTAVYYCARSLARTTAMDYWGQGSLVTVSSDKTHTCPPCPAPELLGGPSVFLFPPKPKDTLMISRTPEVTCVVVDVSHEDPEVKFNWYVDGVEVHNAKTKPREEQYNSTYRVVSVLTVLHQDWLNGKEYKCKVSNKALPAPIEKTISKAKGQPREPQVYTLPPSREEMTKNQVSLWCAVKGFYPSDIAVEWESNGQPENNYKTTPPVLDSDGSFFLVSKLTVDKSRWQQGNVFSCSVMHEALHNHYTQKSLSLSP

SEQ ID NO: 171 - protein, 466 aa, Homo sapiens
QVQLQESGPGLVRPSQTLSLTCTVSGYSITSDHAWSWVRQPPGRGLEWIGYISYSGITTYNPSLKSRVTMLRDTSKNQFSLRLSSVTAADTAVYYCARSLARTTAMDYWGQGSLVTVSSGGGGSGGGGSGGGGSDIQMTQSPSSLSASVGDRVTITCRASQDISSYLNWYQQKPGKAPKLLIYYTSRLHSGVPSRFSGSGSGTDFTFTISSLQPEDIATYYCQQGNTLPYTFGQGTKVEIKDKTHTCPPCPAPELLGGPSVFLFPPKPKDTLMISRTPEVTCVVVDVSHEDPEVKFNWYVDGVEVHNAKTKPREEQYNSTYRVVSVLTVLHQDWLNGKEYKCKVSNKALPAPIEKTISKAKGQPREPQVYTLPPSREEMTKNQVSLTCLVKGFYPSDIAVEWESNGQPENNYKTTPPVLDSDGSFFLYSKLTVDKSRWQQGNVFSCSVMHEALHNHYTQKSLSLSP

SEQ ID NO: 172 - protein, 466 aa, Homo sapiens
QVQLQESGPGLVRPSQTLSLTCTVSGYSITSDHAWSWVRQPPGRGLEWIGYISYSGITTYNPSLKSRVTMLRDTSKNQFSLRLSSVTAADTAVYYCARSLARTTAMDYWGQGSLVTVSSGGGGSGGGGSGGGGSDIQMTQSPSSLSASVGDRVTITCRASQDISSYLNWYQQKPGKAPKLLIYYTSRLHSGVPSRFSGSGSGTDFTFTISSLQPEDIATYYCQQGNTLPYTFGQGTKVEIKDKTHTCPPCPAPELLGGPSVFLFPPKPKDTLMISRTPEVTCVVVDVSHEDPEVKFNWYVDGVEVHNAKTKPREEQYNSTYRVVSVLTVLHQDWLNGKEYKCKVSNKALPAPIEKTISKAKGQPREPRVYTLPPSREEMTENQVSLTCLVKGFYPSDIAVEWESNGQPENNYKTTPPVLVSDGSFTLYSWLTVDKSRWQQGNVFSCSVMHEALHNHYTQKSLSLSP

SEQ ID NO: 173 - protein, 466 aa, Homo sapiens
QVQLQESGPGLVRPSQTLSLTCTVSGYSITSDHAWSWVRQPPGRGLEWIGYISYSGITTYNPSLKSRVTMLRDTSKNQFSLRLSSVTAADTAVYYCARSLARTTAMDYWGQGSLVTVSSGGGGSGGGGSGGGGSDIQMTQSPSSLSASVGDRVTITCRASQDISSYLNWYQQKPGKAPKLLIYYTSRLHSGVPSRFSGSGSGTDFTFTISSLQPEDIATYYCQQGNTLPYTFGQGTKVEIKDKTHTCPPCPAPELLGGPSVFLFPPKPKDTLMISRTPEVTCVVVDVSHEDPEVKFNWYVDGVEVHNAKTKPREEQYNSTYRVVSVLTVLHQDWLNGKEYKCKVSNKALPAPIEKTISKAKGQPREPQVYTLPPSRKEMTKNQVSLTCLVKGFYPSDIAVEWESNGQPENNYDTTPPVLKSDGSFFLYSKLTVDKSRWQQGNVFSCSVMHEALHNHYTQESLSLSP

SEQ ID NO: 174 - protein, 466 aa, Homo sapiens
QVQLQESGPGLVRPSQTLSLTCTVSGYSITSDHAWSWVRQPPGRGLEWIGYISYSGITTYNPSLKSRVTMLRDTSKNQFSLRLSSVTAADTAVYYCARSLARTTAMDYWGQGSLVTVSSGGGGSGGGGSGGGGSDIQMTQSPSSLSASVGDRVTITCRASQDISSYLNWYQQKPGKAPKLLIYYTSRLHSGVPSRFSGSGSGTDFTFTISSLQPEDIATYYCQQGNTLPYTFGQGTKVEIKDKTHTCPPCPAPELLGGPSVFLFPPKPKDTLMISRTPEVTCVVVDVSHEDPEVKFNWYVDGVEVHNAKTKPREEQYNSTYRVVSVLTVLHQDWLNGKEYKCKVSNKALPAPIEKTISKAKGQPREPQVYTLPPSREEMTKNQVSLTCLVKGFYPSDIAVEWESNGQPENNYKTWPPVLDSDGSFALYSKLTVDKSRWQQGNVFSCSVMHEALHNHYTQKSLSLSP

SEQ ID NO: 175 - protein, 466 aa, Homo sapiens
QVQLQESGPGLVRPSQTLSLTCTVSGYSITSDHAWSWVRQPPGRGLEWIGYISYSGITTYNPSLKSRVTMLRDTSKNQFSLRLSSVTAADTAVYYCARSLARTTAMDYWGQGSLVTVSSGGGGSGGGGSGGGGSDIQMTQSPSSLSASVGDRVTITCRASQDISSYLNWYQQKPGKAPKLLIYYTSRLHSGVPSRFSGSGSGTDFTFTISSLQPEDIATYYCQQGNTLPYTFGQGTKVEIKDKTHTCPPCPAPELLGGPSVFLFPPKPKDTLMISRTPEVTCVVVDVSHEDPEVKFNWYVDGVEVHNAKTKPREEQYNSTYRVVSVLTVLHQDWLNGKEYKCKVSNKALPAPIEKTISKAKGQPREPQVYTLPPSREEMTKNQVSLWCAVKGFYPSDIAVEWESNGQPENNYKTTPPVLDSDGSFFLVSKLTVDKSRWQQGNVFSCSVMHEALHNHYTQKSLSLSP

SEQ ID NO: 176 - protein, 447 aa, Homo sapiens
QVQLQESGPGLVRPSQTLSLTCTVSGYSITSDHAWSWVRQPPGRGLEWIGYISYSGITTYNPSLKSRVTMLRDTSKNQFSLRLSSVTAADTAVYYCARSLARTTAMDYWGQGSLVTVSSASTKGPSVFPLAPSSKSTSGGTAALGCLVKDYFPEPVTVSWNSGALTSGVHTFPAVLQSSGLYSLSSVVTVPSSSLGTQTYICNVNHKPSNTKVDKRVEPKSCDKTHTCPPCPAPELLGGPSVFLFPPKPKDTLMISRTPEVTCVVVDVSHEDPEVKFNWYVDGVEVHNAKTKPREEQYNSTYRVVSVLTVLHQDWLNGKEYKCKVSNKALPAPIEKTISKAKGQPREPQVYTLPPSRREMTKNQVSLTCLVKGFYPSDIAVEWESNGQPENNYKTTPPVLKSDGSFFLYSELTVDKSRWQQGNVFSCSVMHEALHNHYTQESLSLSP

SEQ ID NO: 177 - protein, 447 aa, Homo sapiens
QVQLQESGPGLVRPSQTLSLTCTVSGYSITSDHAWSWVRQPPGRGLEWIGYISYSGITTYNPSLKSRVTMLRDTSKNQFSLRLSSVTAADTAVYYCARSLARTTAMDYWGQGSLVTVSSASTKGPSVFPLAPSSKSTSGGTAALGCLVKDYFPEPVTVSWNSGALTSGVHTFPAVLQSSGLYSLSSVVTVPSSSLGTQTYICNVNHKPSNTKVDKRVEPKSCDKTHTCPPCPAPELLGGPSVFLFPPKPKDTLMISRTPEVTCVVVDVSHEDPEVKFNWYVDGVEVHNAKTKPREEQYNSTYRVVSVLTVLHQDWLNGKEYKCKVSNKALPAPIEKTISKAKGQPREPQVYTLPPSRHEMTKNQVSLTCLVKGFYPSDIAVEWESNGQPENNYKTTPPVLKSDGSFFLYSELTVDKSRWQQGNVFSCSVMHEALHNHYTQESLSLSP

SEQ ID NO: 178 - protein, 447 aa, Homo sapiens
QVQLQESGPGLVRPSQTLSLTCTVSGYSITSDHAWSWVRQPPGRGLEWIGYISYSGITTYNPSLKSRVTMLRDTSKNQFSLRLSSVTAADTAVYYCARSLARTTAMDYWGQGSLVTVSSASTKGPSVFPLAPSSKSTSGGTAALGCLVKDYFPEPVTVSWNSGALTSGVHTFPAVLQSSGLYSLSSVVTVPSSSLGTQTYICNVNHKPSNTKVDKRVEPKSCDKTHTCPPCPAPELLGGPSVFLFPPKPKDTLMISRTPEVTCVVVDVSHEDPEVKFNWYVDGVEVHNAKTKPREEQYNSTYRVVSVLTVLHQDWLNGKEYKCKVSNKALPAPIEKTISKAKGQPREPQVYTLPPSRKEMTKNQVSLTCLVKGFYPSDIAVEWESNGQPENNYKTTPPVLRSDGSFFLYSELTVDKSRWQQGNVFSCSVMHEALHNHYTQESLSLSP

SEQ ID NO: 179 - protein, 447 aa, Homo sapiens
QVQLQESGPGLVRPSQTLSLTCTVSGYSITSDHAWSWVRQPPGRGLEWIGYISYSGITTYNPSLKSRVTMLRDTSKNQFSLRLSSVTAADTAVYYCARSLARTTAMDYWGQGSLVTVSSASTKGPSVFPLAPSSKSTSGGTAALGCLVKDYFPEPVTVSWNSGALTSGVHTFPAVLQSSGLYSLSSVVTVPSSSLGTQTYICNVNHKPSNTKVDKRVEPKSCDKTHTCPPCPAPELLGGPSVFLFPPKPKDTLMISRTPEVTCVVVDVSHEDPEVKFNWYVDGVEVHNAKTKPREEQYNSTYRVVSVLTVLHQDWLNGKEYKCKVSNKALPAPIEKTISKAKGQPREPQVYTLPPSRKEMTKNQVSLTCLVKGFYPSDIAVEWESNGQPENNYKTTPPVLHSDGSFFLYSELTVDKSRWQQGNVFSCSVMHEALHNHYTQESLSLSP

SEQ ID NO: 180 - protein, 447 aa, Homo sapiens
QVQLQESGPGLVRPSQTLSLTCTVSGYSITSDHAWSWVRQPPGRGLEWIGYISYSGITTYNPSLKSRVTMLRDTSKNQFSLRLSSVTAADTAVYYCARSLARTTAMDYWGQGSLVTVSSASTKGPSVFPLAPSSKSTSGGTAALGCLVKDYFPEPVTVSWNSGALTSGVHTFPAVLQSSGLYSLSSVVTVPSSSLGTQTYICNVNHKPSNTKVDKRVEPKSCDKTHTCPPCPAPELLGGPSVFLFPPKPKDTLMISRTPEVTCVVVDVSHEDPEVKFNWYVDGVEVHNAKTKPREEQYNSTYRVVSVLTVLHQDWLNGKEYKCKVSNKALPAPIEKTISKAKGQPREPQVYTLPPSRKEMTKNQVSLTCLVKGFYPSDIAVEWESNGQPENNYKTTPPVLKSDGSFFLYSDLTVDKSRWQQGNVFSCSVMHEALHNHYTQESLSLSP

SEQ ID NO: 181 - protein, 447 aa, Homo sapiens
QVQLQESGPGLVRPSQTLSLTCTVSGYSITSDHAWSWVRQPPGRGLEWIGYISYSGITTYNPSLKSRVTMLRDTSKNQFSLRLSSVTAADTAVYYCARSLARTTAMDYWGQGSLVTVSSASTKGPSVFPLAPSSKSTSGGTAALGCLVKDYFPEPVTVSWNSGALTSGVHTFPAVLQSSGLYSLSSVVTVPSSSLGTQTYICNVNHKPSNTKVDKRVEPKSCDKTHTCPPCPAPELLGGPSVFLFPPKPKDTLMISRTPEVTCVVVDVSHEDPEVKFNWYVDGVEVHNAKTKPREEQYNSTYRVVSVLTVLHQDWLNGKEYKCKVSNKALPAPIEKTISKAKGQPREPQVYTLPPSRKEMTKNQVSLTCLVKGFYPSDIAVEWESNGQPENNYKTTPPVLKSDGSFFLYSELTVDKSRWQQGNVFSCSVMHEALHNHYTQDSLSLSP

SEQ ID NO: 182 - protein, 447 aa, Homo sapiens
QVQLQESGPGLVRPSQTLSLTCTVSGYSITSDHAWSWVRQPPGRGLEWIGYISYSGITTYNPSLKSRVTMLRDTSKNQFSLRLSSVTAADTAVYYCARSLARTTAMDYWGQGSLVTVSSASTKGPSVFPLAPSSKSTSGGTAALGCLVKDYFPEPVTVSWNSGALTSGVHTFPAVLQSSGLYSLSSVVTVPSSSLGTQTYICNVNHKPSNTKVDKRVEPKSCDKTHTCPPCPAPELLGGPSVFLFPPKPKDTLMISRTPEVTCVVVDVSHEDPEVKFNWYVDGVEVHNAKTKPREEQYNSTYRVVSVLTVLHQDWLNGKEYKCKVSNKALPAPIEKTISKAKGQPREPQVYTLPPSRKEMTKNQVSLTCLVKGFYPSDIAVEWESNGQPENNYKTTPPVLRSDGSFFLYSDLTVDKSRWQQGNVFSCSVMHEALHNHYTQESLSLSP

SEQ ID NO: 183 - protein, 447 aa, Homo sapiens
QVQLQESGPGLVRPSQTLSLTCTVSGYSITSDHAWSWVRQPPGRGLEWIGYISYSGITTYNPSLKSRVTMLRDTSKNQFSLRLSSVTAADTAVYYCARSLARTTAMDYWGQGSLVTVSSASTKGPSVFPLAPSSKSTSGGTAALGCLVKDYFPEPVTVSWNSGALTSGVHTFPAVLQSSGLYSLSSVVTVPSSSLGTQTYICNVNHKPSNTKVDKRVEPKSCDKTHTCPPCPAPELLGGPSVFLFPPKPKDTLMISRTPEVTCVVVDVSHEDPEVKFNWYVDGVEVHNAKTKPREEQYNSTYRVVSVLTVLHQDWLNGKEYKCKVSNKALPAPIEKTISKAKGQPREPQVYTLPPSRKEMTKNQVSLTCLVKGFYPSDIAVEWESNGQPENNYKTTPPVLHSDGSFFLYSDLTVDKSRWQQGNVFSCSVMHEALHNHYTQESLSLSP

SEQ ID NO: 184 - protein, 447 aa, Homo sapiens
QVQLQESGPGLVRPSQTLSLTCTVSGYSITSDHAWSWVRQPPGRGLEWIGYISYSGITTYNPSLKSRVTMLRDTSKNQFSLRLSSVTAADTAVYYCARSLARTTAMDYWGQGSLVTVSSASTKGPSVFPLAPSSKSTSGGTAALGCLVKDYFPEPVTVSWNSGALTSGVHTFPAVLQSSGLYSLSSVVTVPSSSLGTQTYICNVNHKPSNTKVDKRVEPKSCDKTHTCPPCPAPELLGGPSVFLFPPKPKDTLMISRTPEVTCVVVDVSHEDPEVKFNWYVDGVEVHNAKTKPREEQYNSTYRVVSVLTVLHQDWLNGKEYKCKVSNKALPAPIEKTISKAKGQPREPQVYTLPPSRREMTKNQVSLTCLVKGFYPSDIAVEWESNGQPENNYDTTPPVLKSDGSFFLYSKLTVDKSRWQQGNVFSCSVMHEALHNHYTQESLSLSP

SEQ ID NO: 185 - protein, 447 aa, Homo sapiens
QVQLQESGPGLVRPSQTLSLTCTVSGYSITSDHAWSWVRQPPGRGLEWIGYISYSGITTYNPSLKSRVTMLRDTSKNQFSLRLSSVTAADTAVYYCARSLARTTAMDYWGQGSLVTVSSASTKGPSVFPLAPSSKSTSGGTAALGCLVKDYFPEPVTVSWNSGALTSGVHTFPAVLQSSGLYSLSSVVTVPSSSLGTQTYICNVNHKPSNTKVDKRVEPKSCDKTHTCPPCPAPELLGGPSVFLFPPKPKDTLMISRTPEVTCVVVDVSHEDPEVKFNWYVDGVEVHNAKTKPREEQYNSTYRVVSVLTVLHQDWLNGKEYKCKVSNKALPAPIEKTISKAKGQPREPQVYTLPPSRKEMTKNQVSLTCLVKGFYPSDIAVEWESNGQPENNYDTTPPVLKSDGSFFLYSKLTVDKSRWQQGNVFSCSVMHEALHNHYTQDSLSLSP

SEQ ID NO: 186 - protein, 447 aa, Homo sapiens
QVQLQESGPGLVRPSQTLSLTCTVSGYSITSDHAWSWVRQPPGRGLEWIGYISYSGITTYNPSLKSRVTMLRDTSKNQFSLRLSSVTAADTAVYYCARSLARTTAMDYWGQGSLVTVSSASTKGPSVFPLAPSSKSTSGGTAALGCLVKDYFPEPVTVSWNSGALTSGVHTFPAVLQSSGLYSLSSVVTVPSSSLGTQTYICNVNHKPSNTKVDKRVEPKSCDKTHTCPPCPAPELLGGPSVFLFPPKPKDTLMISRTPEVTCVVVDVSHEDPEVKFNWYVDGVEVHNAKTKPREEQYNSTYRVVSVLTVLHQDWLNGKEYKCKVSNKALPAPIEKTISKAKGQPREPQVYTLPPSRKEMTKNQVSLTCLVKGFYPSDIAVEWESNGQPENNYDTTPPVLRSDGSFFLYSKLTVDKSRWQQGNVFSCSVMHEALHNHYTQESLSLSP

SEQ ID NO: 187 - protein, 447 aa, Homo sapiens
QVQLQESGPGLVRPSQTLSLTCTVSGYSITSDHAWSWVRQPPGRGLEWIGYISYSGITTYNPSLKSRVTMLRDTSKNQFSLRLSSVTAADTAVYYCARSLARTTAMDYWGQGSLVTVSSASTKGPSVFPLAPSSKSTSGGTAALGCLVKDYFPEPVTVSWNSGALTSGVHTFPAVLQSSGLYSLSSVVTVPSSSLGTQTYICNVNHKPSNTKVDKRVEPKSCDKTHTCPPCPAPELLGGPSVFLFPPKPKDTLMISRTPEVTCVVVDVSHEDPEVKFNWYVDGVEVHNAKTKPREEQYNSTYRVVSVLTVLHQDWLNGKEYKCKVSNKALPAPIEKTISKAKGQPREPQVYTLPPSRKEMTKNQVSLTCLVKGFYPSDIAVEWESNGQPENNYETTPPVLKSDGSFFLYSKLTVDKSRWQQGNVFSCSVMHEALHNHYTQESLSLSP

SEQ ID NO: 188 - protein, 447 aa, Homo sapiens
QVQLQESGPGLVRPSQTLSLTCTVSGYSITSDHAWSWVRQPPGRGLEWIGYISYSGITTYNPSLKSRVTMLRDTSKNQFSLRLSSVTAADTAVYYCARSLARTTAMDYWGQGSLVTVSSASTKGPSVFPLAPSSKSTSGGTAALGCLVKDYFPEPVTVSWNSGALTSGVHTFPAVLQSSGLYSLSSVVTVPSSSLGTQTYICNVNHKPSNTKVDKRVEPKSCDKTHTCPPCPAPELLGGPSVFLFPPKPKDTLMISRTPEVTCVVVDVSHEDPEVKFNWYVDGVEVHNAKTKPREEQYNSTYRVVSVLTVLHQDWLNGKEYKCKVSNKALPAPIEKTISKAKGQPREPQVYTLPPSREEMTKNQVSLTCLVKGFYPSDIAVEWESNGQPENNYDTTPPVLRSDGSFFLYSDLTVDKSRWQQGNVFSCSVMHEALHNHYTQKSLSLSP

SEQ ID NO: 189 - protein, 447 aa, Homo sapiens
QVQLQESGPGLVRPSQTLSLTCTVSGYSITSDHAWSWVRQPPGRGLEWIGYISYSGITTYNPSLKSRVTMLRDTSKNQFSLRLSSVTAADTAVYYCARSLARTTAMDYWGQGSLVTVSSASTKGPSVFPLAPSSKSTSGGTAALGCLVKDYFPEPVTVSWNSGALTSGVHTFPAVLQSSGLYSLSSVVTVPSSSLGTQTYICNVNHKPSNTKVDKRVEPKSCDKTHTCPPCPAPELLGGPSVFLFPPKPKDTLMISRTPEVTCVVVDVSHEDPEVKFNWYVDGVEVHNAKTKPREEQYNSTYRVVSVLTVLHQDWLNGKEYKCKVSNKALPAPIEKTISKAKGQPREPQVYTLPPSREEMTKNQVSLTCLVKGFYPSDIAVEWESNGQPENNYDTTPPVLKSDGSFFLYSELTVDKSRWQQGNVFSCSVMHEALHNHYTQKSLSLSP

SEQ ID NO: 190 - protein, 447 aa, Homo sapiens
QVQLQESGPGLVRPSQTLSLTCTVSGYSITSDHAWSWVRQPPGRGLEWIGYISYSGITTYNPSLKSRVTMLRDTSKNQFSLRLSSVTAADTAVYYCARSLARTTAMDYWGQGSLVTVSSASTKGPSVFPLAPSSKSTSGGTAALGCLVKDYFPEPVTVSWNSGALTSGVHTFPAVLQSSGLYSLSSVVTVPSSSLGTQTYICNVNHKPSNTKVDKRVEPKSCDKTHTCPPCPAPELLGGPSVFLFPPKPKDTLMISRTPEVTCVVVDVSHEDPEVKFNWYVDGVEVHNAKTKPREEQYNSTYRVVSVLTVLHQDWLNGKEYKCKVSNKALPAPIEKTISKAKGQPREPQVYTLPPSREEMTKNQVSLTCLVKGFYPSDIAVEWESNGQPENNYETTPPVLKSDGSFFLYSDLTVDKSRWQQGNVFSCSVMHEALHNHYTQKSLSLSP

SEQ ID NO: 191 - protein, 447 aa, Homo sapiens
QVQLQESGPGLVRPSQTLSLTCTVSGYSITSDHAWSWVRQPPGRGLEWIGYISYSGITTYNPSLKSRVTMLRDTSKNQFSLRLSSVTAADTAVYYCARSLARTTAMDYWGQGSLVTVSSASTKGPSVFPLAPSSKSTSGGTAALGCLVKDYFPEPVTVSWNSGALTSGVHTFPAVLQSSGLYSLSSVVTVPSSSLGTQTYICNVNHKPSNTKVDKRVEPKSCDKTHTCPPCPAPELLGGPSVFLFPPKPKDTLMISRTPEVTCVVVDVSHEDPEVKFNWYVDGVEVHNAKTKPREEQYNSTYRVVSVLTVLHQDWLNGKEYKCKVSNKALPAPIEKTISKAKGQPREPQVYTLPPSRKEMTKNQVSLTCLVKGFYPSDIAVEWESNGQPENNYDTTPPVLKSDGSFFLYSELTVDKSRWQQGNVFSCSVMHEALHNHYTQKSLSLSP

SEQ ID NO: 192 - protein, 447 aa, Homo sapiens
QVQLQESGPGLVRPSQTLSLTCTVSGYSITSDHAWSWVRQPPGRGLEWIGYISYSGITTYNPSLKSRVTMLRDTSKNQFSLRLSSVTAADTAVYYCARSLARTTAMDYWGQGSLVTVSSASTKGPSVFPLAPSSKSTSGGTAALGCLVKDYFPEPVTVSWNSGALTSGVHTFPAVLQSSGLYSLSSVVTVPSSSLGTQTYICNVNHKPSNTKVDKRVEPKSCDKTHTCPPCPAPELLGGPSVFLFPPKPKDTLMISRTPEVTCVVVDVSHEDPEVKFNWYVDGVEVHNAKTKPREEQYNSTYRVVSVLTVLHQDWLNGKEYKCKVSNKALPAPIEKTISKAKGQPREPQVYTLPPSRKEMTKNQVSLTCLVKGFYPSDIAVEWESNGQPENNYDTTPPVLRSDGSFFLYSDLTVDKSRWQQGNVFSCSVMHEALHNHYTQKSLSLSP

SEQ ID NO: 193 - protein, 447 aa, Homo sapiens
QVQLQESGPGLVRPSQTLSLTCTVSGYSITSDHAWSWVRQPPGRGLEWIGYISYSGITTYNPSLKSRVTMLRDTSKNQFSLRLSSVTAADTAVYYCARSLARTTAMDYWGQGSLVTVSSASTKGPSVFPLAPSSKSTSGGTAALGCLVKDYFPEPVTVSWNSGALTSGVHTFPAVLQSSGLYSLSSVVTVPSSSLGTQTYICNVNHKPSNTKVDKRVEPKSCDKTHTCPPCPAPELLGGPSVFLFPPKPKDTLMISRTPEVTCVVVDVSHEDPEVKFNWYVDGVEVHNAKTKPREEQYNSTYRVVSVLTVLHQDWLNGKEYKCKVSNKALPAPIEKTISKAKGQPREPQVYTLPPSRREMTKNQVSLTCLVKGFYPSDIAVEWESNGQPENNYDTTPPVLKSDGSFFLYSDLTVDKSRWQQGNVFSCSVMHEALHNHYTQKSLSLSP

SEQ ID NO: 194 - protein, 447 aa, Homo sapiens
QVQLQESGPGLVRPSQTLSLTCTVSGYSITSDHAWSWVRQPPGRGLEWIGYISYSGITTYNPSLKSRVTMLRDTSKNQFSLRLSSVTAADTAVYYCARSLARTTAMDYWGQGSLVTVSSASTKGPSVFPLAPSSKSTSGGTAALGCLVKDYFPEPVTVSWNSGALTSGVHTFPAVLQSSGLYSLSSVVTVPSSSLGTQTYICNVNHKPSNTKVDKRVEPKSCDKTHTCPPCPAPELLGGPSVFLFPPKPKDTLMISRTPEVTCVVVDVSHEDPEVKFNWYVDGVEVHNAKTKPREEQYNSTYRVVSVLTVLHQDWLNGKEYKCKVSNKALPAPIEKTISKAKGQPREPQVYTLPPSRHEMTKNQVSLTCLVKGFYPSDIAVEWESNGQPENNYDTTPPVLKSDGSFFLYSDLTVDKSRWQQGNVFSCSVMHEALHNHYTQKSLSLSP

SEQ ID NO: 195 - protein, 447 aa, Homo sapiens
QVQLQESGPGLVRPSQTLSLTCTVSGYSITSDHAWSWVRQPPGRGLEWIGYISYSGITTYNPSLKSRVTMLRDTSKNQFSLRLSSVTAADTAVYYCARSLARTTAMDYWGQGSLVTVSSASTKGPSVFPLAPSSKSTSGGTAALGCLVKDYFPEPVTVSWNSGALTSGVHTFPAVLQSSGLYSLSSVVTVPSSSLGTQTYICNVNHKPSNTKVDKRVEPKSCDKTHTCPPCPAPELLGGPSVFLFPPKPKDTLMISRTPEVTCVVVDVSHEDPEVKFNWYVDGVEVHNAKTKPREEQYNSTYRVVSVLTVLHQDWLNGKEYKCKVSNKALPAPIEKTISKAKGQPREPQVYTLPPSRKEMTKNQVSLTCLVKGFYPSDIAVEWESNGQPENNYETTPPVLKSDGSFFLYSDLTVDKSRWQQGNVFSCSVMHEALHNHYTQKSLSLSP

SEQ ID NO: 196 - protein, 447 aa, Homo sapiens
QVQLQESGPGLVRPSQTLSLTCTVSGYSITSDHAWSWVRQPPGRGLEWIGYISYSGITTYNPSLKSRVTMLRDTSKNQFSLRLSSVTAADTAVYYCARSLARTTAMDYWGQGSLVTVSSASTKGPSVFPLAPSSKSTSGGTAALGCLVKDYFPEPVTVSWNSGALTSGVHTFPAVLQSSGLYSLSSVVTVPSSSLGTQTYICNVNHKPSNTKVDKRVEPKSCDKTHTCPPCPAPELLGGPSVFLFPPKPKDTLMISRTPEVTCVVVDVSHEDPEVKFNWYVDGVEVHNAKTKPREEQYNSTYRVVSVLTVLHQDWLNGKEYKCKVSNKALPAPIEKTISKAKGQPREPQVYTLPPSRREMTKNQVSLTCLVKGFYPSDIAVEWESNGQPENNYDTTPPVLKSDGSFFLYSKLTVDKSRWQQGNVFSCSVMHEALHNHYTQDSLSLSP

SEQ ID NO: 197 - protein, 447 aa, Homo sapiens
QVQLQESGPGLVRPSQTLSLTCTVSGYSITSDHAWSWVRQPPGRGLEWIGYISYSGITTYNPSLKSRVTMLRDTSKNQFSLRLSSVTAADTAVYYCARSLARTTAMDYWGQGSLVTVSSASTKGPSVFPLAPSSKSTSGGTAALGCLVKDYFPEPVTVSWNSGALTSGVHTFPAVLQSSGLYSLSSVVTVPSSSLGTQTYICNVNHKPSNTKVDKRVEPKSCDKTHTCPPCPAPELLGGPSVFLFPPKPKDTLMISRTPEVTCVVVDVSHEDPEVKFNWYVDGVEVHNAKTKPREEQYNSTYRVVSVLTVLHQDWLNGKEYKCKVSNKALPAPIEKTISKAKGQPREPQVYTLPPSRKEMTKNQVSLTCLVKGFYPSDIAVEWESNGQPENNYDTTPPVLHSDGSFFLYSDLTVDKSRWQQGNVFSCSVMHEALHNHYTQKSLSLSP

SEQ ID NO: 198 - protein, 447 aa, Homo sapiens
QVQLQESGPGLVRPSQTLSLTCTVSGYSITSDHAWSWVRQPPGRGLEWIGYISYSGITTYNPSLKSRVTMLRDTSKNQFSLRLSSVTAADTAVYYCARSLARTTAMDYWGQGSLVTVSSASTKGPSVFPLAPSSKSTSGGTAALGCLVKDYFPEPVTVSWNSGALTSGVHTFPAVLQSSGLYSLSSVVTVPSSSLGTQTYICNVNHKPSNTKVDKRVEPKSCDKTHTCPPCPAPELLGGPSVFLFPPKPKDTLMISRTPEVTCVVVDVSHEDPEVKFNWYVDGVEVHNAKTKPREEQYNSTYRVVSVLTVLHQDWLNGKEYKCKVSNKALPAPIEKTISKAKGQPREPQVYTLPPSRREMTKNQVSLTCLVKGFYPSDIAVEWESNGQPENNYKTTPPVLKSDGSFFLYSELTVDKSRWQQGNVFSCSVMHEALHNHYTQDSLSLSP

SEQ ID NO: 199 - protein, 447 aa, Homo sapiens
QVQLQESGPGLVRPSQTLSLTCTVSGYSITSDHAWSWVRQPPGRGLEWIGYISYSGITTYNPSLKSRVTMLRDTSKNQFSLRLSSVTAADTAVYYCARSLARTTAMDYWGQGSLVTVSSASTKGPSVFPLAPSSKSTSGGTAALGCLVKDYFPEPVTVSWNSGALTSGVHTFPAVLQSSGLYSLSSVVTVPSSSLGTQTYICNVNHKPSNTKVDKRVEPKSCDKTHTCPPCPAPELLGGPSVFLFPPKPKDTLMISRTPEVTCVVVDVSHEDPEVKFNWYVDGVEVHNAKTKPREEQYNSTYRVVSVLTVLHQDWLNGKEYKCKVSNKALPAPIEKTISKAKGQPREPQVYTLPPSRHEMTKNQVSLTCLVKGFYPSDIAVEWESNGQPENNYKTTPPVLKSDGSFFLYSELTVDKSRWQQGNVFSCSVMHEALHNHYTQDSLSLSP

SEQ ID NO: 200 - protein, 447 aa, Homo sapiens
QVQLQESGPGLVRPSQTLSLTCTVSGYSITSDHAWSWVRQPPGRGLEWIGYISYSGITTYNPSLKSRVTMLRDTSKNQFSLRLSSVTAADTAVYYCARSLARTTAMDYWGQGSLVTVSSASTKGPSVFPLAPSSKSTSGGTAALGCLVKDYFPEPVTVSWNSGALTSGVHTFPAVLQSSGLYSLSSVVTVPSSSLGTQTYICNVNHKPSNTKVDKRVEPKSCDKTHTCPPCPAPELLGGPSVFLFPPKPKDTLMISRTPEVTCVVVDVSHEDPEVKFNWYVDGVEVHNAKTKPREEQYNSTYRVVSVLTVLHQDWLNGKEYKCKVSNKALPAPIEKTISKAKGQPREPRVYTLPPSREEMTDNQVSLVCLVKGFYPSDIAVEWESNGQPENNYKTTPPVLMSDGSFFLASVLTVDKSRWQQGNVFSCSVMHEALHNHYTQKSLSLSP

SEQ ID NO: 201 - protein, 447 aa, Homo sapiens
QVQLQESGPGLVRPSQTLSLTCTVSGYSITSDHAWSWVRQPPGRGLEWIGYISYSGITTYNPSLKSRVTMLRDTSKNQFSLRLSSVTAADTAVYYCARSLARTTAMDYWGQGSLVTVSSASTKGPSVFPLAPSSKSTSGGTAALGCLVKDYFPEPVTVSWNSGALTSGVHTFPAVLQSSGLYSLSSVVTVPSSSLGTQTYICNVNHKPSNTKVDKRVEPKSCDKTHTCPPCPAPELLGGPSVFLFPPKPKDTLMISRTPEVTCVVVDVSHEDPEVKFNWYVDGVEVHNAKTKPREEQYNSTYRVVSVLTVLHQDWLNGKEYKCKVSNKALPAPIEKTISKAKGQPRRPKVYTLPPSREEMTDNQVSLVCLVKGFYPSDIAVEWESNGQPENNYKTTPPVLMSDGSFFLASVLTVDKSRWQQGNVFSCSVMHEALHNHYTQKSLSLSP

SEQ ID NO: 202 - protein, 447 aa, Homo sapiens
QVQLQESGPGLVRPSQTLSLTCTVSGYSITSDHAWSWVRQPPGRGLEWIGYISYSGITTYNPSLKSRVTMLRDTSKNQFSLRLSSVTAADTAVYYCARSLARTTAMDYWGQGSLVTVSSASTKGPSVFPLAPSSKSTSGGTAALGCLVKDYFPEPVTVSWNSGALTSGVHTFPAVLQSSGLYSLSSVVTVPSSSLGTQTYICNVNHKPSNTKVDKRVEPKSCDKTHTCPPCPAPELLGGPSVFLFPPKPKDTLMISRTPEVTCVVVDVSHEDPEVKFNWYVDGVEVHNAKTKPREEQYNSTYRVVSVLTVLHQDWLNGKEYKCKVSNKALPAPIEKTISKAKGQPRRPRVYTLPPSREEMTENQVSLVCLVKGFYPSDIAVEWESNGQPENNYKTTPPVLMSDGSFFLASVLTVDKSRWQQGNVFSCSVMHEALHNHYTQKSLSLSP

SEQ ID NO: 203 - protein, 447 aa, Homo sapiens
QVQLQESGPGLVRPSQTLSLTCTVSGYSITSDHAWSWVRQPPGRGLEWIGYISYSGITTYNPSLKSRVTMLRDTSKNQFSLRLSSVTAADTAVYYCARSLARTTAMDYWGQGSLVTVSSASTKGPSVFPLAPSSKSTSGGTAALGCLVKDYFPEPVTVSWNSGALTSGVHTFPAVLQSSGLYSLSSVVTVPSSSLGTQTYICNVNHKPSNTKVDKRVEPKSCDKTHTCPPCPAPELLGGPSVFLFPPKPKDTLMISRTPEVTCVVVDVSHEDPEVKFNWYVDGVEVHNAKTKPREEQYNSTYRVVSVLTVLHQDWLNGKEYKCKVSNKALPAPIEKTISKAKGQPREPKVYTLPPSREEMTDNQVSLVCLVKGFYPSDIAVEWESNGQPENNYKTTPPVLMSDGSFFLASVLTVDKSRWQQGNVFSCSVMHEALHNHYTQKSLSLSP

SEQ ID NO: 204 - protein, 447 aa, Homo sapiens
QVQLQESGPGLVRPSQTLSLTCTVSGYSITSDHAWSWVRQPPGRGLEWIGYISYSGITTYNPSLKSRVTMLRDTSKNQFSLRLSSVTAADTAVYYCARSLARTTAMDYWGQGSLVTVSSASTKGPSVFPLAPSSKSTSGGTAALGCLVKDYFPEPVTVSWNSGALTSGVHTFPAVLQSSGLYSLSSVVTVPSSSLGTQTYICNVNHKPSNTKVDKRVEPKSCDKTHTCPPCPAPELLGGPSVFLFPPKPKDTLMISRTPEVTCVVVDVSHEDPEVKFNWYVDGVEVHNAKTKPREEQYNSTYRVVSVLTVLHQDWLNGKEYKCKVSNKALPAPIEKTISKAKGQPREPRVYTLPPSREEMTENQVSLVCLVKGFYPSDIAVEWESNGQPENNYKTTPPVLMSDGSFFLASVLTVDKSRWQQGNVFSCSVMHEALHNHYTQKSLSLSP

SEQ ID NO: 205 - protein, 447 aa, Homo sapiens
QVQLQESGPGLVRPSQTLSLTCTVSGYSITSDHAWSWVRQPPGRGLEWIGYISYSGITTYNPSLKSRVTMLRDTSKNQFSLRLSSVTAADTAVYYCARSLARTTAMDYWGQGSLVTVSSASTKGPSVFPLAPSSKSTSGGTAALGCLVKDYFPEPVTVSWNSGALTSGVHTFPAVLQSSGLYSLSSVVTVPSSSLGTQTYICNVNHKPSNTKVDKRVEPKSCDKTHTCPPCPAPELLGGPSVFLFPPKPKDTLMISRTPEVTCVVVDVSHEDPEVKFNWYVDGVEVHNAKTKPREEQYNSTYRVVSVLTVLHQDWLNGKEYKCKVSNKALPAPIEKTISKAKGQPREPKVYTLPPSREEMTENQVSLVCLVKGFYPSDIAVEWESNGQPENNYKTTPPVLMSDGSFFLASVLTVDKSRWQQGNVFSCSVMHEALHNHYTQKSLSLSP

SEQ ID NO: 206 - protein, 447 aa, Homo sapiens
QVQLQESGPGLVRPSQTLSLTCTVSGYSITSDHAWSWVRQPPGRGLEWIGYISYSGITTYNPSLKSRVTMLRDTSKNQFSLRLSSVTAADTAVYYCARSLARTTAMDYWGQGSLVTVSSASTKGPSVFPLAPSSKSTSGGTAALGCLVKDYFPEPVTVSWNSGALTSGVHTFPAVLQSSGLYSLSSVVTVPSSSLGTQTYICNVNHKPSNTKVDKRVEPKSCDKTHTCPPCPAPELLGGPSVFLFPPKPKDTLMISRTPEVTCVVVDVSHEDPEVKFNWYVDGVEVHNAKTKPREEQYNSTYRVVSVLTVLHQDWLNGKEYKCKVSNKALPAPIEKTISKAKGQPRRPRVYTLPPSREEMTDNQVSLVCLVKGFYPSDIAVEWESNGQPENNYKTTPPVLQSDGSFFLASQLTVDKSRWQQGNVFSCSVMHEALHNHYTQKSLSLSP

SEQ ID NO: 207 - protein, 447 aa, Homo sapiens
QVQLQESGPGLVRPSQTLSLTCTVSGYSITSDHAWSWVRQPPGRGLEWIGYISYSGITTYNPSLKSRVTMLRDTSKNQFSLRLSSVTAADTAVYYCARSLARTTAMDYWGQGSLVTVSSASTKGPSVFPLAPSSKSTSGGTAALGCLVKDYFPEPVTVSWNSGALTSGVHTFPAVLQSSGLYSLSSVVTVPSSSLGTQTYICNVNHKPSNTKVDKRVEPKSCDKTHTCPPCPAPELLGGPSVFLFPPKPKDTLMISRTPEVTCVVVDVSHEDPEVKFNWYVDGVEVHNAKTKPREEQYNSTYRVVSVLTVLHQDWLNGKEYKCKVSNKALPAPIEKTISKAKGQPRRPRVYTLPPSREEMTDNQVSLVCLVKGFYPSDIAVEWESNGQPENNYKTTPPVLNSDGSFFLASQLTVDKSRWQQGNVFSCSVMHEALHNHYTQKSLSLSP

SEQ ID NO: 208 - protein, 447 aa, Homo sapiens
QVQLQESGPGLVRPSQTLSLTCTVSGYSITSDHAWSWVRQPPGRGLEWIGYISYSGITTYNPSLKSRVTMLRDTSKNQFSLRLSSVTAADTAVYYCARSLARTTAMDYWGQGSLVTVSSASTKGPSVFPLAPSSKSTSGGTAALGCLVKDYFPEPVTVSWNSGALTSGVHTFPAVLQSSGLYSLSSVVTVPSSSLGTQTYICNVNHKPSNTKVDKRVEPKSCDKTHTCPPCPAPELLGGPSVFLFPPKPKDTLMISRTPEVTCVVVDVSHEDPEVKFNWYVDGVEVHNAKTKPREEQYNSTYRVVSVLTVLHQDWLNGKEYKCKVSNKALPAPIEKTISKAKGQPRRPRVYTLPPSREEMTDNQVSLVCLVKGFYPSDIAVEWESNGQPENNYKTTPPVLHSDGSFFLASQLTVDKSRWQQGNVFSCSVMHEALHNHYTQKSLSLSP

SEQ ID NO: 209 - protein, 447 aa, Homo sapiens
QVQLQESGPGLVRPSQTLSLTCTVSGYSITSDHAWSWVRQPPGRGLEWIGYISYSGITTYNPSLKSRVTMLRDTSKNQFSLRLSSVTAADTAVYYCARSLARTTAMDYWGQGSLVTVSSASTKGPSVFPLAPSSKSTSGGTAALGCLVKDYFPEPVTVSWNSGALTSGVHTFPAVLQSSGLYSLSSVVTVPSSSLGTQTYICNVNHKPSNTKVDKRVEPKSCDKTHTCPPCPAPELLGGPSVFLFPPKPKDTLMISRTPEVTCVVVDVSHEDPEVKFNWYVDGVEVHNAKTKPREEQYNSTYRVVSVLTVLHQDWLNGKEYKCKVSNKALPAPIEKTISKAKGQPRRPRVYTLPPSREEMTDNQVSLVCLVKGFYPSDIAVEWESNGQPENNYKTTPPVLISDGSFFLASQLTVDKSRWQQGNVFSCSVMHEALHNHYTQKSLSLSP

SEQ ID NO: 210 - protein, 447 aa, Homo sapiens
QVQLQESGPGLVRPSQTLSLTCTVSGYSITSDHAWSWVRQPPGRGLEWIGYISYSGITTYNPSLKSRVTMLRDTSKNQFSLRLSSVTAADTAVYYCARSLARTTAMDYWGQGSLVTVSSASTKGPSVFPLAPSSKSTSGGTAALGCLVKDYFPEPVTVSWNSGALTSGVHTFPAVLQSSGLYSLSSVVTVPSSSLGTQTYICNVNHKPSNTKVDKRVEPKSCDKTHTCPPCPAPELLGGPSVFLFPPKPKDTLMISRTPEVTCVVVDVSHEDPEVKFNWYVDGVEVHNAKTKPREEQYNSTYRVVSVLTVLHQDWLNGKEYKCKVSNKALPAPIEKTISKAKGQPRRPRVYTLPPSREEMTDNQVSLVCLVKGFYPSDIAVEWESNGQPENNYKTTPPVLFSDGSFFLASQLTVDKSRWQQGNVFSCSVMHEALHNHYTQKSLSLSP

SEQ ID NO: 211 - protein, 447 aa, Homo sapiens
QVQLQESGPGLVRPSQTLSLTCTVSGYSITSDHAWSWVRQPPGRGLEWIGYISYSGITTYNPSLKSRVTMLRDTSKNQFSLRLSSVTAADTAVYYCARSLARTTAMDYWGQGSLVTVSSASTKGPSVFPLAPSSKSTSGGTAALGCLVKDYFPEPVTVSWNSGALTSGVHTFPAVLQSSGLYSLSSVVTVPSSSLGTQTYICNVNHKPSNTKVDKRVEPKSCDKTHTCPPCPAPELLGGPSVFLFPPKPKDTLMISRTPEVTCVVVDVSHEDPEVKFNWYVDGVEVHNAKTKPREEQYNSTYRVVSVLTVLHQDWLNGKEYKCKVSNKALPAPIEKTISKAKGQPRRPRVYTLPPSREEMTDNQVSLVCLVKGFYPSDIAVEWESNGQPENNYKTTPPVLYSDGSFFLASQLTVDKSRWQQGNVFSCSVMHEALHNHYTQKSLSLSP

SEQ ID NO: 212 - protein, 447 aa, Homo sapiens
QVQLQESGPGLVRPSQTLSLTCTVSGYSITSDHAWSWVRQPPGRGLEWIGYISYSGITTYNPSLKSRVTMLRDTSKNQFSLRLSSVTAADTAVYYCARSLARTTAMDYWGQGSLVTVSSASTKGPSVFPLAPSSKSTSGGTAALGCLVKDYFPEPVTVSWNSGALTSGVHTFPAVLQSSGLYSLSSVVTVPSSSLGTQTYICNVNHKPSNTKVDKRVEPKSCDKTHTCPPCPAPELLGGPSVFLFPPKPKDTLMISRTPEVTCVVVDVSHEDPEVKFNWYVDGVEVHNAKTKPREEQYNSTYRVVSVLTVLHQDWLNGKEYKCKVSNKALPAPIEKTISKAKGQPRRPRVYTLPPSREEMTDNQVSLVCLVKGFYPSDIAVEWESNGQPENNYKTTPPVLTSDGSFFLASQLTVDKSRWQQGNVFSCSVMHEALHNHYTQKSLSLSP

SEQ ID NO: 213 - protein, 447 aa, Homo sapiens
QVQLQESGPGLVRPSQTLSLTCTVSGYSITSDHAWSWVRQPPGRGLEWIGYISYSGITTYNPSLKSRVTMLRDTSKNQFSLRLSSVTAADTAVYYCARSLARTTAMDYWGQGSLVTVSSASTKGPSVFPLAPSSKSTSGGTAALGCLVKDYFPEPVTVSWNSGALTSGVHTFPAVLQSSGLYSLSSVVTVPSSSLGTQTYICNVNHKPSNTKVDKRVEPKSCDKTHTCPPCPAPELLGGPSVFLFPPKPKDTLMISRTPEVTCVVVDVSHEDPEVKFNWYVDGVEVHNAKTKPREEQYNSTYRVVSVLTVLHQDWLNGKEYKCKVSNKALPAPIEKTISKAKGQPRRPRVYTLPPSREEMTDNQVSLVCLVKGFYPSDIAVEWESNGQPENNYKTTPPVLSSDGSFFLASQLTVDKSRWQQGNVFSCSVMHEALHNHYTQKSLSLSP

SEQ ID NO: 214 - protein, 447 aa, Homo sapiens
QVQLQESGPGLVRPSQTLSLTCTVSGYSITSDHAWSWVRQPPGRGLEWIGYISYSGITTYNPSLKSRVTMLRDTSKNQFSLRLSSVTAADTAVYYCARSLARTTAMDYWGQGSLVTVSSASTKGPSVFPLAPSSKSTSGGTAALGCLVKDYFPEPVTVSWNSGALTSGVHTFPAVLQSSGLYSLSSVVTVPSSSLGTQTYICNVNHKPSNTKVDKRVEPKSCDKTHTCPPCPAPELLGGPSVFLFPPKPKDTLMISRTPEVTCVVVDVSHEDPEVKFNWYVDGVEVHNAKTKPREEQYNSTYRVVSVLTVLHQDWLNGKEYKCKVSNKALPAPIEKTISKAKGQPRRPRVYTLPPSREEMTDNQVSLVCLVKGFYPSDIAVEWESNGQPENNYKTTPPVLQSDGSFFLASNLTVDKSRWQQGNVFSCSVMHEALHNHYTQKSLSLSP

SEQ ID NO: 215 - protein, 447 aa, Homo sapiens
QVQLQESGPGLVRPSQTLSLTCTVSGYSITSDHAWSWVRQPPGRGLEWIGYISYSGITTYNPSLKSRVTMLRDTSKNQFSLRLSSVTAADTAVYYCARSLARTTAMDYWGQGSLVTVSSASTKGPSVFPLAPSSKSTSGGTAALGCLVKDYFPEPVTVSWNSGALTSGVHTFPAVLQSSGLYSLSSVVTVPSSSLGTQTYICNVNHKPSNTKVDKRVEPKSCDKTHTCPPCPAPELLGGPSVFLFPPKPKDTLMISRTPEVTCVVVDVSHEDPEVKFNWYVDGVEVHNAKTKPREEQYNSTYRVVSVLTVLHQDWLNGKEYKCKVSNKALPAPIEKTISKAKGQPRRPRVYTLPPSREEMTDNQVSLVCLVKGFYPSDIAVEWESNGQPENNYKTTPPVLHSDGSFFLASNLTVDKSRWQQGNVFSCSVMHEALHNHYTQKSLSLSP

SEQ ID NO: 216 - protein, 447 aa, Homo sapiens
QVQLQESGPGLVRPSQTLSLTCTVSGYSITSDHAWSWVRQPPGRGLEWIGYISYSGITTYNPSLKSRVTMLRDTSKNQFSLRLSSVTAADTAVYYCARSLARTTAMDYWGQGSLVTVSSASTKGPSVFPLAPSSKSTSGGTAALGCLVKDYFPEPVTVSWNSGALTSGVHTFPAVLQSSGLYSLSSVVTVPSSSLGTQTYICNVNHKPSNTKVDKRVEPKSCDKTHTCPPCPAPELLGGPSVFLFPPKPKDTLMISRTPEVTCVVVDVSHEDPEVKFNWYVDGVEVHNAKTKPREEQYNSTYRVVSVLTVLHQDWLNGKEYKCKVSNKALPAPIEKTISKAKGQPRRPRVYTLPPSREEMTDNQVSLVCLVKGFYPSDIAVEWESNGQPENNYKTTPPVLVSDGSFFLASNLTVDKSRWQQGNVFSCSVMHEALHNHYTQKSLSLSP

SEQ ID NO: 217 - protein, 447 aa, Homo sapiens
QVQLQESGPGLVRPSQTLSLTCTVSGYSITSDHAWSWVRQPPGRGLEWIGYISYSGITTYNPSLKSRVTMLRDTSKNQFSLRLSSVTAADTAVYYCARSLARTTAMDYWGQGSLVTVSSASTKGPSVFPLAPSSKSTSGGTAALGCLVKDYFPEPVTVSWNSGALTSGVHTFPAVLQSSGLYSLSSVVTVPSSSLGTQTYICNVNHKPSNTKVDKRVEPKSCDKTHTCPPCPAPELLGGPSVFLFPPKPKDTLMISRTPEVTCVVVDVSHEDPEVKFNWYVDGVEVHNAKTKPREEQYNSTYRVVSVLTVLHQDWLNGKEYKCKVSNKALPAPIEKTISKAKGQPRRPRVYTLPPSREEMTDNQVSLVCLVKGFYPSDIAVEWESNGQPENNYKTTPPVLLSDGSFFLASNLTVDKSRWQQGNVFSCSVMHEALHNHYTQKSLSLSP

SEQ ID NO: 218 - protein, 447 aa, Homo sapiens
QVQLQESGPGLVRPSQTLSLTCTVSGYSITSDHAWSWVRQPPGRGLEWIGYISYSGITTYNPSLKSRVTMLRDTSKNQFSLRLSSVTAADTAVYYCARSLARTTAMDYWGQGSLVTVSSASTKGPSVFPLAPSSKSTSGGTAALGCLVKDYFPEPVTVSWNSGALTSGVHTFPAVLQSSGLYSLSSVVTVPSSSLGTQTYICNVNHKPSNTKVDKRVEPKSCDKTHTCPPCPAPELLGGPSVFLFPPKPKDTLMISRTPEVTCVVVDVSHEDPEVKFNWYVDGVEVHNAKTKPREEQYNSTYRVVSVLTVLHQDWLNGKEYKCKVSNKALPAPIEKTISKAKGQPRRPRVYTLPPSREEMTDNQVSLVCLVKGFYPSDIAVEWESNGQPENNYKTTPPVLFSDGSFFLASNLTVDKSRWQQGNVFSCSVMHEALHNHYTQKSLSLSP

SEQ ID NO: 219 - protein, 447 aa, Homo sapiens
QVQLQESGPGLVRPSQTLSLTCTVSGYSITSDHAWSWVRQPPGRGLEWIGYISYSGITTYNPSLKSRVTMLRDTSKNQFSLRLSSVTAADTAVYYCARSLARTTAMDYWGQGSLVTVSSASTKGPSVFPLAPSSKSTSGGTAALGCLVKDYFPEPVTVSWNSGALTSGVHTFPAVLQSSGLYSLSSVVTVPSSSLGTQTYICNVNHKPSNTKVDKRVEPKSCDKTHTCPPCPAPELLGGPSVFLFPPKPKDTLMISRTPEVTCVVVDVSHEDPEVKFNWYVDGVEVHNAKTKPREEQYNSTYRVVSVLTVLHQDWLNGKEYKCKVSNKALPAPIEKTISKAKGQPRRPRVYTLPPSREEMTDNQVSLVCLVKGFYPSDIAVEWESNGQPENNYKTTPPVLYSDGSFFLASNLTVDKSRWQQGNVFSCSVMHEALHNHYTQKSLSLSP

SEQ ID NO: 220 - protein, 447 aa, Homo sapiens
QVQLQESGPGLVRPSQTLSLTCTVSGYSITSDHAWSWVRQPPGRGLEWIGYISYSGITTYNPSLKSRVTMLRDTSKNQFSLRLSSVTAADTAVYYCARSLARTTAMDYWGQGSLVTVSSASTKGPSVFPLAPSSKSTSGGTAALGCLVKDYFPEPVTVSWNSGALTSGVHTFPAVLQSSGLYSLSSVVTVPSSSLGTQTYICNVNHKPSNTKVDKRVEPKSCDKTHTCPPCPAPELLGGPSVFLFPPKPKDTLMISRTPEVTCVVVDVSHEDPEVKFNWYVDGVEVHNAKTKPREEQYNSTYRVVSVLTVLHQDWLNGKEYKCKVSNKALPAPIEKTISKAKGQPRRPRVYTLPPSREEMTDNQVSLVCLVKGFYPSDIAVEWESNGQPENNYKTTPPVLTSDGSFFLASNLTVDKSRWQQGNVFSCSVMHEALHNHYTQKSLSLSP

SEQ ID NO: 221 - protein, 447 aa, Homo sapiens
QVQLQESGPGLVRPSQTLSLTCTVSGYSITSDHAWSWVRQPPGRGLEWIGYISYSGITTYNPSLKSRVTMLRDTSKNQFSLRLSSVTAADTAVYYCARSLARTTAMDYWGQGSLVTVSSASTKGPSVFPLAPSSKSTSGGTAALGCLVKDYFPEPVTVSWNSGALTSGVHTFPAVLQSSGLYSLSSVVTVPSSSLGTQTYICNVNHKPSNTKVDKRVEPKSCDKTHTCPPCPAPELLGGPSVFLFPPKPKDTLMISRTPEVTCVVVDVSHEDPEVKFNWYVDGVEVHNAKTKPREEQYNSTYRVVSVLTVLHQDWLNGKEYKCKVSNKALPAPIEKTISKAKGQPRRPRVYTLPPSREEMTDNQVSLVCLVKGFYPSDIAVEWESNGQPENNYKTTPPVLSSDGSFFLASNLTVDKSRWQQGNVFSCSVMHEALHNHYTQKSLSLSP

SEQ ID NO: 222 - protein, 447 aa, Homo sapiens
QVQLQESGPGLVRPSQTLSLTCTVSGYSITSDHAWSWVRQPPGRGLEWIGYISYSGITTYNPSLKSRVTMLRDTSKNQFSLRLSSVTAADTAVYYCARSLARTTAMDYWGQGSLVTVSSASTKGPSVFPLAPSSKSTSGGTAALGCLVKDYFPEPVTVSWNSGALTSGVHTFPAVLQSSGLYSLSSVVTVPSSSLGTQTYICNVNHKPSNTKVDKRVEPKSCDKTHTCPPCPAPELLGGPSVFLFPPKPKDTLMISRTPEVTCVVVDVSHEDPEVKFNWYVDGVEVHNAKTKPREEQYNSTYRVVSVLTVLHQDWLNGKEYKCKVSNKALPAPIEKTISKAKGQPRRPRVYTLPPSREEMTDNQVSLVCLVKGFYPSDIAVEWESNGQPENNYKTTPPVLQSDGSFFLASHLTVDKSRWQQGNVFSCSVMHEALHNHYTQKSLSLSP

SEQ ID NO: 223 - protein, 447 aa, Homo sapiens
QVQLQESGPGLVRPSQTLSLTCTVSGYSITSDHAWSWVRQPPGRGLEWIGYISYSGITTYNPSLKSRVTMLRDTSKNQFSLRLSSVTAADTAVYYCARSLARTTAMDYWGQGSLVTVSSASTKGPSVFPLAPSSKSTSGGTAALGCLVKDYFPEPVTVSWNSGALTSGVHTFPAVLQSSGLYSLSSVVTVPSSSLGTQTYICNVNHKPSNTKVDKRVEPKSCDKTHTCPPCPAPELLGGPSVFLFPPKPKDTLMISRTPEVTCVVVDVSHEDPEVKFNWYVDGVEVHNAKTKPREEQYNSTYRVVSVLTVLHQDWLNGKEYKCKVSNKALPAPIEKTISKAKGQPRRPRVYTLPPSREEMTDNQVSLVCLVKGFYPSDIAVEWESNGQPENNYKTTPPVLNSDGSFFLASHLTVDKSRWQQGNVFSCSVMHEALHNHYTQKSLSLSP

SEQ ID NO: 224 - protein, 447 aa, Homo sapiens
QVQLQESGPGLVRPSQTLSLTCTVSGYSITSDHAWSWVRQPPGRGLEWIGYISYSGITTYNPSLKSRVTMLRDTSKNQFSLRLSSVTAADTAVYYCARSLARTTAMDYWGQGSLVTVSSASTKGPSVFPLAPSSKSTSGGTAALGCLVKDYFPEPVTVSWNSGALTSGVHTFPAVLQSSGLYSLSSVVTVPSSSLGTQTYICNVNHKPSNTKVDKRVEPKSCDKTHTCPPCPAPELLGGPSVFLFPPKPKDTLMISRTPEVTCVVVDVSHEDPEVKFNWYVDGVEVHNAKTKPREEQYNSTYRVVSVLTVLHQDWLNGKEYKCKVSNKALPAPIEKTISKAKGQPRRPRVYTLPPSREEMTDNQVSLVCLVKGFYPSDIAVEWESNGQPENNYKTTPPVLHSDGSFFLASHLTVDKSRWQQGNVFSCSVMHEALHNHYTQKSLSLSP

SEQ ID NO: 225 - protein, 447 aa, Homo sapiens
QVQLQESGPGLVRPSQTLSLTCTVSGYSITSDHAWSWVRQPPGRGLEWIGYISYSGITTYNPSLKSRVTMLRDTSKNQFSLRLSSVTAADTAVYYCARSLARTTAMDYWGQGSLVTVSSASTKGPSVFPLAPSSKSTSGGTAALGCLVKDYFPEPVTVSWNSGALTSGVHTFPAVLQSSGLYSLSSVVTVPSSSLGTQTYICNVNHKPSNTKVDKRVEPKSCDKTHTCPPCPAPELLGGPSVFLFPPKPKDTLMISRTPEVTCVVVDVSHEDPEVKFNWYVDGVEVHNAKTKPREEQYNSTYRVVSVLTVLHQDWLNGKEYKCKVSNKALPAPIEKTISKAKGQPRRPRVYTLPPSREEMTDNQVSLVCLVKGFYPSDIAVEWESNGQPENNYKTTPPVLVSDGSFFLASHLTVDKSRWQQGNVFSCSVMHEALHNHYTQKSLSLSP

SEQ ID NO: 226 - protein, 447 aa, Homo sapiens
QVQLQESGPGLVRPSQTLSLTCTVSGYSITSDHAWSWVRQPPGRGLEWIGYISYSGITTYNPSLKSRVTMLRDTSKNQFSLRLSSVTAADTAVYYCARSLARTTAMDYWGQGSLVTVSSASTKGPSVFPLAPSSKSTSGGTAALGCLVKDYFPEPVTVSWNSGALTSGVHTFPAVLQSSGLYSLSSVVTVPSSSLGTQTYICNVNHKPSNTKVDKRVEPKSCDKTHTCPPCPAPELLGGPSVFLFPPKPKDTLMISRTPEVTCVVVDVSHEDPEVKFNWYVDGVEVHNAKTKPREEQYNSTYRVVSVLTVLHQDWLNGKEYKCKVSNKALPAPIEKTISKAKGQPRRPRVYTLPPSREEMTDNQVSLVCLVKGFYPSDIAVEWESNGQPENNYKTTPPVLLSDGSFFLASHLTVDKSRWQQGNVFSCSVMHEALHNHYTQKSLSLSP

SEQ ID NO: 227 - protein, 447 aa, Homo sapiens
QVQLQESGPGLVRPSQTLSLTCTVSGYSITSDHAWSWVRQPPGRGLEWIGYISYSGITTYNPSLKSRVTMLRDTSKNQFSLRLSSVTAADTAVYYCARSLARTTAMDYWGQGSLVTVSSASTKGPSVFPLAPSSKSTSGGTAALGCLVKDYFPEPVTVSWNSGALTSGVHTFPAVLQSSGLYSLSSVVTVPSSSLGTQTYICNVNHKPSNTKVDKRVEPKSCDKTHTCPPCPAPELLGGPSVFLFPPKPKDTLMISRTPEVTCVVVDVSHEDPEVKFNWYVDGVEVHNAKTKPREEQYNSTYRVVSVLTVLHQDWLNGKEYKCKVSNKALPAPIEKTISKAKGQPRRPRVYTLPPSREEMTDNQVSLVCLVKGFYPSDIAVEWESNGQPENNYKTTPPVLFSDGSFFLASHLTVDKSRWQQGNVFSCSVMHEALHNHYTQKSLSLSP

SEQ ID NO: 228 - protein, 447 aa, Homo sapiens
QVQLQESGPGLVRPSQTLSLTCTVSGYSITSDHAWSWVRQPPGRGLEWIGYISYSGITTYNPSLKSRVTMLRDTSKNQFSLRLSSVTAADTAVYYCARSLARTTAMDYWGQGSLVTVSSASTKGPSVFPLAPSSKSTSGGTAALGCLVKDYFPEPVTVSWNSGALTSGVHTFPAVLQSSGLYSLSSVVTVPSSSLGTQTYICNVNHKPSNTKVDKRVEPKSCDKTHTCPPCPAPELLGGPSVFLFPPKPKDTLMISRTPEVTCVVVDVSHEDPEVKFNWYVDGVEVHNAKTKPREEQYNSTYRVVSVLTVLHQDWLNGKEYKCKVSNKALPAPIEKTISKAKGQPRRPRVYTLPPSREEMTDNQVSLVCLVKGFYPSDIAVEWESNGQPENNYKTTPPVLYSDGSFFLASHLTVDKSRWQQGNVFSCSVMHEALHNHYTQKSLSLSP

SEQ ID NO: 229 - protein, 447 aa, Homo sapiens
QVQLQESGPGLVRPSQTLSLTCTVSGYSITSDHAWSWVRQPPGRGLEWIGYISYSGITTYNPSLKSRVTMLRDTSKNQFSLRLSSVTAADTAVYYCARSLARTTAMDYWGQGSLVTVSSASTKGPSVFPLAPSSKSTSGGTAALGCLVKDYFPEPVTVSWNSGALTSGVHTFPAVLQSSGLYSLSSVVTVPSSSLGTQTYICNVNHKPSNTKVDKRVEPKSCDKTHTCPPCPAPELLGGPSVFLFPPKPKDTLMISRTPEVTCVVVDVSHEDPEVKFNWYVDGVEVHNAKTKPREEQYNSTYRVVSVLTVLHQDWLNGKEYKCKVSNKALPAPIEKTISKAKGQPRRPRVYTLPPSREEMTDNQVSLVCLVKGFYPSDIAVEWESNGQPENNYKTTPPVLTSDGSFFLASHLTVDKSRWQQGNVFSCSVMHEALHNHYTQKSLSLSP

SEQ ID NO: 230 - protein, 447 aa, Homo sapiens
QVQLQESGPGLVRPSQTLSLTCTVSGYSITSDHAWSWVRQPPGRGLEWIGYISYSGITTYNPSLKSRVTMLRDTSKNQFSLRLSSVTAADTAVYYCARSLARTTAMDYWGQGSLVTVSSASTKGPSVFPLAPSSKSTSGGTAALGCLVKDYFPEPVTVSWNSGALTSGVHTFPAVLQSSGLYSLSSVVTVPSSSLGTQTYICNVNHKPSNTKVDKRVEPKSCDKTHTCPPCPAPELLGGPSVFLFPPKPKDTLMISRTPEVTCVVVDVSHEDPEVKFNWYVDGVEVHNAKTKPREEQYNSTYRVVSVLTVLHQDWLNGKEYKCKVSNKALPAPIEKTISKAKGQPRRPRVYTLPPSREEMTDNQVSLVCLVKGFYPSDIAVEWESNGQPENNYKTTPPVLSSDGSFFLASHLTVDKSRWQQGNVFSCSVMHEALHNHYTQKSLSLSP

SEQ ID NO: 231 - protein, 447 aa, Homo sapiens
QVQLQESGPGLVRPSQTLSLTCTVSGYSITSDHAWSWVRQPPGRGLEWIGYISYSGITTYNPSLKSRVTMLRDTSKNQFSLRLSSVTAADTAVYYCARSLARTTAMDYWGQGSLVTVSSASTKGPSVFPLAPSSKSTSGGTAALGCLVKDYFPEPVTVSWNSGALTSGVHTFPAVLQSSGLYSLSSVVTVPSSSLGTQTYICNVNHKPSNTKVDKRVEPKSCDKTHTCPPCPAPELLGGPSVFLFPPKPKDTLMISRTPEVTCVVVDVSHEDPEVKFNWYVDGVEVHNAKTKPREEQYNSTYRVVSVLTVLHQDWLNGKEYKCKVSNKALPAPIEKTISKAKGQPRRPRVYTLPPSREEMTDNQVSLVCLVKGFYPSDIAVEWESNGQPENNYKTTPPVLQSDGSFFLASVLTVDKSRWQQGNVFSCSVMHEALHNHYTQKSLSLSP

SEQ ID NO: 232 - protein, 447 aa, Homo sapiens
QVQLQESGPGLVRPSQTLSLTCTVSGYSITSDHAWSWVRQPPGRGLEWIGYISYSGITTYNPSLKSRVTMLRDTSKNQFSLRLSSVTAADTAVYYCARSLARTTAMDYWGQGSLVTVSSASTKGPSVFPLAPSSKSTSGGTAALGCLVKDYFPEPVTVSWNSGALTSGVHTFPAVLQSSGLYSLSSVVTVPSSSLGTQTYICNVNHKPSNTKVDKRVEPKSCDKTHTCPPCPAPELLGGPSVFLFPPKPKDTLMISRTPEVTCVVVDVSHEDPEVKFNWYVDGVEVHNAKTKPREEQYNSTYRVVSVLTVLHQDWLNGKEYKCKVSNKALPAPIEKTISKAKGQPRRPRVYTLPPSREEMTDNQVSLVCLVKGFYPSDIAVEWESNGQPENNYKTTPPVLNSDGSFFLASVLTVDKSRWQQGNVFSCSVMHEALHNHYTQKSLSLSP

SEQ ID NO: 233 - protein, 447 aa, Homo sapiens
QVQLQESGPGLVRPSQTLSLTCTVSGYSITSDHAWSWVRQPPGRGLEWIGYISYSGITTYNPSLKSRVTMLRDTSKNQFSLRLSSVTAADTAVYYCARSLARTTAMDYWGQGSLVTVSSASTKGPSVFPLAPSSKSTSGGTAALGCLVKDYFPEPVTVSWNSGALTSGVHTFPAVLQSSGLYSLSSVVTVPSSSLGTQTYICNVNHKPSNTKVDKRVEPKSCDKTHTCPPCPAPELLGGPSVFLFPPKPKDTLMISRTPEVTCVVVDVSHEDPEVKFNWYVDGVEVHNAKTKPREEQYNSTYRVVSVLTVLHQDWLNGKEYKCKVSNKALPAPIEKTISKAKGQPRRPRVYTLPPSREEMTDNQVSLVCLVKGFYPSDIAVEWESNGQPENNYKTTPPVLHSDGSFFLASVLTVDKSRWQQGNVFSCSVMHEALHNHYTQKSLSLSP

SEQ ID NO: 234 - protein, 447 aa, Homo sapiens
QVQLQESGPGLVRPSQTLSLTCTVSGYSITSDHAWSWVRQPPGRGLEWIGYISYSGITTYNPSLKSRVTMLRDTSKNQFSLRLSSVTAADTAVYYCARSLARTTAMDYWGQGSLVTVSSASTKGPSVFPLAPSSKSTSGGTAALGCLVKDYFPEPVTVSWNSGALTSGVHTFPAVLQSSGLYSLSSVVTVPSSSLGTQTYICNVNHKPSNTKVDKRVEPKSCDKTHTCPPCPAPELLGGPSVFLFPPKPKDTLMISRTPEVTCVVVDVSHEDPEVKFNWYVDGVEVHNAKTKPREEQYNSTYRVVSVLTVLHQDWLNGKEYKCKVSNKALPAPIEKTISKAKGQPRRPRVYTLPPSREEMTDNQVSLVCLVKGFYPSDIAVEWESNGQPENNYKTTPPVLVSDGSFFLASVLTVDKSRWQQGNVFSCSVMHEALHNHYTQKSLSLSP

SEQ ID NO: 235 - protein, 447 aa, Homo sapiens
QVQLQESGPGLVRPSQTLSLTCTVSGYSITSDHAWSWVRQPPGRGLEWIGYISYSGITTYNPSLKSRVTMLRDTSKNQFSLRLSSVTAADTAVYYCARSLARTTAMDYWGQGSLVTVSSASTKGPSVFPLAPSSKSTSGGTAALGCLVKDYFPEPVTVSWNSGALTSGVHTFPAVLQSSGLYSLSSVVTVPSSSLGTQTYICNVNHKPSNTKVDKRVEPKSCDKTHTCPPCPAPELLGGPSVFLFPPKPKDTLMISRTPEVTCVVVDVSHEDPEVKFNWYVDGVEVHNAKTKPREEQYNSTYRVVSVLTVLHQDWLNGKEYKCKVSNKALPAPIEKTISKAKGQPRRPRVYTLPPSREEMTDNQVSLVCLVKGFYPSDIAVEWESNGQPENNYKTTPPVLLSDGSFFLASVLTVDKSRWQQGNVFSCSVMHEALHNHYTQKSLSLSP

SEQ ID NO: 236 - protein, 447 aa, Homo sapiens
QVQLQESGPGLVRPSQTLSLTCTVSGYSITSDHAWSWVRQPPGRGLEWIGYISYSGITTYNPSLKSRVTMLRDTSKNQFSLRLSSVTAADTAVYYCARSLARTTAMDYWGQGSLVTVSSASTKGPSVFPLAPSSKSTSGGTAALGCLVKDYFPEPVTVSWNSGALTSGVHTFPAVLQSSGLYSLSSVVTVPSSSLGTQTYICNVNHKPSNTKVDKRVEPKSCDKTHTCPPCPAPELLGGPSVFLFPPKPKDTLMISRTPEVTCVVVDVSHEDPEVKFNWYVDGVEVHNAKTKPREEQYNSTYRVVSVLTVLHQDWLNGKEYKCKVSNKALPAPIEKTISKAKGQPRRPRVYTLPPSREEMTDNQVSLVCLVKGFYPSDIAVEWESNGQPENNYKTTPPVLISDGSFFLASVLTVDKSRWQQGNVFSCSVMHEALHNHYTQKSLSLSP

SEQ ID NO: 237 - protein, 447 aa, Homo sapiens
QVQLQESGPGLVRPSQTLSLTCTVSGYSITSDHAWSWVRQPPGRGLEWIGYISYSGITTYNPSLKSRVTMLRDTSKNQFSLRLSSVTAADTAVYYCARSLARTTAMDYWGQGSLVTVSSASTKGPSVFPLAPSSKSTSGGTAALGCLVKDYFPEPVTVSWNSGALTSGVHTFPAVLQSSGLYSLSSVVTVPSSSLGTQTYICNVNHKPSNTKVDKRVEPKSCDKTHTCPPCPAPELLGGPSVFLFPPKPKDTLMISRTPEVTCVVVDVSHEDPEVKFNWYVDGVEVHNAKTKPREEQYNSTYRVVSVLTVLHQDWLNGKEYKCKVSNKALPAPIEKTISKAKGQPRRPRVYTLPPSREEMTDNQVSLVCLVKGFYPSDIAVEWESNGQPENNYKTTPPVLFSDGSFFLASVLTVDKSRWQQGNVFSCSVMHEALHNHYTQKSLSLSP

SEQ ID NO: 238 - protein, 447 aa, Homo sapiens
QVQLQESGPGLVRPSQTLSLTCTVSGYSITSDHAWSWVRQPPGRGLEWIGYISYSGITTYNPSLKSRVTMLRDTSKNQFSLRLSSVTAADTAVYYCARSLARTTAMDYWGQGSLVTVSSASTKGPSVFPLAPSSKSTSGGTAALGCLVKDYFPEPVTVSWNSGALTSGVHTFPAVLQSSGLYSLSSVVTVPSSSLGTQTYICNVNHKPSNTKVDKRVEPKSCDKTHTCPPCPAPELLGGPSVFLFPPKPKDTLMISRTPEVTCVVVDVSHEDPEVKFNWYVDGVEVHNAKTKPREEQYNSTYRVVSVLTVLHQDWLNGKEYKCKVSNKALPAPIEKTISKAKGQPRRPRVYTLPPSREEMTDNQVSLVCLVKGFYPSDIAVEWESNGQPENNYKTTPPVLYSDGSFFLASVLTVDKSRWQQGNVFSCSVMHEALHNHYTQKSLSLSP

SEQ ID NO: 239 - protein, 447 aa, Homo sapiens
QVQLQESGPGLVRPSQTLSLTCTVSGYSITSDHAWSWVRQPPGRGLEWIGYISYSGITTYNPSLKSRVTMLRDTSKNQFSLRLSSVTAADTAVYYCARSLARTTAMDYWGQGSLVTVSSASTKGPSVFPLAPSSKSTSGGTAALGCLVKDYFPEPVTVSWNSGALTSGVHTFPAVLQSSGLYSLSSVVTVPSSSLGTQTYICNVNHKPSNTKVDKRVEPKSCDKTHTCPPCPAPELLGGPSVFLFPPKPKDTLMISRTPEVTCVVVDVSHEDPEVKFNWYVDGVEVHNAKTKPREEQYNSTYRVVSVLTVLHQDWLNGKEYKCKVSNKALPAPIEKTISKAKGQPRRPRVYTLPPSREEMTDNQVSLVCLVKGFYPSDIAVEWESNGQPENNYKTTPPVLTSDGSFFLASVLTVDKSRWQQGNVFSCSVMHEALHNHYTQKSLSLSP

SEQ ID NO: 240 - protein, 447 aa, Homo sapiens
QVQLQESGPGLVRPSQTLSLTCTVSGYSITSDHAWSWVRQPPGRGLEWIGYISYSGITTYNPSLKSRVTMLRDTSKNQFSLRLSSVTAADTAVYYCARSLARTTAMDYWGQGSLVTVSSASTKGPSVFPLAPSSKSTSGGTAALGCLVKDYFPEPVTVSWNSGALTSGVHTFPAVLQSSGLYSLSSVVTVPSSSLGTQTYICNVNHKPSNTKVDKRVEPKSCDKTHTCPPCPAPELLGGPSVFLFPPKPKDTLMISRTPEVTCVVVDVSHEDPEVKFNWYVDGVEVHNAKTKPREEQYNSTYRVVSVLTVLHQDWLNGKEYKCKVSNKALPAPIEKTISKAKGQPRRPRVYTLPPSREEMTDNQVSLVCLVKGFYPSDIAVEWESNGQPENNYKTTPPVLSSDGSFFLASVLTVDKSRWQQGNVFSCSVMHEALHNHYTQKSLSLSP

SEQ ID NO: 241 - protein, 447 aa, Homo sapiens
QVQLQESGPGLVRPSQTLSLTCTVSGYSITSDHAWSWVRQPPGRGLEWIGYISYSGITTYNPSLKSRVTMLRDTSKNQFSLRLSSVTAADTAVYYCARSLARTTAMDYWGQGSLVTVSSASTKGPSVFPLAPSSKSTSGGTAALGCLVKDYFPEPVTVSWNSGALTSGVHTFPAVLQSSGLYSLSSVVTVPSSSLGTQTYICNVNHKPSNTKVDKRVEPKSCDKTHTCPPCPAPELLGGPSVFLFPPKPKDTLMISRTPEVTCVVVDVSHEDPEVKFNWYVDGVEVHNAKTKPREEQYNSTYRVVSVLTVLHQDWLNGKEYKCKVSNKALPAPIEKTISKAKGQPRRPRVYTLPPSREEMTDNQVSLVCLVKGFYPSDIAVEWESNGQPENNYKTTPPVLQSDGSFFLASLLTVDKSRWQQGNVFSCSVMHEALHNHYTQKSLSLSP

SEQ ID NO: 242 - protein, 447 aa, Homo sapiens
QVQLQESGPGLVRPSQTLSLTCTVSGYSITSDHAWSWVRQPPGRGLEWIGYISYSGITTYNPSLKSRVTMLRDTSKNQFSLRLSSVTAADTAVYYCARSLARTTAMDYWGQGSLVTVSSASTKGPSVFPLAPSSKSTSGGTAALGCLVKDYFPEPVTVSWNSGALTSGVHTFPAVLQSSGLYSLSSVVTVPSSSLGTQTYICNVNHKPSNTKVDKRVEPKSCDKTHTCPPCPAPELLGGPSVFLFPPKPKDTLMISRTPEVTCVVVDVSHEDPEVKFNWYVDGVEVHNAKTKPREEQYNSTYRVVSVLTVLHQDWLNGKEYKCKVSNKALPAPIEKTISKAKGQPRRPRVYTLPPSREEMTDNQVSLVCLVKGFYPSDIAVEWESNGQPENNYKTTPPVLNSDGSFFLASLLTVDKSRWQQGNVFSCSVMHEALHNHYTQKSLSLSP

SEQ ID NO: 243 - protein, 447 aa, Homo sapiens
QVQLQESGPGLVRPSQTLSLTCTVSGYSITSDHAWSWVRQPPGRGLEWIGYISYSGITTYNPSLKSRVTMLRDTSKNQFSLRLSSVTAADTAVYYCARSLARTTAMDYWGQGSLVTVSSASTKGPSVFPLAPSSKSTSGGTAALGCLVKDYFPEPVTVSWNSGALTSGVHTFPAVLQSSGLYSLSSVVTVPSSSLGTQTYICNVNHKPSNTKVDKRVEPKSCDKTHTCPPCPAPELLGGPSVFLFPPKPKDTLMISRTPEVTCVVVDVSHEDPEVKFNWYVDGVEVHNAKTKPREEQYNSTYRVVSVLTVLHQDWLNGKEYKCKVSNKALPAPIEKTISKAKGQPRRPRVYTLPPSREEMTDNQVSLVCLVKGFYPSDIAVEWESNGQPENNYKTTPPVLHSDGSFFLASLLTVDKSRWQQGNVFSCSVMHEALHNHYTQKSLSLSP

SEQ ID NO: 244 - protein, 447 aa, Homo sapiens
QVQLQESGPGLVRPSQTLSLTCTVSGYSITSDHAWSWVRQPPGRGLEWIGYISYSGITTYNPSLKSRVTMLRDTSKNQFSLRLSSVTAADTAVYYCARSLARTTAMDYWGQGSLVTVSSASTKGPSVFPLAPSSKSTSGGTAALGCLVKDYFPEPVTVSWNSGALTSGVHTFPAVLQSSGLYSLSSVVTVPSSSLGTQTYICNVNHKPSNTKVDKRVEPKSCDKTHTCPPCPAPELLGGPSVFLFPPKPKDTLMISRTPEVTCVVVDVSHEDPEVKFNWYVDGVEVHNAKTKPREEQYNSTYRVVSVLTVLHQDWLNGKEYKCKVSNKALPAPIEKTISKAKGQPRRPRVYTLPPSREEMTDNQVSLVCLVKGFYPSDIAVEWESNGQPENNYKTTPPVLISDGSFFLASLLTVDKSRWQQGNVFSCSVMHEALHNHYTQKSLSLSP

SEQ ID NO: 245 - protein, 447 aa, Homo sapiens
QVQLQESGPGLVRPSQTLSLTCTVSGYSITSDHAWSWVRQPPGRGLEWIGYISYSGITTYNPSLKSRVTMLRDTSKNQFSLRLSSVTAADTAVYYCARSLARTTAMDYWGQGSLVTVSSASTKGPSVFPLAPSSKSTSGGTAALGCLVKDYFPEPVTVSWNSGALTSGVHTFPAVLQSSGLYSLSSVVTVPSSSLGTQTYICNVNHKPSNTKVDKRVEPKSCDKTHTCPPCPAPELLGGPSVFLFPPKPKDTLMISRTPEVTCVVVDVSHEDPEVKFNWYVDGVEVHNAKTKPREEQYNSTYRVVSVLTVLHQDWLNGKEYKCKVSNKALPAPIEKTISKAKGQPRRPRVYTLPPSREEMTDNQVSLVCLVKGFYPSDIAVEWESNGQPENNYKTTPPVLFSDGSFFLASLLTVDKSRWQQGNVFSCSVMHEALHNHYTQKSLSLSP

SEQ ID NO: 246 - protein, 447 aa, Homo sapiens
QVQLQESGPGLVRPSQTLSLTCTVSGYSITSDHAWSWVRQPPGRGLEWIGYISYSGITTYNPSLKSRVTMLRDTSKNQFSLRLSSVTAADTAVYYCARSLARTTAMDYWGQGSLVTVSSASTKGPSVFPLAPSSKSTSGGTAALGCLVKDYFPEPVTVSWNSGALTSGVHTFPAVLQSSGLYSLSSVVTVPSSSLGTQTYICNVNHKPSNTKVDKRVEPKSCDKTHTCPPCPAPELLGGPSVFLFPPKPKDTLMISRTPEVTCVVVDVSHEDPEVKFNWYVDGVEVHNAKTKPREEQYNSTYRVVSVLTVLHQDWLNGKEYKCKVSNKALPAPIEKTISKAKGQPRRPRVYTLPPSREEMTDNQVSLVCLVKGFYPSDIAVEWESNGQPENNYKTTPPVLTSDGSFFLASLLTVDKSRWQQGNVFSCSVMHEALHNHYTQKSLSLSP

SEQ ID NO: 247 - protein, 447 aa, Homo sapiens
QVQLQESGPGLVRPSQTLSLTCTVSGYSITSDHAWSWVRQPPGRGLEWIGYISYSGITTYNPSLKSRVTMLRDTSKNQFSLRLSSVTAADTAVYYCARSLARTTAMDYWGQGSLVTVSSASTKGPSVFPLAPSSKSTSGGTAALGCLVKDYFPEPVTVSWNSGALTSGVHTFPAVLQSSGLYSLSSVVTVPSSSLGTQTYICNVNHKPSNTKVDKRVEPKSCDKTHTCPPCPAPELLGGPSVFLFPPKPKDTLMISRTPEVTCVVVDVSHEDPEVKFNWYVDGVEVHNAKTKPREEQYNSTYRVVSVLTVLHQDWLNGKEYKCKVSNKALPAPIEKTISKAKGQPRRPRVYTLPPSREEMTDNQVSLVCLVKGFYPSDIAVEWESNGQPENNYKTTPPVLSSDGSFFLASLLTVDKSRWQQGNVFSCSVMHEALHNHYTQKSLSLSP

SEQ ID NO: 248 - protein, 447 aa, Homo sapiens
QVQLQESGPGLVRPSQTLSLTCTVSGYSITSDHAWSWVRQPPGRGLEWIGYISYSGITTYNPSLKSRVTMLRDTSKNQFSLRLSSVTAADTAVYYCARSLARTTAMDYWGQGSLVTVSSASTKGPSVFPLAPSSKSTSGGTAALGCLVKDYFPEPVTVSWNSGALTSGVHTFPAVLQSSGLYSLSSVVTVPSSSLGTQTYICNVNHKPSNTKVDKRVEPKSCDKTHTCPPCPAPELLGGPSVFLFPPKPKDTLMISRTPEVTCVVVDVSHEDPEVKFNWYVDGVEVHNAKTKPREEQYNSTYRVVSVLTVLHQDWLNGKEYKCKVSNKALPAPIEKTISKAKGQPRRPRVYTLPPSREEMTDNQVSLVCLVKGFYPSDIAVEWESNGQPENNYKTTPPVLQSDGSFFLASILTVDKSRWQQGNVFSCSVMHEALHNHYTQKSLSLSP

SEQ ID NO: 249 - protein, 447 aa, Homo sapiens
QVQLQESGPGLVRPSQTLSLTCTVSGYSITSDHAWSWVRQPPGRGLEWIGYISYSGITTYNPSLKSRVTMLRDTSKNQFSLRLSSVTAADTAVYYCARSLARTTAMDYWGQGSLVTVSSASTKGPSVFPLAPSSKSTSGGTAALGCLVKDYFPEPVTVSWNSGALTSGVHTFPAVLQSSGLYSLSSVVTVPSSSLGTQTYICNVNHKPSNTKVDKRVEPKSCDKTHTCPPCPAPELLGGPSVFLFPPKPKDTLMISRTPEVTCVVVDVSHEDPEVKFNWYVDGVEVHNAKTKPREEQYNSTYRVVSVLTVLHQDWLNGKEYKCKVSNKALPAPIEKTISKAKGQPRRPRVYTLPPSREEMTDNQVSLVCLVKGFYPSDIAVEWESNGQPENNYKTTPPVLNSDGSFFLASILTVDKSRWQQGNVFSCSVMHEALHNHYTQKSLSLSP

SEQ ID NO: 250 - protein, 447 aa, Homo sapiens
QVQLQESGPGLVRPSQTLSLTCTVSGYSITSDHAWSWVRQPPGRGLEWIGYISYSGITTYNPSLKSRVTMLRDTSKNQFSLRLSSVTAADTAVYYCARSLARTTAMDYWGQGSLVTVSSASTKGPSVFPLAPSSKSTSGGTAALGCLVKDYFPEPVTVSWNSGALTSGVHTFPAVLQSSGLYSLSSVVTVPSSSLGTQTYICNVNHKPSNTKVDKRVEPKSCDKTHTCPPCPAPELLGGPSVFLFPPKPKDTLMISRTPEVTCVVVDVSHEDPEVKFNWYVDGVEVHNAKTKPREEQYNSTYRVVSVLTVLHQDWLNGKEYKCKVSNKALPAPIEKTISKAKGQPRRPRVYTLPPSREEMTDNQVSLVCLVKGFYPSDIAVEWESNGQPENNYKTTPPVLHSDGSFFLASILTVDKSRWQQGNVFSCSVMHEALHNHYTQKSLSLSP

SEQ ID NO: 251 - protein, 447 aa, Homo sapiens
QVQLQESGPGLVRPSQTLSLTCTVSGYSITSDHAWSWVRQPPGRGLEWIGYISYSGITTYNPSLKSRVTMLRDTSKNQFSLRLSSVTAADTAVYYCARSLARTTAMDYWGQGSLVTVSSASTKGPSVFPLAPSSKSTSGGTAALGCLVKDYFPEPVTVSWNSGALTSGVHTFPAVLQSSGLYSLSSVVTVPSSSLGTQTYICNVNHKPSNTKVDKRVEPKSCDKTHTCPPCPAPELLGGPSVFLFPPKPKDTLMISRTPEVTCVVVDVSHEDPEVKFNWYVDGVEVHNAKTKPREEQYNSTYRVVSVLTVLHQDWLNGKEYKCKVSNKALPAPIEKTISKAKGQPRRPRVYTLPPSREEMTDNQVSLVCLVKGFYPSDIAVEWESNGQPENNYKTTPPVLVSDGSFFLASILTVDKSRWQQGNVFSCSVMHEALHNHYTQKSLSLSP

SEQ ID NO: 252 - protein, 447 aa, Homo sapiens
QVQLQESGPGLVRPSQTLSLTCTVSGYSITSDHAWSWVRQPPGRGLEWIGYISYSGITTYNPSLKSRVTMLRDTSKNQFSLRLSSVTAADTAVYYCARSLARTTAMDYWGQGSLVTVSSASTKGPSVFPLAPSSKSTSGGTAALGCLVKDYFPEPVTVSWNSGALTSGVHTFPAVLQSSGLYSLSSVVTVPSSSLGTQTYICNVNHKPSNTKVDKRVEPKSCDKTHTCPPCPAPELLGGPSVFLFPPKPKDTLMISRTPEVTCVVVDVSHEDPEVKFNWYVDGVEVHNAKTKPREEQYNSTYRVVSVLTVLHQDWLNGKEYKCKVSNKALPAPIEKTISKAKGQPRRPRVYTLPPSREEMTDNQVSLVCLVKGFYPSDIAVEWESNGQPENNYKTTPPVLLSDGSFFLASILTVDKSRWQQGNVFSCSVMHEALHNHYTQKSLSLSP

SEQ ID NO: 253 - protein, 447 aa, Homo sapiens
QVQLQESGPGLVRPSQTLSLTCTVSGYSITSDHAWSWVRQPPGRGLEWIGYISYSGITTYNPSLKSRVTMLRDTSKNQFSLRLSSVTAADTAVYYCARSLARTTAMDYWGQGSLVTVSSASTKGPSVFPLAPSSKSTSGGTAALGCLVKDYFPEPVTVSWNSGALTSGVHTFPAVLQSSGLYSLSSVVTVPSSSLGTQTYICNVNHKPSNTKVDKRVEPKSCDKTHTCPPCPAPELLGGPSVFLFPPKPKDTLMISRTPEVTCVVVDVSHEDPEVKFNWYVDGVEVHNAKTKPREEQYNSTYRVVSVLTVLHQDWLNGKEYKCKVSNKALPAPIEKTISKAKGQPRRPRVYTLPPSREEMTDNQVSLVCLVKGFYPSDIAVEWESNGQPENNYKTTPPVLFSDGSFFLASILTVDKSRWQQGNVFSCSVMHEALHNHYTQKSLSLSP

SEQ ID NO: 254 - protein, 447 aa, Homo sapiens
QVQLQESGPGLVRPSQTLSLTCTVSGYSITSDHAWSWVRQPPGRGLEWIGYISYSGITTYNPSLKSRVTMLRDTSKNQFSLRLSSVTAADTAVYYCARSLARTTAMDYWGQGSLVTVSSASTKGPSVFPLAPSSKSTSGGTAALGCLVKDYFPEPVTVSWNSGALTSGVHTFPAVLQSSGLYSLSSVVTVPSSSLGTQTYICNVNHKPSNTKVDKRVEPKSCDKTHTCPPCPAPELLGGPSVFLFPPKPKDTLMISRTPEVTCVVVDVSHEDPEVKFNWYVDGVEVHNAKTKPREEQYNSTYRVVSVLTVLHQDWLNGKEYKCKVSNKALPAPIEKTISKAKGQPRRPRVYTLPPSREEMTDNQVSLVCLVKGFYPSDIAVEWESNGQPENNYKTTPPVLYSDGSFFLASILTVDKSRWQQGNVFSCSVMHEALHNHYTQKSLSLSP

SEQ ID NO: 255 - protein, 447 aa, Homo sapiens
QVQLQESGPGLVRPSQTLSLTCTVSGYSITSDHAWSWVRQPPGRGLEWIGYISYSGITTYNPSLKSRVTMLRDTSKNQFSLRLSSVTAADTAVYYCARSLARTTAMDYWGQGSLVTVSSASTKGPSVFPLAPSSKSTSGGTAALGCLVKDYFPEPVTVSWNSGALTSGVHTFPAVLQSSGLYSLSSVVTVPSSSLGTQTYICNVNHKPSNTKVDKRVEPKSCDKTHTCPPCPAPELLGGPSVFLFPPKPKDTLMISRTPEVTCVVVDVSHEDPEVKFNWYVDGVEVHNAKTKPREEQYNSTYRVVSVLTVLHQDWLNGKEYKCKVSNKALPAPIEKTISKAKGQPRRPRVYTLPPSREEMTDNQVSLVCLVKGFYPSDIAVEWESNGQPENNYKTTPPVLTSDGSFFLASILTVDKSRWQQGNVFSCSVMHEALHNHYTQKSLSLSP

SEQ ID NO: 256 - protein, 447 aa, Homo sapiens
QVQLQESGPGLVRPSQTLSLTCTVSGYSITSDHAWSWVRQPPGRGLEWIGYISYSGITTYNPSLKSRVTMLRDTSKNQFSLRLSSVTAADTAVYYCARSLARTTAMDYWGQGSLVTVSSASTKGPSVFPLAPSSKSTSGGTAALGCLVKDYFPEPVTVSWNSGALTSGVHTFPAVLQSSGLYSLSSVVTVPSSSLGTQTYICNVNHKPSNTKVDKRVEPKSCDKTHTCPPCPAPELLGGPSVFLFPPKPKDTLMISRTPEVTCVVVDVSHEDPEVKFNWYVDGVEVHNAKTKPREEQYNSTYRVVSVLTVLHQDWLNGKEYKCKVSNKALPAPIEKTISKAKGQPRRPRVYTLPPSREEMTDNQVSLVCLVKGFYPSDIAVEWESNGQPENNYKTTPPVLSSDGSFFLASILTVDKSRWQQGNVFSCSVMHEALHNHYTQKSLSLSP

SEQ ID NO: 257 - protein, 447 aa, Homo sapiens
QVQLQESGPGLVRPSQTLSLTCTVSGYSITSDHAWSWVRQPPGRGLEWIGYISYSGITTYNPSLKSRVTMLRDTSKNQFSLRLSSVTAADTAVYYCARSLARTTAMDYWGQGSLVTVSSASTKGPSVFPLAPSSKSTSGGTAALGCLVKDYFPEPVTVSWNSGALTSGVHTFPAVLQSSGLYSLSSVVTVPSSSLGTQTYICNVNHKPSNTKVDKRVEPKSCDKTHTCPPCPAPELLGGPSVFLFPPKPKDTLMISRTPEVTCVVVDVSHEDPEVKFNWYVDGVEVHNAKTKPREEQYNSTYRVVSVLTVLHQDWLNGKEYKCKVSNKALPAPIEKTISKAKGQPRRPRVYTLPPSREEMTDNQVSLVCLVKGFYPSDIAVEWESNGQPENNYKTTPPVLQSDGSFFLASFLTVDKSRWQQGNVFSCSVMHEALHNHYTQKSLSLSP

SEQ ID NO: 258 - protein, 447 aa, Homo sapiens
QVQLQESGPGLVRPSQTLSLTCTVSGYSITSDHAWSWVRQPPGRGLEWIGYISYSGITTYNPSLKSRVTMLRDTSKNQFSLRLSSVTAADTAVYYCARSLARTTAMDYWGQGSLVTVSSASTKGPSVFPLAPSSKSTSGGTAALGCLVKDYFPEPVTVSWNSGALTSGVHTFPAVLQSSGLYSLSSVVTVPSSSLGTQTYICNVNHKPSNTKVDKRVEPKSCDKTHTCPPCPAPELLGGPSVFLFPPKPKDTLMISRTPEVTCVVVDVSHEDPEVKFNWYVDGVEVHNAKTKPREEQYNSTYRVVSVLTVLHQDWLNGKEYKCKVSNKALPAPIEKTISKAKGQPRRPRVYTLPPSREEMTDNQVSLVCLVKGFYPSDIAVEWESNGQPENNYKTTPPVLNSDGSFFLASFLTVDKSRWQQGNVFSCSVMHEALHNHYTQKSLSLSP

SEQ ID NO: 259 - protein, 447 aa, Homo sapiens
QVQLQESGPGLVRPSQTLSLTCTVSGYSITSDHAWSWVRQPPGRGLEWIGYISYSGITTYNPSLKSRVTMLRDTSKNQFSLRLSSVTAADTAVYYCARSLARTTAMDYWGQGSLVTVSSASTKGPSVFPLAPSSKSTSGGTAALGCLVKDYFPEPVTVSWNSGALTSGVHTFPAVLQSSGLYSLSSVVTVPSSSLGTQTYICNVNHKPSNTKVDKRVEPKSCDKTHTCPPCPAPELLGGPSVFLFPPKPKDTLMISRTPEVTCVVVDVSHEDPEVKFNWYVDGVEVHNAKTKPREEQYNSTYRVVSVLTVLHQDWLNGKEYKCKVSNKALPAPIEKTISKAKGQPRRPRVYTLPPSREEMTDNQVSLVCLVKGFYPSDIAVEWESNGQPENNYKTTPPVLHSDGSFFLASFLTVDKSRWQQGNVFSCSVMHEALHNHYTQKSLSLSP

SEQ ID NO: 260 - protein, 447 aa, Homo sapiens
QVQLQESGPGLVRPSQTLSLTCTVSGYSITSDHAWSWVRQPPGRGLEWIGYISYSGITTYNPSLKSRVTMLRDTSKNQFSLRLSSVTAADTAVYYCARSLARTTAMDYWGQGSLVTVSSASTKGPSVFPLAPSSKSTSGGTAALGCLVKDYFPEPVTVSWNSGALTSGVHTFPAVLQSSGLYSLSSVVTVPSSSLGTQTYICNVNHKPSNTKVDKRVEPKSCDKTHTCPPCPAPELLGGPSVFLFPPKPKDTLMISRTPEVTCVVVDVSHEDPEVKFNWYVDGVEVHNAKTKPREEQYNSTYRVVSVLTVLHQDWLNGKEYKCKVSNKALPAPIEKTISKAKGQPRRPRVYTLPPSREEMTDNQVSLVCLVKGFYPSDIAVEWESNGQPENNYKTTPPVLVSDGSFFLASFLTVDKSRWQQGNVFSCSVMHEALHNHYTQKSLSLSP

SEQ ID NO: 261 - protein, 447 aa, Homo sapiens
QVQLQESGPGLVRPSQTLSLTCTVSGYSITSDHAWSWVRQPPGRGLEWIGYISYSGITTYNPSLKSRVTMLRDTSKNQFSLRLSSVTAADTAVYYCARSLARTTAMDYWGQGSLVTVSSASTKGPSVFPLAPSSKSTSGGTAALGCLVKDYFPEPVTVSWNSGALTSGVHTFPAVLQSSGLYSLSSVVTVPSSSLGTQTYICNVNHKPSNTKVDKRVEPKSCDKTHTCPPCPAPELLGGPSVFLFPPKPKDTLMISRTPEVTCVVVDVSHEDPEVKFNWYVDGVEVHNAKTKPREEQYNSTYRVVSVLTVLHQDWLNGKEYKCKVSNKALPAPIEKTISKAKGQPRRPRVYTLPPSREEMTDNQVSLVCLVKGFYPSDIAVEWESNGQPENNYKTTPPVLLSDGSFFLASFLTVDKSRWQQGNVFSCSVMHEALHNHYTQKSLSLSP

SEQ ID NO: 262 - protein, 447 aa, Homo sapiens
QVQLQESGPGLVRPSQTLSLTCTVSGYSITSDHAWSWVRQPPGRGLEWIGYISYSGITTYNPSLKSRVTMLRDTSKNQFSLRLSSVTAADTAVYYCARSLARTTAMDYWGQGSLVTVSSASTKGPSVFPLAPSSKSTSGGTAALGCLVKDYFPEPVTVSWNSGALTSGVHTFPAVLQSSGLYSLSSVVTVPSSSLGTQTYICNVNHKPSNTKVDKRVEPKSCDKTHTCPPCPAPELLGGPSVFLFPPKPKDTLMISRTPEVTCVVVDVSHEDPEVKFNWYVDGVEVHNAKTKPREEQYNSTYRVVSVLTVLHQDWLNGKEYKCKVSNKALPAPIEKTISKAKGQPRRPRVYTLPPSREEMTDNQVSLVCLVKGFYPSDIAVEWESNGQPENNYKTTPPVLISDGSFFLASFLTVDKSRWQQGNVFSCSVMHEALHNHYTQKSLSLSP

SEQ ID NO: 263 - protein, 447 aa, Homo sapiens
QVQLQESGPGLVRPSQTLSLTCTVSGYSITSDHAWSWVRQPPGRGLEWIGYISYSGITTYNPSLKSRVTMLRDTSKNQFSLRLSSVTAADTAVYYCARSLARTTAMDYWGQGSLVTVSSASTKGPSVFPLAPSSKSTSGGTAALGCLVKDYFPEPVTVSWNSGALTSGVHTFPAVLQSSGLYSLSSVVTVPSSSLGTQTYICNVNHKPSNTKVDKRVEPKSCDKTHTCPPCPAPELLGGPSVFLFPPKPKDTLMISRTPEVTCVVVDVSHEDPEVKFNWYVDGVEVHNAKTKPREEQYNSTYRVVSVLTVLHQDWLNGKEYKCKVSNKALPAPIEKTISKAKGQPRRPRVYTLPPSREEMTDNQVSLVCLVKGFYPSDIAVEWESNGQPENNYKTTPPVLFSDGSFFLASFLTVDKSRWQQGNVFSCSVMHEALHNHYTQKSLSLSP

SEQ ID NO: 264 - protein, 447 aa, Homo sapiens
QVQLQESGPGLVRPSQTLSLTCTVSGYSITSDHAWSWVRQPPGRGLEWIGYISYSGITTYNPSLKSRVTMLRDTSKNQFSLRLSSVTAADTAVYYCARSLARTTAMDYWGQGSLVTVSSASTKGPSVFPLAPSSKSTSGGTAALGCLVKDYFPEPVTVSWNSGALTSGVHTFPAVLQSSGLYSLSSVVTVPSSSLGTQTYICNVNHKPSNTKVDKRVEPKSCDKTHTCPPCPAPELLGGPSVFLFPPKPKDTLMISRTPEVTCVVVDVSHEDPEVKFNWYVDGVEVHNAKTKPREEQYNSTYRVVSVLTVLHQDWLNGKEYKCKVSNKALPAPIEKTISKAKGQPRRPRVYTLPPSREEMTDNQVSLVCLVKGFYPSDIAVEWESNGQPENNYKTTPPVLYSDGSFFLASFLTVDKSRWQQGNVFSCSVMHEALHNHYTQKSLSLSP

SEQ ID NO: 265 - protein, 447 aa, Homo sapiens
QVQLQESGPGLVRPSQTLSLTCTVSGYSITSDHAWSWVRQPPGRGLEWIGYISYSGITTYNPSLKSRVTMLRDTSKNQFSLRLSSVTAADTAVYYCARSLARTTAMDYWGQGSLVTVSSASTKGPSVFPLAPSSKSTSGGTAALGCLVKDYFPEPVTVSWNSGALTSGVHTFPAVLQSSGLYSLSSVVTVPSSSLGTQTYICNVNHKPSNTKVDKRVEPKSCDKTHTCPPCPAPELLGGPSVFLFPPKPKDTLMISRTPEVTCVVVDVSHEDPEVKFNWYVDGVEVHNAKTKPREEQYNSTYRVVSVLTVLHQDWLNGKEYKCKVSNKALPAPIEKTISKAKGQPRRPRVYTLPPSREEMTDNQVSLVCLVKGFYPSDIAVEWESNGQPENNYKTTPPVLTSDGSFFLASFLTVDKSRWQQGNVFSCSVMHEALHNHYTQKSLSLSP

SEQ ID NO: 266 - protein, 447 aa, Homo sapiens
QVQLQESGPGLVRPSQTLSLTCTVSGYSITSDHAWSWVRQPPGRGLEWIGYISYSGITTYNPSLKSRVTMLRDTSKNQFSLRLSSVTAADTAVYYCARSLARTTAMDYWGQGSLVTVSSASTKGPSVFPLAPSSKSTSGGTAALGCLVKDYFPEPVTVSWNSGALTSGVHTFPAVLQSSGLYSLSSVVTVPSSSLGTQTYICNVNHKPSNTKVDKRVEPKSCDKTHTCPPCPAPELLGGPSVFLFPPKPKDTLMISRTPEVTCVVVDVSHEDPEVKFNWYVDGVEVHNAKTKPREEQYNSTYRVVSVLTVLHQDWLNGKEYKCKVSNKALPAPIEKTISKAKGQPRRPRVYTLPPSREEMTDNQVSLVCLVKGFYPSDIAVEWESNGQPENNYKTTPPVLQSDGSFFLASYLTVDKSRWQQGNVFSCSVMHEALHNHYTQKSLSLSP

SEQ ID NO: 267 - protein, 447 aa, Homo sapiens
QVQLQESGPGLVRPSQTLSLTCTVSGYSITSDHAWSWVRQPPGRGLEWIGYISYSGITTYNPSLKSRVTMLRDTSKNQFSLRLSSVTAADTAVYYCARSLARTTAMDYWGQGSLVTVSSASTKGPSVFPLAPSSKSTSGGTAALGCLVKDYFPEPVTVSWNSGALTSGVHTFPAVLQSSGLYSLSSVVTVPSSSLGTQTYICNVNHKPSNTKVDKRVEPKSCDKTHTCPPCPAPELLGGPSVFLFPPKPKDTLMISRTPEVTCVVVDVSHEDPEVKFNWYVDGVEVHNAKTKPREEQYNSTYRVVSVLTVLHQDWLNGKEYKCKVSNKALPAPIEKTISKAKGQPRRPRVYTLPPSREEMTDNQVSLVCLVKGFYPSDIAVEWESNGQPENNYKTTPPVLHSDGSFFLASYLTVDKSRWQQGNVFSCSVMHEALHNHYTQKSLSLSP

SEQ ID NO: 268 - protein, 447 aa, Homo sapiens
QVQLQESGPGLVRPSQTLSLTCTVSGYSITSDHAWSWVRQPPGRGLEWIGYISYSGITTYNPSLKSRVTMLRDTSKNQFSLRLSSVTAADTAVYYCARSLARTTAMDYWGQGSLVTVSSASTKGPSVFPLAPSSKSTSGGTAALGCLVKDYFPEPVTVSWNSGALTSGVHTFPAVLQSSGLYSLSSVVTVPSSSLGTQTYICNVNHKPSNTKVDKRVEPKSCDKTHTCPPCPAPELLGGPSVFLFPPKPKDTLMISRTPEVTCVVVDVSHEDPEVKFNWYVDGVEVHNAKTKPREEQYNSTYRVVSVLTVLHQDWLNGKEYKCKVSNKALPAPIEKTISKAKGQPRRPRVYTLPPSREEMTDNQVSLVCLVKGFYPSDIAVEWESNGQPENNYKTTPPVLVSDGSFFLASYLTVDKSRWQQGNVFSCSVMHEALHNHYTQKSLSLSP

SEQ ID NO: 269 - protein, 447 aa, Homo sapiens
QVQLQESGPGLVRPSQTLSLTCTVSGYSITSDHAWSWVRQPPGRGLEWIGYISYSGITTYNPSLKSRVTMLRDTSKNQFSLRLSSVTAADTAVYYCARSLARTTAMDYWGQGSLVTVSSASTKGPSVFPLAPSSKSTSGGTAALGCLVKDYFPEPVTVSWNSGALTSGVHTFPAVLQSSGLYSLSSVVTVPSSSLGTQTYICNVNHKPSNTKVDKRVEPKSCDKTHTCPPCPAPELLGGPSVFLFPPKPKDTLMISRTPEVTCVVVDVSHEDPEVKFNWYVDGVEVHNAKTKPREEQYNSTYRVVSVLTVLHQDWLNGKEYKCKVSNKALPAPIEKTISKAKGQPRRPRVYTLPPSREEMTDNQVSLVCLVKGFYPSDIAVEWESNGQPENNYKTTPPVLLSDGSFFLASYLTVDKSRWQQGNVFSCSVMHEALHNHYTQKSLSLSP

SEQ ID NO: 270 - protein, 447 aa, Homo sapiens
QVQLQESGPGLVRPSQTLSLTCTVSGYSITSDHAWSWVRQPPGRGLEWIGYISYSGITTYNPSLKSRVTMLRDTSKNQFSLRLSSVTAADTAVYYCARSLARTTAMDYWGQGSLVTVSSASTKGPSVFPLAPSSKSTSGGTAALGCLVKDYFPEPVTVSWNSGALTSGVHTFPAVLQSSGLYSLSSVVTVPSSSLGTQTYICNVNHKPSNTKVDKRVEPKSCDKTHTCPPCPAPELLGGPSVFLFPPKPKDTLMISRTPEVTCVVVDVSHEDPEVKFNWYVDGVEVHNAKTKPREEQYNSTYRVVSVLTVLHQDWLNGKEYKCKVSNKALPAPIEKTISKAKGQPRRPRVYTLPPSREEMTDNQVSLVCLVKGFYPSDIAVEWESNGQPENNYKTTPPVLISDGSFFLASYLTVDKSRWQQGNVFSCSVMHEALHNHYTQKSLSLSP

SEQ ID NO: 271 - protein, 447 aa, Homo sapiens
QVQLQESGPGLVRPSQTLSLTCTVSGYSITSDHAWSWVRQPPGRGLEWIGYISYSGITTYNPSLKSRVTMLRDTSKNQFSLRLSSVTAADTAVYYCARSLARTTAMDYWGQGSLVTVSSASTKGPSVFPLAPSSKSTSGGTAALGCLVKDYFPEPVTVSWNSGALTSGVHTFPAVLQSSGLYSLSSVVTVPSSSLGTQTYICNVNHKPSNTKVDKRVEPKSCDKTHTCPPCPAPELLGGPSVFLFPPKPKDTLMISRTPEVTCVVVDVSHEDPEVKFNWYVDGVEVHNAKTKPREEQYNSTYRVVSVLTVLHQDWLNGKEYKCKVSNKALPAPIEKTISKAKGQPRRPRVYTLPPSREEMTDNQVSLVCLVKGFYPSDIAVEWESNGQPENNYKTTPPVLFSDGSFFLASYLTVDKSRWQQGNVFSCSVMHEALHNHYTQKSLSLSP

SEQ ID NO: 272 - protein, 447 aa, Homo sapiens
QVQLQESGPGLVRPSQTLSLTCTVSGYSITSDHAWSWVRQPPGRGLEWIGYISYSGITTYNPSLKSRVTMLRDTSKNQFSLRLSSVTAADTAVYYCARSLARTTAMDYWGQGSLVTVSSASTKGPSVFPLAPSSKSTSGGTAALGCLVKDYFPEPVTVSWNSGALTSGVHTFPAVLQSSGLYSLSSVVTVPSSSLGTQTYICNVNHKPSNTKVDKRVEPKSCDKTHTCPPCPAPELLGGPSVFLFPPKPKDTLMISRTPEVTCVVVDVSHEDPEVKFNWYVDGVEVHNAKTKPREEQYNSTYRVVSVLTVLHQDWLNGKEYKCKVSNKALPAPIEKTISKAKGQPRRPRVYTLPPSREEMTDNQVSLVCLVKGFYPSDIAVEWESNGQPENNYKTTPPVLYSDGSFFLASYLTVDKSRWQQGNVFSCSVMHEALHNHYTQKSLSLSP

SEQ ID NO: 273 - protein, 447 aa, Homo sapiens
QVQLQESGPGLVRPSQTLSLTCTVSGYSITSDHAWSWVRQPPGRGLEWIGYISYSGITTYNPSLKSRVTMLRDTSKNQFSLRLSSVTAADTAVYYCARSLARTTAMDYWGQGSLVTVSSASTKGPSVFPLAPSSKSTSGGTAALGCLVKDYFPEPVTVSWNSGALTSGVHTFPAVLQSSGLYSLSSVVTVPSSSLGTQTYICNVNHKPSNTKVDKRVEPKSCDKTHTCPPCPAPELLGGPSVFLFPPKPKDTLMISRTPEVTCVVVDVSHEDPEVKFNWYVDGVEVHNAKTKPREEQYNSTYRVVSVLTVLHQDWLNGKEYKCKVSNKALPAPIEKTISKAKGQPRRPRVYTLPPSREEMTDNQVSLVCLVKGFYPSDIAVEWESNGQPENNYKTTPPVLSSDGSFFLASYLTVDKSRWQQGNVFSCSVMHEALHNHYTQKSLSLSP

SEQ ID NO: 274 - protein, 447 aa, Homo sapiens
QVQLQESGPGLVRPSQTLSLTCTVSGYSITSDHAWSWVRQPPGRGLEWIGYISYSGITTYNPSLKSRVTMLRDTSKNQFSLRLSSVTAADTAVYYCARSLARTTAMDYWGQGSLVTVSSASTKGPSVFPLAPSSKSTSGGTAALGCLVKDYFPEPVTVSWNSGALTSGVHTFPAVLQSSGLYSLSSVVTVPSSSLGTQTYICNVNHKPSNTKVDKRVEPKSCDKTHTCPPCPAPELLGGPSVFLFPPKPKDTLMISRTPEVTCVVVDVSHEDPEVKFNWYVDGVEVHNAKTKPREEQYNSTYRVVSVLTVLHQDWLNGKEYKCKVSNKALPAPIEKTISKAKGQPRRPRVYTLPPSREEMTDNQVSLVCLVKGFYPSDIAVEWESNGQPENNYKTTPPVLNSDGSFFLASTLTVDKSRWQQGNVFSCSVMHEALHNHYTQKSLSLSP

SEQ ID NO: 275 - protein, 447 aa, Homo sapiens
QVQLQESGPGLVRPSQTLSLTCTVSGYSITSDHAWSWVRQPPGRGLEWIGYISYSGITTYNPSLKSRVTMLRDTSKNQFSLRLSSVTAADTAVYYCARSLARTTAMDYWGQGSLVTVSSASTKGPSVFPLAPSSKSTSGGTAALGCLVKDYFPEPVTVSWNSGALTSGVHTFPAVLQSSGLYSLSSVVTVPSSSLGTQTYICNVNHKPSNTKVDKRVEPKSCDKTHTCPPCPAPELLGGPSVFLFPPKPKDTLMISRTPEVTCVVVDVSHEDPEVKFNWYVDGVEVHNAKTKPREEQYNSTYRVVSVLTVLHQDWLNGKEYKCKVSNKALPAPIEKTISKAKGQPRRPRVYTLPPSREEMTDNQVSLVCLVKGFYPSDIAVEWESNGQPENNYKTTPPVLHSDGSFFLASTLTVDKSRWQQGNVFSCSVMHEALHNHYTQKSLSLSP

SEQ ID NO: 276 - protein, 447 aa, Homo sapiens
QVQLQESGPGLVRPSQTLSLTCTVSGYSITSDHAWSWVRQPPGRGLEWIGYISYSGITTYNPSLKSRVTMLRDTSKNQFSLRLSSVTAADTAVYYCARSLARTTAMDYWGQGSLVTVSSASTKGPSVFPLAPSSKSTSGGTAALGCLVKDYFPEPVTVSWNSGALTSGVHTFPAVLQSSGLYSLSSVVTVPSSSLGTQTYICNVNHKPSNTKVDKRVEPKSCDKTHTCPPCPAPELLGGPSVFLFPPKPKDTLMISRTPEVTCVVVDVSHEDPEVKFNWYVDGVEVHNAKTKPREEQYNSTYRVVSVLTVLHQDWLNGKEYKCKVSNKALPAPIEKTISKAKGQPRRPRVYTLPPSREEMTDNQVSLVCLVKGFYPSDIAVEWESNGQPENNYKTTPPVLVSDGSFFLASTLTVDKSRWQQGNVFSCSVMHEALHNHYTQKSLSLSP

SEQ ID NO: 277 - protein, 447 aa, Homo sapiens
QVQLQESGPGLVRPSQTLSLTCTVSGYSITSDHAWSWVRQPPGRGLEWIGYISYSGITTYNPSLKSRVTMLRDTSKNQFSLRLSSVTAADTAVYYCARSLARTTAMDYWGQGSLVTVSSASTKGPSVFPLAPSSKSTSGGTAALGCLVKDYFPEPVTVSWNSGALTSGVHTFPAVLQSSGLYSLSSVVTVPSSSLGTQTYICNVNHKPSNTKVDKRVEPKSCDKTHTCPPCPAPELLGGPSVFLFPPKPKDTLMISRTPEVTCVVVDVSHEDPEVKFNWYVDGVEVHNAKTKPREEQYNSTYRVVSVLTVLHQDWLNGKEYKCKVSNKALPAPIEKTISKAKGQPRRPRVYTLPPSREEMTDNQVSLVCLVKGFYPSDIAVEWESNGQPENNYKTTPPVLLSDGSFFLASTLTVDKSRWQQGNVFSCSVMHEALHNHYTQKSLSLSP

SEQ ID NO: 278 - protein, 447 aa, Homo sapiens
QVQLQESGPGLVRPSQTLSLTCTVSGYSITSDHAWSWVRQPPGRGLEWIGYISYSGITTYNPSLKSRVTMLRDTSKNQFSLRLSSVTAADTAVYYCARSLARTTAMDYWGQGSLVTVSSASTKGPSVFPLAPSSKSTSGGTAALGCLVKDYFPEPVTVSWNSGALTSGVHTFPAVLQSSGLYSLSSVVTVPSSSLGTQTYICNVNHKPSNTKVDKRVEPKSCDKTHTCPPCPAPELLGGPSVFLFPPKPKDTLMISRTPEVTCVVVDVSHEDPEVKFNWYVDGVEVHNAKTKPREEQYNSTYRVVSVLTVLHQDWLNGKEYKCKVSNKALPAPIEKTISKAKGQPRRPRVYTLPPSREEMTDNQVSLVCLVKGFYPSDIAVEWESNGQPENNYKTTPPVLISDGSFFLASTLTVDKSRWQQGNVFSCSVMHEALHNHYTQKSLSLSP

SEQ ID NO: 279 - protein, 447 aa, Homo sapiens
QVQLQESGPGLVRPSQTLSLTCTVSGYSITSDHAWSWVRQPPGRGLEWIGYISYSGITTYNPSLKSRVTMLRDTSKNQFSLRLSSVTAADTAVYYCARSLARTTAMDYWGQGSLVTVSSASTKGPSVFPLAPSSKSTSGGTAALGCLVKDYFPEPVTVSWNSGALTSGVHTFPAVLQSSGLYSLSSVVTVPSSSLGTQTYICNVNHKPSNTKVDKRVEPKSCDKTHTCPPCPAPELLGGPSVFLFPPKPKDTLMISRTPEVTCVVVDVSHEDPEVKFNWYVDGVEVHNAKTKPREEQYNSTYRVVSVLTVLHQDWLNGKEYKCKVSNKALPAPIEKTISKAKGQPRRPRVYTLPPSREEMTDNQVSLVCLVKGFYPSDIAVEWESNGQPENNYKTTPPVLFSDGSFFLASTLTVDKSRWQQGNVFSCSVMHEALHNHYTQKSLSLSP

SEQ ID NO: 280 - protein, 447 aa, Homo sapiens
QVQLQESGPGLVRPSQTLSLTCTVSGYSITSDHAWSWVRQPPGRGLEWIGYISYSGITTYNPSLKSRVTMLRDTSKNQFSLRLSSVTAADTAVYYCARSLARTTAMDYWGQGSLVTVSSASTKGPSVFPLAPSSKSTSGGTAALGCLVKDYFPEPVTVSWNSGALTSGVHTFPAVLQSSGLYSLSSVVTVPSSSLGTQTYICNVNHKPSNTKVDKRVEPKSCDKTHTCPPCPAPELLGGPSVFLFPPKPKDTLMISRTPEVTCVVVDVSHEDPEVKFNWYVDGVEVHNAKTKPREEQYNSTYRVVSVLTVLHQDWLNGKEYKCKVSNKALPAPIEKTISKAKGQPRRPRVYTLPPSREEMTDNQVSLVCLVKGFYPSDIAVEWESNGQPENNYKTTPPVLYSDGSFFLASTLTVDKSRWQQGNVFSCSVMHEALHNHYTQKSLSLSP

SEQ ID NO: 281 - protein, 447 aa, Homo sapiens
QVQLQESGPGLVRPSQTLSLTCTVSGYSITSDHAWSWVRQPPGRGLEWIGYISYSGITTYNPSLKSRVTMLRDTSKNQFSLRLSSVTAADTAVYYCARSLARTTAMDYWGQGSLVTVSSASTKGPSVFPLAPSSKSTSGGTAALGCLVKDYFPEPVTVSWNSGALTSGVHTFPAVLQSSGLYSLSSVVTVPSSSLGTQTYICNVNHKPSNTKVDKRVEPKSCDKTHTCPPCPAPELLGGPSVFLFPPKPKDTLMISRTPEVTCVVVDVSHEDPEVKFNWYVDGVEVHNAKTKPREEQYNSTYRVVSVLTVLHQDWLNGKEYKCKVSNKALPAPIEKTISKAKGQPRRPRVYTLPPSREEMTDNQVSLVCLVKGFYPSDIAVEWESNGQPENNYKTTPPVLTSDGSFFLASTLTVDKSRWQQGNVFSCSVMHEALHNHYTQKSLSLSP

SEQ ID NO: 282 - protein, 447 aa, Homo sapiens
QVQLQESGPGLVRPSQTLSLTCTVSGYSITSDHAWSWVRQPPGRGLEWIGYISYSGITTYNPSLKSRVTMLRDTSKNQFSLRLSSVTAADTAVYYCARSLARTTAMDYWGQGSLVTVSSASTKGPSVFPLAPSSKSTSGGTAALGCLVKDYFPEPVTVSWNSGALTSGVHTFPAVLQSSGLYSLSSVVTVPSSSLGTQTYICNVNHKPSNTKVDKRVEPKSCDKTHTCPPCPAPELLGGPSVFLFPPKPKDTLMISRTPEVTCVVVDVSHEDPEVKFNWYVDGVEVHNAKTKPREEQYNSTYRVVSVLTVLHQDWLNGKEYKCKVSNKALPAPIEKTISKAKGQPRRPRVYTLPPSREEMTDNQVSLVCLVKGFYPSDIAVEWESNGQPENNYKTTPPVLSSDGSFFLASTLTVDKSRWQQGNVFSCSVMHEALHNHYTQKSLSLSP

SEQ ID NO: 283 - protein, 447 aa, Homo sapiens
QVQLQESGPGLVRPSQTLSLTCTVSGYSITSDHAWSWVRQPPGRGLEWIGYISYSGITTYNPSLKSRVTMLRDTSKNQFSLRLSSVTAADTAVYYCARSLARTTAMDYWGQGSLVTVSSASTKGPSVFPLAPSSKSTSGGTAALGCLVKDYFPEPVTVSWNSGALTSGVHTFPAVLQSSGLYSLSSVVTVPSSSLGTQTYICNVNHKPSNTKVDKRVEPKSCDKTHTCPPCPAPELLGGPSVFLFPPKPKDTLMISRTPEVTCVVVDVSHEDPEVKFNWYVDGVEVHNAKTKPREEQYNSTYRVVSVLTVLHQDWLNGKEYKCKVSNKALPAPIEKTISKAKGQPRRPRVYTLPPSREEMTDNQVSLVCLVKGFYPSDIAVEWESNGQPENNYKTTPPVLQSDGSFFLASSLTVDKSRWQQGNVFSCSVMHEALHNHYTQKSLSLSP

SEQ ID NO: 284 - protein, 447 aa, Homo sapiens
QVQLQESGPGLVRPSQTLSLTCTVSGYSITSDHAWSWVRQPPGRGLEWIGYISYSGITTYNPSLKSRVTMLRDTSKNQFSLRLSSVTAADTAVYYCARSLARTTAMDYWGQGSLVTVSSASTKGPSVFPLAPSSKSTSGGTAALGCLVKDYFPEPVTVSWNSGALTSGVHTFPAVLQSSGLYSLSSVVTVPSSSLGTQTYICNVNHKPSNTKVDKRVEPKSCDKTHTCPPCPAPELLGGPSVFLFPPKPKDTLMISRTPEVTCVVVDVSHEDPEVKFNWYVDGVEVHNAKTKPREEQYNSTYRVVSVLTVLHQDWLNGKEYKCKVSNKALPAPIEKTISKAKGQPRRPRVYTLPPSREEMTDNQVSLVCLVKGFYPSDIAVEWESNGQPENNYKTTPPVLNSDGSFFLASSLTVDKSRWQQGNVFSCSVMHEALHNHYTQKSLSLSP

SEQ ID NO: 285 - protein, 447 aa, Homo sapiens
QVQLQESGPGLVRPSQTLSLTCTVSGYSITSDHAWSWVRQPPGRGLEWIGYISYSGITTYNPSLKSRVTMLRDTSKNQFSLRLSSVTAADTAVYYCARSLARTTAMDYWGQGSLVTVSSASTKGPSVFPLAPSSKSTSGGTAALGCLVKDYFPEPVTVSWNSGALTSGVHTFPAVLQSSGLYSLSSVVTVPSSSLGTQTYICNVNHKPSNTKVDKRVEPKSCDKTHTCPPCPAPELLGGPSVFLFPPKPKDTLMISRTPEVTCVVVDVSHEDPEVKFNWYVDGVEVHNAKTKPREEQYNSTYRVVSVLTVLHQDWLNGKEYKCKVSNKALPAPIEKTISKAKGQPRRPRVYTLPPSREEMTDNQVSLVCLVKGFYPSDIAVEWESNGQPENNYKTTPPVLHSDGSFFLASSLTVDKSRWQQGNVFSCSVMHEALHNHYTQKSLSLSP

SEQ ID NO: 286 - protein, 447 aa, Homo sapiens
QVQLQESGPGLVRPSQTLSLTCTVSGYSITSDHAWSWVRQPPGRGLEWIGYISYSGITTYNPSLKSRVTMLRDTSKNQFSLRLSSVTAADTAVYYCARSLARTTAMDYWGQGSLVTVSSASTKGPSVFPLAPSSKSTSGGTAALGCLVKDYFPEPVTVSWNSGALTSGVHTFPAVLQSSGLYSLSSVVTVPSSSLGTQTYICNVNHKPSNTKVDKRVEPKSCDKTHTCPPCPAPELLGGPSVFLFPPKPKDTLMISRTPEVTCVVVDVSHEDPEVKFNWYVDGVEVHNAKTKPREEQYNSTYRVVSVLTVLHQDWLNGKEYKCKVSNKALPAPIEKTISKAKGQPRRPRVYTLPPSREEMTDNQVSLVCLVKGFYPSDIAVEWESNGQPENNYKTTPPVLVSDGSFFLASSLTVDKSRWQQGNVFSCSVMHEALHNHYTQKSLSLSP

SEQ ID NO: 287 - protein, 447 aa, Homo sapiens
QVQLQESGPGLVRPSQTLSLTCTVSGYSITSDHAWSWVRQPPGRGLEWIGYISYSGITTYNPSLKSRVTMLRDTSKNQFSLRLSSVTAADTAVYYCARSLARTTAMDYWGQGSLVTVSSASTKGPSVFPLAPSSKSTSGGTAALGCLVKDYFPEPVTVSWNSGALTSGVHTFPAVLQSSGLYSLSSVVTVPSSSLGTQTYICNVNHKPSNTKVDKRVEPKSCDKTHTCPPCPAPELLGGPSVFLFPPKPKDTLMISRTPEVTCVVVDVSHEDPEVKFNWYVDGVEVHNAKTKPREEQYNSTYRVVSVLTVLHQDWLNGKEYKCKVSNKALPAPIEKTISKAKGQPRRPRVYTLPPSREEMTDNQVSLVCLVKGFYPSDIAVEWESNGQPENNYKTTPPVLLSDGSFFLASSLTVDKSRWQQGNVFSCSVMHEALHNHYTQKSLSLSP

SEQ ID NO: 288 - protein, 447 aa, Homo sapiens
QVQLQESGPGLVRPSQTLSLTCTVSGYSITSDHAWSWVRQPPGRGLEWIGYISYSGITTYNPSLKSRVTMLRDTSKNQFSLRLSSVTAADTAVYYCARSLARTTAMDYWGQGSLVTVSSASTKGPSVFPLAPSSKSTSGGTAALGCLVKDYFPEPVTVSWNSGALTSGVHTFPAVLQSSGLYSLSSVVTVPSSSLGTQTYICNVNHKPSNTKVDKRVEPKSCDKTHTCPPCPAPELLGGPSVFLFPPKPKDTLMISRTPEVTCVVVDVSHEDPEVKFNWYVDGVEVHNAKTKPREEQYNSTYRVVSVLTVLHQDWLNGKEYKCKVSNKALPAPIEKTISKAKGQPRRPRVYTLPPSREEMTDNQVSLVCLVKGFYPSDIAVEWESNGQPENNYKTTPPVLISDGSFFLASSLTVDKSRWQQGNVFSCSVMHEALHNHYTQKSLSLSP

SEQ ID NO: 289 - protein, 447 aa, Homo sapiens
QVQLQESGPGLVRPSQTLSLTCTVSGYSITSDHAWSWVRQPPGRGLEWIGYISYSGITTYNPSLKSRVTMLRDTSKNQFSLRLSSVTAADTAVYYCARSLARTTAMDYWGQGSLVTVSSASTKGPSVFPLAPSSKSTSGGTAALGCLVKDYFPEPVTVSWNSGALTSGVHTFPAVLQSSGLYSLSSVVTVPSSSLGTQTYICNVNHKPSNTKVDKRVEPKSCDKTHTCPPCPAPELLGGPSVFLFPPKPKDTLMISRTPEVTCVVVDVSHEDPEVKFNWYVDGVEVHNAKTKPREEQYNSTYRVVSVLTVLHQDWLNGKEYKCKVSNKALPAPIEKTISKAKGQPRRPRVYTLPPSREEMTDNQVSLVCLVKGFYPSDIAVEWESNGQPENNYKTTPPVLFSDGSFFLASSLTVDKSRWQQGNVFSCSVMHEALHNHYTQKSLSLSP

SEQ ID NO: 290 - protein, 447 aa, Homo sapiens
QVQLQESGPGLVRPSQTLSLTCTVSGYSITSDHAWSWVRQPPGRGLEWIGYISYSGITTYNPSLKSRVTMLRDTSKNQFSLRLSSVTAADTAVYYCARSLARTTAMDYWGQGSLVTVSSASTKGPSVFPLAPSSKSTSGGTAALGCLVKDYFPEPVTVSWNSGALTSGVHTFPAVLQSSGLYSLSSVVTVPSSSLGTQTYICNVNHKPSNTKVDKRVEPKSCDKTHTCPPCPAPELLGGPSVFLFPPKPKDTLMISRTPEVTCVVVDVSHEDPEVKFNWYVDGVEVHNAKTKPREEQYNSTYRVVSVLTVLHQDWLNGKEYKCKVSNKALPAPIEKTISKAKGQPRRPRVYTLPPSREEMTDNQVSLVCLVKGFYPSDIAVEWESNGQPENNYKTTPPVLYSDGSFFLASSLTVDKSRWQQGNVFSCSVMHEALHNHYTQKSLSLSP

SEQ ID NO: 291 - protein, 447 aa, Homo sapiens
QVQLQESGPGLVRPSQTLSLTCTVSGYSITSDHAWSWVRQPPGRGLEWIGYISYSGITTYNPSLKSRVTMLRDTSKNQFSLRLSSVTAADTAVYYCARSLARTTAMDYWGQGSLVTVSSASTKGPSVFPLAPSSKSTSGGTAALGCLVKDYFPEPVTVSWNSGALTSGVHTFPAVLQSSGLYSLSSVVTVPSSSLGTQTYICNVNHKPSNTKVDKRVEPKSCDKTHTCPPCPAPELLGGPSVFLFPPKPKDTLMISRTPEVTCVVVDVSHEDPEVKFNWYVDGVEVHNAKTKPREEQYNSTYRVVSVLTVLHQDWLNGKEYKCKVSNKALPAPIEKTISKAKGQPRRPRVYTLPPSREEMTDNQVSLVCLVKGFYPSDIAVEWESNGQPENNYKTTPPVLTSDGSFFLASSLTVDKSRWQQGNVFSCSVMHEALHNHYTQKSLSLSP

SEQ ID NO: 292 - protein, 447 aa, Homo sapiens
QVQLQESGPGLVRPSQTLSLTCTVSGYSITSDHAWSWVRQPPGRGLEWIGYISYSGITTYNPSLKSRVTMLRDTSKNQFSLRLSSVTAADTAVYYCARSLARTTAMDYWGQGSLVTVSSASTKGPSVFPLAPSSKSTSGGTAALGCLVKDYFPEPVTVSWNSGALTSGVHTFPAVLQSSGLYSLSSVVTVPSSSLGTQTYICNVNHKPSNTKVDKRVEPKSCDKTHTCPPCPAPELLGGPSVFLFPPKPKDTLMISRTPEVTCVVVDVSHEDPEVKFNWYVDGVEVHNAKTKPREEQYNSTYRVVSVLTVLHQDWLNGKEYKCKVSNKALPAPIEKTISKAKGQPRRPRVYTLPPSREEMTDNQVSLVCLVKGFYPSDIAVEWESNGQPENNYKTTPPVLSSDGSFFLASSLTVDKSRWQQGNVFSCSVMHEALHNHYTQKSLSLSP

SEQ ID NO: 293 - protein, 447 aa, Homo sapiens
QVQLQESGPGLVRPSQTLSLTCTVSGYSITSDHAWSWVRQPPGRGLEWIGYISYSGITTYNPSLKSRVTMLRDTSKNQFSLRLSSVTAADTAVYYCARSLARTTAMDYWGQGSLVTVSSASTKGPSVFPLAPSSKSTSGGTAALGCLVKDYFPEPVTVSWNSGALTSGVHTFPAVLQSSGLYSLSSVVTVPSSSLGTQTYICNVNHKPSNTKVDKRVEPKSCDKTHTCPPCPAPELLGGPSVFLFPPKPKDTLMISRTPEVTCVVVDVSHEDPEVKFNWYVDGVEVHNAKTKPREEQYNSTYRVVSVLTVLHQDWLNGKEYKCKVSNKALPAPIEKTISKAKGQPRRPRVYTLPPSREEMTDNQVSLVCLVKGFYPSDIAVEWESNGQPENNYKTTPPVLMSDGSFFLASQLTVDKSRWQQGNVFSCSVMHEALHNHYTQKSLSLSP

SEQ ID NO: 294 - protein, 447 aa, Homo sapiens
QVQLQESGPGLVRPSQTLSLTCTVSGYSITSDHAWSWVRQPPGRGLEWIGYISYSGITTYNPSLKSRVTMLRDTSKNQFSLRLSSVTAADTAVYYCARSLARTTAMDYWGQGSLVTVSSASTKGPSVFPLAPSSKSTSGGTAALGCLVKDYFPEPVTVSWNSGALTSGVHTFPAVLQSSGLYSLSSVVTVPSSSLGTQTYICNVNHKPSNTKVDKRVEPKSCDKTHTCPPCPAPELLGGPSVFLFPPKPKDTLMISRTPEVTCVVVDVSHEDPEVKFNWYVDGVEVHNAKTKPREEQYNSTYRVVSVLTVLHQDWLNGKEYKCKVSNKALPAPIEKTISKAKGQPRRPRVYTLPPSREEMTDNQVSLVCLVKGFYPSDIAVEWESNGQPENNYKTTPPVLMSDGSFFLASNLTVDKSRWQQGNVFSCSVMHEALHNHYTQKSLSLSP

SEQ ID NO: 295 - protein, 447 aa, Homo sapiens
QVQLQESGPGLVRPSQTLSLTCTVSGYSITSDHAWSWVRQPPGRGLEWIGYISYSGITTYNPSLKSRVTMLRDTSKNQFSLRLSSVTAADTAVYYCARSLARTTAMDYWGQGSLVTVSSASTKGPSVFPLAPSSKSTSGGTAALGCLVKDYFPEPVTVSWNSGALTSGVHTFPAVLQSSGLYSLSSVVTVPSSSLGTQTYICNVNHKPSNTKVDKRVEPKSCDKTHTCPPCPAPELLGGPSVFLFPPKPKDTLMISRTPEVTCVVVDVSHEDPEVKFNWYVDGVEVHNAKTKPREEQYNSTYRVVSVLTVLHQDWLNGKEYKCKVSNKALPAPIEKTISKAKGQPRRPRVYTLPPSREEMTDNQVSLVCLVKGFYPSDIAVEWESNGQPENNYKTTPPVLMSDGSFFLASHLTVDKSRWQQGNVFSCSVMHEALHNHYTQKSLSLSP

SEQ ID NO: 296 - protein, 447 aa, Homo sapiens
QVQLQESGPGLVRPSQTLSLTCTVSGYSITSDHAWSWVRQPPGRGLEWIGYISYSGITTYNPSLKSRVTMLRDTSKNQFSLRLSSVTAADTAVYYCARSLARTTAMDYWGQGSLVTVSSASTKGPSVFPLAPSSKSTSGGTAALGCLVKDYFPEPVTVSWNSGALTSGVHTFPAVLQSSGLYSLSSVVTVPSSSLGTQTYICNVNHKPSNTKVDKRVEPKSCDKTHTCPPCPAPELLGGPSVFLFPPKPKDTLMISRTPEVTCVVVDVSHEDPEVKFNWYVDGVEVHNAKTKPREEQYNSTYRVVSVLTVLHQDWLNGKEYKCKVSNKALPAPIEKTISKAKGQPRRPRVYTLPPSREEMTDNQVSLVCLVKGFYPSDIAVEWESNGQPENNYKTTPPVLMSDGSFFLASLLTVDKSRWQQGNVFSCSVMHEALHNHYTQKSLSLSP

SEQ ID NO: 297 - protein, 447 aa, Homo sapiens
QVQLQESGPGLVRPSQTLSLTCTVSGYSITSDHAWSWVRQPPGRGLEWIGYISYSGITTYNPSLKSRVTMLRDTSKNQFSLRLSSVTAADTAVYYCARSLARTTAMDYWGQGSLVTVSSASTKGPSVFPLAPSSKSTSGGTAALGCLVKDYFPEPVTVSWNSGALTSGVHTFPAVLQSSGLYSLSSVVTVPSSSLGTQTYICNVNHKPSNTKVDKRVEPKSCDKTHTCPPCPAPELLGGPSVFLFPPKPKDTLMISRTPEVTCVVVDVSHEDPEVKFNWYVDGVEVHNAKTKPREEQYNSTYRVVSVLTVLHQDWLNGKEYKCKVSNKALPAPIEKTISKAKGQPRRPRVYTLPPSREEMTDNQVSLVCLVKGFYPSDIAVEWESNGQPENNYKTTPPVLMSDGSFFLASILTVDKSRWQQGNVFSCSVMHEALHNHYTQKSLSLSP

SEQ ID NO: 298 - protein, 447 aa, Homo sapiens
QVQLQESGPGLVRPSQTLSLTCTVSGYSITSDHAWSWVRQPPGRGLEWIGYISYSGITTYNPSLKSRVTMLRDTSKNQFSLRLSSVTAADTAVYYCARSLARTTAMDYWGQGSLVTVSSASTKGPSVFPLAPSSKSTSGGTAALGCLVKDYFPEPVTVSWNSGALTSGVHTFPAVLQSSGLYSLSSVVTVPSSSLGTQTYICNVNHKPSNTKVDKRVEPKSCDKTHTCPPCPAPELLGGPSVFLFPPKPKDTLMISRTPEVTCVVVDVSHEDPEVKFNWYVDGVEVHNAKTKPREEQYNSTYRVVSVLTVLHQDWLNGKEYKCKVSNKALPAPIEKTISKAKGQPRRPRVYTLPPSREEMTDNQVSLVCLVKGFYPSDIAVEWESNGQPENNYKTTPPVLMSDGSFFLASFLTVDKSRWQQGNVFSCSVMHEALHNHYTQKSLSLSP

SEQ ID NO: 299 - protein, 447 aa, Homo sapiens
QVQLQESGPGLVRPSQTLSLTCTVSGYSITSDHAWSWVRQPPGRGLEWIGYISYSGITTYNPSLKSRVTMLRDTSKNQFSLRLSSVTAADTAVYYCARSLARTTAMDYWGQGSLVTVSSASTKGPSVFPLAPSSKSTSGGTAALGCLVKDYFPEPVTVSWNSGALTSGVHTFPAVLQSSGLYSLSSVVTVPSSSLGTQTYICNVNHKPSNTKVDKRVEPKSCDKTHTCPPCPAPELLGGPSVFLFPPKPKDTLMISRTPEVTCVVVDVSHEDPEVKFNWYVDGVEVHNAKTKPREEQYNSTYRVVSVLTVLHQDWLNGKEYKCKVSNKALPAPIEKTISKAKGQPRRPRVYTLPPSREEMTDNQVSLVCLVKGFYPSDIAVEWESNGQPENNYKTTPPVLMSDGSFFLASYLTVDKSRWQQGNVFSCSVMHEALHNHYTQKSLSLSP

SEQ ID NO: 300 - protein, 447 aa, Homo sapiens
QVQLQESGPGLVRPSQTLSLTCTVSGYSITSDHAWSWVRQPPGRGLEWIGYISYSGITTYNPSLKSRVTMLRDTSKNQFSLRLSSVTAADTAVYYCARSLARTTAMDYWGQGSLVTVSSASTKGPSVFPLAPSSKSTSGGTAALGCLVKDYFPEPVTVSWNSGALTSGVHTFPAVLQSSGLYSLSSVVTVPSSSLGTQTYICNVNHKPSNTKVDKRVEPKSCDKTHTCPPCPAPELLGGPSVFLFPPKPKDTLMISRTPEVTCVVVDVSHEDPEVKFNWYVDGVEVHNAKTKPREEQYNSTYRVVSVLTVLHQDWLNGKEYKCKVSNKALPAPIEKTISKAKGQPRRPRVYTLPPSREEMTDNQVSLVCLVKGFYPSDIAVEWESNGQPENNYKTTPPVLMSDGSFFLASTLTVDKSRWQQGNVFSCSVMHEALHNHYTQKSLSLSP

SEQ ID NO: 301 - protein, 447 aa, Homo sapiens
QVQLQESGPGLVRPSQTLSLTCTVSGYSITSDHAWSWVRQPPGRGLEWIGYISYSGITTYNPSLKSRVTMLRDTSKNQFSLRLSSVTAADTAVYYCARSLARTTAMDYWGQGSLVTVSSASTKGPSVFPLAPSSKSTSGGTAALGCLVKDYFPEPVTVSWNSGALTSGVHTFPAVLQSSGLYSLSSVVTVPSSSLGTQTYICNVNHKPSNTKVDKRVEPKSCDKTHTCPPCPAPELLGGPSVFLFPPKPKDTLMISRTPEVTCVVVDVSHEDPEVKFNWYVDGVEVHNAKTKPREEQYNSTYRVVSVLTVLHQDWLNGKEYKCKVSNKALPAPIEKTISKAKGQPRRPRVYTLPPSREEMTDNQVSLVCLVKGFYPSDIAVEWESNGQPENNYKTTPPVLMSDGSFFLASSLTVDKSRWQQGNVFSCSVMHEALHNHYTQKSLSLSP

SEQ ID NO: 302 - protein, 447 aa, Homo sapiens
QVQLQESGPGLVRPSQTLSLTCTVSGYSITSDHAWSWVRQPPGRGLEWIGYISYSGITTYNPSLKSRVTMLRDTSKNQFSLRLSSVTAADTAVYYCARSLARTTAMDYWGQGSLVTVSSASTKGPSVFPLAPSSKSTSGGTAALGCLVKDYFPEPVTVSWNSGALTSGVHTFPAVLQSSGLYSLSSVVTVPSSSLGTQTYICNVNHKPSNTKVDKRVEPKSCDKTHTCPPCPAPELLGGPSVFLFPPKPKDTLMISRTPEVTCVVVDVSHEDPEVKFNWYVDGVEVHNAKTKPREEQYNSTYRVVSVLTVLHQDWLNGKEYKCKVSNKALPAPIEKTISKAKGQPRRPRVYTLPPSREEMTDNQVSLVCLVKGFYPSDIAVEWESNGQPENNYKTTPPVLVSDGSFFLASQLTVDKSRWQQGNVFSCSVMHEALHNHYTQKSLSLSP

SEQ ID NO: 303 - protein, 447 aa, Homo sapiens
QVQLQESGPGLVRPSQTLSLTCTVSGYSITSDHAWSWVRQPPGRGLEWIGYISYSGITTYNPSLKSRVTMLRDTSKNQFSLRLSSVTAADTAVYYCARSLARTTAMDYWGQGSLVTVSSASTKGPSVFPLAPSSKSTSGGTAALGCLVKDYFPEPVTVSWNSGALTSGVHTFPAVLQSSGLYSLSSVVTVPSSSLGTQTYICNVNHKPSNTKVDKRVEPKSCDKTHTCPPCPAPELLGGPSVFLFPPKPKDTLMISRTPEVTCVVVDVSHEDPEVKFNWYVDGVEVHNAKTKPREEQYNSTYRVVSVLTVLHQDWLNGKEYKCKVSNKALPAPIEKTISKAKGQPRRPRVYTLPPSREEMTDNQVSLVCLVKGFYPSDIAVEWESNGQPENNYKTTPPVLLSDGSFFLASQLTVDKSRWQQGNVFSCSVMHEALHNHYTQKSLSLSP

SEQ ID NO: 304 - protein, 447 aa, Homo sapiens
QVQLQESGPGLVRPSQTLSLTCTVSGYSITSDHAWSWVRQPPGRGLEWIGYISYSGITTYNPSLKSRVTMLRDTSKNQFSLRLSSVTAADTAVYYCARSLARTTAMDYWGQGSLVTVSSASTKGPSVFPLAPSSKSTSGGTAALGCLVKDYFPEPVTVSWNSGALTSGVHTFPAVLQSSGLYSLSSVVTVPSSSLGTQTYICNVNHKPSNTKVDKRVEPKSCDKTHTCPPCPAPELLGGPSVFLFPPKPKDTLMISRTPEVTCVVVDVSHEDPEVKFNWYVDGVEVHNAKTKPREEQYNSTYRVVSVLTVLHQDWLNGKEYKCKVSNKALPAPIEKTISKAKGQPRRPRVYTLPPSREEMTDNQVSLVCLVKGFYPSDIAVEWESNGQPENNYKTTPPVLISDGSFFLASNLTVDKSRWQQGNVFSCSVMHEALHNHYTQKSLSLSP

SEQ ID NO: 305 - protein, 447 aa, Homo sapiens
QVQLQESGPGLVRPSQTLSLTCTVSGYSITSDHAWSWVRQPPGRGLEWIGYISYSGITTYNPSLKSRVTMLRDTSKNQFSLRLSSVTAADTAVYYCARSLARTTAMDYWGQGSLVTVSSASTKGPSVFPLAPSSKSTSGGTAALGCLVKDYFPEPVTVSWNSGALTSGVHTFPAVLQSSGLYSLSSVVTVPSSSLGTQTYICNVNHKPSNTKVDKRVEPKSCDKTHTCPPCPAPELLGGPSVFLFPPKPKDTLMISRTPEVTCVVVDVSHEDPEVKFNWYVDGVEVHNAKTKPREEQYNSTYRVVSVLTVLHQDWLNGKEYKCKVSNKALPAPIEKTISKAKGQPRRPRVYTLPPSREEMTDNQVSLVCLVKGFYPSDIAVEWESNGQPENNYKTTPPVLISDGSFFLASHLTVDKSRWQQGNVFSCSVMHEALHNHYTQKSLSLSP

SEQ ID NO: 306 - protein, 447 aa, Homo sapiens
QVQLQESGPGLVRPSQTLSLTCTVSGYSITSDHAWSWVRQPPGRGLEWIGYISYSGITTYNPSLKSRVTMLRDTSKNQFSLRLSSVTAADTAVYYCARSLARTTAMDYWGQGSLVTVSSASTKGPSVFPLAPSSKSTSGGTAALGCLVKDYFPEPVTVSWNSGALTSGVHTFPAVLQSSGLYSLSSVVTVPSSSLGTQTYICNVNHKPSNTKVDKRVEPKSCDKTHTCPPCPAPELLGGPSVFLFPPKPKDTLMISRTPEVTCVVVDVSHEDPEVKFNWYVDGVEVHNAKTKPREEQYNSTYRVVSVLTVLHQDWLNGKEYKCKVSNKALPAPIEKTISKAKGQPRRPRVYTLPPSREEMTDNQVSLVCLVKGFYPSDIAVEWESNGQPENNYKTTPPVLVSDGSFFLASLLTVDKSRWQQGNVFSCSVMHEALHNHYTQKSLSLSP

SEQ ID NO: 307 - protein, 447 aa, Homo sapiens
QVQLQESGPGLVRPSQTLSLTCTVSGYSITSDHAWSWVRQPPGRGLEWIGYISYSGITTYNPSLKSRVTMLRDTSKNQFSLRLSSVTAADTAVYYCARSLARTTAMDYWGQGSLVTVSSASTKGPSVFPLAPSSKSTSGGTAALGCLVKDYFPEPVTVSWNSGALTSGVHTFPAVLQSSGLYSLSSVVTVPSSSLGTQTYICNVNHKPSNTKVDKRVEPKSCDKTHTCPPCPAPELLGGPSVFLFPPKPKDTLMISRTPEVTCVVVDVSHEDPEVKFNWYVDGVEVHNAKTKPREEQYNSTYRVVSVLTVLHQDWLNGKEYKCKVSNKALPAPIEKTISKAKGQPRRPRVYTLPPSREEMTDNQVSLVCLVKGFYPSDIAVEWESNGQPENNYKTTPPVLYSDGSFFLASLLTVDKSRWQQGNVFSCSVMHEALHNHYTQKSLSLSP

SEQ ID NO: 308 - protein, 447 aa, Homo sapiens
QVQLQESGPGLVRPSQTLSLTCTVSGYSITSDHAWSWVRQPPGRGLEWIGYISYSGITTYNPSLKSRVTMLRDTSKNQFSLRLSSVTAADTAVYYCARSLARTTAMDYWGQGSLVTVSSASTKGPSVFPLAPSSKSTSGGTAALGCLVKDYFPEPVTVSWNSGALTSGVHTFPAVLQSSGLYSLSSVVTVPSSSLGTQTYICNVNHKPSNTKVDKRVEPKSCDKTHTCPPCPAPELLGGPSVFLFPPKPKDTLMISRTPEVTCVVVDVSHEDPEVKFNWYVDGVEVHNAKTKPREEQYNSTYRVVSVLTVLHQDWLNGKEYKCKVSNKALPAPIEKTISKAKGQPRRPRVYTLPPSREEMTDNQVSLVCLVKGFYPSDIAVEWESNGQPENNYKTTPPVLSSDGSFFLASFLTVDKSRWQQGNVFSCSVMHEALHNHYTQKSLSLSP

SEQ ID NO: 309 - protein, 447 aa, Homo sapiens
QVQLQESGPGLVRPSQTLSLTCTVSGYSITSDHAWSWVRQPPGRGLEWIGYISYSGITTYNPSLKSRVTMLRDTSKNQFSLRLSSVTAADTAVYYCARSLARTTAMDYWGQGSLVTVSSASTKGPSVFPLAPSSKSTSGGTAALGCLVKDYFPEPVTVSWNSGALTSGVHTFPAVLQSSGLYSLSSVVTVPSSSLGTQTYICNVNHKPSNTKVDKRVEPKSCDKTHTCPPCPAPELLGGPSVFLFPPKPKDTLMISRTPEVTCVVVDVSHEDPEVKFNWYVDGVEVHNAKTKPREEQYNSTYRVVSVLTVLHQDWLNGKEYKCKVSNKALPAPIEKTISKAKGQPRRPRVYTLPPSREEMTDNQVSLVCLVKGFYPSDIAVEWESNGQPENNYKTTPPVLNSDGSFFLASYLTVDKSRWQQGNVFSCSVMHEALHNHYTQKSLSLSP

SEQ ID NO: 310 - protein, 447 aa, Homo sapiens
QVQLQESGPGLVRPSQTLSLTCTVSGYSITSDHAWSWVRQPPGRGLEWIGYISYSGITTYNPSLKSRVTMLRDTSKNQFSLRLSSVTAADTAVYYCARSLARTTAMDYWGQGSLVTVSSASTKGPSVFPLAPSSKSTSGGTAALGCLVKDYFPEPVTVSWNSGALTSGVHTFPAVLQSSGLYSLSSVVTVPSSSLGTQTYICNVNHKPSNTKVDKRVEPKSCDKTHTCPPCPAPELLGGPSVFLFPPKPKDTLMISRTPEVTCVVVDVSHEDPEVKFNWYVDGVEVHNAKTKPREEQYNSTYRVVSVLTVLHQDWLNGKEYKCKVSNKALPAPIEKTISKAKGQPRRPRVYTLPPSREEMTDNQVSLVCLVKGFYPSDIAVEWESNGQPENNYKTTPPVLTSDGSFFLASYLTVDKSRWQQGNVFSCSVMHEALHNHYTQKSLSLSP

SEQ ID NO: 311 - protein, 447 aa, Homo sapiens
QVQLQESGPGLVRPSQTLSLTCTVSGYSITSDHAWSWVRQPPGRGLEWIGYISYSGITTYNPSLKSRVTMLRDTSKNQFSLRLSSVTAADTAVYYCARSLARTTAMDYWGQGSLVTVSSASTKGPSVFPLAPSSKSTSGGTAALGCLVKDYFPEPVTVSWNSGALTSGVHTFPAVLQSSGLYSLSSVVTVPSSSLGTQTYICNVNHKPSNTKVDKRVEPKSCDKTHTCPPCPAPELLGGPSVFLFPPKPKDTLMISRTPEVTCVVVDVSHEDPEVKFNWYVDGVEVHNAKTKPREEQYNSTYRVVSVLTVLHQDWLNGKEYKCKVSNKALPAPIEKTISKAKGQPRRPRVYTLPPSREEMTDNQVSLVCLVKGFYPSDIAVEWESNGQPENNYKTTPPVLQSDGSFFLASTLTVDKSRWQQGNVFSCSVMHEALHNHYTQKSLSLSP

SEQ ID NO: 312 - protein, 447 aa, Homo sapiens
QVQLQESGPGLVRPSQTLSLTCTVSGYSITSDHAWSWVRQPPGRGLEWIGYISYSGITTYNPSLKSRVTMLRDTSKNQFSLRLSSVTAADTAVYYCARSLARTTAMDYWGQGSLVTVSSASTKGPSVFPLAPSSKSTSGGTAALGCLVKDYFPEPVTVSWNSGALTSGVHTFPAVLQSSGLYSLSSVVTVPSSSLGTQTYICNVNHKPSNTKVDKRVEPKSCDKTHTCPPCPAPELLGGPSVFLFPPKPKDTLMISRTPEVTCVVVDVSHEDPEVKFNWYVDGVEVHNAKTKPREEQYNSTYRVVSVLTVLHQDWLNGKEYKCKVSNKALPAPIEKTISKAKGQPRRPRVYTLPPSREEMTDNQVSLVCLVKGFYPSDIAVEWESNGQPENNYKTTPPVLNSDGSFFLASNLTVDKSRWQQGNVFSCSVMHEALHNHYTQKSLSLSP

SEQ ID NO: 313 - protein, 447 aa, Homo sapiens
QVQLQESGPGLVRPSQTLSLTCTVSGYSITSDHAWSWVRQPPGRGLEWIGYISYSGITTYNPSLKSRVTMLRDTSKNQFSLRLSSVTAADTAVYYCARSLARTTAMDYWGQGSLVTVSSASTKGPSVFPLAPSSKSTSGGTAALGCLVKDYFPEPVTVSWNSGALTSGVHTFPAVLQSSGLYSLSSVVTVPSSSLGTQTYICNVNHKPSNTKVDKRVEPKSCDKTHTCPPCPAPELLGGPSVFLFPPKPKDTLMISRTPEVTCVVVDVSHEDPEVKFNWYVDGVEVHNAKTKPREEQYNSTYRVVSVLTVLHQDWLNGKEYKCKVSNKALPAPIEKTISKAKGQPREPRVYTLPPSREEMTENQVSLTCLVKGFYPSDIAVEWESNGQPENNYKTTPPVLVSDGSFTLYSFLTVDKSRWQQGNVFSCSVMHEALHNHYTQKSLSLSP

SEQ ID NO: 314 - protein, 447 aa, Homo sapiens
QVQLQESGPGLVRPSQTLSLTCTVSGYSITSDHAWSWVRQPPGRGLEWIGYISYSGITTYNPSLKSRVTMLRDTSKNQFSLRLSSVTAADTAVYYCARSLARTTAMDYWGQGSLVTVSSASTKGPSVFPLAPSSKSTSGGTAALGCLVKDYFPEPVTVSWNSGALTSGVHTFPAVLQSSGLYSLSSVVTVPSSSLGTQTYICNVNHKPSNTKVDKRVEPKSCDKTHTCPPCPAPELLGGPSVFLFPPKPKDTLMISRTPEVTCVVVDVSHEDPEVKFNWYVDGVEVHNAKTKPREEQYNSTYRVVSVLTVLHQDWLNGKEYKCKVSNKALPAPIEKTISKAKGQPREPKVYTLPPSREEMTENQVSLTCLVKGFYPSDIAVEWESNGQPENNYKTTPPVLVSDGSFTLYSWLTVDKSRWQQGNVFSCSVMHEALHNHYTQKSLSLSP

SEQ ID NO: 315 - protein, 447 aa, Homo sapiens
QVQLQESGPGLVRPSQTLSLTCTVSGYSITSDHAWSWVRQPPGRGLEWIGYISYSGITTYNPSLKSRVTMLRDTSKNQFSLRLSSVTAADTAVYYCARSLARTTAMDYWGQGSLVTVSSASTKGPSVFPLAPSSKSTSGGTAALGCLVKDYFPEPVTVSWNSGALTSGVHTFPAVLQSSGLYSLSSVVTVPSSSLGTQTYICNVNHKPSNTKVDKRVEPKSCDKTHTCPPCPAPELLGGPSVFLFPPKPKDTLMISRTPEVTCVVVDVSHEDPEVKFNWYVDGVEVHNAKTKPREEQYNSTYRVVSVLTVLHQDWLNGKEYKCKVSNKALPAPIEKTISKAKGQPREPYVYTLPPSREEMTENQVSLTCLVKGFYPSDIAVEWESNGQPENNYKTTPPVLVSDGSFTLYSWLTVDKSRWQQGNVFSCSVMHEALHNHYTQKSLSLSP

SEQ ID NO: 316 - protein, 447 aa, Homo sapiens
QVQLQESGPGLVRPSQTLSLTCTVSGYSITSDHAWSWVRQPPGRGLEWIGYISYSGITTYNPSLKSRVTMLRDTSKNQFSLRLSSVTAADTAVYYCARSLARTTAMDYWGQGSLVTVSSASTKGPSVFPLAPSSKSTSGGTAALGCLVKDYFPEPVTVSWNSGALTSGVHTFPAVLQSSGLYSLSSVVTVPSSSLGTQTYICNVNHKPSNTKVDKRVEPKSCDKTHTCPPCPAPELLGGPSVFLFPPKPKDTLMISRTPEVTCVVVDVSHEDPEVKFNWYVDGVEVHNAKTKPREEQYNSTYRVVSVLTVLHQDWLNGKEYKCKVSNKALPAPIEKTISKAKGQPREPRVYTLPPSREEMTDNQVSLTCLVKGFYPSDIAVEWESNGQPENNYKTTPPVLVSDGSFTLYSWLTVDKSRWQQGNVFSCSVMHEALHNHYTQKSLSLSP

SEQ ID NO: 317 - protein, 447 aa, Homo sapiens
QVQLQESGPGLVRPSQTLSLTCTVSGYSITSDHAWSWVRQPPGRGLEWIGYISYSGITTYNPSLKSRVTMLRDTSKNQFSLRLSSVTAADTAVYYCARSLARTTAMDYWGQGSLVTVSSASTKGPSVFPLAPSSKSTSGGTAALGCLVKDYFPEPVTVSWNSGALTSGVHTFPAVLQSSGLYSLSSVVTVPSSSLGTQTYICNVNHKPSNTKVDKRVEPKSCDKTHTCPPCPAPELLGGPSVFLFPPKPKDTLMISRTPEVTCVVVDVSHEDPEVKFNWYVDGVEVHNAKTKPREEQYNSTYRVVSVLTVLHQDWLNGKEYKCKVSNKALPAPIEKTISKAKGQPREPKVYTLPPSREEMTDNQVSLTCLVKGFYPSDIAVEWESNGQPENNYKTTPPVLVSDGSFTLYSWLTVDKSRWQQGNVFSCSVMHEALHNHYTQKSLSLSP

SEQ ID NO: 318 - protein, 447 aa, Homo sapiens
QVQLQESGPGLVRPSQTLSLTCTVSGYSITSDHAWSWVRQPPGRGLEWIGYISYSGITTYNPSLKSRVTMLRDTSKNQFSLRLSSVTAADTAVYYCARSLARTTAMDYWGQGSLVTVSSASTKGPSVFPLAPSSKSTSGGTAALGCLVKDYFPEPVTVSWNSGALTSGVHTFPAVLQSSGLYSLSSVVTVPSSSLGTQTYICNVNHKPSNTKVDKRVEPKSCDKTHTCPPCPAPELLGGPSVFLFPPKPKDTLMISRTPEVTCVVVDVSHEDPEVKFNWYVDGVEVHNAKTKPREEQYNSTYRVVSVLTVLHQDWLNGKEYKCKVSNKALPAPIEKTISKAKGQPREPHVYTLPPSREEMTDNQVSLTCLVKGFYPSDIAVEWESNGQPENNYKTTPPVLVSDGSFTLYSWLTVDKSRWQQGNVFSCSVMHEALHNHYTQKSLSLSP

SEQ ID NO: 319 - protein, 447 aa, Homo sapiens
QVQLQESGPGLVRPSQTLSLTCTVSGYSITSDHAWSWVRQPPGRGLEWIGYISYSGITTYNPSLKSRVTMLRDTSKNQFSLRLSSVTAADTAVYYCARSLARTTAMDYWGQGSLVTVSSASTKGPSVFPLAPSSKSTSGGTAALGCLVKDYFPEPVTVSWNSGALTSGVHTFPAVLQSSGLYSLSSVVTVPSSSLGTQTYICNVNHKPSNTKVDKRVEPKSCDKTHTCPPCPAPELLGGPSVFLFPPKPKDTLMISRTPEVTCVVVDVSHEDPEVKFNWYVDGVEVHNAKTKPREEQYNSTYRVVSVLTVLHQDWLNGKEYKCKVSNKALPAPIEKTISKAKGQPREPYVYTLPPSREEMTDNQVSLTCLVKGFYPSDIAVEWESNGQPENNYKTTPPVLVSDGSFTLYSWLTVDKSRWQQGNVFSCSVMHEALHNHYTQKSLSLSP

SEQ ID NO: 320 - protein, 447 aa, Homo sapiens
QVQLQESGPGLVRPSQTLSLTCTVSGYSITSDHAWSWVRQPPGRGLEWIGYISYSGITTYNPSLKSRVTMLRDTSKNQFSLRLSSVTAADTAVYYCARSLARTTAMDYWGQGSLVTVSSASTKGPSVFPLAPSSKSTSGGTAALGCLVKDYFPEPVTVSWNSGALTSGVHTFPAVLQSSGLYSLSSVVTVPSSSLGTQTYICNVNHKPSNTKVDKRVEPKSCDKTHTCPPCPAPELLGGPSVFLFPPKPKDTLMISRTPEVTCVVVDVSHEDPEVKFNWYVDGVEVHNAKTKPREEQYNSTYRVVSVLTVLHQDWLNGKEYKCKVSNKALPAPIEKTISKAKGQPREPRVYTLPPSREEMTENQVSLTCLVKGFYPSDIAVEWESNGQPENNYKTTPPVLLSDGSFTLYSWLTVDKSRWQQGNVFSCSVMHEALHNHYTQKSLSLSP

SEQ ID NO: 321 - protein, 447 aa, Homo sapiens
QVQLQESGPGLVRPSQTLSLTCTVSGYSITSDHAWSWVRQPPGRGLEWIGYISYSGITTYNPSLKSRVTMLRDTSKNQFSLRLSSVTAADTAVYYCARSLARTTAMDYWGQGSLVTVSSASTKGPSVFPLAPSSKSTSGGTAALGCLVKDYFPEPVTVSWNSGALTSGVHTFPAVLQSSGLYSLSSVVTVPSSSLGTQTYICNVNHKPSNTKVDKRVEPKSCDKTHTCPPCPAPELLGGPSVFLFPPKPKDTLMISRTPEVTCVVVDVSHEDPEVKFNWYVDGVEVHNAKTKPREEQYNSTYRVVSVLTVLHQDWLNGKEYKCKVSNKALPAPIEKTISKAKGQPREPRVYTLPPSREEMTENQVSLTCLVKGFYPSDIAVEWESNGQPENNYKTTPPVLISDGSFTLYSWLTVDKSRWQQGNVFSCSVMHEALHNHYTQKSLSLSP

SEQ ID NO: 322 - protein, 447 aa, Homo sapiens
QVQLQESGPGLVRPSQTLSLTCTVSGYSITSDHAWSWVRQPPGRGLEWIGYISYSGITTYNPSLKSRVTMLRDTSKNQFSLRLSSVTAADTAVYYCARSLARTTAMDYWGQGSLVTVSSASTKGPSVFPLAPSSKSTSGGTAALGCLVKDYFPEPVTVSWNSGALTSGVHTFPAVLQSSGLYSLSSVVTVPSSSLGTQTYICNVNHKPSNTKVDKRVEPKSCDKTHTCPPCPAPELLGGPSVFLFPPKPKDTLMISRTPEVTCVVVDVSHEDPEVKFNWYVDGVEVHNAKTKPREEQYNSTYRVVSVLTVLHQDWLNGKEYKCKVSNKALPAPIEKTISKAKGQPREPRVYTLPPSREEMTENQVSLTCLVKGFYPSDIAVEWESNGQPENNYKTTPPVLMSDGSFTLYSWLTVDKSRWQQGNVFSCSVMHEALHNHYTQKSLSLSP

SEQ ID NO: 323 - protein, 447 aa, Homo sapiens
QVQLQESGPGLVRPSQTLSLTCTVSGYSITSDHAWSWVRQPPGRGLEWIGYISYSGITTYNPSLKSRVTMLRDTSKNQFSLRLSSVTAADTAVYYCARSLARTTAMDYWGQGSLVTVSSASTKGPSVFPLAPSSKSTSGGTAALGCLVKDYFPEPVTVSWNSGALTSGVHTFPAVLQSSGLYSLSSVVTVPSSSLGTQTYICNVNHKPSNTKVDKRVEPKSCDKTHTCPPCPAPELLGGPSVFLFPPKPKDTLMISRTPEVTCVVVDVSHEDPEVKFNWYVDGVEVHNAKTKPREEQYNSTYRVVSVLTVLHQDWLNGKEYKCKVSNKALPAPIEKTISKAKGQPREPRVYTLPPSREEMTENQVSLTCLVKGFYPSDIAVEWESNGQPENNYKTTPPVLSSDGSFTLYSWLTVDKSRWQQGNVFSCSVMHEALHNHYTQKSLSLSP

SEQ ID NO: 324 - protein, 447 aa, Homo sapiens
QVQLQESGPGLVRPSQTLSLTCTVSGYSITSDHAWSWVRQPPGRGLEWIGYISYSGITTYNPSLKSRVTMLRDTSKNQFSLRLSSVTAADTAVYYCARSLARTTAMDYWGQGSLVTVSSASTKGPSVFPLAPSSKSTSGGTAALGCLVKDYFPEPVTVSWNSGALTSGVHTFPAVLQSSGLYSLSSVVTVPSSSLGTQTYICNVNHKPSNTKVDKRVEPKSCDKTHTCPPCPAPELLGGPSVFLFPPKPKDTLMISRTPEVTCVVVDVSHEDPEVKFNWYVDGVEVHNAKTKPREEQYNSTYRVVSVLTVLHQDWLNGKEYKCKVSNKALPAPIEKTISKAKGQPREPRVYTLPPSREEMTENQVSLTCLVKGFYPSDIAVEWESNGQPENNYKTTPPVLTSDGSFTLYSWLTVDKSRWQQGNVFSCSVMHEALHNHYTQKSLSLSP

SEQ ID NO: 325 - protein, 447 aa, Homo sapiens
QVQLQESGPGLVRPSQTLSLTCTVSGYSITSDHAWSWVRQPPGRGLEWIGYISYSGITTYNPSLKSRVTMLRDTSKNQFSLRLSSVTAADTAVYYCARSLARTTAMDYWGQGSLVTVSSASTKGPSVFPLAPSSKSTSGGTAALGCLVKDYFPEPVTVSWNSGALTSGVHTFPAVLQSSGLYSLSSVVTVPSSSLGTQTYICNVNHKPSNTKVDKRVEPKSCDKTHTCPPCPAPELLGGPSVFLFPPKPKDTLMISRTPEVTCVVVDVSHEDPEVKFNWYVDGVEVHNAKTKPREEQYNSTYRVVSVLTVLHQDWLNGKEYKCKVSNKALPAPIEKTISKAKGQPREPRVYTLPPSREEMTENQVSLTCLVKGFYPSDIAVEWESNGQPENNYKTTPPVLCSDGSFTLYSWLTVDKSRWQQGNVFSCSVMHEALHNHYTQKSLSLSP

SEQ ID NO: 326 - protein, 447 aa, Homo sapiens
QVQLQESGPGLVRPSQTLSLTCTVSGYSITSDHAWSWVRQPPGRGLEWIGYISYSGITTYNPSLKSRVTMLRDTSKNQFSLRLSSVTAADTAVYYCARSLARTTAMDYWGQGSLVTVSSASTKGPSVFPLAPSSKSTSGGTAALGCLVKDYFPEPVTVSWNSGALTSGVHTFPAVLQSSGLYSLSSVVTVPSSSLGTQTYICNVNHKPSNTKVDKRVEPKSCDKTHTCPPCPAPELLGGPSVFLFPPKPKDTLMISRTPEVTCVVVDVSHEDPEVKFNWYVDGVEVHNAKTKPREEQYNSTYRVVSVLTVLHQDWLNGKEYKCKVSNKALPAPIEKTISKAKGQPREPRVYTLPPSREEMTENQVSLTCLVKGFYPSDIAVEWESNGQPENNYKTTPPVLHSDGSFTLYSWLTVDKSRWQQGNVFSCSVMHEALHNHYTQKSLSLSP

SEQ ID NO: 327 - protein, 447 aa, Homo sapiens
QVQLQESGPGLVRPSQTLSLTCTVSGYSITSDHAWSWVRQPPGRGLEWIGYISYSGITTYNPSLKSRVTMLRDTSKNQFSLRLSSVTAADTAVYYCARSLARTTAMDYWGQGSLVTVSSASTKGPSVFPLAPSSKSTSGGTAALGCLVKDYFPEPVTVSWNSGALTSGVHTFPAVLQSSGLYSLSSVVTVPSSSLGTQTYICNVNHKPSNTKVDKRVEPKSCDKTHTCPPCPAPELLGGPSVFLFPPKPKDTLMISRTPEVTCVVVDVSHEDPEVKFNWYVDGVEVHNAKTKPREEQYNSTYRVVSVLTVLHQDWLNGKEYKCKVSNKALPAPIEKTISKAKGQPREPRVYTLPPSREEMTENQVSLTCLVKGFYPSDIAVEWESNGQPENNYKTTPPVLVSDGSFALYSWLTVDKSRWQQGNVFSCSVMHEALHNHYTQKSLSLSP

SEQ ID NO: 328 - protein, 447 aa, Homo sapiens
QVQLQESGPGLVRPSQTLSLTCTVSGYSITSDHAWSWVRQPPGRGLEWIGYISYSGITTYNPSLKSRVTMLRDTSKNQFSLRLSSVTAADTAVYYCARSLARTTAMDYWGQGSLVTVSSASTKGPSVFPLAPSSKSTSGGTAALGCLVKDYFPEPVTVSWNSGALTSGVHTFPAVLQSSGLYSLSSVVTVPSSSLGTQTYICNVNHKPSNTKVDKRVEPKSCDKTHTCPPCPAPELLGGPSVFLFPPKPKDTLMISRTPEVTCVVVDVSHEDPEVKFNWYVDGVEVHNAKTKPREEQYNSTYRVVSVLTVLHQDWLNGKEYKCKVSNKALPAPIEKTISKAKGQPREPRVYTLPPSREEMTENQVSLTCLVKGFYPSDIAVEWESNGQPENNYKTTPPVLVSDGSFVLYSWLTVDKSRWQQGNVFSCSVMHEALHNHYTQKSLSLSP

SEQ ID NO: 329 - protein, 447 aa, Homo sapiens
QVQLQESGPGLVRPSQTLSLTCTVSGYSITSDHAWSWVRQPPGRGLEWIGYISYSGITTYNPSLKSRVTMLRDTSKNQFSLRLSSVTAADTAVYYCARSLARTTAMDYWGQGSLVTVSSASTKGPSVFPLAPSSKSTSGGTAALGCLVKDYFPEPVTVSWNSGALTSGVHTFPAVLQSSGLYSLSSVVTVPSSSLGTQTYICNVNHKPSNTKVDKRVEPKSCDKTHTCPPCPAPELLGGPSVFLFPPKPKDTLMISRTPEVTCVVVDVSHEDPEVKFNWYVDGVEVHNAKTKPREEQYNSTYRVVSVLTVLHQDWLNGKEYKCKVSNKALPAPIEKTISKAKGQPREPRVYTLPPSREEMTENQVSLTCLVKGFYPSDIAVEWESNGQPENNYKTTPPVLVSDGSFSLYSWLTVDKSRWQQGNVFSCSVMHEALHNHYTQKSLSLSP

SEQ ID NO: 330 - protein, 447 aa, Homo sapiens
QVQLQESGPGLVRPSQTLSLTCTVSGYSITSDHAWSWVRQPPGRGLEWIGYISYSGITTYNPSLKSRVTMLRDTSKNQFSLRLSSVTAADTAVYYCARSLARTTAMDYWGQGSLVTVSSASTKGPSVFPLAPSSKSTSGGTAALGCLVKDYFPEPVTVSWNSGALTSGVHTFPAVLQSSGLYSLSSVVTVPSSSLGTQTYICNVNHKPSNTKVDKRVEPKSCDKTHTCPPCPAPELLGGPSVFLFPPKPKDTLMISRTPEVTCVVVDVSHEDPEVKFNWYVDGVEVHNAKTKPREEQYNSTYRVVSVLTVLHQDWLNGKEYKCKVSNKALPAPIEKTISKAKGQPREPRVYTLPPSREEMTENQVSLTCLVKGFYPSDIAVEWESNGQPENNYKTTPPVLVSDGSFCLYSWLTVDKSRWQQGNVFSCSVMHEALHNHYTQKSLSLSP

SEQ ID NO: 331 - protein, 447 aa, Homo sapiens
QVQLQESGPGLVRPSQTLSLTCTVSGYSITSDHAWSWVRQPPGRGLEWIGYISYSGITTYNPSLKSRVTMLRDTSKNQFSLRLSSVTAADTAVYYCARSLARTTAMDYWGQGSLVTVSSASTKGPSVFPLAPSSKSTSGGTAALGCLVKDYFPEPVTVSWNSGALTSGVHTFPAVLQSSGLYSLSSVVTVPSSSLGTQTYICNVNHKPSNTKVDKRVEPKSCDKTHTCPPCPAPELLGGPSVFLFPPKPKDTLMISRTPEVTCVVVDVSHEDPEVKFNWYVDGVEVHNAKTKPREEQYNSTYRVVSVLTVLHQDWLNGKEYKCKVSNKALPAPIEKTISKAKGQPREPRVYTLPPSREEMTENQVSLTCLVKGFYPSDIAVEWESNGQPENNYKTTPPVLVSDGSFNLYSWLTVDKSRWQQGNVFSCSVMHEALHNHYTQKSLSLSP

SEQ ID NO: 332 - protein, 447 aa, Homo sapiens
QVQLQESGPGLVRPSQTLSLTCTVSGYSITSDHAWSWVRQPPGRGLEWIGYISYSGITTYNPSLKSRVTMLRDTSKNQFSLRLSSVTAADTAVYYCARSLARTTAMDYWGQGSLVTVSSASTKGPSVFPLAPSSKSTSGGTAALGCLVKDYFPEPVTVSWNSGALTSGVHTFPAVLQSSGLYSLSSVVTVPSSSLGTQTYICNVNHKPSNTKVDKRVEPKSCDKTHTCPPCPAPELLGGPSVFLFPPKPKDTLMISRTPEVTCVVVDVSHEDPEVKFNWYVDGVEVHNAKTKPREEQYNSTYRVVSVLTVLHQDWLNGKEYKCKVSNKALPAPIEKTISKAKGQPREPRVYTLPPSREEMTENQVSLTCLVKGFYPSDIAVEWESNGQPENNYKTTPPVLVSDGSFDLYSWLTVDKSRWQQGNVFSCSVMHEALHNHYTQKSLSLSP

SEQ ID NO: 333 - protein, 447 aa, Homo sapiens
QVQLQESGPGLVRPSQTLSLTCTVSGYSITSDHAWSWVRQPPGRGLEWIGYISYSGITTYNPSLKSRVTMLRDTSKNQFSLRLSSVTAADTAVYYCARSLARTTAMDYWGQGSLVTVSSASTKGPSVFPLAPSSKSTSGGTAALGCLVKDYFPEPVTVSWNSGALTSGVHTFPAVLQSSGLYSLSSVVTVPSSSLGTQTYICNVNHKPSNTKVDKRVEPKSCDKTHTCPPCPAPELLGGPSVFLFPPKPKDTLMISRTPEVTCVVVDVSHEDPEVKFNWYVDGVEVHNAKTKPREEQYNSTYRVVSVLTVLHQDWLNGKEYKCKVSNKALPAPIEKTISKAKGQPREPRVYTLPPSREEMTENQVSLTCLVKGFYPSDIAVEWESNGQPENNYKTTPPVLVSDGSFTLYSYLTVDKSRWQQGNVFSCSVMHEALHNHYTQKSLSLSP

SEQ ID NO: 334 - protein, 447 aa, Homo sapiens
QVQLQESGPGLVRPSQTLSLTCTVSGYSITSDHAWSWVRQPPGRGLEWIGYISYSGITTYNPSLKSRVTMLRDTSKNQFSLRLSSVTAADTAVYYCARSLARTTAMDYWGQGSLVTVSSASTKGPSVFPLAPSSKSTSGGTAALGCLVKDYFPEPVTVSWNSGALTSGVHTFPAVLQSSGLYSLSSVVTVPSSSLGTQTYICNVNHKPSNTKVDKRVEPKSCDKTHTCPPCPAPELLGGPSVFLFPPKPKDTLMISRTPEVTCVVVDVSHEDPEVKFNWYVDGVEVHNAKTKPREEQYNSTYRVVSVLTVLHQDWLNGKEYKCKVSNKALPAPIEKTISKAKGQPREPRVYTLPPSREEMTENQVSLTCLVKGFYPSDIAVEWESNGQPENNYKTTPPVLVSDGSFTLYSHLTVDKSRWQQGNVFSCSVMHEALHNHYTQKSLSLSP

SEQ ID NO: 335 - protein, 447 aa, Homo sapiens
QVQLQESGPGLVRPSQTLSLTCTVSGYSITSDHAWSWVRQPPGRGLEWIGYISYSGITTYNPSLKSRVTMLRDTSKNQFSLRLSSVTAADTAVYYCARSLARTTAMDYWGQGSLVTVSSASTKGPSVFPLAPSSKSTSGGTAALGCLVKDYFPEPVTVSWNSGALTSGVHTFPAVLQSSGLYSLSSVVTVPSSSLGTQTYICNVNHKPSNTKVDKRVEPKSCDKTHTCPPCPAPELLGGPSVFLFPPKPKDTLMISRTPEVTCVVVDVSHEDPEVKFNWYVDGVEVHNAKTKPREEQYNSTYRVVSVLTVLHQDWLNGKEYKCKVSNKALPAPIEKTISKAKGQPREPRVYTLPPSREEMTENQVSLTCLVKGFYPSDIAVEWESNGQPENNYKTTPPVLASDGSFTLYSFLTVDKSRWQQGNVFSCSVMHEALHNHYTQKSLSLSP

SEQ ID NO: 336 - protein, 447 aa, Homo sapiens
QVQLQESGPGLVRPSQTLSLTCTVSGYSITSDHAWSWVRQPPGRGLEWIGYISYSGITTYNPSLKSRVTMLRDTSKNQFSLRLSSVTAADTAVYYCARSLARTTAMDYWGQGSLVTVSSASTKGPSVFPLAPSSKSTSGGTAALGCLVKDYFPEPVTVSWNSGALTSGVHTFPAVLQSSGLYSLSSVVTVPSSSLGTQTYICNVNHKPSNTKVDKRVEPKSCDKTHTCPPCPAPELLGGPSVFLFPPKPKDTLMISRTPEVTCVVVDVSHEDPEVKFNWYVDGVEVHNAKTKPREEQYNSTYRVVSVLTVLHQDWLNGKEYKCKVSNKALPAPIEKTISKAKGQPREPRVYTLPPSREEMTENQVSLTCLVKGFYPSDIAVEWESNGQPENNYKTTPPVLLSDGSFTLYSFLTVDKSRWQQGNVFSCSVMHEALHNHYTQKSLSLSP

SEQ ID NO: 337 - protein, 447 aa, Homo sapiens
QVQLQESGPGLVRPSQTLSLTCTVSGYSITSDHAWSWVRQPPGRGLEWIGYISYSGITTYNPSLKSRVTMLRDTSKNQFSLRLSSVTAADTAVYYCARSLARTTAMDYWGQGSLVTVSSASTKGPSVFPLAPSSKSTSGGTAALGCLVKDYFPEPVTVSWNSGALTSGVHTFPAVLQSSGLYSLSSVVTVPSSSLGTQTYICNVNHKPSNTKVDKRVEPKSCDKTHTCPPCPAPELLGGPSVFLFPPKPKDTLMISRTPEVTCVVVDVSHEDPEVKFNWYVDGVEVHNAKTKPREEQYNSTYRVVSVLTVLHQDWLNGKEYKCKVSNKALPAPIEKTISKAKGQPREPRVYTLPPSREEMTENQVSLTCLVKGFYPSDIAVEWESNGQPENNYKTTPPVLISDGSFTLYSFLTVDKSRWQQGNVFSCSVMHEALHNHYTQKSLSLSP

SEQ ID NO: 338 - protein, 447 aa, Homo sapiens
QVQLQESGPGLVRPSQTLSLTCTVSGYSITSDHAWSWVRQPPGRGLEWIGYISYSGITTYNPSLKSRVTMLRDTSKNQFSLRLSSVTAADTAVYYCARSLARTTAMDYWGQGSLVTVSSASTKGPSVFPLAPSSKSTSGGTAALGCLVKDYFPEPVTVSWNSGALTSGVHTFPAVLQSSGLYSLSSVVTVPSSSLGTQTYICNVNHKPSNTKVDKRVEPKSCDKTHTCPPCPAPELLGGPSVFLFPPKPKDTLMISRTPEVTCVVVDVSHEDPEVKFNWYVDGVEVHNAKTKPREEQYNSTYRVVSVLTVLHQDWLNGKEYKCKVSNKALPAPIEKTISKAKGQPREPRVYTLPPSREEMTENQVSLTCLVKGFYPSDIAVEWESNGQPENNYKTTPPVLMSDGSFTLYSFLTVDKSRWQQGNVFSCSVMHEALHNHYTQKSLSLSP

SEQ ID NO: 339 - protein, 447 aa, Homo sapiens
QVQLQESGPGLVRPSQTLSLTCTVSGYSITSDHAWSWVRQPPGRGLEWIGYISYSGITTYNPSLKSRVTMLRDTSKNQFSLRLSSVTAADTAVYYCARSLARTTAMDYWGQGSLVTVSSASTKGPSVFPLAPSSKSTSGGTAALGCLVKDYFPEPVTVSWNSGALTSGVHTFPAVLQSSGLYSLSSVVTVPSSSLGTQTYICNVNHKPSNTKVDKRVEPKSCDKTHTCPPCPAPELLGGPSVFLFPPKPKDTLMISRTPEVTCVVVDVSHEDPEVKFNWYVDGVEVHNAKTKPREEQYNSTYRVVSVLTVLHQDWLNGKEYKCKVSNKALPAPIEKTISKAKGQPREPRVYTLPPSREEMTENQVSLTCLVKGFYPSDIAVEWESNGQPENNYKTTPPVLTSDGSFTLYSFLTVDKSRWQQGNVFSCSVMHEALHNHYTQKSLSLSP

SEQ ID NO: 340 - protein, 447 aa, Homo sapiens
QVQLQESGPGLVRPSQTLSLTCTVSGYSITSDHAWSWVRQPPGRGLEWIGYISYSGITTYNPSLKSRVTMLRDTSKNQFSLRLSSVTAADTAVYYCARSLARTTAMDYWGQGSLVTVSSASTKGPSVFPLAPSSKSTSGGTAALGCLVKDYFPEPVTVSWNSGALTSGVHTFPAVLQSSGLYSLSSVVTVPSSSLGTQTYICNVNHKPSNTKVDKRVEPKSCDKTHTCPPCPAPELLGGPSVFLFPPKPKDTLMISRTPEVTCVVVDVSHEDPEVKFNWYVDGVEVHNAKTKPREEQYNSTYRVVSVLTVLHQDWLNGKEYKCKVSNKALPAPIEKTISKAKGQPREPRVYTLPPSREEMTENQVSLTCLVKGFYPSDIAVEWESNGQPENNYKTTPPVLCSDGSFTLYSFLTVDKSRWQQGNVFSCSVMHEALHNHYTQKSLSLSP

SEQ ID NO: 341 - protein, 447 aa, Homo sapiens
QVQLQESGPGLVRPSQTLSLTCTVSGYSITSDHAWSWVRQPPGRGLEWIGYISYSGITTYNPSLKSRVTMLRDTSKNQFSLRLSSVTAADTAVYYCARSLARTTAMDYWGQGSLVTVSSASTKGPSVFPLAPSSKSTSGGTAALGCLVKDYFPEPVTVSWNSGALTSGVHTFPAVLQSSGLYSLSSVVTVPSSSLGTQTYICNVNHKPSNTKVDKRVEPKSCDKTHTCPPCPAPELLGGPSVFLFPPKPKDTLMISRTPEVTCVVVDVSHEDPEVKFNWYVDGVEVHNAKTKPREEQYNSTYRVVSVLTVLHQDWLNGKEYKCKVSNKALPAPIEKTISKAKGQPREPRVYTLPPSREEMTENQVSLTCLVKGFYPSDIAVEWESNGQPENNYKTTPPVLNSDGSFTLYSFLTVDKSRWQQGNVFSCSVMHEALHNHYTQKSLSLSP

SEQ ID NO: 342 - protein, 447 aa, Homo sapiens
QVQLQESGPGLVRPSQTLSLTCTVSGYSITSDHAWSWVRQPPGRGLEWIGYISYSGITTYNPSLKSRVTMLRDTSKNQFSLRLSSVTAADTAVYYCARSLARTTAMDYWGQGSLVTVSSASTKGPSVFPLAPSSKSTSGGTAALGCLVKDYFPEPVTVSWNSGALTSGVHTFPAVLQSSGLYSLSSVVTVPSSSLGTQTYICNVNHKPSNTKVDKRVEPKSCDKTHTCPPCPAPELLGGPSVFLFPPKPKDTLMISRTPEVTCVVVDVSHEDPEVKFNWYVDGVEVHNAKTKPREEQYNSTYRVVSVLTVLHQDWLNGKEYKCKVSNKALPAPIEKTISKAKGQPREPRVYTLPPSREEMTENQVSLTCLVKGFYPSDIAVEWESNGQPENNYKTTPPVLQSDGSFTLYSFLTVDKSRWQQGNVFSCSVMHEALHNHYTQKSLSLSP

SEQ ID NO: 343 - protein, 447 aa, Homo sapiens
QVQLQESGPGLVRPSQTLSLTCTVSGYSITSDHAWSWVRQPPGRGLEWIGYISYSGITTYNPSLKSRVTMLRDTSKNQFSLRLSSVTAADTAVYYCARSLARTTAMDYWGQGSLVTVSSASTKGPSVFPLAPSSKSTSGGTAALGCLVKDYFPEPVTVSWNSGALTSGVHTFPAVLQSSGLYSLSSVVTVPSSSLGTQTYICNVNHKPSNTKVDKRVEPKSCDKTHTCPPCPAPELLGGPSVFLFPPKPKDTLMISRTPEVTCVVVDVSHEDPEVKFNWYVDGVEVHNAKTKPREEQYNSTYRVVSVLTVLHQDWLNGKEYKCKVSNKALPAPIEKTISKAKGQPREPRVYTLPPSREEMTENQVSLTCLVKGFYPSDIAVEWESNGQPENNYKTTPPVLHSDGSFTLYSFLTVDKSRWQQGNVFSCSVMHEALHNHYTQKSLSLSP

SEQ ID NO: 344 - protein, 447 aa, Homo sapiens
QVQLQESGPGLVRPSQTLSLTCTVSGYSITSDHAWSWVRQPPGRGLEWIGYISYSGITTYNPSLKSRVTMLRDTSKNQFSLRLSSVTAADTAVYYCARSLARTTAMDYWGQGSLVTVSSASTKGPSVFPLAPSSKSTSGGTAALGCLVKDYFPEPVTVSWNSGALTSGVHTFPAVLQSSGLYSLSSVVTVPSSSLGTQTYICNVNHKPSNTKVDKRVEPKSCDKTHTCPPCPAPELLGGPSVFLFPPKPKDTLMISRTPEVTCVVVDVSHEDPEVKFNWYVDGVEVHNAKTKPREEQYNSTYRVVSVLTVLHQDWLNGKEYKCKVSNKALPAPIEKTISKAKGQPREPRVYTLPPSREEMTENQVSLTCLVKGFYPSDIAVEWESNGQPENNYKTTPPVLASDGSFTLYSYLTVDKSRWQQGNVFSCSVMHEALHNHYTQKSLSLSP

SEQ ID NO: 345 - protein, 447 aa, Homo sapiens
QVQLQESGPGLVRPSQTLSLTCTVSGYSITSDHAWSWVRQPPGRGLEWIGYISYSGITTYNPSLKSRVTMLRDTSKNQFSLRLSSVTAADTAVYYCARSLARTTAMDYWGQGSLVTVSSASTKGPSVFPLAPSSKSTSGGTAALGCLVKDYFPEPVTVSWNSGALTSGVHTFPAVLQSSGLYSLSSVVTVPSSSLGTQTYICNVNHKPSNTKVDKRVEPKSCDKTHTCPPCPAPELLGGPSVFLFPPKPKDTLMISRTPEVTCVVVDVSHEDPEVKFNWYVDGVEVHNAKTKPREEQYNSTYRVVSVLTVLHQDWLNGKEYKCKVSNKALPAPIEKTISKAKGQPREPRVYTLPPSREEMTENQVSLTCLVKGFYPSDIAVEWESNGQPENNYKTTPPVLLSDGSFTLYSYLTVDKSRWQQGNVFSCSVMHEALHNHYTQKSLSLSP

SEQ ID NO: 346 - protein, 447 aa, Homo sapiens
QVQLQESGPGLVRPSQTLSLTCTVSGYSITSDHAWSWVRQPPGRGLEWIGYISYSGITTYNPSLKSRVTMLRDTSKNQFSLRLSSVTAADTAVYYCARSLARTTAMDYWGQGSLVTVSSASTKGPSVFPLAPSSKSTSGGTAALGCLVKDYFPEPVTVSWNSGALTSGVHTFPAVLQSSGLYSLSSVVTVPSSSLGTQTYICNVNHKPSNTKVDKRVEPKSCDKTHTCPPCPAPELLGGPSVFLFPPKPKDTLMISRTPEVTCVVVDVSHEDPEVKFNWYVDGVEVHNAKTKPREEQYNSTYRVVSVLTVLHQDWLNGKEYKCKVSNKALPAPIEKTISKAKGQPREPRVYTLPPSREEMTENQVSLTCLVKGFYPSDIAVEWESNGQPENNYKTTPPVLMSDGSFTLYSYLTVDKSRWQQGNVFSCSVMHEALHNHYTQKSLSLSP

SEQ ID NO: 347 - protein, 447 aa, Homo sapiens
QVQLQESGPGLVRPSQTLSLTCTVSGYSITSDHAWSWVRQPPGRGLEWIGYISYSGITTYNPSLKSRVTMLRDTSKNQFSLRLSSVTAADTAVYYCARSLARTTAMDYWGQGSLVTVSSASTKGPSVFPLAPSSKSTSGGTAALGCLVKDYFPEPVTVSWNSGALTSGVHTFPAVLQSSGLYSLSSVVTVPSSSLGTQTYICNVNHKPSNTKVDKRVEPKSCDKTHTCPPCPAPELLGGPSVFLFPPKPKDTLMISRTPEVTCVVVDVSHEDPEVKFNWYVDGVEVHNAKTKPREEQYNSTYRVVSVLTVLHQDWLNGKEYKCKVSNKALPAPIEKTISKAKGQPREPRVYTLPPSREEMTENQVSLTCLVKGFYPSDIAVEWESNGQPENNYKTTPPVLSSDGSFTLYSYLTVDKSRWQQGNVFSCSVMHEALHNHYTQKSLSLSP

SEQ ID NO: 348 - protein, 447 aa, Homo sapiens
QVQLQESGPGLVRPSQTLSLTCTVSGYSITSDHAWSWVRQPPGRGLEWIGYISYSGITTYNPSLKSRVTMLRDTSKNQFSLRLSSVTAADTAVYYCARSLARTTAMDYWGQGSLVTVSSASTKGPSVFPLAPSSKSTSGGTAALGCLVKDYFPEPVTVSWNSGALTSGVHTFPAVLQSSGLYSLSSVVTVPSSSLGTQTYICNVNHKPSNTKVDKRVEPKSCDKTHTCPPCPAPELLGGPSVFLFPPKPKDTLMISRTPEVTCVVVDVSHEDPEVKFNWYVDGVEVHNAKTKPREEQYNSTYRVVSVLTVLHQDWLNGKEYKCKVSNKALPAPIEKTISKAKGQPREPRVYTLPPSREEMTENQVSLTCLVKGFYPSDIAVEWESNGQPENNYKTTPPVLTSDGSFTLYSYLTVDKSRWQQGNVFSCSVMHEALHNHYTQKSLSLSP

SEQ ID NO: 349 - protein, 447 aa, Homo sapiens
QVQLQESGPGLVRPSQTLSLTCTVSGYSITSDHAWSWVRQPPGRGLEWIGYISYSGITTYNPSLKSRVTMLRDTSKNQFSLRLSSVTAADTAVYYCARSLARTTAMDYWGQGSLVTVSSASTKGPSVFPLAPSSKSTSGGTAALGCLVKDYFPEPVTVSWNSGALTSGVHTFPAVLQSSGLYSLSSVVTVPSSSLGTQTYICNVNHKPSNTKVDKRVEPKSCDKTHTCPPCPAPELLGGPSVFLFPPKPKDTLMISRTPEVTCVVVDVSHEDPEVKFNWYVDGVEVHNAKTKPREEQYNSTYRVVSVLTVLHQDWLNGKEYKCKVSNKALPAPIEKTISKAKGQPREPRVYTLPPSREEMTENQVSLTCLVKGFYPSDIAVEWESNGQPENNYKTTPPVLCSDGSFTLYSYLTVDKSRWQQGNVFSCSVMHEALHNHYTQKSLSLSP

SEQ ID NO: 350 - protein, 447 aa, Homo sapiens
QVQLQESGPGLVRPSQTLSLTCTVSGYSITSDHAWSWVRQPPGRGLEWIGYISYSGITTYNPSLKSRVTMLRDTSKNQFSLRLSSVTAADTAVYYCARSLARTTAMDYWGQGSLVTVSSASTKGPSVFPLAPSSKSTSGGTAALGCLVKDYFPEPVTVSWNSGALTSGVHTFPAVLQSSGLYSLSSVVTVPSSSLGTQTYICNVNHKPSNTKVDKRVEPKSCDKTHTCPPCPAPELLGGPSVFLFPPKPKDTLMISRTPEVTCVVVDVSHEDPEVKFNWYVDGVEVHNAKTKPREEQYNSTYRVVSVLTVLHQDWLNGKEYKCKVSNKALPAPIEKTISKAKGQPREPRVYTLPPSREEMTENQVSLTCLVKGFYPSDIAVEWESNGQPENNYKTTPPVLNSDGSFTLYSYLTVDKSRWQQGNVFSCSVMHEALHNHYTQKSLSLSP

SEQ ID NO: 351 - protein, 447 aa, Homo sapiens
QVQLQESGPGLVRPSQTLSLTCTVSGYSITSDHAWSWVRQPPGRGLEWIGYISYSGITTYNPSLKSRVTMLRDTSKNQFSLRLSSVTAADTAVYYCARSLARTTAMDYWGQGSLVTVSSASTKGPSVFPLAPSSKSTSGGTAALGCLVKDYFPEPVTVSWNSGALTSGVHTFPAVLQSSGLYSLSSVVTVPSSSLGTQTYICNVNHKPSNTKVDKRVEPKSCDKTHTCPPCPAPELLGGPSVFLFPPKPKDTLMISRTPEVTCVVVDVSHEDPEVKFNWYVDGVEVHNAKTKPREEQYNSTYRVVSVLTVLHQDWLNGKEYKCKVSNKALPAPIEKTISKAKGQPREPRVYTLPPSREEMTENQVSLTCLVKGFYPSDIAVEWESNGQPENNYKTTPPVLQSDGSFTLYSYLTVDKSRWQQGNVFSCSVMHEALHNHYTQKSLSLSP

SEQ ID NO: 352 - protein, 447 aa, Homo sapiens
QVQLQESGPGLVRPSQTLSLTCTVSGYSITSDHAWSWVRQPPGRGLEWIGYISYSGITTYNPSLKSRVTMLRDTSKNQFSLRLSSVTAADTAVYYCARSLARTTAMDYWGQGSLVTVSSASTKGPSVFPLAPSSKSTSGGTAALGCLVKDYFPEPVTVSWNSGALTSGVHTFPAVLQSSGLYSLSSVVTVPSSSLGTQTYICNVNHKPSNTKVDKRVEPKSCDKTHTCPPCPAPELLGGPSVFLFPPKPKDTLMISRTPEVTCVVVDVSHEDPEVKFNWYVDGVEVHNAKTKPREEQYNSTYRVVSVLTVLHQDWLNGKEYKCKVSNKALPAPIEKTISKAKGQPREPRVYTLPPSREEMTENQVSLTCLVKGFYPSDIAVEWESNGQPENNYKTTPPVLHSDGSFTLYSYLTVDKSRWQQGNVFSCSVMHEALHNHYTQKSLSLSP

SEQ ID NO: 353 - protein, 447 aa, Homo sapiens
QVQLQESGPGLVRPSQTLSLTCTVSGYSITSDHAWSWVRQPPGRGLEWIGYISYSGITTYNPSLKSRVTMLRDTSKNQFSLRLSSVTAADTAVYYCARSLARTTAMDYWGQGSLVTVSSASTKGPSVFPLAPSSKSTSGGTAALGCLVKDYFPEPVTVSWNSGALTSGVHTFPAVLQSSGLYSLSSVVTVPSSSLGTQTYICNVNHKPSNTKVDKRVEPKSCDKTHTCPPCPAPELLGGPSVFLFPPKPKDTLMISRTPEVTCVVVDVSHEDPEVKFNWYVDGVEVHNAKTKPREEQYNSTYRVVSVLTVLHQDWLNGKEYKCKVSNKALPAPIEKTISKAKGQPREPRVYTLPPSREEMTENQVSLTCLVKGFYPSDIAVEWESNGQPENNYKTTPPVLVSDGSFALYSFLTVDKSRWQQGNVFSCSVMHEALHNHYTQKSLSLSP

SEQ ID NO: 354 - protein, 447 aa, Homo sapiens
QVQLQESGPGLVRPSQTLSLTCTVSGYSITSDHAWSWVRQPPGRGLEWIGYISYSGITTYNPSLKSRVTMLRDTSKNQFSLRLSSVTAADTAVYYCARSLARTTAMDYWGQGSLVTVSSASTKGPSVFPLAPSSKSTSGGTAALGCLVKDYFPEPVTVSWNSGALTSGVHTFPAVLQSSGLYSLSSVVTVPSSSLGTQTYICNVNHKPSNTKVDKRVEPKSCDKTHTCPPCPAPELLGGPSVFLFPPKPKDTLMISRTPEVTCVVVDVSHEDPEVKFNWYVDGVEVHNAKTKPREEQYNSTYRVVSVLTVLHQDWLNGKEYKCKVSNKALPAPIEKTISKAKGQPREPRVYTLPPSREEMTENQVSLTCLVKGFYPSDIAVEWESNGQPENNYKTTPPVLVSDGSFVLYSFLTVDKSRWQQGNVFSCSVMHEALHNHYTQKSLSLSP

SEQ ID NO: 355 - protein, 447 aa, Homo sapiens
QVQLQESGPGLVRPSQTLSLTCTVSGYSITSDHAWSWVRQPPGRGLEWIGYISYSGITTYNPSLKSRVTMLRDTSKNQFSLRLSSVTAADTAVYYCARSLARTTAMDYWGQGSLVTVSSASTKGPSVFPLAPSSKSTSGGTAALGCLVKDYFPEPVTVSWNSGALTSGVHTFPAVLQSSGLYSLSSVVTVPSSSLGTQTYICNVNHKPSNTKVDKRVEPKSCDKTHTCPPCPAPELLGGPSVFLFPPKPKDTLMISRTPEVTCVVVDVSHEDPEVKFNWYVDGVEVHNAKTKPREEQYNSTYRVVSVLTVLHQDWLNGKEYKCKVSNKALPAPIEKTISKAKGQPREPRVYTLPPSREEMTENQVSLTCLVKGFYPSDIAVEWESNGQPENNYKTTPPVLVSDGSFSLYSFLTVDKSRWQQGNVFSCSVMHEALHNHYTQKSLSLSP

SEQ ID NO: 356 - protein, 447 aa, Homo sapiens
QVQLQESGPGLVRPSQTLSLTCTVSGYSITSDHAWSWVRQPPGRGLEWIGYISYSGITTYNPSLKSRVTMLRDTSKNQFSLRLSSVTAADTAVYYCARSLARTTAMDYWGQGSLVTVSSASTKGPSVFPLAPSSKSTSGGTAALGCLVKDYFPEPVTVSWNSGALTSGVHTFPAVLQSSGLYSLSSVVTVPSSSLGTQTYICNVNHKPSNTKVDKRVEPKSCDKTHTCPPCPAPELLGGPSVFLFPPKPKDTLMISRTPEVTCVVVDVSHEDPEVKFNWYVDGVEVHNAKTKPREEQYNSTYRVVSVLTVLHQDWLNGKEYKCKVSNKALPAPIEKTISKAKGQPREPRVYTLPPSREEMTENQVSLTCLVKGFYPSDIAVEWESNGQPENNYKTTPPVLVSDGSFCLYSFLTVDKSRWQQGNVFSCSVMHEALHNHYTQKSLSLSP

SEQ ID NO: 357 - protein, 447 aa, Homo sapiens
QVQLQESGPGLVRPSQTLSLTCTVSGYSITSDHAWSWVRQPPGRGLEWIGYISYSGITTYNPSLKSRVTMLRDTSKNQFSLRLSSVTAADTAVYYCARSLARTTAMDYWGQGSLVTVSSASTKGPSVFPLAPSSKSTSGGTAALGCLVKDYFPEPVTVSWNSGALTSGVHTFPAVLQSSGLYSLSSVVTVPSSSLGTQTYICNVNHKPSNTKVDKRVEPKSCDKTHTCPPCPAPELLGGPSVFLFPPKPKDTLMISRTPEVTCVVVDVSHEDPEVKFNWYVDGVEVHNAKTKPREEQYNSTYRVVSVLTVLHQDWLNGKEYKCKVSNKALPAPIEKTISKAKGQPREPRVYTLPPSREEMTENQVSLTCLVKGFYPSDIAVEWESNGQPENNYKTTPPVLVSDGSFDLYSFLTVDKSRWQQGNVFSCSVMHEALHNHYTQKSLSLSP

SEQ ID NO: 358 - protein, 447 aa, Homo sapiens
QVQLQESGPGLVRPSQTLSLTCTVSGYSITSDHAWSWVRQPPGRGLEWIGYISYSGITTYNPSLKSRVTMLRDTSKNQFSLRLSSVTAADTAVYYCARSLARTTAMDYWGQGSLVTVSSASTKGPSVFPLAPSSKSTSGGTAALGCLVKDYFPEPVTVSWNSGALTSGVHTFPAVLQSSGLYSLSSVVTVPSSSLGTQTYICNVNHKPSNTKVDKRVEPKSCDKTHTCPPCPAPELLGGPSVFLFPPKPKDTLMISRTPEVTCVVVDVSHEDPEVKFNWYVDGVEVHNAKTKPREEQYNSTYRVVSVLTVLHQDWLNGKEYKCKVSNKALPAPIEKTISKAKGQPREPRVYTLPPSREEMTENQVSLTCLVKGFYPSDIAVEWESNGQPENNYKTTPPVLVSDGSFALYSYLTVDKSRWQQGNVFSCSVMHEALHNHYTQKSLSLSP

SEQ ID NO: 359 - protein, 447 aa, Homo sapiens
QVQLQESGPGLVRPSQTLSLTCTVSGYSITSDHAWSWVRQPPGRGLEWIGYISYSGITTYNPSLKSRVTMLRDTSKNQFSLRLSSVTAADTAVYYCARSLARTTAMDYWGQGSLVTVSSASTKGPSVFPLAPSSKSTSGGTAALGCLVKDYFPEPVTVSWNSGALTSGVHTFPAVLQSSGLYSLSSVVTVPSSSLGTQTYICNVNHKPSNTKVDKRVEPKSCDKTHTCPPCPAPELLGGPSVFLFPPKPKDTLMISRTPEVTCVVVDVSHEDPEVKFNWYVDGVEVHNAKTKPREEQYNSTYRVVSVLTVLHQDWLNGKEYKCKVSNKALPAPIEKTISKAKGQPREPRVYTLPPSREEMTENQVSLTCLVKGFYPSDIAVEWESNGQPENNYKTTPPVLVSDGSFCLYSYLTVDKSRWQQGNVFSCSVMHEALHNHYTQKSLSLSP

SEQ ID NO: 360 - protein, 447 aa, Homo sapiens
QVQLQESGPGLVRPSQTLSLTCTVSGYSITSDHAWSWVRQPPGRGLEWIGYISYSGITTYNPSLKSRVTMLRDTSKNQFSLRLSSVTAADTAVYYCARSLARTTAMDYWGQGSLVTVSSASTKGPSVFPLAPSSKSTSGGTAALGCLVKDYFPEPVTVSWNSGALTSGVHTFPAVLQSSGLYSLSSVVTVPSSSLGTQTYICNVNHKPSNTKVDKRVEPKSCDKTHTCPPCPAPELLGGPSVFLFPPKPKDTLMISRTPEVTCVVVDVSHEDPEVKFNWYVDGVEVHNAKTKPREEQYNSTYRVVSVLTVLHQDWLNGKEYKCKVSNKALPAPIEKTISKAKGQPREPRVYTLPPSREEMTENQVSLTCLVKGFYPSDIAVEWESNGQPENNYKTTPPVLVSDGSFNLYSYLTVDKSRWQQGNVFSCSVMHEALHNHYTQKSLSLSP

SEQ ID NO: 361 - protein, 447 aa, Homo sapiens
QVQLQESGPGLVRPSQTLSLTCTVSGYSITSDHAWSWVRQPPGRGLEWIGYISYSGITTYNPSLKSRVTMLRDTSKNQFSLRLSSVTAADTAVYYCARSLARTTAMDYWGQGSLVTVSSASTKGPSVFPLAPSSKSTSGGTAALGCLVKDYFPEPVTVSWNSGALTSGVHTFPAVLQSSGLYSLSSVVTVPSSSLGTQTYICNVNHKPSNTKVDKRVEPKSCDKTHTCPPCPAPELLGGPSVFLFPPKPKDTLMISRTPEVTCVVVDVSHEDPEVKFNWYVDGVEVHNAKTKPREEQYNSTYRVVSVLTVLHQDWLNGKEYKCKVSNKALPAPIEKTISKAKGQPREPRVYTLPPSREEMTENQVSLTCLVKGFYPSDIAVEWESNGQPENNYKTTPPVLVSDGSFDLYSYLTVDKSRWQQGNVFSCSVMHEALHNHYTQKSLSLSP

SEQ ID NO: 362 - protein, 447 aa, Homo sapiens
QVQLQESGPGLVRPSQTLSLTCTVSGYSITSDHAWSWVRQPPGRGLEWIGYISYSGITTYNPSLKSRVTMLRDTSKNQFSLRLSSVTAADTAVYYCARSLARTTAMDYWGQGSLVTVSSASTKGPSVFPLAPSSKSTSGGTAALGCLVKDYFPEPVTVSWNSGALTSGVHTFPAVLQSSGLYSLSSVVTVPSSSLGTQTYICNVNHKPSNTKVDKRVEPKSCDKTHTCPPCPAPELLGGPSVFLFPPKPKDTLMISRTPEVTCVVVDVSHEDPEVKFNWYVDGVEVHNAKTKPREEQYNSTYRVVSVLTVLHQDWLNGKEYKCKVSNKALPAPIEKTISKAKGQPREPRVYTLPPSREEMTENQVSLTCLVKGFYPSDIAVEWESNGQPENNYKTTPPVLLSDGSFALYSWLTVDKSRWQQGNVFSCSVMHEALHNHYTQKSLSLSP

SEQ ID NO: 363 - protein, 447 aa, Homo sapiens
QVQLQESGPGLVRPSQTLSLTCTVSGYSITSDHAWSWVRQPPGRGLEWIGYISYSGITTYNPSLKSRVTMLRDTSKNQFSLRLSSVTAADTAVYYCARSLARTTAMDYWGQGSLVTVSSASTKGPSVFPLAPSSKSTSGGTAALGCLVKDYFPEPVTVSWNSGALTSGVHTFPAVLQSSGLYSLSSVVTVPSSSLGTQTYICNVNHKPSNTKVDKRVEPKSCDKTHTCPPCPAPELLGGPSVFLFPPKPKDTLMISRTPEVTCVVVDVSHEDPEVKFNWYVDGVEVHNAKTKPREEQYNSTYRVVSVLTVLHQDWLNGKEYKCKVSNKALPAPIEKTISKAKGQPREPRVYTLPPSREEMTENQVSLTCLVKGFYPSDIAVEWESNGQPENNYKTTPPVLLSDGSFSLYSWLTVDKSRWQQGNVFSCSVMHEALHNHYTQKSLSLSP

SEQ ID NO: 364 - protein, 447 aa, Homo sapiens
QVQLQESGPGLVRPSQTLSLTCTVSGYSITSDHAWSWVRQPPGRGLEWIGYISYSGITTYNPSLKSRVTMLRDTSKNQFSLRLSSVTAADTAVYYCARSLARTTAMDYWGQGSLVTVSSASTKGPSVFPLAPSSKSTSGGTAALGCLVKDYFPEPVTVSWNSGALTSGVHTFPAVLQSSGLYSLSSVVTVPSSSLGTQTYICNVNHKPSNTKVDKRVEPKSCDKTHTCPPCPAPELLGGPSVFLFPPKPKDTLMISRTPEVTCVVVDVSHEDPEVKFNWYVDGVEVHNAKTKPREEQYNSTYRVVSVLTVLHQDWLNGKEYKCKVSNKALPAPIEKTISKAKGQPREPRVYTLPPSREEMTENQVSLTCLVKGFYPSDIAVEWESNGQPENNYKTTPPVLLSDGSFCLYSWLTVDKSRWQQGNVFSCSVMHEALHNHYTQKSLSLSP

SEQ ID NO: 365 - protein, 447 aa, Homo sapiens
QVQLQESGPGLVRPSQTLSLTCTVSGYSITSDHAWSWVRQPPGRGLEWIGYISYSGITTYNPSLKSRVTMLRDTSKNQFSLRLSSVTAADTAVYYCARSLARTTAMDYWGQGSLVTVSSASTKGPSVFPLAPSSKSTSGGTAALGCLVKDYFPEPVTVSWNSGALTSGVHTFPAVLQSSGLYSLSSVVTVPSSSLGTQTYICNVNHKPSNTKVDKRVEPKSCDKTHTCPPCPAPELLGGPSVFLFPPKPKDTLMISRTPEVTCVVVDVSHEDPEVKFNWYVDGVEVHNAKTKPREEQYNSTYRVVSVLTVLHQDWLNGKEYKCKVSNKALPAPIEKTISKAKGQPREPRVYTLPPSREEMTENQVSLTCLVKGFYPSDIAVEWESNGQPENNYKTTPPVLISDGSFSLYSWLTVDKSRWQQGNVFSCSVMHEALHNHYTQKSLSLSP

SEQ ID NO: 366 - protein, 447 aa, Homo sapiens
QVQLQESGPGLVRPSQTLSLTCTVSGYSITSDHAWSWVRQPPGRGLEWIGYISYSGITTYNPSLKSRVTMLRDTSKNQFSLRLSSVTAADTAVYYCARSLARTTAMDYWGQGSLVTVSSASTKGPSVFPLAPSSKSTSGGTAALGCLVKDYFPEPVTVSWNSGALTSGVHTFPAVLQSSGLYSLSSVVTVPSSSLGTQTYICNVNHKPSNTKVDKRVEPKSCDKTHTCPPCPAPELLGGPSVFLFPPKPKDTLMISRTPEVTCVVVDVSHEDPEVKFNWYVDGVEVHNAKTKPREEQYNSTYRVVSVLTVLHQDWLNGKEYKCKVSNKALPAPIEKTISKAKGQPREPRVYTLPPSREEMTENQVSLTCLVKGFYPSDIAVEWESNGQPENNYKTTPPVLISDGSFCLYSWLTVDKSRWQQGNVFSCSVMHEALHNHYTQKSLSLSP

SEQ ID NO: 367 - protein, 447 aa, Homo sapiens
QVQLQESGPGLVRPSQTLSLTCTVSGYSITSDHAWSWVRQPPGRGLEWIGYISYSGITTYNPSLKSRVTMLRDTSKNQFSLRLSSVTAADTAVYYCARSLARTTAMDYWGQGSLVTVSSASTKGPSVFPLAPSSKSTSGGTAALGCLVKDYFPEPVTVSWNSGALTSGVHTFPAVLQSSGLYSLSSVVTVPSSSLGTQTYICNVNHKPSNTKVDKRVEPKSCDKTHTCPPCPAPELLGGPSVFLFPPKPKDTLMISRTPEVTCVVVDVSHEDPEVKFNWYVDGVEVHNAKTKPREEQYNSTYRVVSVLTVLHQDWLNGKEYKCKVSNKALPAPIEKTISKAKGQPREPRVYTLPPSREEMTENQVSLTCLVKGFYPSDIAVEWESNGQPENNYKTTPPVLMSDGSFALYSWLTVDKSRWQQGNVFSCSVMHEALHNHYTQKSLSLSP

SEQ ID NO: 368 - protein, 447 aa, Homo sapiens
QVQLQESGPGLVRPSQTLSLTCTVSGYSITSDHAWSWVRQPPGRGLEWIGYISYSGITTYNPSLKSRVTMLRDTSKNQFSLRLSSVTAADTAVYYCARSLARTTAMDYWGQGSLVTVSSASTKGPSVFPLAPSSKSTSGGTAALGCLVKDYFPEPVTVSWNSGALTSGVHTFPAVLQSSGLYSLSSVVTVPSSSLGTQTYICNVNHKPSNTKVDKRVEPKSCDKTHTCPPCPAPELLGGPSVFLFPPKPKDTLMISRTPEVTCVVVDVSHEDPEVKFNWYVDGVEVHNAKTKPREEQYNSTYRVVSVLTVLHQDWLNGKEYKCKVSNKALPAPIEKTISKAKGQPREPRVYTLPPSREEMTENQVSLTCLVKGFYPSDIAVEWESNGQPENNYKTTPPVLMSDGSFSLYSWLTVDKSRWQQGNVFSCSVMHEALHNHYTQKSLSLSP

SEQ ID NO: 369 - protein, 447 aa, Homo sapiens
QVQLQESGPGLVRPSQTLSLTCTVSGYSITSDHAWSWVRQPPGRGLEWIGYISYSGITTYNPSLKSRVTMLRDTSKNQFSLRLSSVTAADTAVYYCARSLARTTAMDYWGQGSLVTVSSASTKGPSVFPLAPSSKSTSGGTAALGCLVKDYFPEPVTVSWNSGALTSGVHTFPAVLQSSGLYSLSSVVTVPSSSLGTQTYICNVNHKPSNTKVDKRVEPKSCDKTHTCPPCPAPELLGGPSVFLFPPKPKDTLMISRTPEVTCVVVDVSHEDPEVKFNWYVDGVEVHNAKTKPREEQYNSTYRVVSVLTVLHQDWLNGKEYKCKVSNKALPAPIEKTISKAKGQPREPRVYTLPPSREEMTENQVSLTCLVKGFYPSDIAVEWESNGQPENNYKTTPPVLMSDGSFCLYSWLTVDKSRWQQGNVFSCSVMHEALHNHYTQKSLSLSP

SEQ ID NO: 370 - protein, 447 aa, Homo sapiens
QVQLQESGPGLVRPSQTLSLTCTVSGYSITSDHAWSWVRQPPGRGLEWIGYISYSGITTYNPSLKSRVTMLRDTSKNQFSLRLSSVTAADTAVYYCARSLARTTAMDYWGQGSLVTVSSASTKGPSVFPLAPSSKSTSGGTAALGCLVKDYFPEPVTVSWNSGALTSGVHTFPAVLQSSGLYSLSSVVTVPSSSLGTQTYICNVNHKPSNTKVDKRVEPKSCDKTHTCPPCPAPELLGGPSVFLFPPKPKDTLMISRTPEVTCVVVDVSHEDPEVKFNWYVDGVEVHNAKTKPREEQYNSTYRVVSVLTVLHQDWLNGKEYKCKVSNKALPAPIEKTISKAKGQPREPRVYTLPPSREEMTENQVSLTCLVKGFYPSDIAVEWESNGQPENNYKTTPPVLGSDGSFTLYSWLTVDKSRWQQGNVFSCSVMHEALHNHYTQKSLSLSP

SEQ ID NO: 371 - protein, 447 aa, Homo sapiens
QVQLQESGPGLVRPSQTLSLTCTVSGYSITSDHAWSWVRQPPGRGLEWIGYISYSGITTYNPSLKSRVTMLRDTSKNQFSLRLSSVTAADTAVYYCARSLARTTAMDYWGQGSLVTVSSASTKGPSVFPLAPSSKSTSGGTAALGCLVKDYFPEPVTVSWNSGALTSGVHTFPAVLQSSGLYSLSSVVTVPSSSLGTQTYICNVNHKPSNTKVDKRVEPKSCDKTHTCPPCPAPELLGGPSVFLFPPKPKDTLMISRTPEVTCVVVDVSHEDPEVKFNWYVDGVEVHNAKTKPREEQYNSTYRVVSVLTVLHQDWLNGKEYKCKVSNKALPAPIEKTISKAKGQPREPHVYTLPPSREEMTENQVSLTCLVKGFYPSDIAVEWESNGQPENNYKTTPPVLVSDGSFTLYSWLTVDKSRWQQGNVFSCSVMHEALHNHYTQKSLSLSP

SEQ ID NO: 372 - protein, 447 aa, Homo sapiens
QVQLQESGPGLVRPSQTLSLTCTVSGYSITSDHAWSWVRQPPGRGLEWIGYISYSGITTYNPSLKSRVTMLRDTSKNQFSLRLSSVTAADTAVYYCARSLARTTAMDYWGQGSLVTVSSASTKGPSVFPLAPSSKSTSGGTAALGCLVKDYFPEPVTVSWNSGALTSGVHTFPAVLQSSGLYSLSSVVTVPSSSLGTQTYICNVNHKPSNTKVDKRVEPKSCDKTHTCPPCPAPELLGGPSVFLFPPKPKDTLMISRTPEVTCVVVDVSHEDPEVKFNWYVDGVEVHNAKTKPREEQYNSTYRVVSVLTVLHQDWLNGKEYKCKVSNKALPAPIEKTISKAKGQPREPRVYTLPPSREEMTENQVSLTCLVKGFYPSDIAVEWESNGQPENNYKTTPPVLASDGSFTLYSWLTVDKSRWQQGNVFSCSVMHEALHNHYTQKSLSLSP

SEQ ID NO: 373 - protein, 447 aa, Homo sapiens
QVQLQESGPGLVRPSQTLSLTCTVSGYSITSDHAWSWVRQPPGRGLEWIGYISYSGITTYNPSLKSRVTMLRDTSKNQFSLRLSSVTAADTAVYYCARSLARTTAMDYWGQGSLVTVSSASTKGPSVFPLAPSSKSTSGGTAALGCLVKDYFPEPVTVSWNSGALTSGVHTFPAVLQSSGLYSLSSVVTVPSSSLGTQTYICNVNHKPSNTKVDKRVEPKSCDKTHTCPPCPAPELLGGPSVFLFPPKPKDTLMISRTPEVTCVVVDVSHEDPEVKFNWYVDGVEVHNAKTKPREEQYNSTYRVVSVLTVLHQDWLNGKEYKCKVSNKALPAPIEKTISKAKGQPREPRVYTLPPSREEMTENQVSLTCLVKGFYPSDIAVEWESNGQPENNYKTTPPVLNSDGSFTLYSWLTVDKSRWQQGNVFSCSVMHEALHNHYTQKSLSLSP

SEQ ID NO: 374 - protein, 447 aa, Homo sapiens
QVQLQESGPGLVRPSQTLSLTCTVSGYSITSDHAWSWVRQPPGRGLEWIGYISYSGITTYNPSLKSRVTMLRDTSKNQFSLRLSSVTAADTAVYYCARSLARTTAMDYWGQGSLVTVSSASTKGPSVFPLAPSSKSTSGGTAALGCLVKDYFPEPVTVSWNSGALTSGVHTFPAVLQSSGLYSLSSVVTVPSSSLGTQTYICNVNHKPSNTKVDKRVEPKSCDKTHTCPPCPAPELLGGPSVFLFPPKPKDTLMISRTPEVTCVVVDVSHEDPEVKFNWYVDGVEVHNAKTKPREEQYNSTYRVVSVLTVLHQDWLNGKEYKCKVSNKALPAPIEKTISKAKGQPREPRVYTLPPSREEMTENQVSLTCLVKGFYPSDIAVEWESNGQPENNYKTTPPVLQSDGSFTLYSWLTVDKSRWQQGNVFSCSVMHEALHNHYTQKSLSLSP

SEQ ID NO: 375 - protein, 447 aa, Homo sapiens
QVQLQESGPGLVRPSQTLSLTCTVSGYSITSDHAWSWVRQPPGRGLEWIGYISYSGITTYNPSLKSRVTMLRDTSKNQFSLRLSSVTAADTAVYYCARSLARTTAMDYWGQGSLVTVSSASTKGPSVFPLAPSSKSTSGGTAALGCLVKDYFPEPVTVSWNSGALTSGVHTFPAVLQSSGLYSLSSVVTVPSSSLGTQTYICNVNHKPSNTKVDKRVEPKSCDKTHTCPPCPAPELLGGPSVFLFPPKPKDTLMISRTPEVTCVVVDVSHEDPEVKFNWYVDGVEVHNAKTKPREEQYNSTYRVVSVLTVLHQDWLNGKEYKCKVSNKALPAPIEKTISKAKGQPREPRVYTLPPSREEMTENQVSLTCLVKGFYPSDIAVEWESNGQPENNYKTTPPVLSSDGSFTLYSFLTVDKSRWQQGNVFSCSVMHEALHNHYTQKSLSLSP

SEQ ID NO: 376 - protein, 447 aa, Homo sapiens
QVQLQESGPGLVRPSQTLSLTCTVSGYSITSDHAWSWVRQPPGRGLEWIGYISYSGITTYNPSLKSRVTMLRDTSKNQFSLRLSSVTAADTAVYYCARSLARTTAMDYWGQGSLVTVSSASTKGPSVFPLAPSSKSTSGGTAALGCLVKDYFPEPVTVSWNSGALTSGVHTFPAVLQSSGLYSLSSVVTVPSSSLGTQTYICNVNHKPSNTKVDKRVEPKSCDKTHTCPPCPAPELLGGPSVFLFPPKPKDTLMISRTPEVTCVVVDVSHEDPEVKFNWYVDGVEVHNAKTKPREEQYNSTYRVVSVLTVLHQDWLNGKEYKCKVSNKALPAPIEKTISKAKGQPREPRVYTLPPSREEMTENQVSLTCLVKGFYPSDIAVEWESNGQPENNYKTTPPVLVSDGSFNLYSFLTVDKSRWQQGNVFSCSVMHEALHNHYTQKSLSLSP

SEQ ID NO: 377 - protein, 447 aa, Homo sapiens
QVQLQESGPGLVRPSQTLSLTCTVSGYSITSDHAWSWVRQPPGRGLEWIGYISYSGITTYNPSLKSRVTMLRDTSKNQFSLRLSSVTAADTAVYYCARSLARTTAMDYWGQGSLVTVSSASTKGPSVFPLAPSSKSTSGGTAALGCLVKDYFPEPVTVSWNSGALTSGVHTFPAVLQSSGLYSLSSVVTVPSSSLGTQTYICNVNHKPSNTKVDKRVEPKSCDKTHTCPPCPAPELLGGPSVFLFPPKPKDTLMISRTPEVTCVVVDVSHEDPEVKFNWYVDGVEVHNAKTKPREEQYNSTYRVVSVLTVLHQDWLNGKEYKCKVSNKALPAPIEKTISKAKGQPREPRVYTLPPSREEMTENQVSLTCLVKGFYPSDIAVEWESNGQPENNYKTTPPVLVSDGSFVLYSYLTVDKSRWQQGNVFSCSVMHEALHNHYTQKSLSLSP

SEQ ID NO: 378 - protein, 447 aa, Homo sapiens
QVQLQESGPGLVRPSQTLSLTCTVSGYSITSDHAWSWVRQPPGRGLEWIGYISYSGITTYNPSLKSRVTMLRDTSKNQFSLRLSSVTAADTAVYYCARSLARTTAMDYWGQGSLVTVSSASTKGPSVFPLAPSSKSTSGGTAALGCLVKDYFPEPVTVSWNSGALTSGVHTFPAVLQSSGLYSLSSVVTVPSSSLGTQTYICNVNHKPSNTKVDKRVEPKSCDKTHTCPPCPAPELLGGPSVFLFPPKPKDTLMISRTPEVTCVVVDVSHEDPEVKFNWYVDGVEVHNAKTKPREEQYNSTYRVVSVLTVLHQDWLNGKEYKCKVSNKALPAPIEKTISKAKGQPREPRVYTLPPSREEMTENQVSLTCLVKGFYPSDIAVEWESNGQPENNYKTTPPVLVSDGSFSLYSYLTVDKSRWQQGNVFSCSVMHEALHNHYTQKSLSLSP

SEQ ID NO: 379 - protein, 447 aa, Homo sapiens
QVQLQESGPGLVRPSQTLSLTCTVSGYSITSDHAWSWVRQPPGRGLEWIGYISYSGITTYNPSLKSRVTMLRDTSKNQFSLRLSSVTAADTAVYYCARSLARTTAMDYWGQGSLVTVSSASTKGPSVFPLAPSSKSTSGGTAALGCLVKDYFPEPVTVSWNSGALTSGVHTFPAVLQSSGLYSLSSVVTVPSSSLGTQTYICNVNHKPSNTKVDKRVEPKSCDKTHTCPPCPAPELLGGPSVFLFPPKPKDTLMISRTPEVTCVVVDVSHEDPEVKFNWYVDGVEVHNAKTKPREEQYNSTYRVVSVLTVLHQDWLNGKEYKCKVSNKALPAPIEKTISKAKGQPREPRVYTLPPSREEMTENQVSLTCLVKGFYPSDIAVEWESNGQPENNYKTTPPVLISDGSFALYSWLTVDKSRWQQGNVFSCSVMHEALHNHYTQKSLSLSP

SEQ ID NO: 380 - protein, 447 aa, Homo sapiens
QVQLQESGPGLVRPSQTLSLTCTVSGYSITSDHAWSWVRQPPGRGLEWIGYISYSGITTYNPSLKSRVTMLRDTSKNQFSLRLSSVTAADTAVYYCARSLARTTAMDYWGQGSLVTVSSASTKGPSVFPLAPSSKSTSGGTAALGCLVKDYFPEPVTVSWNSGALTSGVHTFPAVLQSSGLYSLSSVVTVPSSSLGTQTYICNVNHKPSNTKVDKRVEPKSCDKTHTCPPCPAPELLGGPSVFLFPPKPKDTLMISRTPEVTCVVVDVSHEDPEVKFNWYVDGVEVHNAKTKPREEQYNSTYRVVSVLTVLHQDWLNGKEYKCKVSNKALPAPIEKTISKAKGQPREPRVYTLPPSREEMTENQVSLTCLVKGFYPSDIAVEWESNGQPENNYKTTPPVLVSDGSFGLYSWLTVDKSRWQQGNVFSCSVMHEALHNHYTQKSLSLSP

SEQ ID NO: 381 - protein, 447 aa, Homo sapiens
QVQLQESGPGLVRPSQTLSLTCTVSGYSITSDHAWSWVRQPPGRGLEWIGYISYSGITTYNPSLKSRVTMLRDTSKNQFSLRLSSVTAADTAVYYCARSLARTTAMDYWGQGSLVTVSSASTKGPSVFPLAPSSKSTSGGTAALGCLVKDYFPEPVTVSWNSGALTSGVHTFPAVLQSSGLYSLSSVVTVPSSSLGTQTYICNVNHKPSNTKVDKRVEPKSCDKTHTCPPCPAPELLGGPSVFLFPPKPKDTLMISRTPEVTCVVVDVSHEDPEVKFNWYVDGVEVHNAKTKPREEQYNSTYRVVSVLTVLHQDWLNGKEYKCKVSNKALPAPIEKTISKAKGQPREPQVYTLPPSREEMTKNQVSLTCLVKGFYPSDIAVEWESNGQPENNYKTWPPVLDSDGSFSLYSKLTVDKSRWQQGNVFSCSVMHEALHNHYTQKSLSLSP

SEQ ID NO: 382 - protein, 447 aa, Homo sapiens
QVQLQESGPGLVRPSQTLSLTCTVSGYSITSDHAWSWVRQPPGRGLEWIGYISYSGITTYNPSLKSRVTMLRDTSKNQFSLRLSSVTAADTAVYYCARSLARTTAMDYWGQGSLVTVSSASTKGPSVFPLAPSSKSTSGGTAALGCLVKDYFPEPVTVSWNSGALTSGVHTFPAVLQSSGLYSLSSVVTVPSSSLGTQTYICNVNHKPSNTKVDKRVEPKSCDKTHTCPPCPAPELLGGPSVFLFPPKPKDTLMISRTPEVTCVVVDVSHEDPEVKFNWYVDGVEVHNAKTKPREEQYNSTYRVVSVLTVLHQDWLNGKEYKCKVSNKALPAPIEKTISKAKGQPREPQVYTLPPSREEMTKNQVSLTCLVKGFYPSDIAVEWESNGQPENNYKTWPPVLDSDGSFTLYSKLTVDKSRWQQGNVFSCSVMHEALHNHYTQKSLSLSP

SEQ ID NO: 383 - protein, 447 aa, Homo sapiens
QVQLQESGPGLVRPSQTLSLTCTVSGYSITSDHAWSWVRQPPGRGLEWIGYISYSGITTYNPSLKSRVTMLRDTSKNQFSLRLSSVTAADTAVYYCARSLARTTAMDYWGQGSLVTVSSASTKGPSVFPLAPSSKSTSGGTAALGCLVKDYFPEPVTVSWNSGALTSGVHTFPAVLQSSGLYSLSSVVTVPSSSLGTQTYICNVNHKPSNTKVDKRVEPKSCDKTHTCPPCPAPELLGGPSVFLFPPKPKDTLMISRTPEVTCVVVDVSHEDPEVKFNWYVDGVEVHNAKTKPREEQYNSTYRVVSVLTVLHQDWLNGKEYKCKVSNKALPAPIEKTISKAKGQPREPQVYTLPPSREEMTKNQVSLTCLVKGFYPSDIAVEWESNGQPENNYKTYPPVLDSDGSFALYSKLTVDKSRWQQGNVFSCSVMHEALHNHYTQKSLSLSP

SEQ ID NO: 384 - protein, 447 aa, Homo sapiens
QVQLQESGPGLVRPSQTLSLTCTVSGYSITSDHAWSWVRQPPGRGLEWIGYISYSGITTYNPSLKSRVTMLRDTSKNQFSLRLSSVTAADTAVYYCARSLARTTAMDYWGQGSLVTVSSASTKGPSVFPLAPSSKSTSGGTAALGCLVKDYFPEPVTVSWNSGALTSGVHTFPAVLQSSGLYSLSSVVTVPSSSLGTQTYICNVNHKPSNTKVDKRVEPKSCDKTHTCPPCPAPELLGGPSVFLFPPKPKDTLMISRTPEVTCVVVDVSHEDPEVKFNWYVDGVEVHNAKTKPREEQYNSTYRVVSVLTVLHQDWLNGKEYKCKVSNKALPAPIEKTISKAKGQPREPQVYTLPPSREEMTKNQVSLTCLVKGFYPSDIAVEWESNGQPENNYKTHPPVLDSDGSFALYSKLTVDKSRWQQGNVFSCSVMHEALHNHYTQKSLSLSP

SEQ ID NO: 385 - protein, 447 aa, Homo sapiens
QVQLQESGPGLVRPSQTLSLTCTVSGYSITSDHAWSWVRQPPGRGLEWIGYISYSGITTYNPSLKSRVTMLRDTSKNQFSLRLSSVTAADTAVYYCARSLARTTAMDYWGQGSLVTVSSASTKGPSVFPLAPSSKSTSGGTAALGCLVKDYFPEPVTVSWNSGALTSGVHTFPAVLQSSGLYSLSSVVTVPSSSLGTQTYICNVNHKPSNTKVDKRVEPKSCDKTHTCPPCPAPELLGGPSVFLFPPKPKDTLMISRTPEVTCVVVDVSHEDPEVKFNWYVDGVEVHNAKTKPREEQYNSTYRVVSVLTVLHQDWLNGKEYKCKVSNKALPAPIEKTISKAKGQPREPQVYTLPPSREEMTKNQVSLTCLVKGFYPSDIAVEWESNGQPENNYKTYPPVLDSDGSFTLYSKLTVDKSRWQQGNVFSCSVMHEALHNHYTQKSLSLSP

SEQ ID NO: 386 - protein, 447 aa, Homo sapiens
QVQLQESGPGLVRPSQTLSLTCTVSGYSITSDHAWSWVRQPPGRGLEWIGYISYSGITTYNPSLKSRVTMLRDTSKNQFSLRLSSVTAADTAVYYCARSLARTTAMDYWGQGSLVTVSSASTKGPSVFPLAPSSKSTSGGTAALGCLVKDYFPEPVTVSWNSGALTSGVHTFPAVLQSSGLYSLSSVVTVPSSSLGTQTYICNVNHKPSNTKVDKRVEPKSCDKTHTCPPCPAPELLGGPSVFLFPPKPKDTLMISRTPEVTCVVVDVSHEDPEVKFNWYVDGVEVHNAKTKPREEQYNSTYRVVSVLTVLHQDWLNGKEYKCKVSNKALPAPIEKTISKAKGQPREPQVYTLPPSREEMTKNQVSLTCLVKGFYPSDIAVEWESNGQPENNYKTYPPVLDSDGSFCLYSKLTVDKSRWQQGNVFSCSVMHEALHNHYTQKSLSLSP

SEQ ID NO: 387 - protein, 447 aa, Homo sapiens
QVQLQESGPGLVRPSQTLSLTCTVSGYSITSDHAWSWVRQPPGRGLEWIGYISYSGITTYNPSLKSRVTMLRDTSKNQFSLRLSSVTAADTAVYYCARSLARTTAMDYWGQGSLVTVSSASTKGPSVFPLAPSSKSTSGGTAALGCLVKDYFPEPVTVSWNSGALTSGVHTFPAVLQSSGLYSLSSVVTVPSSSLGTQTYICNVNHKPSNTKVDKRVEPKSCDKTHTCPPCPAPELLGGPSVFLFPPKPKDTLMISRTPEVTCVVVDVSHEDPEVKFNWYVDGVEVHNAKTKPREEQYNSTYRVVSVLTVLHQDWLNGKEYKCKVSNKALPAPIEKTISKAKGQPREPQVYTLPPSREEMTKNQVSLTCLVKGFYPSDIAVEWESNGQPENNYKTYPPVLDSDGSFVLYSKLTVDKSRWQQGNVFSCSVMHEALHNHYTQKSLSLSP

SEQ ID NO: 388 - protein, 447 aa, Homo sapiens
QVQLQESGPGLVRPSQTLSLTCTVSGYSITSDHAWSWVRQPPGRGLEWIGYISYSGITTYNPSLKSRVTMLRDTSKNQFSLRLSSVTAADTAVYYCARSLARTTAMDYWGQGSLVTVSSASTKGPSVFPLAPSSKSTSGGTAALGCLVKDYFPEPVTVSWNSGALTSGVHTFPAVLQSSGLYSLSSVVTVPSSSLGTQTYICNVNHKPSNTKVDKRVEPKSCDKTHTCPPCPAPELLGGPSVFLFPPKPKDTLMISRTPEVTCVVVDVSHEDPEVKFNWYVDGVEVHNAKTKPREEQYNSTYRVVSVLTVLHQDWLNGKEYKCKVSNKALPAPIEKTISKAKGQPREPQVYTLPPSREEMTKNQVSLTCLVKGFYPSDIAVEWESNGQPENNYKTFPPVLDSDGSFGLYSKLTVDKSRWQQGNVFSCSVMHEALHNHYTQKSLSLSP

SEQ ID NO: 389 - protein, 447 aa, Homo sapiens
QVQLQESGPGLVRPSQTLSLTCTVSGYSITSDHAWSWVRQPPGRGLEWIGYISYSGITTYNPSLKSRVTMLRDTSKNQFSLRLSSVTAADTAVYYCARSLARTTAMDYWGQGSLVTVSSASTKGPSVFPLAPSSKSTSGGTAALGCLVKDYFPEPVTVSWNSGALTSGVHTFPAVLQSSGLYSLSSVVTVPSSSLGTQTYICNVNHKPSNTKVDKRVEPKSCDKTHTCPPCPAPELLGGPSVFLFPPKPKDTLMISRTPEVTCVVVDVSHEDPEVKFNWYVDGVEVHNAKTKPREEQYNSTYRVVSVLTVLHQDWLNGKEYKCKVSNKALPAPIEKTISKAKGQPREPQVYTLPPSREEMTKNQVSLTCLVKGFYPSDIAVEWESNGQPENNYKTFPPVLDSDGSFCLYSKLTVDKSRWQQGNVFSCSVMHEALHNHYTQKSLSLSP

SEQ ID NO: 390 - protein, 447 aa, Homo sapiens
QVQLQESGPGLVRPSQTLSLTCTVSGYSITSDHAWSWVRQPPGRGLEWIGYISYSGITTYNPSLKSRVTMLRDTSKNQFSLRLSSVTAADTAVYYCARSLARTTAMDYWGQGSLVTVSSASTKGPSVFPLAPSSKSTSGGTAALGCLVKDYFPEPVTVSWNSGALTSGVHTFPAVLQSSGLYSLSSVVTVPSSSLGTQTYICNVNHKPSNTKVDKRVEPKSCDKTHTCPPCPAPELLGGPSVFLFPPKPKDTLMISRTPEVTCVVVDVSHEDPEVKFNWYVDGVEVHNAKTKPREEQYNSTYRVVSVLTVLHQDWLNGKEYKCKVSNKALPAPIEKTISKAKGQPREPQVYTLPPSREEMTKNQVSLTCLVKGFYPSDIAVEWESNGQPENNYKTFPPVLDSDGSFVLYSKLTVDKSRWQQGNVFSCSVMHEALHNHYTQKSLSLSP

SEQ ID NO: 391 - protein, 447 aa, Homo sapiens
QVQLQESGPGLVRPSQTLSLTCTVSGYSITSDHAWSWVRQPPGRGLEWIGYISYSGITTYNPSLKSRVTMLRDTSKNQFSLRLSSVTAADTAVYYCARSLARTTAMDYWGQGSLVTVSSASTKGPSVFPLAPSSKSTSGGTAALGCLVKDYFPEPVTVSWNSGALTSGVHTFPAVLQSSGLYSLSSVVTVPSSSLGTQTYICNVNHKPSNTKVDKRVEPKSCDKTHTCPPCPAPELLGGPSVFLFPPKPKDTLMISRTPEVTCVVVDVSHEDPEVKFNWYVDGVEVHNAKTKPREEQYNSTYRVVSVLTVLHQDWLNGKEYKCKVSNKALPAPIEKTISKAKGQPREPQVYTLPPSREEMTKNQVSLTCLVKGFYPSDIAVEWESNGQPENNYKTHPPVLDSDGSFGLYSKLTVDKSRWQQGNVFSCSVMHEALHNHYTQKSLSLSP

SEQ ID NO: 392 - protein, 447 aa, Homo sapiens
QVQLQESGPGLVRPSQTLSLTCTVSGYSITSDHAWSWVRQPPGRGLEWIGYISYSGITTYNPSLKSRVTMLRDTSKNQFSLRLSSVTAADTAVYYCARSLARTTAMDYWGQGSLVTVSSASTKGPSVFPLAPSSKSTSGGTAALGCLVKDYFPEPVTVSWNSGALTSGVHTFPAVLQSSGLYSLSSVVTVPSSSLGTQTYICNVNHKPSNTKVDKRVEPKSCDKTHTCPPCPAPELLGGPSVFLFPPKPKDTLMISRTPEVTCVVVDVSHEDPEVKFNWYVDGVEVHNAKTKPREEQYNSTYRVVSVLTVLHQDWLNGKEYKCKVSNKALPAPIEKTISKAKGQPREPQVYTLPPSREEMTKNQVSLTCLVKGFYPSDIAVEWESNGQPENNYKTHPPVLDSDGSFSLYSKLTVDKSRWQQGNVFSCSVMHEALHNHYTQKSLSLSP

SEQ ID NO: 393 - protein, 447 aa, Homo sapiens
QVQLQESGPGLVRPSQTLSLTCTVSGYSITSDHAWSWVRQPPGRGLEWIGYISYSGITTYNPSLKSRVTMLRDTSKNQFSLRLSSVTAADTAVYYCARSLARTTAMDYWGQGSLVTVSSASTKGPSVFPLAPSSKSTSGGTAALGCLVKDYFPEPVTVSWNSGALTSGVHTFPAVLQSSGLYSLSSVVTVPSSSLGTQTYICNVNHKPSNTKVDKRVEPKSCDKTHTCPPCPAPELLGGPSVFLFPPKPKDTLMISRTPEVTCVVVDVSHEDPEVKFNWYVDGVEVHNAKTKPREEQYNSTYRVVSVLTVLHQDWLNGKEYKCKVSNKALPAPIEKTISKAKGQPREPQVYTLPPSREEMTKNQVSLTCLVKGFYPSDIAVEWESNGQPENNYKTHPPVLDSDGSFTLYSKLTVDKSRWQQGNVFSCSVMHEALHNHYTQKSLSLSP

SEQ ID NO: 394 - protein, 447 aa, Homo sapiens
QVQLQESGPGLVRPSQTLSLTCTVSGYSITSDHAWSWVRQPPGRGLEWIGYISYSGITTYNPSLKSRVTMLRDTSKNQFSLRLSSVTAADTAVYYCARSLARTTAMDYWGQGSLVTVSSASTKGPSVFPLAPSSKSTSGGTAALGCLVKDYFPEPVTVSWNSGALTSGVHTFPAVLQSSGLYSLSSVVTVPSSSLGTQTYICNVNHKPSNTKVDKRVEPKSCDKTHTCPPCPAPELLGGPSVFLFPPKPKDTLMISRTPEVTCVVVDVSHEDPEVKFNWYVDGVEVHNAKTKPREEQYNSTYRVVSVLTVLHQDWLNGKEYKCKVSNKALPAPIEKTISKAKGQPREPQVYTLPPSREEMTKNQVSLTCLVKGFYPSDIAVEWESNGQPENNYKTHPPVLDSDGSFCLYSKLTVDKSRWQQGNVFSCSVMHEALHNHYTQKSLSLSP

SEQ ID NO: 395 - protein, 447 aa, Homo sapiens
QVQLQESGPGLVRPSQTLSLTCTVSGYSITSDHAWSWVRQPPGRGLEWIGYISYSGITTYNPSLKSRVTMLRDTSKNQFSLRLSSVTAADTAVYYCARSLARTTAMDYWGQGSLVTVSSASTKGPSVFPLAPSSKSTSGGTAALGCLVKDYFPEPVTVSWNSGALTSGVHTFPAVLQSSGLYSLSSVVTVPSSSLGTQTYICNVNHKPSNTKVDKRVEPKSCDKTHTCPPCPAPELLGGPSVFLFPPKPKDTLMISRTPEVTCVVVDVSHEDPEVKFNWYVDGVEVHNAKTKPREEQYNSTYRVVSVLTVLHQDWLNGKEYKCKVSNKALPAPIEKTISKAKGQPREPQVYTLPPSREEMTKNQVSLTCLVKGFYPSDIAVEWESNGQPENNYKTCPPVLDSDGSFCLYSKLTVDKSRWQQGNVFSCSVMHEALHNHYTQKSLSLSP

SEQ ID NO: 396 - protein, 447 aa, Homo sapiens
QVQLQESGPGLVRPSQTLSLTCTVSGYSITSDHAWSWVRQPPGRGLEWIGYISYSGITTYNPSLKSRVTMLRDTSKNQFSLRLSSVTAADTAVYYCARSLARTTAMDYWGQGSLVTVSSASTKGPSVFPLAPSSKSTSGGTAALGCLVKDYFPEPVTVSWNSGALTSGVHTFPAVLQSSGLYSLSSVVTVPSSSLGTQTYICNVNHKPSNTKVDKRVEPKSCDKTHTCPPCPAPELLGGPSVFLFPPKPKDTLMISRTPEVTCVVVDVSHEDPEVKFNWYVDGVEVHNAKTKPREEQYNSTYRVVSVLTVLHQDWLNGKEYKCKVSNKALPAPIEKTISKAKGQPREPQVYTLPPSREEMTKNQVSLTCLVKGFYPSDIAVEWESNGQPENNYKTWPPVLDSDGSFCLYSKLTVDKSRWQQGNVFSCSVMHEALHNHYTQKSLSLSP

SEQ ID NO: 397 - protein, 447 aa, Homo sapiens
QVQLQESGPGLVRPSQTLSLTCTVSGYSITSDHAWSWVRQPPGRGLEWIGYISYSGITTYNPSLKSRVTMLRDTSKNQFSLRLSSVTAADTAVYYCARSLARTTAMDYWGQGSLVTVSSASTKGPSVFPLAPSSKSTSGGTAALGCLVKDYFPEPVTVSWNSGALTSGVHTFPAVLQSSGLYSLSSVVTVPSSSLGTQTYICNVNHKPSNTKVDKRVEPKSCDKTHTCPPCPAPELLGGPSVFLFPPKPKDTLMISRTPEVTCVVVDVSHEDPEVKFNWYVDGVEVHNAKTKPREEQYNSTYRVVSVLTVLHQDWLNGKEYKCKVSNKALPAPIEKTISKAKGQPREPQVYTLPPSREEMTKNQVSLTCLVKGFYPSDIAVEWESNGQPENNYKTWPPVLDSDGSFVLYSKLTVDKSRWQQGNVFSCSVMHEALHNHYTQKSLSLSP

SEQ ID NO: 398 - protein, 447 aa, Homo sapiens
QVQLQESGPGLVRPSQTLSLTCTVSGYSITSDHAWSWVRQPPGRGLEWIGYISYSGITTYNPSLKSRVTMLRDTSKNQFSLRLSSVTAADTAVYYCARSLARTTAMDYWGQGSLVTVSSASTKGPSVFPLAPSSKSTSGGTAALGCLVKDYFPEPVTVSWNSGALTSGVHTFPAVLQSSGLYSLSSVVTVPSSSLGTQTYICNVNHKPSNTKVDKRVEPKSCDKTHTCPPCPAPELLGGPSVFLFPPKPKDTLMISRTPEVTCVVVDVSHEDPEVKFNWYVDGVEVHNAKTKPREEQYNSTYRVVSVLTVLHQDWLNGKEYKCKVSNKALPAPIEKTISKAKGQPREPQVYTLPPSREEMTKNQVSLTCLVKGFYPSDIAVEWESNGQPENNYKTYPPVLDSDGSFGLYSKLTVDKSRWQQGNVFSCSVMHEALHNHYTQKSLSLSP

SEQ ID NO: 399 - protein, 447 aa, Homo sapiens
QVQLQESGPGLVRPSQTLSLTCTVSGYSITSDHAWSWVRQPPGRGLEWIGYISYSGITTYNPSLKSRVTMLRDTSKNQFSLRLSSVTAADTAVYYCARSLARTTAMDYWGQGSLVTVSSASTKGPSVFPLAPSSKSTSGGTAALGCLVKDYFPEPVTVSWNSGALTSGVHTFPAVLQSSGLYSLSSVVTVPSSSLGTQTYICNVNHKPSNTKVDKRVEPKSCDKTHTCPPCPAPELLGGPSVFLFPPKPKDTLMISRTPEVTCVVVDVSHEDPEVKFNWYVDGVEVHNAKTKPREEQYNSTYRVVSVLTVLHQDWLNGKEYKCKVSNKALPAPIEKTISKAKGQPREPQVYTLPPSREEMTKNQVSLTCLVKGFYPSDIAVEWESNGQPENNYKTYPPVLDSDGSFSLYSKLTVDKSRWQQGNVFSCSVMHEALHNHYTQKSLSLSP

SEQ ID NO: 400 - protein, 447 aa, Homo sapiens
QVQLQESGPGLVRPSQTLSLTCTVSGYSITSDHAWSWVRQPPGRGLEWIGYISYSGITTYNPSLKSRVTMLRDTSKNQFSLRLSSVTAADTAVYYCARSLARTTAMDYWGQGSLVTVSSASTKGPSVFPLAPSSKSTSGGTAALGCLVKDYFPEPVTVSWNSGALTSGVHTFPAVLQSSGLYSLSSVVTVPSSSLGTQTYICNVNHKPSNTKVDKRVEPKSCDKTHTCPPCPAPELLGGPSVFLFPPKPKDTLMISRTPEVTCVVVDVSHEDPEVKFNWYVDGVEVHNAKTKPREEQYNSTYRVVSVLTVLHQDWLNGKEYKCKVSNKALPAPIEKTISKAKGQPREPQVYTLPPSREEMTKNQVSLTCLVKGFYPSDIAVEWESNGQPENNYKTFPPVLDSDGSFSLYSKLTVDKSRWQQGNVFSCSVMHEALHNHYTQKSLSLSP

SEQ ID NO: 401 - protein, 447 aa, Homo sapiens
QVQLQESGPGLVRPSQTLSLTCTVSGYSITSDHAWSWVRQPPGRGLEWIGYISYSGITTYNPSLKSRVTMLRDTSKNQFSLRLSSVTAADTAVYYCARSLARTTAMDYWGQGSLVTVSSASTKGPSVFPLAPSSKSTSGGTAALGCLVKDYFPEPVTVSWNSGALTSGVHTFPAVLQSSGLYSLSSVVTVPSSSLGTQTYICNVNHKPSNTKVDKRVEPKSCDKTHTCPPCPAPELLGGPSVFLFPPKPKDTLMISRTPEVTCVVVDVSHEDPEVKFNWYVDGVEVHNAKTKPREEQYNSTYRVVSVLTVLHQDWLNGKEYKCKVSNKALPAPIEKTISKAKGQPREPQVYTLPPSREEMTKNQVSLTCLVKGFYPSDIAVEWESNGQPENNYKTFPPVLDSDGSFTLYSKLTVDKSRWQQGNVFSCSVMHEALHNHYTQKSLSLSP

SEQ ID NO: 402 - protein, 447 aa, Homo sapiens
QVQLQESGPGLVRPSQTLSLTCTVSGYSITSDHAWSWVRQPPGRGLEWIGYISYSGITTYNPSLKSRVTMLRDTSKNQFSLRLSSVTAADTAVYYCARSLARTTAMDYWGQGSLVTVSSASTKGPSVFPLAPSSKSTSGGTAALGCLVKDYFPEPVTVSWNSGALTSGVHTFPAVLQSSGLYSLSSVVTVPSSSLGTQTYICNVNHKPSNTKVDKRVEPKSCDKTHTCPPCPAPELLGGPSVFLFPPKPKDTLMISRTPEVTCVVVDVSHEDPEVKFNWYVDGVEVHNAKTKPREEQYNSTYRVVSVLTVLHQDWLNGKEYKCKVSNKALPAPIEKTISKAKGQPREPQVYTLPPSREEMTKNQVSLTCLVKGFYPSDIAVEWESNGQPENNYKTHPPVLDSDGSFVLYSKLTVDKSRWQQGNVFSCSVMHEALHNHYTQKSLSLSP

SEQ ID NO: 403 - protein, 447 aa, Homo sapiens
QVQLQESGPGLVRPSQTLSLTCTVSGYSITSDHAWSWVRQPPGRGLEWIGYISYSGITTYNPSLKSRVTMLRDTSKNQFSLRLSSVTAADTAVYYCARSLARTTAMDYWGQGSLVTVSSASTKGPSVFPLAPSSKSTSGGTAALGCLVKDYFPEPVTVSWNSGALTSGVHTFPAVLQSSGLYSLSSVVTVPSSSLGTQTYICNVNHKPSNTKVDKRVEPKSCDKTHTCPPCPAPELLGGPSVFLFPPKPKDTLMISRTPEVTCVVVDVSHEDPEVKFNWYVDGVEVHNAKTKPREEQYNSTYRVVSVLTVLHQDWLNGKEYKCKVSNKALPAPIEKTISKAKGQPREPQVYTLPPSREEMTKNQVSLTCLVKGFYPSDIAVEWESNGQPENNYKTWPPVLDSDGSFGLYSKLTVDKSRWQQGNVFSCSVMHEALHNHYTQKSLSLSP

SEQ ID NO: 404 - protein, 447 aa, Homo sapiens
QVQLQESGPGLVRPSQTLSLTCTVSGYSITSDHAWSWVRQPPGRGLEWIGYISYSGITTYNPSLKSRVTMLRDTSKNQFSLRLSSVTAADTAVYYCARSLARTTAMDYWGQGSLVTVSSASTKGPSVFPLAPSSKSTSGGTAALGCLVKDYFPEPVTVSWNSGALTSGVHTFPAVLQSSGLYSLSSVVTVPSSSLGTQTYICNVNHKPSNTKVDKRVEPKSCDKTHTCPPCPAPELLGGPSVFLFPPKPKDTLMISRTPEVTCVVVDVSHEDPEVKFNWYVDGVEVHNAKTKPREEQYNSTYRVVSVLTVLHQDWLNGKEYKCKVSNKALPAPIEKTISKAKGQPREPQVYTLPPSREEMTKNQVSLWCSVKGFYPSDIAVEWESNGQPENNYKTTPPVLDSDGSFFLVSKLTVDKSRWQQGNVFSCSVMHEALHNHYTQKSLSLSP

SEQ ID NO: 405 - protein, 447 aa, Homo sapiens
QVQLQESGPGLVRPSQTLSLTCTVSGYSITSDHAWSWVRQPPGRGLEWIGYISYSGITTYNPSLKSRVTMLRDTSKNQFSLRLSSVTAADTAVYYCARSLARTTAMDYWGQGSLVTVSSASTKGPSVFPLAPSSKSTSGGTAALGCLVKDYFPEPVTVSWNSGALTSGVHTFPAVLQSSGLYSLSSVVTVPSSSLGTQTYICNVNHKPSNTKVDKRVEPKSCDKTHTCPPCPAPELLGGPSVFLFPPKPKDTLMISRTPEVTCVVVDVSHEDPEVKFNWYVDGVEVHNAKTKPREEQYNSTYRVVSVLTVLHQDWLNGKEYKCKVSNKALPAPIEKTISKAKGQPREPQVYTLPPSREEMTKNQVSLWCTVKGFYPSDIAVEWESNGQPENNYKTTPPVLDSDGSFFLVSKLTVDKSRWQQGNVFSCSVMHEALHNHYTQKSLSLSP

SEQ ID NO: 406 - protein, 447 aa, Homo sapiens
QVQLQESGPGLVRPSQTLSLTCTVSGYSITSDHAWSWVRQPPGRGLEWIGYISYSGITTYNPSLKSRVTMLRDTSKNQFSLRLSSVTAADTAVYYCARSLARTTAMDYWGQGSLVTVSSASTKGPSVFPLAPSSKSTSGGTAALGCLVKDYFPEPVTVSWNSGALTSGVHTFPAVLQSSGLYSLSSVVTVPSSSLGTQTYICNVNHKPSNTKVDKRVEPKSCDKTHTCPPCPAPELLGGPSVFLFPPKPKDTLMISRTPEVTCVVVDVSHEDPEVKFNWYVDGVEVHNAKTKPREEQYNSTYRVVSVLTVLHQDWLNGKEYKCKVSNKALPAPIEKTISKAKGQPREPQVYTLPPSREEMTKNQVSLWCCVKGFYPSDIAVEWESNGQPENNYKTTPPVLDSDGSFFLVSKLTVDKSRWQQGNVFSCSVMHEALHNHYTQKSLSLSP

SEQ ID NO: 407 - protein, 447 aa, Homo sapiens
QVQLQESGPGLVRPSQTLSLTCTVSGYSITSDHAWSWVRQPPGRGLEWIGYISYSGITTYNPSLKSRVTMLRDTSKNQFSLRLSSVTAADTAVYYCARSLARTTAMDYWGQGSLVTVSSASTKGPSVFPLAPSSKSTSGGTAALGCLVKDYFPEPVTVSWNSGALTSGVHTFPAVLQSSGLYSLSSVVTVPSSSLGTQTYICNVNHKPSNTKVDKRVEPKSCDKTHTCPPCPAPELLGGPSVFLFPPKPKDTLMISRTPEVTCVVVDVSHEDPEVKFNWYVDGVEVHNAKTKPREEQYNSTYRVVSVLTVLHQDWLNGKEYKCKVSNKALPAPIEKTISKAKGQPREPQVYTLPPSREEMTKNQVSLWCVVKGFYPSDIAVEWESNGQPENNYKTTPPVLDSDGSFFLVSKLTVDKSRWQQGNVFSCSVMHEALHNHYTQKSLSLSP

SEQ ID NO: 408 - protein, 447 aa, Homo sapiens
QVQLQESGPGLVRPSQTLSLTCTVSGYSITSDHAWSWVRQPPGRGLEWIGYISYSGITTYNPSLKSRVTMLRDTSKNQFSLRLSSVTAADTAVYYCARSLARTTAMDYWGQGSLVTVSSASTKGPSVFPLAPSSKSTSGGTAALGCLVKDYFPEPVTVSWNSGALTSGVHTFPAVLQSSGLYSLSSVVTVPSSSLGTQTYICNVNHKPSNTKVDKRVEPKSCDKTHTCPPCPAPELLGGPSVFLFPPKPKDTLMISRTPEVTCVVVDVSHEDPEVKFNWYVDGVEVHNAKTKPREEQYNSTYRVVSVLTVLHQDWLNGKEYKCKVSNKALPAPIEKTISKAKGQPREPQVYTLPPSREEMTKNQVSLWCGVKGFYPSDIAVEWESNGQPENNYKTTPPVLDSDGSFFLVSKLTVDKSRWQQGNVFSCSVMHEALHNHYTQKSLSLSP

SEQ ID NO: 409 - protein, 447 aa, Homo sapiens
QVQLQESGPGLVRPSQTLSLTCTVSGYSITSDHAWSWVRQPPGRGLEWIGYISYSGITTYNPSLKSRVTMLRDTSKNQFSLRLSSVTAADTAVYYCARSLARTTAMDYWGQGSLVTVSSASTKGPSVFPLAPSSKSTSGGTAALGCLVKDYFPEPVTVSWNSGALTSGVHTFPAVLQSSGLYSLSSVVTVPSSSLGTQTYICNVNHKPSNTKVDKRVEPKSCDKTHTCPPCPAPELLGGPSVFLFPPKPKDTLMISRTPEVTCVVVDVSHEDPEVKFNWYVDGVEVHNAKTKPREEQYNSTYRVVSVLTVLHQDWLNGKEYKCKVSNKALPAPIEKTISKAKGQPREPQVYTLPPSREEMTKNQVSLYCAVKGFYPSDIAVEWESNGQPENNYKTTPPVLDSDGSFFLVSKLTVDKSRWQQGNVFSCSVMHEALHNHYTQKSLSLSP

SEQ ID NO: 410 - protein, 447 aa, Homo sapiens
QVQLQESGPGLVRPSQTLSLTCTVSGYSITSDHAWSWVRQPPGRGLEWIGYISYSGITTYNPSLKSRVTMLRDTSKNQFSLRLSSVTAADTAVYYCARSLARTTAMDYWGQGSLVTVSSASTKGPSVFPLAPSSKSTSGGTAALGCLVKDYFPEPVTVSWNSGALTSGVHTFPAVLQSSGLYSLSSVVTVPSSSLGTQTYICNVNHKPSNTKVDKRVEPKSCDKTHTCPPCPAPELLGGPSVFLFPPKPKDTLMISRTPEVTCVVVDVSHEDPEVKFNWYVDGVEVHNAKTKPREEQYNSTYRVVSVLTVLHQDWLNGKEYKCKVSNKALPAPIEKTISKAKGQPREPQVYTLPPSREEMTKNQVSLFCAVKGFYPSDIAVEWESNGQPENNYKTTPPVLDSDGSFFLVSKLTVDKSRWQQGNVFSCSVMHEALHNHYTQKSLSLSP

SEQ ID NO: 411 - protein, 447 aa, Homo sapiens
QVQLQESGPGLVRPSQTLSLTCTVSGYSITSDHAWSWVRQPPGRGLEWIGYISYSGITTYNPSLKSRVTMLRDTSKNQFSLRLSSVTAADTAVYYCARSLARTTAMDYWGQGSLVTVSSASTKGPSVFPLAPSSKSTSGGTAALGCLVKDYFPEPVTVSWNSGALTSGVHTFPAVLQSSGLYSLSSVVTVPSSSLGTQTYICNVNHKPSNTKVDKRVEPKSCDKTHTCPPCPAPELLGGPSVFLFPPKPKDTLMISRTPEVTCVVVDVSHEDPEVKFNWYVDGVEVHNAKTKPREEQYNSTYRVVSVLTVLHQDWLNGKEYKCKVSNKALPAPIEKTISKAKGQPREPQVYTLPPSREEMTKNQVSLHCAVKGFYPSDIAVEWESNGQPENNYKTTPPVLDSDGSFFLVSKLTVDKSRWQQGNVFSCSVMHEALHNHYTQKSLSLSP

SEQ ID NO: 412 - protein, 447 aa, Homo sapiens
QVQLQESGPGLVRPSQTLSLTCTVSGYSITSDHAWSWVRQPPGRGLEWIGYISYSGITTYNPSLKSRVTMLRDTSKNQFSLRLSSVTAADTAVYYCARSLARTTAMDYWGQGSLVTVSSASTKGPSVFPLAPSSKSTSGGTAALGCLVKDYFPEPVTVSWNSGALTSGVHTFPAVLQSSGLYSLSSVVTVPSSSLGTQTYICNVNHKPSNTKVDKRVEPKSCDKTHTCPPCPAPELLGGPSVFLFPPKPKDTLMISRTPEVTCVVVDVSHEDPEVKFNWYVDGVEVHNAKTKPREEQYNSTYRVVSVLTVLHQDWLNGKEYKCKVSNKALPAPIEKTISKAKGQPREPQVYTLPPSREEMTKNQVSLWCAVKGFYPSDIAVEWESNGQPENNYKTTPPVLDSDGSFFLLSKLTVDKSRWQQGNVFSCSVMHEALHNHYTQKSLSLSP

SEQ ID NO: 413 - protein, 447 aa, Homo sapiens
QVQLQESGPGLVRPSQTLSLTCTVSGYSITSDHAWSWVRQPPGRGLEWIGYISYSGITTYNPSLKSRVTMLRDTSKNQFSLRLSSVTAADTAVYYCARSLARTTAMDYWGQGSLVTVSSASTKGPSVFPLAPSSKSTSGGTAALGCLVKDYFPEPVTVSWNSGALTSGVHTFPAVLQSSGLYSLSSVVTVPSSSLGTQTYICNVNHKPSNTKVDKRVEPKSCDKTHTCPPCPAPELLGGPSVFLFPPKPKDTLMISRTPEVTCVVVDVSHEDPEVKFNWYVDGVEVHNAKTKPREEQYNSTYRVVSVLTVLHQDWLNGKEYKCKVSNKALPAPIEKTISKAKGQPREPQVYTLPPSREEMTKNQVSLWCAVKGFYPSDIAVEWESNGQPENNYKTTPPVLDSDGSFFLISKLTVDKSRWQQGNVFSCSVMHEALHNHYTQKSLSLSP

SEQ ID NO: 414 - protein, 447 aa, Homo sapiens
QVQLQESGPGLVRPSQTLSLTCTVSGYSITSDHAWSWVRQPPGRGLEWIGYISYSGITTYNPSLKSRVTMLRDTSKNQFSLRLSSVTAADTAVYYCARSLARTTAMDYWGQGSLVTVSSASTKGPSVFPLAPSSKSTSGGTAALGCLVKDYFPEPVTVSWNSGALTSGVHTFPAVLQSSGLYSLSSVVTVPSSSLGTQTYICNVNHKPSNTKVDKRVEPKSCDKTHTCPPCPAPELLGGPSVFLFPPKPKDTLMISRTPEVTCVVVDVSHEDPEVKFNWYVDGVEVHNAKTKPREEQYNSTYRVVSVLTVLHQDWLNGKEYKCKVSNKALPAPIEKTISKAKGQPREPQVYTLPPSREEMTKNQVSLWCAVKGFYPSDIAVEWESNGQPENNYKTTPPVLDSDGSFFLMSKLTVDKSRWQQGNVFSCSVMHEALHNHYTQKSLSLSP

SEQ ID NO: 415 - protein, 447 aa, Homo sapiens
QVQLQESGPGLVRPSQTLSLTCTVSGYSITSDHAWSWVRQPPGRGLEWIGYISYSGITTYNPSLKSRVTMLRDTSKNQFSLRLSSVTAADTAVYYCARSLARTTAMDYWGQGSLVTVSSASTKGPSVFPLAPSSKSTSGGTAALGCLVKDYFPEPVTVSWNSGALTSGVHTFPAVLQSSGLYSLSSVVTVPSSSLGTQTYICNVNHKPSNTKVDKRVEPKSCDKTHTCPPCPAPELLGGPSVFLFPPKPKDTLMISRTPEVTCVVVDVSHEDPEVKFNWYVDGVEVHNAKTKPREEQYNSTYRVVSVLTVLHQDWLNGKEYKCKVSNKALPAPIEKTISKAKGQPREPQVYTLPPSREEMTKNQVSLWCAVKGFYPSDIAVEWESNGQPENNYKTTPPVLDSDGSFFLASKLTVDKSRWQQGNVFSCSVMHEALHNHYTQKSLSLSP

SEQ ID NO: 416 - protein, 447 aa, Homo sapiens
QVQLQESGPGLVRPSQTLSLTCTVSGYSITSDHAWSWVRQPPGRGLEWIGYISYSGITTYNPSLKSRVTMLRDTSKNQFSLRLSSVTAADTAVYYCARSLARTTAMDYWGQGSLVTVSSASTKGPSVFPLAPSSKSTSGGTAALGCLVKDYFPEPVTVSWNSGALTSGVHTFPAVLQSSGLYSLSSVVTVPSSSLGTQTYICNVNHKPSNTKVDKRVEPKSCDKTHTCPPCPAPELLGGPSVFLFPPKPKDTLMISRTPEVTCVVVDVSHEDPEVKFNWYVDGVEVHNAKTKPREEQYNSTYRVVSVLTVLHQDWLNGKEYKCKVSNKALPAPIEKTISKAKGQPREPQVYTLPPSREEMTKNQVSLWCAVKGFYPSDIAVEWESNGQPENNYKTTPPVLDSDGSFFLSSKLTVDKSRWQQGNVFSCSVMHEALHNHYTQKSLSLSP

SEQ ID NO: 417 - protein, 447 aa, Homo sapiens
QVQLQESGPGLVRPSQTLSLTCTVSGYSITSDHAWSWVRQPPGRGLEWIGYISYSGITTYNPSLKSRVTMLRDTSKNQFSLRLSSVTAADTAVYYCARSLARTTAMDYWGQGSLVTVSSASTKGPSVFPLAPSSKSTSGGTAALGCLVKDYFPEPVTVSWNSGALTSGVHTFPAVLQSSGLYSLSSVVTVPSSSLGTQTYICNVNHKPSNTKVDKRVEPKSCDKTHTCPPCPAPELLGGPSVFLFPPKPKDTLMISRTPEVTCVVVDVSHEDPEVKFNWYVDGVEVHNAKTKPREEQYNSTYRVVSVLTVLHQDWLNGKEYKCKVSNKALPAPIEKTISKAKGQPREPQVYTLPPSREEMTKNQVSLWCAVKGFYPSDIAVEWESNGQPENNYKTTPPVLDSDGSFFLTSKLTVDKSRWQQGNVFSCSVMHEALHNHYTQKSLSLSP

SEQ ID NO: 418 - protein, 447 aa, Homo sapiens
QVQLQESGPGLVRPSQTLSLTCTVSGYSITSDHAWSWVRQPPGRGLEWIGYISYSGITTYNPSLKSRVTMLRDTSKNQFSLRLSSVTAADTAVYYCARSLARTTAMDYWGQGSLVTVSSASTKGPSVFPLAPSSKSTSGGTAALGCLVKDYFPEPVTVSWNSGALTSGVHTFPAVLQSSGLYSLSSVVTVPSSSLGTQTYICNVNHKPSNTKVDKRVEPKSCDKTHTCPPCPAPELLGGPSVFLFPPKPKDTLMISRTPEVTCVVVDVSHEDPEVKFNWYVDGVEVHNAKTKPREEQYNSTYRVVSVLTVLHQDWLNGKEYKCKVSNKALPAPIEKTISKAKGQPREPQVYTLPPSREEMTKNQVSLWCAVKGFYPSDIAVEWESNGQPENNYKTTPPVLDSDGSFFLCSKLTVDKSRWQQGNVFSCSVMHEALHNHYTQKSLSLSP

SEQ ID NO: 419 - protein, 447 aa, Homo sapiens
QVQLQESGPGLVRPSQTLSLTCTVSGYSITSDHAWSWVRQPPGRGLEWIGYISYSGITTYNPSLKSRVTMLRDTSKNQFSLRLSSVTAADTAVYYCARSLARTTAMDYWGQGSLVTVSSASTKGPSVFPLAPSSKSTSGGTAALGCLVKDYFPEPVTVSWNSGALTSGVHTFPAVLQSSGLYSLSSVVTVPSSSLGTQTYICNVNHKPSNTKVDKRVEPKSCDKTHTCPPCPAPELLGGPSVFLFPPKPKDTLMISRTPEVTCVVVDVSHEDPEVKFNWYVDGVEVHNAKTKPREEQYNSTYRVVSVLTVLHQDWLNGKEYKCKVSNKALPAPIEKTISKAKGQPREPQVYTLPPSREEMTKNQVSLWCAVKGFYPSDIAVEWESNGQPENNYKTTPPVLDSDGSFFLHSKLTVDKSRWQQGNVFSCSVMHEALHNHYTQKSLSLSP

SEQ ID NO: 420 - protein, 447 aa, Homo sapiens
QVQLQESGPGLVRPSQTLSLTCTVSGYSITSDHAWSWVRQPPGRGLEWIGYISYSGITTYNPSLKSRVTMLRDTSKNQFSLRLSSVTAADTAVYYCARSLARTTAMDYWGQGSLVTVSSASTKGPSVFPLAPSSKSTSGGTAALGCLVKDYFPEPVTVSWNSGALTSGVHTFPAVLQSSGLYSLSSVVTVPSSSLGTQTYICNVNHKPSNTKVDKRVEPKSCDKTHTCPPCPAPELLGGPSVFLFPPKPKDTLMISRTPEVTCVVVDVSHEDPEVKFNWYVDGVEVHNAKTKPREEQYNSTYRVVSVLTVLHQDWLNGKEYKCKVSNKALPAPIEKTISKAKGQPREPQVYTLPPSREEMTKNQVSLWCAVKGFYPSDIAVEWESNGQPENNYKTTPPVLDSDGSFFLNSKLTVDKSRWQQGNVFSCSVMHEALHNHYTQKSLSLSP

SEQ ID NO: 421 - protein, 447 aa, Homo sapiens
QVQLQESGPGLVRPSQTLSLTCTVSGYSITSDHAWSWVRQPPGRGLEWIGYISYSGITTYNPSLKSRVTMLRDTSKNQFSLRLSSVTAADTAVYYCARSLARTTAMDYWGQGSLVTVSSASTKGPSVFPLAPSSKSTSGGTAALGCLVKDYFPEPVTVSWNSGALTSGVHTFPAVLQSSGLYSLSSVVTVPSSSLGTQTYICNVNHKPSNTKVDKRVEPKSCDKTHTCPPCPAPELLGGPSVFLFPPKPKDTLMISRTPEVTCVVVDVSHEDPEVKFNWYVDGVEVHNAKTKPREEQYNSTYRVVSVLTVLHQDWLNGKEYKCKVSNKALPAPIEKTISKAKGQPREPQVYTLPPSREEMTKNQVSLWCCVKGFYPSDIAVEWESNGQPENNYKTTPPVLDSDGSFFLCSKLTVDKSRWQQGNVFSCSVMHEALHNHYTQKSLSLSP

SEQ ID NO: 422 - protein, 447 aa, Homo sapiens
QVQLQESGPGLVRPSQTLSLTCTVSGYSITSDHAWSWVRQPPGRGLEWIGYISYSGITTYNPSLKSRVTMLRDTSKNQFSLRLSSVTAADTAVYYCARSLARTTAMDYWGQGSLVTVSSASTKGPSVFPLAPSSKSTSGGTAALGCLVKDYFPEPVTVSWNSGALTSGVHTFPAVLQSSGLYSLSSVVTVPSSSLGTQTYICNVNHKPSNTKVDKRVEPKSCDKTHTCPPCPAPELLGGPSVFLFPPKPKDTLMISRTPEVTCVVVDVSHEDPEVKFNWYVDGVEVHNAKTKPREEQYNSTYRVVSVLTVLHQDWLNGKEYKCKVSNKALPAPIEKTISKAKGQPREPQVYTLPPSREEMTKNQVSLCCAVKGFYPSDIAVEWESNGQPENNYKTTPPVLDSDGSFFLCSKLTVDKSRWQQGNVFSCSVMHEALHNHYTQKSLSLSP

SEQ ID NO: 423 - protein, 447 aa, Homo sapiens
QVQLQESGPGLVRPSQTLSLTCTVSGYSITSDHAWSWVRQPPGRGLEWIGYISYSGITTYNPSLKSRVTMLRDTSKNQFSLRLSSVTAADTAVYYCARSLARTTAMDYWGQGSLVTVSSASTKGPSVFPLAPSSKSTSGGTAALGCLVKDYFPEPVTVSWNSGALTSGVHTFPAVLQSSGLYSLSSVVTVPSSSLGTQTYICNVNHKPSNTKVDKRVEPKSCDKTHTCPPCPAPELLGGPSVFLFPPKPKDTLMISRTPEVTCVVVDVSHEDPEVKFNWYVDGVEVHNAKTKPREEQYNSTYRVVSVLTVLHQDWLNGKEYKCKVSNKALPAPIEKTISKAKGQPREPQVYTLPPSREEMTKNQVSLWCSVKGFYPSDIAVEWESNGQPENNYKTTPPVLDSDGSFFLLSKLTVDKSRWQQGNVFSCSVMHEALHNHYTQKSLSLSP

SEQ ID NO: 424 - protein, 447 aa, Homo sapiens
QVQLQESGPGLVRPSQTLSLTCTVSGYSITSDHAWSWVRQPPGRGLEWIGYISYSGITTYNPSLKSRVTMLRDTSKNQFSLRLSSVTAADTAVYYCARSLARTTAMDYWGQGSLVTVSSASTKGPSVFPLAPSSKSTSGGTAALGCLVKDYFPEPVTVSWNSGALTSGVHTFPAVLQSSGLYSLSSVVTVPSSSLGTQTYICNVNHKPSNTKVDKRVEPKSCDKTHTCPPCPAPELLGGPSVFLFPPKPKDTLMISRTPEVTCVVVDVSHEDPEVKFNWYVDGVEVHNAKTKPREEQYNSTYRVVSVLTVLHQDWLNGKEYKCKVSNKALPAPIEKTISKAKGQPREPQVYTLPPSREEMTKNQVSLWCTVKGFYPSDIAVEWESNGQPENNYKTTPPVLDSDGSFFLLSKLTVDKSRWQQGNVFSCSVMHEALHNHYTQKSLSLSP

SEQ ID NO: 425 - protein, 447 aa, Homo sapiens
QVQLQESGPGLVRPSQTLSLTCTVSGYSITSDHAWSWVRQPPGRGLEWIGYISYSGITTYNPSLKSRVTMLRDTSKNQFSLRLSSVTAADTAVYYCARSLARTTAMDYWGQGSLVTVSSASTKGPSVFPLAPSSKSTSGGTAALGCLVKDYFPEPVTVSWNSGALTSGVHTFPAVLQSSGLYSLSSVVTVPSSSLGTQTYICNVNHKPSNTKVDKRVEPKSCDKTHTCPPCPAPELLGGPSVFLFPPKPKDTLMISRTPEVTCVVVDVSHEDPEVKFNWYVDGVEVHNAKTKPREEQYNSTYRVVSVLTVLHQDWLNGKEYKCKVSNKALPAPIEKTISKAKGQPREPQVYTLPPSREEMTKNQVSLWCCVKGFYPSDIAVEWESNGQPENNYKTTPPVLDSDGSFFLLSKLTVDKSRWQQGNVFSCSVMHEALHNHYTQKSLSLSP

SEQ ID NO: 426 - protein, 447 aa, Homo sapiens
QVQLQESGPGLVRPSQTLSLTCTVSGYSITSDHAWSWVRQPPGRGLEWIGYISYSGITTYNPSLKSRVTMLRDTSKNQFSLRLSSVTAADTAVYYCARSLARTTAMDYWGQGSLVTVSSASTKGPSVFPLAPSSKSTSGGTAALGCLVKDYFPEPVTVSWNSGALTSGVHTFPAVLQSSGLYSLSSVVTVPSSSLGTQTYICNVNHKPSNTKVDKRVEPKSCDKTHTCPPCPAPELLGGPSVFLFPPKPKDTLMISRTPEVTCVVVDVSHEDPEVKFNWYVDGVEVHNAKTKPREEQYNSTYRVVSVLTVLHQDWLNGKEYKCKVSNKALPAPIEKTISKAKGQPREPQVYTLPPSREEMTKNQVSLWCVVKGFYPSDIAVEWESNGQPENNYKTTPPVLDSDGSFFLLSKLTVDKSRWQQGNVFSCSVMHEALHNHYTQKSLSLSP

SEQ ID NO: 427 - protein, 447 aa, Homo sapiens
QVQLQESGPGLVRPSQTLSLTCTVSGYSITSDHAWSWVRQPPGRGLEWIGYISYSGITTYNPSLKSRVTMLRDTSKNQFSLRLSSVTAADTAVYYCARSLARTTAMDYWGQGSLVTVSSASTKGPSVFPLAPSSKSTSGGTAALGCLVKDYFPEPVTVSWNSGALTSGVHTFPAVLQSSGLYSLSSVVTVPSSSLGTQTYICNVNHKPSNTKVDKRVEPKSCDKTHTCPPCPAPELLGGPSVFLFPPKPKDTLMISRTPEVTCVVVDVSHEDPEVKFNWYVDGVEVHNAKTKPREEQYNSTYRVVSVLTVLHQDWLNGKEYKCKVSNKALPAPIEKTISKAKGQPREPQVYTLPPSREEMTKNQVSLWCGVKGFYPSDIAVEWESNGQPENNYKTTPPVLDSDGSFFLLSKLTVDKSRWQQGNVFSCSVMHEALHNHYTQKSLSLSP

SEQ ID NO: 428 - protein, 447 aa, Homo sapiens
QVQLQESGPGLVRPSQTLSLTCTVSGYSITSDHAWSWVRQPPGRGLEWIGYISYSGITTYNPSLKSRVTMLRDTSKNQFSLRLSSVTAADTAVYYCARSLARTTAMDYWGQGSLVTVSSASTKGPSVFPLAPSSKSTSGGTAALGCLVKDYFPEPVTVSWNSGALTSGVHTFPAVLQSSGLYSLSSVVTVPSSSLGTQTYICNVNHKPSNTKVDKRVEPKSCDKTHTCPPCPAPELLGGPSVFLFPPKPKDTLMISRTPEVTCVVVDVSHEDPEVKFNWYVDGVEVHNAKTKPREEQYNSTYRVVSVLTVLHQDWLNGKEYKCKVSNKALPAPIEKTISKAKGQPREPQVYTLPPSREEMTKNQVSLWCSVKGFYPSDIAVEWESNGQPENNYKTTPPVLDSDGSFFLISKLTVDKSRWQQGNVFSCSVMHEALHNHYTQKSLSLSP

SEQ ID NO: 429 - protein, 447 aa, Homo sapiens
QVQLQESGPGLVRPSQTLSLTCTVSGYSITSDHAWSWVRQPPGRGLEWIGYISYSGITTYNPSLKSRVTMLRDTSKNQFSLRLSSVTAADTAVYYCARSLARTTAMDYWGQGSLVTVSSASTKGPSVFPLAPSSKSTSGGTAALGCLVKDYFPEPVTVSWNSGALTSGVHTFPAVLQSSGLYSLSSVVTVPSSSLGTQTYICNVNHKPSNTKVDKRVEPKSCDKTHTCPPCPAPELLGGPSVFLFPPKPKDTLMISRTPEVTCVVVDVSHEDPEVKFNWYVDGVEVHNAKTKPREEQYNSTYRVVSVLTVLHQDWLNGKEYKCKVSNKALPAPIEKTISKAKGQPREPQVYTLPPSREEMTKNQVSLWCCVKGFYPSDIAVEWESNGQPENNYKTTPPVLDSDGSFFLISKLTVDKSRWQQGNVFSCSVMHEALHNHYTQKSLSLSP

SEQ ID NO: 430 - protein, 447 aa, Homo sapiens
QVQLQESGPGLVRPSQTLSLTCTVSGYSITSDHAWSWVRQPPGRGLEWIGYISYSGITTYNPSLKSRVTMLRDTSKNQFSLRLSSVTAADTAVYYCARSLARTTAMDYWGQGSLVTVSSASTKGPSVFPLAPSSKSTSGGTAALGCLVKDYFPEPVTVSWNSGALTSGVHTFPAVLQSSGLYSLSSVVTVPSSSLGTQTYICNVNHKPSNTKVDKRVEPKSCDKTHTCPPCPAPELLGGPSVFLFPPKPKDTLMISRTPEVTCVVVDVSHEDPEVKFNWYVDGVEVHNAKTKPREEQYNSTYRVVSVLTVLHQDWLNGKEYKCKVSNKALPAPIEKTISKAKGQPREPQVYTLPPSREEMTKNQVSLWCVVKGFYPSDIAVEWESNGQPENNYKTTPPVLDSDGSFFLISKLTVDKSRWQQGNVFSCSVMHEALHNHYTQKSLSLSP

SEQ ID NO: 431 - protein, 447 aa, Homo sapiens
QVQLQESGPGLVRPSQTLSLTCTVSGYSITSDHAWSWVRQPPGRGLEWIGYISYSGITTYNPSLKSRVTMLRDTSKNQFSLRLSSVTAADTAVYYCARSLARTTAMDYWGQGSLVTVSSASTKGPSVFPLAPSSKSTSGGTAALGCLVKDYFPEPVTVSWNSGALTSGVHTFPAVLQSSGLYSLSSVVTVPSSSLGTQTYICNVNHKPSNTKVDKRVEPKSCDKTHTCPPCPAPELLGGPSVFLFPPKPKDTLMISRTPEVTCVVVDVSHEDPEVKFNWYVDGVEVHNAKTKPREEQYNSTYRVVSVLTVLHQDWLNGKEYKCKVSNKALPAPIEKTISKAKGQPREPQVYTLPPSREEMTKNQVSLWCGVKGFYPSDIAVEWESNGQPENNYKTTPPVLDSDGSFFLISKLTVDKSRWQQGNVFSCSVMHEALHNHYTQKSLSLSP

SEQ ID NO: 432 - protein, 447 aa, Homo sapiens
QVQLQESGPGLVRPSQTLSLTCTVSGYSITSDHAWSWVRQPPGRGLEWIGYISYSGITTYNPSLKSRVTMLRDTSKNQFSLRLSSVTAADTAVYYCARSLARTTAMDYWGQGSLVTVSSASTKGPSVFPLAPSSKSTSGGTAALGCLVKDYFPEPVTVSWNSGALTSGVHTFPAVLQSSGLYSLSSVVTVPSSSLGTQTYICNVNHKPSNTKVDKRVEPKSCDKTHTCPPCPAPELLGGPSVFLFPPKPKDTLMISRTPEVTCVVVDVSHEDPEVKFNWYVDGVEVHNAKTKPREEQYNSTYRVVSVLTVLHQDWLNGKEYKCKVSNKALPAPIEKTISKAKGQPREPQVYTLPPSREEMTKNQVSLWCSVKGFYPSDIAVEWESNGQPENNYKTTPPVLDSDGSFFLMSKLTVDKSRWQQGNVFSCSVMHEALHNHYTQKSLSLSP

SEQ ID NO: 433 - protein, 447 aa, Homo sapiens
QVQLQESGPGLVRPSQTLSLTCTVSGYSITSDHAWSWVRQPPGRGLEWIGYISYSGITTYNPSLKSRVTMLRDTSKNQFSLRLSSVTAADTAVYYCARSLARTTAMDYWGQGSLVTVSSASTKGPSVFPLAPSSKSTSGGTAALGCLVKDYFPEPVTVSWNSGALTSGVHTFPAVLQSSGLYSLSSVVTVPSSSLGTQTYICNVNHKPSNTKVDKRVEPKSCDKTHTCPPCPAPELLGGPSVFLFPPKPKDTLMISRTPEVTCVVVDVSHEDPEVKFNWYVDGVEVHNAKTKPREEQYNSTYRVVSVLTVLHQDWLNGKEYKCKVSNKALPAPIEKTISKAKGQPREPQVYTLPPSREEMTKNQVSLWCTVKGFYPSDIAVEWESNGQPENNYKTTPPVLDSDGSFFLMSKLTVDKSRWQQGNVFSCSVMHEALHNHYTQKSLSLSP

SEQ ID NO: 434 - protein, 447 aa, Homo sapiens
QVQLQESGPGLVRPSQTLSLTCTVSGYSITSDHAWSWVRQPPGRGLEWIGYISYSGITTYNPSLKSRVTMLRDTSKNQFSLRLSSVTAADTAVYYCARSLARTTAMDYWGQGSLVTVSSASTKGPSVFPLAPSSKSTSGGTAALGCLVKDYFPEPVTVSWNSGALTSGVHTFPAVLQSSGLYSLSSVVTVPSSSLGTQTYICNVNHKPSNTKVDKRVEPKSCDKTHTCPPCPAPELLGGPSVFLFPPKPKDTLMISRTPEVTCVVVDVSHEDPEVKFNWYVDGVEVHNAKTKPREEQYNSTYRVVSVLTVLHQDWLNGKEYKCKVSNKALPAPIEKTISKAKGQPREPQVYTLPPSREEMTKNQVSLWCCVKGFYPSDIAVEWESNGQPENNYKTTPPVLDSDGSFFLMSKLTVDKSRWQQGNVFSCSVMHEALHNHYTQKSLSLSP

SEQ ID NO: 435 - protein, 447 aa, Homo sapiens
QVQLQESGPGLVRPSQTLSLTCTVSGYSITSDHAWSWVRQPPGRGLEWIGYISYSGITTYNPSLKSRVTMLRDTSKNQFSLRLSSVTAADTAVYYCARSLARTTAMDYWGQGSLVTVSSASTKGPSVFPLAPSSKSTSGGTAALGCLVKDYFPEPVTVSWNSGALTSGVHTFPAVLQSSGLYSLSSVVTVPSSSLGTQTYICNVNHKPSNTKVDKRVEPKSCDKTHTCPPCPAPELLGGPSVFLFPPKPKDTLMISRTPEVTCVVVDVSHEDPEVKFNWYVDGVEVHNAKTKPREEQYNSTYRVVSVLTVLHQDWLNGKEYKCKVSNKALPAPIEKTISKAKGQPREPQVYTLPPSREEMTKNQVSLWCVVKGFYPSDIAVEWESNGQPENNYKTTPPVLDSDGSFFLMSKLTVDKSRWQQGNVFSCSVMHEALHNHYTQKSLSLSP

SEQ ID NO: 436 - protein, 447 aa, Homo sapiens
QVQLQESGPGLVRPSQTLSLTCTVSGYSITSDHAWSWVRQPPGRGLEWIGYISYSGITTYNPSLKSRVTMLRDTSKNQFSLRLSSVTAADTAVYYCARSLARTTAMDYWGQGSLVTVSSASTKGPSVFPLAPSSKSTSGGTAALGCLVKDYFPEPVTVSWNSGALTSGVHTFPAVLQSSGLYSLSSVVTVPSSSLGTQTYICNVNHKPSNTKVDKRVEPKSCDKTHTCPPCPAPELLGGPSVFLFPPKPKDTLMISRTPEVTCVVVDVSHEDPEVKFNWYVDGVEVHNAKTKPREEQYNSTYRVVSVLTVLHQDWLNGKEYKCKVSNKALPAPIEKTISKAKGQPREPQVYTLPPSREEMTKNQVSLWCGVKGFYPSDIAVEWESNGQPENNYKTTPPVLDSDGSFFLMSKLTVDKSRWQQGNVFSCSVMHEALHNHYTQKSLSLSP

SEQ ID NO: 437 - protein, 447 aa, Homo sapiens
QVQLQESGPGLVRPSQTLSLTCTVSGYSITSDHAWSWVRQPPGRGLEWIGYISYSGITTYNPSLKSRVTMLRDTSKNQFSLRLSSVTAADTAVYYCARSLARTTAMDYWGQGSLVTVSSASTKGPSVFPLAPSSKSTSGGTAALGCLVKDYFPEPVTVSWNSGALTSGVHTFPAVLQSSGLYSLSSVVTVPSSSLGTQTYICNVNHKPSNTKVDKRVEPKSCDKTHTCPPCPAPELLGGPSVFLFPPKPKDTLMISRTPEVTCVVVDVSHEDPEVKFNWYVDGVEVHNAKTKPREEQYNSTYRVVSVLTVLHQDWLNGKEYKCKVSNKALPAPIEKTISKAKGQPREPQVYTLPPSREEMTKNQVSLWCSVKGFYPSDIAVEWESNGQPENNYKTTPPVLDSDGSFFLASKLTVDKSRWQQGNVFSCSVMHEALHNHYTQKSLSLSP

SEQ ID NO: 438 - protein, 447 aa, Homo sapiens
QVQLQESGPGLVRPSQTLSLTCTVSGYSITSDHAWSWVRQPPGRGLEWIGYISYSGITTYNPSLKSRVTMLRDTSKNQFSLRLSSVTAADTAVYYCARSLARTTAMDYWGQGSLVTVSSASTKGPSVFPLAPSSKSTSGGTAALGCLVKDYFPEPVTVSWNSGALTSGVHTFPAVLQSSGLYSLSSVVTVPSSSLGTQTYICNVNHKPSNTKVDKRVEPKSCDKTHTCPPCPAPELLGGPSVFLFPPKPKDTLMISRTPEVTCVVVDVSHEDPEVKFNWYVDGVEVHNAKTKPREEQYNSTYRVVSVLTVLHQDWLNGKEYKCKVSNKALPAPIEKTISKAKGQPREPQVYTLPPSREEMTKNQVSLWCTVKGFYPSDIAVEWESNGQPENNYKTTPPVLDSDGSFFLASKLTVDKSRWQQGNVFSCSVMHEALHNHYTQKSLSLSP

SEQ ID NO: 439 - protein, 447 aa, Homo sapiens
QVQLQESGPGLVRPSQTLSLTCTVSGYSITSDHAWSWVRQPPGRGLEWIGYISYSGITTYNPSLKSRVTMLRDTSKNQFSLRLSSVTAADTAVYYCARSLARTTAMDYWGQGSLVTVSSASTKGPSVFPLAPSSKSTSGGTAALGCLVKDYFPEPVTVSWNSGALTSGVHTFPAVLQSSGLYSLSSVVTVPSSSLGTQTYICNVNHKPSNTKVDKRVEPKSCDKTHTCPPCPAPELLGGPSVFLFPPKPKDTLMISRTPEVTCVVVDVSHEDPEVKFNWYVDGVEVHNAKTKPREEQYNSTYRVVSVLTVLHQDWLNGKEYKCKVSNKALPAPIEKTISKAKGQPREPQVYTLPPSREEMTKNQVSLWCCVKGFYPSDIAVEWESNGQPENNYKTTPPVLDSDGSFFLASKLTVDKSRWQQGNVFSCSVMHEALHNHYTQKSLSLSP

SEQ ID NO: 440 - protein, 447 aa, Homo sapiens
QVQLQESGPGLVRPSQTLSLTCTVSGYSITSDHAWSWVRQPPGRGLEWIGYISYSGITTYNPSLKSRVTMLRDTSKNQFSLRLSSVTAADTAVYYCARSLARTTAMDYWGQGSLVTVSSASTKGPSVFPLAPSSKSTSGGTAALGCLVKDYFPEPVTVSWNSGALTSGVHTFPAVLQSSGLYSLSSVVTVPSSSLGTQTYICNVNHKPSNTKVDKRVEPKSCDKTHTCPPCPAPELLGGPSVFLFPPKPKDTLMISRTPEVTCVVVDVSHEDPEVKFNWYVDGVEVHNAKTKPREEQYNSTYRVVSVLTVLHQDWLNGKEYKCKVSNKALPAPIEKTISKAKGQPREPQVYTLPPSREEMTKNQVSLWCVVKGFYPSDIAVEWESNGQPENNYKTTPPVLDSDGSFFLASKLTVDKSRWQQGNVFSCSVMHEALHNHYTQKSLSLSP

SEQ ID NO: 441 - protein, 447 aa, Homo sapiens
QVQLQESGPGLVRPSQTLSLTCTVSGYSITSDHAWSWVRQPPGRGLEWIGYISYSGITTYNPSLKSRVTMLRDTSKNQFSLRLSSVTAADTAVYYCARSLARTTAMDYWGQGSLVTVSSASTKGPSVFPLAPSSKSTSGGTAALGCLVKDYFPEPVTVSWNSGALTSGVHTFPAVLQSSGLYSLSSVVTVPSSSLGTQTYICNVNHKPSNTKVDKRVEPKSCDKTHTCPPCPAPELLGGPSVFLFPPKPKDTLMISRTPEVTCVVVDVSHEDPEVKFNWYVDGVEVHNAKTKPREEQYNSTYRVVSVLTVLHQDWLNGKEYKCKVSNKALPAPIEKTISKAKGQPREPQVYTLPPSREEMTKNQVSLWCGVKGFYPSDIAVEWESNGQPENNYKTTPPVLDSDGSFFLASKLTVDKSRWQQGNVFSCSVMHEALHNHYTQKSLSLSP

SEQ ID NO: 442 - protein, 447 aa, Homo sapiens
QVQLQESGPGLVRPSQTLSLTCTVSGYSITSDHAWSWVRQPPGRGLEWIGYISYSGITTYNPSLKSRVTMLRDTSKNQFSLRLSSVTAADTAVYYCARSLARTTAMDYWGQGSLVTVSSASTKGPSVFPLAPSSKSTSGGTAALGCLVKDYFPEPVTVSWNSGALTSGVHTFPAVLQSSGLYSLSSVVTVPSSSLGTQTYICNVNHKPSNTKVDKRVEPKSCDKTHTCPPCPAPELLGGPSVFLFPPKPKDTLMISRTPEVTCVVVDVSHEDPEVKFNWYVDGVEVHNAKTKPREEQYNSTYRVVSVLTVLHQDWLNGKEYKCKVSNKALPAPIEKTISKAKGQPREPQVYTLPPSREEMTKNQVSLWCSVKGFYPSDIAVEWESNGQPENNYKTTPPVLDSDGSFFLTSKLTVDKSRWQQGNVFSCSVMHEALHNHYTQKSLSLSP

SEQ ID NO: 443 - protein, 447 aa, Homo sapiens
QVQLQESGPGLVRPSQTLSLTCTVSGYSITSDHAWSWVRQPPGRGLEWIGYISYSGITTYNPSLKSRVTMLRDTSKNQFSLRLSSVTAADTAVYYCARSLARTTAMDYWGQGSLVTVSSASTKGPSVFPLAPSSKSTSGGTAALGCLVKDYFPEPVTVSWNSGALTSGVHTFPAVLQSSGLYSLSSVVTVPSSSLGTQTYICNVNHKPSNTKVDKRVEPKSCDKTHTCPPCPAPELLGGPSVFLFPPKPKDTLMISRTPEVTCVVVDVSHEDPEVKFNWYVDGVEVHNAKTKPREEQYNSTYRVVSVLTVLHQDWLNGKEYKCKVSNKALPAPIEKTISKAKGQPREPQVYTLPPSREEMTKNQVSLWCTVKGFYPSDIAVEWESNGQPENNYKTTPPVLDSDGSFFLTSKLTVDKSRWQQGNVFSCSVMHEALHNHYTQKSLSLSP

SEQ ID NO: 444 - protein, 447 aa, Homo sapiens
QVQLQESGPGLVRPSQTLSLTCTVSGYSITSDHAWSWVRQPPGRGLEWIGYISYSGITTYNPSLKSRVTMLRDTSKNQFSLRLSSVTAADTAVYYCARSLARTTAMDYWGQGSLVTVSSASTKGPSVFPLAPSSKSTSGGTAALGCLVKDYFPEPVTVSWNSGALTSGVHTFPAVLQSSGLYSLSSVVTVPSSSLGTQTYICNVNHKPSNTKVDKRVEPKSCDKTHTCPPCPAPELLGGPSVFLFPPKPKDTLMISRTPEVTCVVVDVSHEDPEVKFNWYVDGVEVHNAKTKPREEQYNSTYRVVSVLTVLHQDWLNGKEYKCKVSNKALPAPIEKTISKAKGQPREPQVYTLPPSREEMTKNQVSLWCCVKGFYPSDIAVEWESNGQPENNYKTTPPVLDSDGSFFLTSKLTVDKSRWQQGNVFSCSVMHEALHNHYTQKSLSLSP

SEQ ID NO: 445 - protein, 447 aa, Homo sapiens
QVQLQESGPGLVRPSQTLSLTCTVSGYSITSDHAWSWVRQPPGRGLEWIGYISYSGITTYNPSLKSRVTMLRDTSKNQFSLRLSSVTAADTAVYYCARSLARTTAMDYWGQGSLVTVSSASTKGPSVFPLAPSSKSTSGGTAALGCLVKDYFPEPVTVSWNSGALTSGVHTFPAVLQSSGLYSLSSVVTVPSSSLGTQTYICNVNHKPSNTKVDKRVEPKSCDKTHTCPPCPAPELLGGPSVFLFPPKPKDTLMISRTPEVTCVVVDVSHEDPEVKFNWYVDGVEVHNAKTKPREEQYNSTYRVVSVLTVLHQDWLNGKEYKCKVSNKALPAPIEKTISKAKGQPREPQVYTLPPSREEMTKNQVSLWCVVKGFYPSDIAVEWESNGQPENNYKTTPPVLDSDGSFFLTSKLTVDKSRWQQGNVFSCSVMHEALHNHYTQKSLSLSP

SEQ ID NO: 446 - protein, 447 aa, Homo sapiens
QVQLQESGPGLVRPSQTLSLTCTVSGYSITSDHAWSWVRQPPGRGLEWIGYISYSGITTYNPSLKSRVTMLRDTSKNQFSLRLSSVTAADTAVYYCARSLARTTAMDYWGQGSLVTVSSASTKGPSVFPLAPSSKSTSGGTAALGCLVKDYFPEPVTVSWNSGALTSGVHTFPAVLQSSGLYSLSSVVTVPSSSLGTQTYICNVNHKPSNTKVDKRVEPKSCDKTHTCPPCPAPELLGGPSVFLFPPKPKDTLMISRTPEVTCVVVDVSHEDPEVKFNWYVDGVEVHNAKTKPREEQYNSTYRVVSVLTVLHQDWLNGKEYKCKVSNKALPAPIEKTISKAKGQPREPQVYTLPPSREEMTKNQVSLWCGVKGFYPSDIAVEWESNGQPENNYKTTPPVLDSDGSFFLTSKLTVDKSRWQQGNVFSCSVMHEALHNHYTQKSLSLSP

SEQ ID NO: 447 - protein, 447 aa, Homo sapiens
QVQLQESGPGLVRPSQTLSLTCTVSGYSITSDHAWSWVRQPPGRGLEWIGYISYSGITTYNPSLKSRVTMLRDTSKNQFSLRLSSVTAADTAVYYCARSLARTTAMDYWGQGSLVTVSSASTKGPSVFPLAPSSKSTSGGTAALGCLVKDYFPEPVTVSWNSGALTSGVHTFPAVLQSSGLYSLSSVVTVPSSSLGTQTYICNVNHKPSNTKVDKRVEPKSCDKTHTCPPCPAPELLGGPSVFLFPPKPKDTLMISRTPEVTCVVVDVSHEDPEVKFNWYVDGVEVHNAKTKPREEQYNSTYRVVSVLTVLHQDWLNGKEYKCKVSNKALPAPIEKTISKAKGQPREPQVYTLPPSREEMTKNQVSLWCSVKGFYPSDIAVEWESNGQPENNYKTTPPVLDSDGSFFLCSKLTVDKSRWQQGNVFSCSVMHEALHNHYTQKSLSLSP

SEQ ID NO: 448 - protein, 447 aa, Homo sapiens
QVQLQESGPGLVRPSQTLSLTCTVSGYSITSDHAWSWVRQPPGRGLEWIGYISYSGITTYNPSLKSRVTMLRDTSKNQFSLRLSSVTAADTAVYYCARSLARTTAMDYWGQGSLVTVSSASTKGPSVFPLAPSSKSTSGGTAALGCLVKDYFPEPVTVSWNSGALTSGVHTFPAVLQSSGLYSLSSVVTVPSSSLGTQTYICNVNHKPSNTKVDKRVEPKSCDKTHTCPPCPAPELLGGPSVFLFPPKPKDTLMISRTPEVTCVVVDVSHEDPEVKFNWYVDGVEVHNAKTKPREEQYNSTYRVVSVLTVLHQDWLNGKEYKCKVSNKALPAPIEKTISKAKGQPREPQVYTLPPSREEMTKNQVSLWCTVKGFYPSDIAVEWESNGQPENNYKTTPPVLDSDGSFFLCSKLTVDKSRWQQGNVFSCSVMHEALHNHYTQKSLSLSP

SEQ ID NO: 449 - protein, 447 aa, Homo sapiens
QVQLQESGPGLVRPSQTLSLTCTVSGYSITSDHAWSWVRQPPGRGLEWIGYISYSGITTYNPSLKSRVTMLRDTSKNQFSLRLSSVTAADTAVYYCARSLARTTAMDYWGQGSLVTVSSASTKGPSVFPLAPSSKSTSGGTAALGCLVKDYFPEPVTVSWNSGALTSGVHTFPAVLQSSGLYSLSSVVTVPSSSLGTQTYICNVNHKPSNTKVDKRVEPKSCDKTHTCPPCPAPELLGGPSVFLFPPKPKDTLMISRTPEVTCVVVDVSHEDPEVKFNWYVDGVEVHNAKTKPREEQYNSTYRVVSVLTVLHQDWLNGKEYKCKVSNKALPAPIEKTISKAKGQPREPQVYTLPPSREEMTKNQVSLWCVVKGFYPSDIAVEWESNGQPENNYKTTPPVLDSDGSFFLCSKLTVDKSRWQQGNVFSCSVMHEALHNHYTQKSLSLSP

SEQ ID NO: 450 - protein, 447 aa, Homo sapiens
QVQLQESGPGLVRPSQTLSLTCTVSGYSITSDHAWSWVRQPPGRGLEWIGYISYSGITTYNPSLKSRVTMLRDTSKNQFSLRLSSVTAADTAVYYCARSLARTTAMDYWGQGSLVTVSSASTKGPSVFPLAPSSKSTSGGTAALGCLVKDYFPEPVTVSWNSGALTSGVHTFPAVLQSSGLYSLSSVVTVPSSSLGTQTYICNVNHKPSNTKVDKRVEPKSCDKTHTCPPCPAPELLGGPSVFLFPPKPKDTLMISRTPEVTCVVVDVSHEDPEVKFNWYVDGVEVHNAKTKPREEQYNSTYRVVSVLTVLHQDWLNGKEYKCKVSNKALPAPIEKTISKAKGQPREPQVYTLPPSREEMTKNQVSLWCGVKGFYPSDIAVEWESNGQPENNYKTTPPVLDSDGSFFLCSKLTVDKSRWQQGNVFSCSVMHEALHNHYTQKSLSLSP

SEQ ID NO: 451 - protein, 447 aa, Homo sapiens
QVQLQESGPGLVRPSQTLSLTCTVSGYSITSDHAWSWVRQPPGRGLEWIGYISYSGITTYNPSLKSRVTMLRDTSKNQFSLRLSSVTAADTAVYYCARSLARTTAMDYWGQGSLVTVSSASTKGPSVFPLAPSSKSTSGGTAALGCLVKDYFPEPVTVSWNSGALTSGVHTFPAVLQSSGLYSLSSVVTVPSSSLGTQTYICNVNHKPSNTKVDKRVEPKSCDKTHTCPPCPAPELLGGPSVFLFPPKPKDTLMISRTPEVTCVVVDVSHEDPEVKFNWYVDGVEVHNAKTKPREEQYNSTYRVVSVLTVLHQDWLNGKEYKCKVSNKALPAPIEKTISKAKGQPREPQVYTLPPSREEMTKNQVSLWCSVKGFYPSDIAVEWESNGQPENNYKTTPPVLDSDGSFFLHSKLTVDKSRWQQGNVFSCSVMHEALHNHYTQKSLSLSP

SEQ ID NO: 452 - protein, 447 aa, Homo sapiens
QVQLQESGPGLVRPSQTLSLTCTVSGYSITSDHAWSWVRQPPGRGLEWIGYISYSGITTYNPSLKSRVTMLRDTSKNQFSLRLSSVTAADTAVYYCARSLARTTAMDYWGQGSLVTVSSASTKGPSVFPLAPSSKSTSGGTAALGCLVKDYFPEPVTVSWNSGALTSGVHTFPAVLQSSGLYSLSSVVTVPSSSLGTQTYICNVNHKPSNTKVDKRVEPKSCDKTHTCPPCPAPELLGGPSVFLFPPKPKDTLMISRTPEVTCVVVDVSHEDPEVKFNWYVDGVEVHNAKTKPREEQYNSTYRVVSVLTVLHQDWLNGKEYKCKVSNKALPAPIEKTISKAKGQPREPQVYTLPPSREEMTKNQVSLWCTVKGFYPSDIAVEWESNGQPENNYKTTPPVLDSDGSFFLHSKLTVDKSRWQQGNVFSCSVMHEALHNHYTQKSLSLSP

SEQ ID NO: 453 - protein, 447 aa, Homo sapiens
QVQLQESGPGLVRPSQTLSLTCTVSGYSITSDHAWSWVRQPPGRGLEWIGYISYSGITTYNPSLKSRVTMLRDTSKNQFSLRLSSVTAADTAVYYCARSLARTTAMDYWGQGSLVTVSSASTKGPSVFPLAPSSKSTSGGTAALGCLVKDYFPEPVTVSWNSGALTSGVHTFPAVLQSSGLYSLSSVVTVPSSSLGTQTYICNVNHKPSNTKVDKRVEPKSCDKTHTCPPCPAPELLGGPSVFLFPPKPKDTLMISRTPEVTCVVVDVSHEDPEVKFNWYVDGVEVHNAKTKPREEQYNSTYRVVSVLTVLHQDWLNGKEYKCKVSNKALPAPIEKTISKAKGQPREPQVYTLPPSREEMTKNQVSLWCVVKGFYPSDIAVEWESNGQPENNYKTTPPVLDSDGSFFLHSKLTVDKSRWQQGNVFSCSVMHEALHNHYTQKSLSLSP

SEQ ID NO: 454 - protein, 447 aa, Homo sapiens
QVQLQESGPGLVRPSQTLSLTCTVSGYSITSDHAWSWVRQPPGRGLEWIGYISYSGITTYNPSLKSRVTMLRDTSKNQFSLRLSSVTAADTAVYYCARSLARTTAMDYWGQGSLVTVSSASTKGPSVFPLAPSSKSTSGGTAALGCLVKDYFPEPVTVSWNSGALTSGVHTFPAVLQSSGLYSLSSVVTVPSSSLGTQTYICNVNHKPSNTKVDKRVEPKSCDKTHTCPPCPAPELLGGPSVFLFPPKPKDTLMISRTPEVTCVVVDVSHEDPEVKFNWYVDGVEVHNAKTKPREEQYNSTYRVVSVLTVLHQDWLNGKEYKCKVSNKALPAPIEKTISKAKGQPREPQVYTLPPSREEMTKNQVSLWCGVKGFYPSDIAVEWESNGQPENNYKTTPPVLDSDGSFFLHSKLTVDKSRWQQGNVFSCSVMHEALHNHYTQKSLSLSP

SEQ ID NO: 455 - protein, 447 aa, Homo sapiens
QVQLQESGPGLVRPSQTLSLTCTVSGYSITSDHAWSWVRQPPGRGLEWIGYISYSGITTYNPSLKSRVTMLRDTSKNQFSLRLSSVTAADTAVYYCARSLARTTAMDYWGQGSLVTVSSASTKGPSVFPLAPSSKSTSGGTAALGCLVKDYFPEPVTVSWNSGALTSGVHTFPAVLQSSGLYSLSSVVTVPSSSLGTQTYICNVNHKPSNTKVDKRVEPKSCDKTHTCPPCPAPELLGGPSVFLFPPKPKDTLMISRTPEVTCVVVDVSHEDPEVKFNWYVDGVEVHNAKTKPREEQYNSTYRVVSVLTVLHQDWLNGKEYKCKVSNKALPAPIEKTISKAKGQPREPQVYTLPPSREEMTKNQVSLWCSVKGFYPSDIAVEWESNGQPENNYKTTPPVLDSDGSFFLNSKLTVDKSRWQQGNVFSCSVMHEALHNHYTQKSLSLSP

SEQ ID NO: 456 - protein, 447 aa, Homo sapiens
QVQLQESGPGLVRPSQTLSLTCTVSGYSITSDHAWSWVRQPPGRGLEWIGYISYSGITTYNPSLKSRVTMLRDTSKNQFSLRLSSVTAADTAVYYCARSLARTTAMDYWGQGSLVTVSSASTKGPSVFPLAPSSKSTSGGTAALGCLVKDYFPEPVTVSWNSGALTSGVHTFPAVLQSSGLYSLSSVVTVPSSSLGTQTYICNVNHKPSNTKVDKRVEPKSCDKTHTCPPCPAPELLGGPSVFLFPPKPKDTLMISRTPEVTCVVVDVSHEDPEVKFNWYVDGVEVHNAKTKPREEQYNSTYRVVSVLTVLHQDWLNGKEYKCKVSNKALPAPIEKTISKAKGQPREPQVYTLPPSREEMTKNQVSLWCTVKGFYPSDIAVEWESNGQPENNYKTTPPVLDSDGSFFLNSKLTVDKSRWQQGNVFSCSVMHEALHNHYTQKSLSLSP

SEQ ID NO: 457 - protein, 447 aa, Homo sapiens
QVQLQESGPGLVRPSQTLSLTCTVSGYSITSDHAWSWVRQPPGRGLEWIGYISYSGITTYNPSLKSRVTMLRDTSKNQFSLRLSSVTAADTAVYYCARSLARTTAMDYWGQGSLVTVSSASTKGPSVFPLAPSSKSTSGGTAALGCLVKDYFPEPVTVSWNSGALTSGVHTFPAVLQSSGLYSLSSVVTVPSSSLGTQTYICNVNHKPSNTKVDKRVEPKSCDKTHTCPPCPAPELLGGPSVFLFPPKPKDTLMISRTPEVTCVVVDVSHEDPEVKFNWYVDGVEVHNAKTKPREEQYNSTYRVVSVLTVLHQDWLNGKEYKCKVSNKALPAPIEKTISKAKGQPREPQVYTLPPSREEMTKNQVSLWCCVKGFYPSDIAVEWESNGQPENNYKTTPPVLDSDGSFFLNSKLTVDKSRWQQGNVFSCSVMHEALHNHYTQKSLSLSP

SEQ ID NO: 458 - protein, 447 aa, Homo sapiens
QVQLQESGPGLVRPSQTLSLTCTVSGYSITSDHAWSWVRQPPGRGLEWIGYISYSGITTYNPSLKSRVTMLRDTSKNQFSLRLSSVTAADTAVYYCARSLARTTAMDYWGQGSLVTVSSASTKGPSVFPLAPSSKSTSGGTAALGCLVKDYFPEPVTVSWNSGALTSGVHTFPAVLQSSGLYSLSSVVTVPSSSLGTQTYICNVNHKPSNTKVDKRVEPKSCDKTHTCPPCPAPELLGGPSVFLFPPKPKDTLMISRTPEVTCVVVDVSHEDPEVKFNWYVDGVEVHNAKTKPREEQYNSTYRVVSVLTVLHQDWLNGKEYKCKVSNKALPAPIEKTISKAKGQPREPQVYTLPPSREEMTKNQVSLWCGVKGFYPSDIAVEWESNGQPENNYKTTPPVLDSDGSFFLNSKLTVDKSRWQQGNVFSCSVMHEALHNHYTQKSLSLSP

SEQ ID NO: 459 - protein, 447 aa, Homo sapiens
QVQLQESGPGLVRPSQTLSLTCTVSGYSITSDHAWSWVRQPPGRGLEWIGYISYSGITTYNPSLKSRVTMLRDTSKNQFSLRLSSVTAADTAVYYCARSLARTTAMDYWGQGSLVTVSSASTKGPSVFPLAPSSKSTSGGTAALGCLVKDYFPEPVTVSWNSGALTSGVHTFPAVLQSSGLYSLSSVVTVPSSSLGTQTYICNVNHKPSNTKVDKRVEPKSCDKTHTCPPCPAPELLGGPSVFLFPPKPKDTLMISRTPEVTCVVVDVSHEDPEVKFNWYVDGVEVHNAKTKPREEQYNSTYRVVSVLTVLHQDWLNGKEYKCKVSNKALPAPIEKTISKAKGQPREPQVYTLPPSREEMTKNQVSLWCSVKGFYPSDIAVEWESNGQPENNYKTTPPVLDSDGSFFLQSKLTVDKSRWQQGNVFSCSVMHEALHNHYTQKSLSLSP

SEQ ID NO: 460 - protein, 447 aa, Homo sapiens
QVQLQESGPGLVRPSQTLSLTCTVSGYSITSDHAWSWVRQPPGRGLEWIGYISYSGITTYNPSLKSRVTMLRDTSKNQFSLRLSSVTAADTAVYYCARSLARTTAMDYWGQGSLVTVSSASTKGPSVFPLAPSSKSTSGGTAALGCLVKDYFPEPVTVSWNSGALTSGVHTFPAVLQSSGLYSLSSVVTVPSSSLGTQTYICNVNHKPSNTKVDKRVEPKSCDKTHTCPPCPAPELLGGPSVFLFPPKPKDTLMISRTPEVTCVVVDVSHEDPEVKFNWYVDGVEVHNAKTKPREEQYNSTYRVVSVLTVLHQDWLNGKEYKCKVSNKALPAPIEKTISKAKGQPREPQVYTLPPSREEMTKNQVSLWCTVKGFYPSDIAVEWESNGQPENNYKTTPPVLDSDGSFFLQSKLTVDKSRWQQGNVFSCSVMHEALHNHYTQKSLSLSP

SEQ ID NO: 461 - protein, 447 aa, Homo sapiens
QVQLQESGPGLVRPSQTLSLTCTVSGYSITSDHAWSWVRQPPGRGLEWIGYISYSGITTYNPSLKSRVTMLRDTSKNQFSLRLSSVTAADTAVYYCARSLARTTAMDYWGQGSLVTVSSASTKGPSVFPLAPSSKSTSGGTAALGCLVKDYFPEPVTVSWNSGALTSGVHTFPAVLQSSGLYSLSSVVTVPSSSLGTQTYICNVNHKPSNTKVDKRVEPKSCDKTHTCPPCPAPELLGGPSVFLFPPKPKDTLMISRTPEVTCVVVDVSHEDPEVKFNWYVDGVEVHNAKTKPREEQYNSTYRVVSVLTVLHQDWLNGKEYKCKVSNKALPAPIEKTISKAKGQPREPQVYTLPPSREEMTKNQVSLWCCVKGFYPSDIAVEWESNGQPENNYKTTPPVLDSDGSFFLQSKLTVDKSRWQQGNVFSCSVMHEALHNHYTQKSLSLSP

SEQ ID NO: 462 - protein, 447 aa, Homo sapiens
QVQLQESGPGLVRPSQTLSLTCTVSGYSITSDHAWSWVRQPPGRGLEWIGYISYSGITTYNPSLKSRVTMLRDTSKNQFSLRLSSVTAADTAVYYCARSLARTTAMDYWGQGSLVTVSSASTKGPSVFPLAPSSKSTSGGTAALGCLVKDYFPEPVTVSWNSGALTSGVHTFPAVLQSSGLYSLSSVVTVPSSSLGTQTYICNVNHKPSNTKVDKRVEPKSCDKTHTCPPCPAPELLGGPSVFLFPPKPKDTLMISRTPEVTCVVVDVSHEDPEVKFNWYVDGVEVHNAKTKPREEQYNSTYRVVSVLTVLHQDWLNGKEYKCKVSNKALPAPIEKTISKAKGQPREPQVYTLPPSREEMTKNQVSLWCVVKGFYPSDIAVEWESNGQPENNYKTTPPVLDSDGSFFLQSKLTVDKSRWQQGNVFSCSVMHEALHNHYTQKSLSLSP

SEQ ID NO: 463 - protein, 447 aa, Homo sapiens
QVQLQESGPGLVRPSQTLSLTCTVSGYSITSDHAWSWVRQPPGRGLEWIGYISYSGITTYNPSLKSRVTMLRDTSKNQFSLRLSSVTAADTAVYYCARSLARTTAMDYWGQGSLVTVSSASTKGPSVFPLAPSSKSTSGGTAALGCLVKDYFPEPVTVSWNSGALTSGVHTFPAVLQSSGLYSLSSVVTVPSSSLGTQTYICNVNHKPSNTKVDKRVEPKSCDKTHTCPPCPAPELLGGPSVFLFPPKPKDTLMISRTPEVTCVVVDVSHEDPEVKFNWYVDGVEVHNAKTKPREEQYNSTYRVVSVLTVLHQDWLNGKEYKCKVSNKALPAPIEKTISKAKGQPREPQVYTLPPSREEMTKNQVSLWCGVKGFYPSDIAVEWESNGQPENNYKTTPPVLDSDGSFFLQSKLTVDKSRWQQGNVFSCSVMHEALHNHYTQKSLSLSP

SEQ ID NO: 464 - protein, 447 aa, Homo sapiens
QVQLQESGPGLVRPSQTLSLTCTVSGYSITSDHAWSWVRQPPGRGLEWIGYISYSGITTYNPSLKSRVTMLRDTSKNQFSLRLSSVTAADTAVYYCARSLARTTAMDYWGQGSLVTVSSASTKGPSVFPLAPSSKSTSGGTAALGCLVKDYFPEPVTVSWNSGALTSGVHTFPAVLQSSGLYSLSSVVTVPSSSLGTQTYICNVNHKPSNTKVDKRVEPKSCDKTHTCPPCPAPELLGGPSVFLFPPKPKDTLMISRTPEVTCVVVDVSHEDPEVKFNWYVDGVEVHNAKTKPREEQYNSTYRVVSVLTVLHQDWLNGKEYKCKVSNKALPAPIEKTISKAKGQPREPQVYTLPPSREEMTKNQVSLYCSVKGFYPSDIAVEWESNGQPENNYKTTPPVLDSDGSFFLLSKLTVDKSRWQQGNVFSCSVMHEALHNHYTQKSLSLSP

SEQ ID NO: 465 - protein, 447 aa, Homo sapiens
QVQLQESGPGLVRPSQTLSLTCTVSGYSITSDHAWSWVRQPPGRGLEWIGYISYSGITTYNPSLKSRVTMLRDTSKNQFSLRLSSVTAADTAVYYCARSLARTTAMDYWGQGSLVTVSSASTKGPSVFPLAPSSKSTSGGTAALGCLVKDYFPEPVTVSWNSGALTSGVHTFPAVLQSSGLYSLSSVVTVPSSSLGTQTYICNVNHKPSNTKVDKRVEPKSCDKTHTCPPCPAPELLGGPSVFLFPPKPKDTLMISRTPEVTCVVVDVSHEDPEVKFNWYVDGVEVHNAKTKPREEQYNSTYRVVSVLTVLHQDWLNGKEYKCKVSNKALPAPIEKTISKAKGQPREPQVYTLPPSREEMTKNQVSLYCCVKGFYPSDIAVEWESNGQPENNYKTTPPVLDSDGSFFLLSKLTVDKSRWQQGNVFSCSVMHEALHNHYTQKSLSLSP

SEQ ID NO: 466 - protein, 447 aa, Homo sapiens
QVQLQESGPGLVRPSQTLSLTCTVSGYSITSDHAWSWVRQPPGRGLEWIGYISYSGITTYNPSLKSRVTMLRDTSKNQFSLRLSSVTAADTAVYYCARSLARTTAMDYWGQGSLVTVSSASTKGPSVFPLAPSSKSTSGGTAALGCLVKDYFPEPVTVSWNSGALTSGVHTFPAVLQSSGLYSLSSVVTVPSSSLGTQTYICNVNHKPSNTKVDKRVEPKSCDKTHTCPPCPAPELLGGPSVFLFPPKPKDTLMISRTPEVTCVVVDVSHEDPEVKFNWYVDGVEVHNAKTKPREEQYNSTYRVVSVLTVLHQDWLNGKEYKCKVSNKALPAPIEKTISKAKGQPREPQVYTLPPSREEMTKNQVSLYCVVKGFYPSDIAVEWESNGQPENNYKTTPPVLDSDGSFFLLSKLTVDKSRWQQGNVFSCSVMHEALHNHYTQKSLSLSP

SEQ ID NO: 467 - protein, 447 aa, Homo sapiens
QVQLQESGPGLVRPSQTLSLTCTVSGYSITSDHAWSWVRQPPGRGLEWIGYISYSGITTYNPSLKSRVTMLRDTSKNQFSLRLSSVTAADTAVYYCARSLARTTAMDYWGQGSLVTVSSASTKGPSVFPLAPSSKSTSGGTAALGCLVKDYFPEPVTVSWNSGALTSGVHTFPAVLQSSGLYSLSSVVTVPSSSLGTQTYICNVNHKPSNTKVDKRVEPKSCDKTHTCPPCPAPELLGGPSVFLFPPKPKDTLMISRTPEVTCVVVDVSHEDPEVKFNWYVDGVEVHNAKTKPREEQYNSTYRVVSVLTVLHQDWLNGKEYKCKVSNKALPAPIEKTISKAKGQPREPQVYTLPPSREEMTKNQVSLYCGVKGFYPSDIAVEWESNGQPENNYKTTPPVLDSDGSFFLLSKLTVDKSRWQQGNVFSCSVMHEALHNHYTQKSLSLSP

SEQ ID NO: 468 - protein, 447 aa, Homo sapiens
QVQLQESGPGLVRPSQTLSLTCTVSGYSITSDHAWSWVRQPPGRGLEWIGYISYSGITTYNPSLKSRVTMLRDTSKNQFSLRLSSVTAADTAVYYCARSLARTTAMDYWGQGSLVTVSSASTKGPSVFPLAPSSKSTSGGTAALGCLVKDYFPEPVTVSWNSGALTSGVHTFPAVLQSSGLYSLSSVVTVPSSSLGTQTYICNVNHKPSNTKVDKRVEPKSCDKTHTCPPCPAPELLGGPSVFLFPPKPKDTLMISRTPEVTCVVVDVSHEDPEVKFNWYVDGVEVHNAKTKPREEQYNSTYRVVSVLTVLHQDWLNGKEYKCKVSNKALPAPIEKTISKAKGQPREPQVYTLPPSREEMTKNQVSLYCSVKGFYPSDIAVEWESNGQPENNYKTTPPVLDSDGSFFLISKLTVDKSRWQQGNVFSCSVMHEALHNHYTQKSLSLSP

SEQ ID NO: 469 - protein, 447 aa, Homo sapiens
QVQLQESGPGLVRPSQTLSLTCTVSGYSITSDHAWSWVRQPPGRGLEWIGYISYSGITTYNPSLKSRVTMLRDTSKNQFSLRLSSVTAADTAVYYCARSLARTTAMDYWGQGSLVTVSSASTKGPSVFPLAPSSKSTSGGTAALGCLVKDYFPEPVTVSWNSGALTSGVHTFPAVLQSSGLYSLSSVVTVPSSSLGTQTYICNVNHKPSNTKVDKRVEPKSCDKTHTCPPCPAPELLGGPSVFLFPPKPKDTLMISRTPEVTCVVVDVSHEDPEVKFNWYVDGVEVHNAKTKPREEQYNSTYRVVSVLTVLHQDWLNGKEYKCKVSNKALPAPIEKTISKAKGQPREPQVYTLPPSREEMTKNQVSLYCCVKGFYPSDIAVEWESNGQPENNYKTTPPVLDSDGSFFLISKLTVDKSRWQQGNVFSCSVMHEALHNHYTQKSLSLSP

SEQ ID NO: 470 - protein, 447 aa, Homo sapiens
QVQLQESGPGLVRPSQTLSLTCTVSGYSITSDHAWSWVRQPPGRGLEWIGYISYSGITTYNPSLKSRVTMLRDTSKNQFSLRLSSVTAADTAVYYCARSLARTTAMDYWGQGSLVTVSSASTKGPSVFPLAPSSKSTSGGTAALGCLVKDYFPEPVTVSWNSGALTSGVHTFPAVLQSSGLYSLSSVVTVPSSSLGTQTYICNVNHKPSNTKVDKRVEPKSCDKTHTCPPCPAPELLGGPSVFLFPPKPKDTLMISRTPEVTCVVVDVSHEDPEVKFNWYVDGVEVHNAKTKPREEQYNSTYRVVSVLTVLHQDWLNGKEYKCKVSNKALPAPIEKTISKAKGQPREPQVYTLPPSREEMTKNQVSLYCVVKGFYPSDIAVEWESNGQPENNYKTTPPVLDSDGSFFLISKLTVDKSRWQQGNVFSCSVMHEALHNHYTQKSLSLSP

SEQ ID NO: 471 - protein, 447 aa, Homo sapiens
QVQLQESGPGLVRPSQTLSLTCTVSGYSITSDHAWSWVRQPPGRGLEWIGYISYSGITTYNPSLKSRVTMLRDTSKNQFSLRLSSVTAADTAVYYCARSLARTTAMDYWGQGSLVTVSSASTKGPSVFPLAPSSKSTSGGTAALGCLVKDYFPEPVTVSWNSGALTSGVHTFPAVLQSSGLYSLSSVVTVPSSSLGTQTYICNVNHKPSNTKVDKRVEPKSCDKTHTCPPCPAPELLGGPSVFLFPPKPKDTLMISRTPEVTCVVVDVSHEDPEVKFNWYVDGVEVHNAKTKPREEQYNSTYRVVSVLTVLHQDWLNGKEYKCKVSNKALPAPIEKTISKAKGQPREPQVYTLPPSREEMTKNQVSLYCGVKGFYPSDIAVEWESNGQPENNYKTTPPVLDSDGSFFLISKLTVDKSRWQQGNVFSCSVMHEALHNHYTQKSLSLSP

SEQ ID NO: 472 - protein, 447 aa, Homo sapiens
QVQLQESGPGLVRPSQTLSLTCTVSGYSITSDHAWSWVRQPPGRGLEWIGYISYSGITTYNPSLKSRVTMLRDTSKNQFSLRLSSVTAADTAVYYCARSLARTTAMDYWGQGSLVTVSSASTKGPSVFPLAPSSKSTSGGTAALGCLVKDYFPEPVTVSWNSGALTSGVHTFPAVLQSSGLYSLSSVVTVPSSSLGTQTYICNVNHKPSNTKVDKRVEPKSCDKTHTCPPCPAPELLGGPSVFLFPPKPKDTLMISRTPEVTCVVVDVSHEDPEVKFNWYVDGVEVHNAKTKPREEQYNSTYRVVSVLTVLHQDWLNGKEYKCKVSNKALPAPIEKTISKAKGQPREPQVYTLPPSREEMTKNQVSLYCGVKGFYPSDIAVEWESNGQPENNYKTTPPVLDSDGSFFLMSKLTVDKSRWQQGNVFSCSVMHEALHNHYTQKSLSLSP

SEQ ID NO: 473 - protein, 447 aa, Homo sapiens
QVQLQESGPGLVRPSQTLSLTCTVSGYSITSDHAWSWVRQPPGRGLEWIGYISYSGITTYNPSLKSRVTMLRDTSKNQFSLRLSSVTAADTAVYYCARSLARTTAMDYWGQGSLVTVSSASTKGPSVFPLAPSSKSTSGGTAALGCLVKDYFPEPVTVSWNSGALTSGVHTFPAVLQSSGLYSLSSVVTVPSSSLGTQTYICNVNHKPSNTKVDKRVEPKSCDKTHTCPPCPAPELLGGPSVFLFPPKPKDTLMISRTPEVTCVVVDVSHEDPEVKFNWYVDGVEVHNAKTKPREEQYNSTYRVVSVLTVLHQDWLNGKEYKCKVSNKALPAPIEKTISKAKGQPREPQVYTLPPSREEMTKNQVSLYCVVKGFYPSDIAVEWESNGQPENNYKTTPPVLDSDGSFFLASKLTVDKSRWQQGNVFSCSVMHEALHNHYTQKSLSLSP

SEQ ID NO: 474 - protein, 447 aa, Homo sapiens
QVQLQESGPGLVRPSQTLSLTCTVSGYSITSDHAWSWVRQPPGRGLEWIGYISYSGITTYNPSLKSRVTMLRDTSKNQFSLRLSSVTAADTAVYYCARSLARTTAMDYWGQGSLVTVSSASTKGPSVFPLAPSSKSTSGGTAALGCLVKDYFPEPVTVSWNSGALTSGVHTFPAVLQSSGLYSLSSVVTVPSSSLGTQTYICNVNHKPSNTKVDKRVEPKSCDKTHTCPPCPAPELLGGPSVFLFPPKPKDTLMISRTPEVTCVVVDVSHEDPEVKFNWYVDGVEVHNAKTKPREEQYNSTYRVVSVLTVLHQDWLNGKEYKCKVSNKALPAPIEKTISKAKGQPREPQVYTLPPSREEMTKNQVSLYCGVKGFYPSDIAVEWESNGQPENNYKTTPPVLDSDGSFFLASKLTVDKSRWQQGNVFSCSVMHEALHNHYTQKSLSLSP

SEQ ID NO: 475 - protein, 447 aa, Homo sapiens
QVQLQESGPGLVRPSQTLSLTCTVSGYSITSDHAWSWVRQPPGRGLEWIGYISYSGITTYNPSLKSRVTMLRDTSKNQFSLRLSSVTAADTAVYYCARSLARTTAMDYWGQGSLVTVSSASTKGPSVFPLAPSSKSTSGGTAALGCLVKDYFPEPVTVSWNSGALTSGVHTFPAVLQSSGLYSLSSVVTVPSSSLGTQTYICNVNHKPSNTKVDKRVEPKSCDKTHTCPPCPAPELLGGPSVFLFPPKPKDTLMISRTPEVTCVVVDVSHEDPEVKFNWYVDGVEVHNAKTKPREEQYNSTYRVVSVLTVLHQDWLNGKEYKCKVSNKALPAPIEKTISKAKGQPREPQVYTLPPSREEMTKNQVSLYCSVKGFYPSDIAVEWESNGQPENNYKTTPPVLDSDGSFFLTSKLTVDKSRWQQGNVFSCSVMHEALHNHYTQKSLSLSP

SEQ ID NO: 476 - protein, 447 aa, Homo sapiens
QVQLQESGPGLVRPSQTLSLTCTVSGYSITSDHAWSWVRQPPGRGLEWIGYISYSGITTYNPSLKSRVTMLRDTSKNQFSLRLSSVTAADTAVYYCARSLARTTAMDYWGQGSLVTVSSASTKGPSVFPLAPSSKSTSGGTAALGCLVKDYFPEPVTVSWNSGALTSGVHTFPAVLQSSGLYSLSSVVTVPSSSLGTQTYICNVNHKPSNTKVDKRVEPKSCDKTHTCPPCPAPELLGGPSVFLFPPKPKDTLMISRTPEVTCVVVDVSHEDPEVKFNWYVDGVEVHNAKTKPREEQYNSTYRVVSVLTVLHQDWLNGKEYKCKVSNKALPAPIEKTISKAKGQPREPQVYTLPPSREEMTKNQVSLYCTVKGFYPSDIAVEWESNGQPENNYKTTPPVLDSDGSFFLTSKLTVDKSRWQQGNVFSCSVMHEALHNHYTQKSLSLSP

SEQ ID NO: 477 - protein, 447 aa, Homo sapiens
QVQLQESGPGLVRPSQTLSLTCTVSGYSITSDHAWSWVRQPPGRGLEWIGYISYSGITTYNPSLKSRVTMLRDTSKNQFSLRLSSVTAADTAVYYCARSLARTTAMDYWGQGSLVTVSSASTKGPSVFPLAPSSKSTSGGTAALGCLVKDYFPEPVTVSWNSGALTSGVHTFPAVLQSSGLYSLSSVVTVPSSSLGTQTYICNVNHKPSNTKVDKRVEPKSCDKTHTCPPCPAPELLGGPSVFLFPPKPKDTLMISRTPEVTCVVVDVSHEDPEVKFNWYVDGVEVHNAKTKPREEQYNSTYRVVSVLTVLHQDWLNGKEYKCKVSNKALPAPIEKTISKAKGQPREPQVYTLPPSREEMTKNQVSLYCCVKGFYPSDIAVEWESNGQPENNYKTTPPVLDSDGSFFLTSKLTVDKSRWQQGNVFSCSVMHEALHNHYTQKSLSLSP

SEQ ID NO: 478 - protein, 447 aa, Homo sapiens
QVQLQESGPGLVRPSQTLSLTCTVSGYSITSDHAWSWVRQPPGRGLEWIGYISYSGITTYNPSLKSRVTMLRDTSKNQFSLRLSSVTAADTAVYYCARSLARTTAMDYWGQGSLVTVSSASTKGPSVFPLAPSSKSTSGGTAALGCLVKDYFPEPVTVSWNSGALTSGVHTFPAVLQSSGLYSLSSVVTVPSSSLGTQTYICNVNHKPSNTKVDKRVEPKSCDKTHTCPPCPAPELLGGPSVFLFPPKPKDTLMISRTPEVTCVVVDVSHEDPEVKFNWYVDGVEVHNAKTKPREEQYNSTYRVVSVLTVLHQDWLNGKEYKCKVSNKALPAPIEKTISKAKGQPREPQVYTLPPSREEMTKNQVSLYCVVKGFYPSDIAVEWESNGQPENNYKTTPPVLDSDGSFFLTSKLTVDKSRWQQGNVFSCSVMHEALHNHYTQKSLSLSP

SEQ ID NO: 479 - protein, 447 aa, Homo sapiens
QVQLQESGPGLVRPSQTLSLTCTVSGYSITSDHAWSWVRQPPGRGLEWIGYISYSGITTYNPSLKSRVTMLRDTSKNQFSLRLSSVTAADTAVYYCARSLARTTAMDYWGQGSLVTVSSASTKGPSVFPLAPSSKSTSGGTAALGCLVKDYFPEPVTVSWNSGALTSGVHTFPAVLQSSGLYSLSSVVTVPSSSLGTQTYICNVNHKPSNTKVDKRVEPKSCDKTHTCPPCPAPELLGGPSVFLFPPKPKDTLMISRTPEVTCVVVDVSHEDPEVKFNWYVDGVEVHNAKTKPREEQYNSTYRVVSVLTVLHQDWLNGKEYKCKVSNKALPAPIEKTISKAKGQPREPQVYTLPPSREEMTKNQVSLYCGVKGFYPSDIAVEWESNGQPENNYKTTPPVLDSDGSFFLTSKLTVDKSRWQQGNVFSCSVMHEALHNHYTQKSLSLSP

SEQ ID NO: 480 - protein, 447 aa, Homo sapiens
QVQLQESGPGLVRPSQTLSLTCTVSGYSITSDHAWSWVRQPPGRGLEWIGYISYSGITTYNPSLKSRVTMLRDTSKNQFSLRLSSVTAADTAVYYCARSLARTTAMDYWGQGSLVTVSSASTKGPSVFPLAPSSKSTSGGTAALGCLVKDYFPEPVTVSWNSGALTSGVHTFPAVLQSSGLYSLSSVVTVPSSSLGTQTYICNVNHKPSNTKVDKRVEPKSCDKTHTCPPCPAPELLGGPSVFLFPPKPKDTLMISRTPEVTCVVVDVSHEDPEVKFNWYVDGVEVHNAKTKPREEQYNSTYRVVSVLTVLHQDWLNGKEYKCKVSNKALPAPIEKTISKAKGQPREPQVYTLPPSREEMTKNQVSLYCTVKGFYPSDIAVEWESNGQPENNYKTTPPVLDSDGSFFLCSKLTVDKSRWQQGNVFSCSVMHEALHNHYTQKSLSLSP

SEQ ID NO: 481 - protein, 447 aa, Homo sapiens
QVQLQESGPGLVRPSQTLSLTCTVSGYSITSDHAWSWVRQPPGRGLEWIGYISYSGITTYNPSLKSRVTMLRDTSKNQFSLRLSSVTAADTAVYYCARSLARTTAMDYWGQGSLVTVSSASTKGPSVFPLAPSSKSTSGGTAALGCLVKDYFPEPVTVSWNSGALTSGVHTFPAVLQSSGLYSLSSVVTVPSSSLGTQTYICNVNHKPSNTKVDKRVEPKSCDKTHTCPPCPAPELLGGPSVFLFPPKPKDTLMISRTPEVTCVVVDVSHEDPEVKFNWYVDGVEVHNAKTKPREEQYNSTYRVVSVLTVLHQDWLNGKEYKCKVSNKALPAPIEKTISKAKGQPREPQVYTLPPSREEMTKNQVSLYCVVKGFYPSDIAVEWESNGQPENNYKTTPPVLDSDGSFFLCSKLTVDKSRWQQGNVFSCSVMHEALHNHYTQKSLSLSP

SEQ ID NO: 482 - protein, 447 aa, Homo sapiens
QVQLQESGPGLVRPSQTLSLTCTVSGYSITSDHAWSWVRQPPGRGLEWIGYISYSGITTYNPSLKSRVTMLRDTSKNQFSLRLSSVTAADTAVYYCARSLARTTAMDYWGQGSLVTVSSASTKGPSVFPLAPSSKSTSGGTAALGCLVKDYFPEPVTVSWNSGALTSGVHTFPAVLQSSGLYSLSSVVTVPSSSLGTQTYICNVNHKPSNTKVDKRVEPKSCDKTHTCPPCPAPELLGGPSVFLFPPKPKDTLMISRTPEVTCVVVDVSHEDPEVKFNWYVDGVEVHNAKTKPREEQYNSTYRVVSVLTVLHQDWLNGKEYKCKVSNKALPAPIEKTISKAKGQPREPQVYTLPPSREEMTKNQVSLYCGVKGFYPSDIAVEWESNGQPENNYKTTPPVLDSDGSFFLCSKLTVDKSRWQQGNVFSCSVMHEALHNHYTQKSLSLSP

SEQ ID NO: 483 - protein, 447 aa, Homo sapiens
QVQLQESGPGLVRPSQTLSLTCTVSGYSITSDHAWSWVRQPPGRGLEWIGYISYSGITTYNPSLKSRVTMLRDTSKNQFSLRLSSVTAADTAVYYCARSLARTTAMDYWGQGSLVTVSSASTKGPSVFPLAPSSKSTSGGTAALGCLVKDYFPEPVTVSWNSGALTSGVHTFPAVLQSSGLYSLSSVVTVPSSSLGTQTYICNVNHKPSNTKVDKRVEPKSCDKTHTCPPCPAPELLGGPSVFLFPPKPKDTLMISRTPEVTCVVVDVSHEDPEVKFNWYVDGVEVHNAKTKPREEQYNSTYRVVSVLTVLHQDWLNGKEYKCKVSNKALPAPIEKTISKAKGQPREPQVYTLPPSREEMTKNQVSLYCSVKGFYPSDIAVEWESNGQPENNYKTTPPVLDSDGSFFLHSKLTVDKSRWQQGNVFSCSVMHEALHNHYTQKSLSLSP

SEQ ID NO: 484 - protein, 447 aa, Homo sapiens
QVQLQESGPGLVRPSQTLSLTCTVSGYSITSDHAWSWVRQPPGRGLEWIGYISYSGITTYNPSLKSRVTMLRDTSKNQFSLRLSSVTAADTAVYYCARSLARTTAMDYWGQGSLVTVSSASTKGPSVFPLAPSSKSTSGGTAALGCLVKDYFPEPVTVSWNSGALTSGVHTFPAVLQSSGLYSLSSVVTVPSSSLGTQTYICNVNHKPSNTKVDKRVEPKSCDKTHTCPPCPAPELLGGPSVFLFPPKPKDTLMISRTPEVTCVVVDVSHEDPEVKFNWYVDGVEVHNAKTKPREEQYNSTYRVVSVLTVLHQDWLNGKEYKCKVSNKALPAPIEKTISKAKGQPREPQVYTLPPSREEMTKNQVSLYCTVKGFYPSDIAVEWESNGQPENNYKTTPPVLDSDGSFFLHSKLTVDKSRWQQGNVFSCSVMHEALHNHYTQKSLSLSP

SEQ ID NO: 485 - protein, 447 aa, Homo sapiens
QVQLQESGPGLVRPSQTLSLTCTVSGYSITSDHAWSWVRQPPGRGLEWIGYISYSGITTYNPSLKSRVTMLRDTSKNQFSLRLSSVTAADTAVYYCARSLARTTAMDYWGQGSLVTVSSASTKGPSVFPLAPSSKSTSGGTAALGCLVKDYFPEPVTVSWNSGALTSGVHTFPAVLQSSGLYSLSSVVTVPSSSLGTQTYICNVNHKPSNTKVDKRVEPKSCDKTHTCPPCPAPELLGGPSVFLFPPKPKDTLMISRTPEVTCVVVDVSHEDPEVKFNWYVDGVEVHNAKTKPREEQYNSTYRVVSVLTVLHQDWLNGKEYKCKVSNKALPAPIEKTISKAKGQPREPQVYTLPPSREEMTKNQVSLYCCVKGFYPSDIAVEWESNGQPENNYKTTPPVLDSDGSFFLHSKLTVDKSRWQQGNVFSCSVMHEALHNHYTQKSLSLSP

SEQ ID NO: 486 - protein, 447 aa, Homo sapiens
QVQLQESGPGLVRPSQTLSLTCTVSGYSITSDHAWSWVRQPPGRGLEWIGYISYSGITTYNPSLKSRVTMLRDTSKNQFSLRLSSVTAADTAVYYCARSLARTTAMDYWGQGSLVTVSSASTKGPSVFPLAPSSKSTSGGTAALGCLVKDYFPEPVTVSWNSGALTSGVHTFPAVLQSSGLYSLSSVVTVPSSSLGTQTYICNVNHKPSNTKVDKRVEPKSCDKTHTCPPCPAPELLGGPSVFLFPPKPKDTLMISRTPEVTCVVVDVSHEDPEVKFNWYVDGVEVHNAKTKPREEQYNSTYRVVSVLTVLHQDWLNGKEYKCKVSNKALPAPIEKTISKAKGQPREPQVYTLPPSREEMTKNQVSLYCVVKGFYPSDIAVEWESNGQPENNYKTTPPVLDSDGSFFLHSKLTVDKSRWQQGNVFSCSVMHEALHNHYTQKSLSLSP

SEQ ID NO: 487 - protein, 447 aa, Homo sapiens
QVQLQESGPGLVRPSQTLSLTCTVSGYSITSDHAWSWVRQPPGRGLEWIGYISYSGITTYNPSLKSRVTMLRDTSKNQFSLRLSSVTAADTAVYYCARSLARTTAMDYWGQGSLVTVSSASTKGPSVFPLAPSSKSTSGGTAALGCLVKDYFPEPVTVSWNSGALTSGVHTFPAVLQSSGLYSLSSVVTVPSSSLGTQTYICNVNHKPSNTKVDKRVEPKSCDKTHTCPPCPAPELLGGPSVFLFPPKPKDTLMISRTPEVTCVVVDVSHEDPEVKFNWYVDGVEVHNAKTKPREEQYNSTYRVVSVLTVLHQDWLNGKEYKCKVSNKALPAPIEKTISKAKGQPREPQVYTLPPSREEMTKNQVSLYCGVKGFYPSDIAVEWESNGQPENNYKTTPPVLDSDGSFFLHSKLTVDKSRWQQGNVFSCSVMHEALHNHYTQKSLSLSP

SEQ ID NO: 488 - protein, 447 aa, Homo sapiens
QVQLQESGPGLVRPSQTLSLTCTVSGYSITSDHAWSWVRQPPGRGLEWIGYISYSGITTYNPSLKSRVTMLRDTSKNQFSLRLSSVTAADTAVYYCARSLARTTAMDYWGQGSLVTVSSASTKGPSVFPLAPSSKSTSGGTAALGCLVKDYFPEPVTVSWNSGALTSGVHTFPAVLQSSGLYSLSSVVTVPSSSLGTQTYICNVNHKPSNTKVDKRVEPKSCDKTHTCPPCPAPELLGGPSVFLFPPKPKDTLMISRTPEVTCVVVDVSHEDPEVKFNWYVDGVEVHNAKTKPREEQYNSTYRVVSVLTVLHQDWLNGKEYKCKVSNKALPAPIEKTISKAKGQPREPQVYTLPPSREEMTKNQVSLYCSVKGFYPSDIAVEWESNGQPENNYKTTPPVLDSDGSFFLNSKLTVDKSRWQQGNVFSCSVMHEALHNHYTQKSLSLSP

SEQ ID NO: 489 - protein, 447 aa, Homo sapiens
QVQLQESGPGLVRPSQTLSLTCTVSGYSITSDHAWSWVRQPPGRGLEWIGYISYSGITTYNPSLKSRVTMLRDTSKNQFSLRLSSVTAADTAVYYCARSLARTTAMDYWGQGSLVTVSSASTKGPSVFPLAPSSKSTSGGTAALGCLVKDYFPEPVTVSWNSGALTSGVHTFPAVLQSSGLYSLSSVVTVPSSSLGTQTYICNVNHKPSNTKVDKRVEPKSCDKTHTCPPCPAPELLGGPSVFLFPPKPKDTLMISRTPEVTCVVVDVSHEDPEVKFNWYVDGVEVHNAKTKPREEQYNSTYRVVSVLTVLHQDWLNGKEYKCKVSNKALPAPIEKTISKAKGQPREPQVYTLPPSREEMTKNQVSLYCTVKGFYPSDIAVEWESNGQPENNYKTTPPVLDSDGSFFLNSKLTVDKSRWQQGNVFSCSVMHEALHNHYTQKSLSLSP

SEQ ID NO: 490 - protein, 447 aa, Homo sapiens
QVQLQESGPGLVRPSQTLSLTCTVSGYSITSDHAWSWVRQPPGRGLEWIGYISYSGITTYNPSLKSRVTMLRDTSKNQFSLRLSSVTAADTAVYYCARSLARTTAMDYWGQGSLVTVSSASTKGPSVFPLAPSSKSTSGGTAALGCLVKDYFPEPVTVSWNSGALTSGVHTFPAVLQSSGLYSLSSVVTVPSSSLGTQTYICNVNHKPSNTKVDKRVEPKSCDKTHTCPPCPAPELLGGPSVFLFPPKPKDTLMISRTPEVTCVVVDVSHEDPEVKFNWYVDGVEVHNAKTKPREEQYNSTYRVVSVLTVLHQDWLNGKEYKCKVSNKALPAPIEKTISKAKGQPREPQVYTLPPSREEMTKNQVSLYCCVKGFYPSDIAVEWESNGQPENNYKTTPPVLDSDGSFFLNSKLTVDKSRWQQGNVFSCSVMHEALHNHYTQKSLSLSP

SEQ ID NO: 491 - protein, 447 aa, Homo sapiens
QVQLQESGPGLVRPSQTLSLTCTVSGYSITSDHAWSWVRQPPGRGLEWIGYISYSGITTYNPSLKSRVTMLRDTSKNQFSLRLSSVTAADTAVYYCARSLARTTAMDYWGQGSLVTVSSASTKGPSVFPLAPSSKSTSGGTAALGCLVKDYFPEPVTVSWNSGALTSGVHTFPAVLQSSGLYSLSSVVTVPSSSLGTQTYICNVNHKPSNTKVDKRVEPKSCDKTHTCPPCPAPELLGGPSVFLFPPKPKDTLMISRTPEVTCVVVDVSHEDPEVKFNWYVDGVEVHNAKTKPREEQYNSTYRVVSVLTVLHQDWLNGKEYKCKVSNKALPAPIEKTISKAKGQPREPQVYTLPPSREEMTKNQVSLYCVVKGFYPSDIAVEWESNGQPENNYKTTPPVLDSDGSFFLNSKLTVDKSRWQQGNVFSCSVMHEALHNHYTQKSLSLSP

SEQ ID NO: 492 - protein, 447 aa, Homo sapiens
QVQLQESGPGLVRPSQTLSLTCTVSGYSITSDHAWSWVRQPPGRGLEWIGYISYSGITTYNPSLKSRVTMLRDTSKNQFSLRLSSVTAADTAVYYCARSLARTTAMDYWGQGSLVTVSSASTKGPSVFPLAPSSKSTSGGTAALGCLVKDYFPEPVTVSWNSGALTSGVHTFPAVLQSSGLYSLSSVVTVPSSSLGTQTYICNVNHKPSNTKVDKRVEPKSCDKTHTCPPCPAPELLGGPSVFLFPPKPKDTLMISRTPEVTCVVVDVSHEDPEVKFNWYVDGVEVHNAKTKPREEQYNSTYRVVSVLTVLHQDWLNGKEYKCKVSNKALPAPIEKTISKAKGQPREPQVYTLPPSREEMTKNQVSLYCGVKGFYPSDIAVEWESNGQPENNYKTTPPVLDSDGSFFLNSKLTVDKSRWQQGNVFSCSVMHEALHNHYTQKSLSLSP

SEQ ID NO: 493 - protein, 447 aa, Homo sapiens
QVQLQESGPGLVRPSQTLSLTCTVSGYSITSDHAWSWVRQPPGRGLEWIGYISYSGITTYNPSLKSRVTMLRDTSKNQFSLRLSSVTAADTAVYYCARSLARTTAMDYWGQGSLVTVSSASTKGPSVFPLAPSSKSTSGGTAALGCLVKDYFPEPVTVSWNSGALTSGVHTFPAVLQSSGLYSLSSVVTVPSSSLGTQTYICNVNHKPSNTKVDKRVEPKSCDKTHTCPPCPAPELLGGPSVFLFPPKPKDTLMISRTPEVTCVVVDVSHEDPEVKFNWYVDGVEVHNAKTKPREEQYNSTYRVVSVLTVLHQDWLNGKEYKCKVSNKALPAPIEKTISKAKGQPREPQVYTLPPSREEMTKNQVSLYCSVKGFYPSDIAVEWESNGQPENNYKTTPPVLDSDGSFFLQSKLTVDKSRWQQGNVFSCSVMHEALHNHYTQKSLSLSP

SEQ ID NO: 494 - protein, 447 aa, Homo sapiens
QVQLQESGPGLVRPSQTLSLTCTVSGYSITSDHAWSWVRQPPGRGLEWIGYISYSGITTYNPSLKSRVTMLRDTSKNQFSLRLSSVTAADTAVYYCARSLARTTAMDYWGQGSLVTVSSASTKGPSVFPLAPSSKSTSGGTAALGCLVKDYFPEPVTVSWNSGALTSGVHTFPAVLQSSGLYSLSSVVTVPSSSLGTQTYICNVNHKPSNTKVDKRVEPKSCDKTHTCPPCPAPELLGGPSVFLFPPKPKDTLMISRTPEVTCVVVDVSHEDPEVKFNWYVDGVEVHNAKTKPREEQYNSTYRVVSVLTVLHQDWLNGKEYKCKVSNKALPAPIEKTISKAKGQPREPQVYTLPPSREEMTKNQVSLYCTVKGFYPSDIAVEWESNGQPENNYKTTPPVLDSDGSFFLQSKLTVDKSRWQQGNVFSCSVMHEALHNHYTQKSLSLSP

SEQ ID NO: 495 - protein, 447 aa, Homo sapiens
QVQLQESGPGLVRPSQTLSLTCTVSGYSITSDHAWSWVRQPPGRGLEWIGYISYSGITTYNPSLKSRVTMLRDTSKNQFSLRLSSVTAADTAVYYCARSLARTTAMDYWGQGSLVTVSSASTKGPSVFPLAPSSKSTSGGTAALGCLVKDYFPEPVTVSWNSGALTSGVHTFPAVLQSSGLYSLSSVVTVPSSSLGTQTYICNVNHKPSNTKVDKRVEPKSCDKTHTCPPCPAPELLGGPSVFLFPPKPKDTLMISRTPEVTCVVVDVSHEDPEVKFNWYVDGVEVHNAKTKPREEQYNSTYRVVSVLTVLHQDWLNGKEYKCKVSNKALPAPIEKTISKAKGQPREPQVYTLPPSREEMTKNQVSLYCCVKGFYPSDIAVEWESNGQPENNYKTTPPVLDSDGSFFLQSKLTVDKSRWQQGNVFSCSVMHEALHNHYTQKSLSLSP

SEQ ID NO: 496 - protein, 447 aa, Homo sapiens
QVQLQESGPGLVRPSQTLSLTCTVSGYSITSDHAWSWVRQPPGRGLEWIGYISYSGITTYNPSLKSRVTMLRDTSKNQFSLRLSSVTAADTAVYYCARSLARTTAMDYWGQGSLVTVSSASTKGPSVFPLAPSSKSTSGGTAALGCLVKDYFPEPVTVSWNSGALTSGVHTFPAVLQSSGLYSLSSVVTVPSSSLGTQTYICNVNHKPSNTKVDKRVEPKSCDKTHTCPPCPAPELLGGPSVFLFPPKPKDTLMISRTPEVTCVVVDVSHEDPEVKFNWYVDGVEVHNAKTKPREEQYNSTYRVVSVLTVLHQDWLNGKEYKCKVSNKALPAPIEKTISKAKGQPREPQVYTLPPSREEMTKNQVSLWCAVKGFYPSDIAVEWESNGQPENNYKTTPPVLDSDGSFFLQSKLTVDKSRWQQGNVFSCSVMHEALHNHYTQKSLSLSP

SEQ ID NO: 497 - protein, 447 aa, Homo sapiens
QVQLQESGPGLVRPSQTLSLTCTVSGYSITSDHAWSWVRQPPGRGLEWIGYISYSGITTYNPSLKSRVTMLRDTSKNQFSLRLSSVTAADTAVYYCARSLARTTAMDYWGQGSLVTVSSASTKGPSVFPLAPSSKSTSGGTAALGCLVKDYFPEPVTVSWNSGALTSGVHTFPAVLQSSGLYSLSSVVTVPSSSLGTQTYICNVNHKPSNTKVDKRVEPKSCDKTHTCPPCPAPELLGGPSVFLFPPKPKDTLMISRTPEVTCVVVDVSHEDPEVKFNWYVDGVEVHNAKTKPREEQYNSTYRVVSVLTVLHQDWLNGKEYKCKVSNKALPAPIEKTISKAKGQPREPQVYTLPPSREEMTKNQVSLWCTVKGFYPSDIAVEWESNGQPENNYKTTPPVLDSDGSFFLISKLTVDKSRWQQGNVFSCSVMHEALHNHYTQKSLSLSP

SEQ ID NO: 498 - protein, 447 aa, Homo sapiens
QVQLQESGPGLVRPSQTLSLTCTVSGYSITSDHAWSWVRQPPGRGLEWIGYISYSGITTYNPSLKSRVTMLRDTSKNQFSLRLSSVTAADTAVYYCARSLARTTAMDYWGQGSLVTVSSASTKGPSVFPLAPSSKSTSGGTAALGCLVKDYFPEPVTVSWNSGALTSGVHTFPAVLQSSGLYSLSSVVTVPSSSLGTQTYICNVNHKPSNTKVDKRVEPKSCDKTHTCPPCPAPELLGGPSVFLFPPKPKDTLMISRTPEVTCVVVDVSHEDPEVKFNWYVDGVEVHNAKTKPREEQYNSTYRVVSVLTVLHQDWLNGKEYKCKVSNKALPAPIEKTISKAKGQPREPQVYTLPPSREEMTKNQVSLWCCVKGFYPSDIAVEWESNGQPENNYKTTPPVLDSDGSFFLHSKLTVDKSRWQQGNVFSCSVMHEALHNHYTQKSLSLSP

SEQ ID NO: 499 - protein, 447 aa, Homo sapiens
QVQLQESGPGLVRPSQTLSLTCTVSGYSITSDHAWSWVRQPPGRGLEWIGYISYSGITTYNPSLKSRVTMLRDTSKNQFSLRLSSVTAADTAVYYCARSLARTTAMDYWGQGSLVTVSSASTKGPSVFPLAPSSKSTSGGTAALGCLVKDYFPEPVTVSWNSGALTSGVHTFPAVLQSSGLYSLSSVVTVPSSSLGTQTYICNVNHKPSNTKVDKRVEPKSCDKTHTCPPCPAPELLGGPSVFLFPPKPKDTLMISRTPEVTCVVVDVSHEDPEVKFNWYVDGVEVHNAKTKPREEQYNSTYRVVSVLTVLHQDWLNGKEYKCKVSNKALPAPIEKTISKAKGQPREPQVYTLPPSREEMTKNQVSLWCVVKGFYPSDIAVEWESNGQPENNYKTTPPVLDSDGSFFLNSKLTVDKSRWQQGNVFSCSVMHEALHNHYTQKSLSLSP

SEQ ID NO: 500 - protein, 447 aa, Homo sapiens
QVQLQESGPGLVRPSQTLSLTCTVSGYSITSDHAWSWVRQPPGRGLEWIGYISYSGITTYNPSLKSRVTMLRDTSKNQFSLRLSSVTAADTAVYYCARSLARTTAMDYWGQGSLVTVSSASTKGPSVFPLAPSSKSTSGGTAALGCLVKDYFPEPVTVSWNSGALTSGVHTFPAVLQSSGLYSLSSVVTVPSSSLGTQTYICNVNHKPSNTKVDKRVEPKSCDKTHTCPPCPAPELLGGPSVFLFPPKPKDTLMISRTPEVTCVVVDVSHEDPEVKFNWYVDGVEVHNAKTKPREEQYNSTYRVVSVLTVLHQDWLNGKEYKCKVSNKALPAPIEKTISKAKGQPREPQVYTLPPSREEMTKNQVSLYCTVKGFYPSDIAVEWESNGQPENNYKTTPPVLDSDGSFFLLSKLTVDKSRWQQGNVFSCSVMHEALHNHYTQKSLSLSP

SEQ ID NO: 501 - protein, 447 aa, Homo sapiens
QVQLQESGPGLVRPSQTLSLTCTVSGYSITSDHAWSWVRQPPGRGLEWIGYISYSGITTYNPSLKSRVTMLRDTSKNQFSLRLSSVTAADTAVYYCARSLARTTAMDYWGQGSLVTVSSASTKGPSVFPLAPSSKSTSGGTAALGCLVKDYFPEPVTVSWNSGALTSGVHTFPAVLQSSGLYSLSSVVTVPSSSLGTQTYICNVNHKPSNTKVDKRVEPKSCDKTHTCPPCPAPELLGGPSVFLFPPKPKDTLMISRTPEVTCVVVDVSHEDPEVKFNWYVDGVEVHNAKTKPREEQYNSTYRVVSVLTVLHQDWLNGKEYKCKVSNKALPAPIEKTISKAKGQPREPQVYTLPPSREEMTKNQVSLYCCVKGFYPSDIAVEWESNGQPENNYKTTPPVLDSDGSFFLCSKLTVDKSRWQQGNVFSCSVMHEALHNHYTQKSLSLSP

SEQ ID NO: 502 - protein, 447 aa, Homo sapiens
QVQLQESGPGLVRPSQTLSLTCTVSGYSITSDHAWSWVRQPPGRGLEWIGYISYSGITTYNPSLKSRVTMLRDTSKNQFSLRLSSVTAADTAVYYCARSLARTTAMDYWGQGSLVTVSSASTKGPSVFPLAPSSKSTSGGTAALGCLVKDYFPEPVTVSWNSGALTSGVHTFPAVLQSSGLYSLSSVVTVPSSSLGTQTYICNVNHKPSNTKVDKRVEPKSCDKTHTCPPCPAPELLGGPSVFLFPPKPKDTLMISRTPEVTCVVVDVSHEDPEVKFNWYVDGVEVHNAKTKPREEQYNSTYRVVSVLTVLHQDWLNGKEYKCKVSNKALPAPIEKTISKAKGQPREPQVYTLPPSREEMTKNQVSLFCSVKGFYPSDIAVEWESNGQPENNYKTTPPVLDSDGSFFLLSKLTVDKSRWQQGNVFSCSVMHEALHNHYTQKSLSLSP

SEQ ID NO: 503 - protein, 447 aa, Homo sapiens
QVQLQESGPGLVRPSQTLSLTCTVSGYSITSDHAWSWVRQPPGRGLEWIGYISYSGITTYNPSLKSRVTMLRDTSKNQFSLRLSSVTAADTAVYYCARSLARTTAMDYWGQGSLVTVSSASTKGPSVFPLAPSSKSTSGGTAALGCLVKDYFPEPVTVSWNSGALTSGVHTFPAVLQSSGLYSLSSVVTVPSSSLGTQTYICNVNHKPSNTKVDKRVEPKSCDKTHTCPPCPAPELLGGPSVFLFPPKPKDTLMISRTPEVTCVVVDVSHEDPEVKFNWYVDGVEVHNAKTKPREEQYNSTYRVVSVLTVLHQDWLNGKEYKCKVSNKALPAPIEKTISKAKGQPREPQVYTLPPSREEMTKNQVSLFCTVKGFYPSDIAVEWESNGQPENNYKTTPPVLDSDGSFFLLSKLTVDKSRWQQGNVFSCSVMHEALHNHYTQKSLSLSP

SEQ ID NO: 504 - protein, 447 aa, Homo sapiens
QVQLQESGPGLVRPSQTLSLTCTVSGYSITSDHAWSWVRQPPGRGLEWIGYISYSGITTYNPSLKSRVTMLRDTSKNQFSLRLSSVTAADTAVYYCARSLARTTAMDYWGQGSLVTVSSASTKGPSVFPLAPSSKSTSGGTAALGCLVKDYFPEPVTVSWNSGALTSGVHTFPAVLQSSGLYSLSSVVTVPSSSLGTQTYICNVNHKPSNTKVDKRVEPKSCDKTHTCPPCPAPELLGGPSVFLFPPKPKDTLMISRTPEVTCVVVDVSHEDPEVKFNWYVDGVEVHNAKTKPREEQYNSTYRVVSVLTVLHQDWLNGKEYKCKVSNKALPAPIEKTISKAKGQPREPQVYTLPPSREEMTKNQVSLFCCVKGFYPSDIAVEWESNGQPENNYKTTPPVLDSDGSFFLLSKLTVDKSRWQQGNVFSCSVMHEALHNHYTQKSLSLSP

SEQ ID NO: 505 - protein, 447 aa, Homo sapiens
QVQLQESGPGLVRPSQTLSLTCTVSGYSITSDHAWSWVRQPPGRGLEWIGYISYSGITTYNPSLKSRVTMLRDTSKNQFSLRLSSVTAADTAVYYCARSLARTTAMDYWGQGSLVTVSSASTKGPSVFPLAPSSKSTSGGTAALGCLVKDYFPEPVTVSWNSGALTSGVHTFPAVLQSSGLYSLSSVVTVPSSSLGTQTYICNVNHKPSNTKVDKRVEPKSCDKTHTCPPCPAPELLGGPSVFLFPPKPKDTLMISRTPEVTCVVVDVSHEDPEVKFNWYVDGVEVHNAKTKPREEQYNSTYRVVSVLTVLHQDWLNGKEYKCKVSNKALPAPIEKTISKAKGQPREPQVYTLPPSREEMTKNQVSLFCVVKGFYPSDIAVEWESNGQPENNYKTTPPVLDSDGSFFLLSKLTVDKSRWQQGNVFSCSVMHEALHNHYTQKSLSLSP

SEQ ID NO: 506 - protein, 447 aa, Homo sapiens
QVQLQESGPGLVRPSQTLSLTCTVSGYSITSDHAWSWVRQPPGRGLEWIGYISYSGITTYNPSLKSRVTMLRDTSKNQFSLRLSSVTAADTAVYYCARSLARTTAMDYWGQGSLVTVSSASTKGPSVFPLAPSSKSTSGGTAALGCLVKDYFPEPVTVSWNSGALTSGVHTFPAVLQSSGLYSLSSVVTVPSSSLGTQTYICNVNHKPSNTKVDKRVEPKSCDKTHTCPPCPAPELLGGPSVFLFPPKPKDTLMISRTPEVTCVVVDVSHEDPEVKFNWYVDGVEVHNAKTKPREEQYNSTYRVVSVLTVLHQDWLNGKEYKCKVSNKALPAPIEKTISKAKGQPREPQVYTLPPSREEMTKNQVSLFCGVKGFYPSDIAVEWESNGQPENNYKTTPPVLDSDGSFFLLSKLTVDKSRWQQGNVFSCSVMHEALHNHYTQKSLSLSP

SEQ ID NO: 507 - protein, 447 aa, Homo sapiens
QVQLQESGPGLVRPSQTLSLTCTVSGYSITSDHAWSWVRQPPGRGLEWIGYISYSGITTYNPSLKSRVTMLRDTSKNQFSLRLSSVTAADTAVYYCARSLARTTAMDYWGQGSLVTVSSASTKGPSVFPLAPSSKSTSGGTAALGCLVKDYFPEPVTVSWNSGALTSGVHTFPAVLQSSGLYSLSSVVTVPSSSLGTQTYICNVNHKPSNTKVDKRVEPKSCDKTHTCPPCPAPELLGGPSVFLFPPKPKDTLMISRTPEVTCVVVDVSHEDPEVKFNWYVDGVEVHNAKTKPREEQYNSTYRVVSVLTVLHQDWLNGKEYKCKVSNKALPAPIEKTISKAKGQPREPQVYTLPPSREEMTKNQVSLFCSVKGFYPSDIAVEWESNGQPENNYKTTPPVLDSDGSFFLISKLTVDKSRWQQGNVFSCSVMHEALHNHYTQKSLSLSP

SEQ ID NO: 508 - protein, 447 aa, Homo sapiens
QVQLQESGPGLVRPSQTLSLTCTVSGYSITSDHAWSWVRQPPGRGLEWIGYISYSGITTYNPSLKSRVTMLRDTSKNQFSLRLSSVTAADTAVYYCARSLARTTAMDYWGQGSLVTVSSASTKGPSVFPLAPSSKSTSGGTAALGCLVKDYFPEPVTVSWNSGALTSGVHTFPAVLQSSGLYSLSSVVTVPSSSLGTQTYICNVNHKPSNTKVDKRVEPKSCDKTHTCPPCPAPELLGGPSVFLFPPKPKDTLMISRTPEVTCVVVDVSHEDPEVKFNWYVDGVEVHNAKTKPREEQYNSTYRVVSVLTVLHQDWLNGKEYKCKVSNKALPAPIEKTISKAKGQPREPQVYTLPPSREEMTKNQVSLFCTVKGFYPSDIAVEWESNGQPENNYKTTPPVLDSDGSFFLISKLTVDKSRWQQGNVFSCSVMHEALHNHYTQKSLSLSP

SEQ ID NO: 509 - protein, 447 aa, Homo sapiens
QVQLQESGPGLVRPSQTLSLTCTVSGYSITSDHAWSWVRQPPGRGLEWIGYISYSGITTYNPSLKSRVTMLRDTSKNQFSLRLSSVTAADTAVYYCARSLARTTAMDYWGQGSLVTVSSASTKGPSVFPLAPSSKSTSGGTAALGCLVKDYFPEPVTVSWNSGALTSGVHTFPAVLQSSGLYSLSSVVTVPSSSLGTQTYICNVNHKPSNTKVDKRVEPKSCDKTHTCPPCPAPELLGGPSVFLFPPKPKDTLMISRTPEVTCVVVDVSHEDPEVKFNWYVDGVEVHNAKTKPREEQYNSTYRVVSVLTVLHQDWLNGKEYKCKVSNKALPAPIEKTISKAKGQPREPQVYTLPPSREEMTKNQVSLFCCVKGFYPSDIAVEWESNGQPENNYKTTPPVLDSDGSFFLISKLTVDKSRWQQGNVFSCSVMHEALHNHYTQKSLSLSP

SEQ ID NO: 510 - protein, 447 aa, Homo sapiens
QVQLQESGPGLVRPSQTLSLTCTVSGYSITSDHAWSWVRQPPGRGLEWIGYISYSGITTYNPSLKSRVTMLRDTSKNQFSLRLSSVTAADTAVYYCARSLARTTAMDYWGQGSLVTVSSASTKGPSVFPLAPSSKSTSGGTAALGCLVKDYFPEPVTVSWNSGALTSGVHTFPAVLQSSGLYSLSSVVTVPSSSLGTQTYICNVNHKPSNTKVDKRVEPKSCDKTHTCPPCPAPELLGGPSVFLFPPKPKDTLMISRTPEVTCVVVDVSHEDPEVKFNWYVDGVEVHNAKTKPREEQYNSTYRVVSVLTVLHQDWLNGKEYKCKVSNKALPAPIEKTISKAKGQPREPQVYTLPPSREEMTKNQVSLFCVVKGFYPSDIAVEWESNGQPENNYKTTPPVLDSDGSFFLISKLTVDKSRWQQGNVFSCSVMHEALHNHYTQKSLSLSP

SEQ ID NO: 511 - protein, 447 aa, Homo sapiens
QVQLQESGPGLVRPSQTLSLTCTVSGYSITSDHAWSWVRQPPGRGLEWIGYISYSGITTYNPSLKSRVTMLRDTSKNQFSLRLSSVTAADTAVYYCARSLARTTAMDYWGQGSLVTVSSASTKGPSVFPLAPSSKSTSGGTAALGCLVKDYFPEPVTVSWNSGALTSGVHTFPAVLQSSGLYSLSSVVTVPSSSLGTQTYICNVNHKPSNTKVDKRVEPKSCDKTHTCPPCPAPELLGGPSVFLFPPKPKDTLMISRTPEVTCVVVDVSHEDPEVKFNWYVDGVEVHNAKTKPREEQYNSTYRVVSVLTVLHQDWLNGKEYKCKVSNKALPAPIEKTISKAKGQPREPQVYTLPPSREEMTKNQVSLFCGVKGFYPSDIAVEWESNGQPENNYKTTPPVLDSDGSFFLISKLTVDKSRWQQGNVFSCSVMHEALHNHYTQKSLSLSP

SEQ ID NO: 512 - protein, 447 aa, Homo sapiens
QVQLQESGPGLVRPSQTLSLTCTVSGYSITSDHAWSWVRQPPGRGLEWIGYISYSGITTYNPSLKSRVTMLRDTSKNQFSLRLSSVTAADTAVYYCARSLARTTAMDYWGQGSLVTVSSASTKGPSVFPLAPSSKSTSGGTAALGCLVKDYFPEPVTVSWNSGALTSGVHTFPAVLQSSGLYSLSSVVTVPSSSLGTQTYICNVNHKPSNTKVDKRVEPKSCDKTHTCPPCPAPELLGGPSVFLFPPKPKDTLMISRTPEVTCVVVDVSHEDPEVKFNWYVDGVEVHNAKTKPREEQYNSTYRVVSVLTVLHQDWLNGKEYKCKVSNKALPAPIEKTISKAKGQPREPQVYTLPPSREEMTKNQVSLFCSVKGFYPSDIAVEWESNGQPENNYKTTPPVLDSDGSFFLMSKLTVDKSRWQQGNVFSCSVMHEALHNHYTQKSLSLSP

SEQ ID NO: 513 - protein, 447 aa, Homo sapiens
QVQLQESGPGLVRPSQTLSLTCTVSGYSITSDHAWSWVRQPPGRGLEWIGYISYSGITTYNPSLKSRVTMLRDTSKNQFSLRLSSVTAADTAVYYCARSLARTTAMDYWGQGSLVTVSSASTKGPSVFPLAPSSKSTSGGTAALGCLVKDYFPEPVTVSWNSGALTSGVHTFPAVLQSSGLYSLSSVVTVPSSSLGTQTYICNVNHKPSNTKVDKRVEPKSCDKTHTCPPCPAPELLGGPSVFLFPPKPKDTLMISRTPEVTCVVVDVSHEDPEVKFNWYVDGVEVHNAKTKPREEQYNSTYRVVSVLTVLHQDWLNGKEYKCKVSNKALPAPIEKTISKAKGQPREPQVYTLPPSREEMTKNQVSLFCTVKGFYPSDIAVEWESNGQPENNYKTTPPVLDSDGSFFLMSKLTVDKSRWQQGNVFSCSVMHEALHNHYTQKSLSLSP

SEQ ID NO: 514 - protein, 447 aa, Homo sapiens
QVQLQESGPGLVRPSQTLSLTCTVSGYSITSDHAWSWVRQPPGRGLEWIGYISYSGITTYNPSLKSRVTMLRDTSKNQFSLRLSSVTAADTAVYYCARSLARTTAMDYWGQGSLVTVSSASTKGPSVFPLAPSSKSTSGGTAALGCLVKDYFPEPVTVSWNSGALTSGVHTFPAVLQSSGLYSLSSVVTVPSSSLGTQTYICNVNHKPSNTKVDKRVEPKSCDKTHTCPPCPAPELLGGPSVFLFPPKPKDTLMISRTPEVTCVVVDVSHEDPEVKFNWYVDGVEVHNAKTKPREEQYNSTYRVVSVLTVLHQDWLNGKEYKCKVSNKALPAPIEKTISKAKGQPREPQVYTLPPSREEMTKNQVSLFCCVKGFYPSDIAVEWESNGQPENNYKTTPPVLDSDGSFFLMSKLTVDKSRWQQGNVFSCSVMHEALHNHYTQKSLSLSP

SEQ ID NO: 515 - protein, 447 aa, Homo sapiens
QVQLQESGPGLVRPSQTLSLTCTVSGYSITSDHAWSWVRQPPGRGLEWIGYISYSGITTYNPSLKSRVTMLRDTSKNQFSLRLSSVTAADTAVYYCARSLARTTAMDYWGQGSLVTVSSASTKGPSVFPLAPSSKSTSGGTAALGCLVKDYFPEPVTVSWNSGALTSGVHTFPAVLQSSGLYSLSSVVTVPSSSLGTQTYICNVNHKPSNTKVDKRVEPKSCDKTHTCPPCPAPELLGGPSVFLFPPKPKDTLMISRTPEVTCVVVDVSHEDPEVKFNWYVDGVEVHNAKTKPREEQYNSTYRVVSVLTVLHQDWLNGKEYKCKVSNKALPAPIEKTISKAKGQPREPQVYTLPPSREEMTKNQVSLFCVVKGFYPSDIAVEWESNGQPENNYKTTPPVLDSDGSFFLMSKLTVDKSRWQQGNVFSCSVMHEALHNHYTQKSLSLSP

SEQ ID NO: 516 - protein, 447 aa, Homo sapiens
QVQLQESGPGLVRPSQTLSLTCTVSGYSITSDHAWSWVRQPPGRGLEWIGYISYSGITTYNPSLKSRVTMLRDTSKNQFSLRLSSVTAADTAVYYCARSLARTTAMDYWGQGSLVTVSSASTKGPSVFPLAPSSKSTSGGTAALGCLVKDYFPEPVTVSWNSGALTSGVHTFPAVLQSSGLYSLSSVVTVPSSSLGTQTYICNVNHKPSNTKVDKRVEPKSCDKTHTCPPCPAPELLGGPSVFLFPPKPKDTLMISRTPEVTCVVVDVSHEDPEVKFNWYVDGVEVHNAKTKPREEQYNSTYRVVSVLTVLHQDWLNGKEYKCKVSNKALPAPIEKTISKAKGQPREPQVYTLPPSREEMTKNQVSLFCGVKGFYPSDIAVEWESNGQPENNYKTTPPVLDSDGSFFLMSKLTVDKSRWQQGNVFSCSVMHEALHNHYTQKSLSLSP

SEQ ID NO: 517 - protein, 447 aa, Homo sapiens
QVQLQESGPGLVRPSQTLSLTCTVSGYSITSDHAWSWVRQPPGRGLEWIGYISYSGITTYNPSLKSRVTMLRDTSKNQFSLRLSSVTAADTAVYYCARSLARTTAMDYWGQGSLVTVSSASTKGPSVFPLAPSSKSTSGGTAALGCLVKDYFPEPVTVSWNSGALTSGVHTFPAVLQSSGLYSLSSVVTVPSSSLGTQTYICNVNHKPSNTKVDKRVEPKSCDKTHTCPPCPAPELLGGPSVFLFPPKPKDTLMISRTPEVTCVVVDVSHEDPEVKFNWYVDGVEVHNAKTKPREEQYNSTYRVVSVLTVLHQDWLNGKEYKCKVSNKALPAPIEKTISKAKGQPREPQVYTLPPSREEMTKNQVSLFCSVKGFYPSDIAVEWESNGQPENNYKTTPPVLDSDGSFFLASKLTVDKSRWQQGNVFSCSVMHEALHNHYTQKSLSLSP

SEQ ID NO: 518 - protein, 447 aa, Homo sapiens
QVQLQESGPGLVRPSQTLSLTCTVSGYSITSDHAWSWVRQPPGRGLEWIGYISYSGITTYNPSLKSRVTMLRDTSKNQFSLRLSSVTAADTAVYYCARSLARTTAMDYWGQGSLVTVSSASTKGPSVFPLAPSSKSTSGGTAALGCLVKDYFPEPVTVSWNSGALTSGVHTFPAVLQSSGLYSLSSVVTVPSSSLGTQTYICNVNHKPSNTKVDKRVEPKSCDKTHTCPPCPAPELLGGPSVFLFPPKPKDTLMISRTPEVTCVVVDVSHEDPEVKFNWYVDGVEVHNAKTKPREEQYNSTYRVVSVLTVLHQDWLNGKEYKCKVSNKALPAPIEKTISKAKGQPREPQVYTLPPSREEMTKNQVSLFCTVKGFYPSDIAVEWESNGQPENNYKTTPPVLDSDGSFFLASKLTVDKSRWQQGNVFSCSVMHEALHNHYTQKSLSLSP

SEQ ID NO: 519 - protein, 447 aa, Homo sapiens
QVQLQESGPGLVRPSQTLSLTCTVSGYSITSDHAWSWVRQPPGRGLEWIGYISYSGITTYNPSLKSRVTMLRDTSKNQFSLRLSSVTAADTAVYYCARSLARTTAMDYWGQGSLVTVSSASTKGPSVFPLAPSSKSTSGGTAALGCLVKDYFPEPVTVSWNSGALTSGVHTFPAVLQSSGLYSLSSVVTVPSSSLGTQTYICNVNHKPSNTKVDKRVEPKSCDKTHTCPPCPAPELLGGPSVFLFPPKPKDTLMISRTPEVTCVVVDVSHEDPEVKFNWYVDGVEVHNAKTKPREEQYNSTYRVVSVLTVLHQDWLNGKEYKCKVSNKALPAPIEKTISKAKGQPREPQVYTLPPSREEMTKNQVSLFCCVKGFYPSDIAVEWESNGQPENNYKTTPPVLDSDGSFFLASKLTVDKSRWQQGNVFSCSVMHEALHNHYTQKSLSLSP

SEQ ID NO: 520 - protein, 447 aa, Homo sapiens
QVQLQESGPGLVRPSQTLSLTCTVSGYSITSDHAWSWVRQPPGRGLEWIGYISYSGITTYNPSLKSRVTMLRDTSKNQFSLRLSSVTAADTAVYYCARSLARTTAMDYWGQGSLVTVSSASTKGPSVFPLAPSSKSTSGGTAALGCLVKDYFPEPVTVSWNSGALTSGVHTFPAVLQSSGLYSLSSVVTVPSSSLGTQTYICNVNHKPSNTKVDKRVEPKSCDKTHTCPPCPAPELLGGPSVFLFPPKPKDTLMISRTPEVTCVVVDVSHEDPEVKFNWYVDGVEVHNAKTKPREEQYNSTYRVVSVLTVLHQDWLNGKEYKCKVSNKALPAPIEKTISKAKGQPREPQVYTLPPSREEMTKNQVSLFCVVKGFYPSDIAVEWESNGQPENNYKTTPPVLDSDGSFFLASKLTVDKSRWQQGNVFSCSVMHEALHNHYTQKSLSLSP

SEQ ID NO: 521 - protein, 447 aa, Homo sapiens
QVQLQESGPGLVRPSQTLSLTCTVSGYSITSDHAWSWVRQPPGRGLEWIGYISYSGITTYNPSLKSRVTMLRDTSKNQFSLRLSSVTAADTAVYYCARSLARTTAMDYWGQGSLVTVSSASTKGPSVFPLAPSSKSTSGGTAALGCLVKDYFPEPVTVSWNSGALTSGVHTFPAVLQSSGLYSLSSVVTVPSSSLGTQTYICNVNHKPSNTKVDKRVEPKSCDKTHTCPPCPAPELLGGPSVFLFPPKPKDTLMISRTPEVTCVVVDVSHEDPEVKFNWYVDGVEVHNAKTKPREEQYNSTYRVVSVLTVLHQDWLNGKEYKCKVSNKALPAPIEKTISKAKGQPREPQVYTLPPSREEMTKNQVSLFCGVKGFYPSDIAVEWESNGQPENNYKTTPPVLDSDGSFFLASKLTVDKSRWQQGNVFSCSVMHEALHNHYTQKSLSLSP

SEQ ID NO: 522 - protein, 447 aa, Homo sapiens
QVQLQESGPGLVRPSQTLSLTCTVSGYSITSDHAWSWVRQPPGRGLEWIGYISYSGITTYNPSLKSRVTMLRDTSKNQFSLRLSSVTAADTAVYYCARSLARTTAMDYWGQGSLVTVSSASTKGPSVFPLAPSSKSTSGGTAALGCLVKDYFPEPVTVSWNSGALTSGVHTFPAVLQSSGLYSLSSVVTVPSSSLGTQTYICNVNHKPSNTKVDKRVEPKSCDKTHTCPPCPAPELLGGPSVFLFPPKPKDTLMISRTPEVTCVVVDVSHEDPEVKFNWYVDGVEVHNAKTKPREEQYNSTYRVVSVLTVLHQDWLNGKEYKCKVSNKALPAPIEKTISKAKGQPREPQVYTLPPSREEMTKNQVSLFCSVKGFYPSDIAVEWESNGQPENNYKTTPPVLDSDGSFFLTSKLTVDKSRWQQGNVFSCSVMHEALHNHYTQKSLSLSP

SEQ ID NO: 523 - protein, 447 aa, Homo sapiens
QVQLQESGPGLVRPSQTLSLTCTVSGYSITSDHAWSWVRQPPGRGLEWIGYISYSGITTYNPSLKSRVTMLRDTSKNQFSLRLSSVTAADTAVYYCARSLARTTAMDYWGQGSLVTVSSASTKGPSVFPLAPSSKSTSGGTAALGCLVKDYFPEPVTVSWNSGALTSGVHTFPAVLQSSGLYSLSSVVTVPSSSLGTQTYICNVNHKPSNTKVDKRVEPKSCDKTHTCPPCPAPELLGGPSVFLFPPKPKDTLMISRTPEVTCVVVDVSHEDPEVKFNWYVDGVEVHNAKTKPREEQYNSTYRVVSVLTVLHQDWLNGKEYKCKVSNKALPAPIEKTISKAKGQPREPQVYTLPPSREEMTKNQVSLFCTVKGFYPSDIAVEWESNGQPENNYKTTPPVLDSDGSFFLTSKLTVDKSRWQQGNVFSCSVMHEALHNHYTQKSLSLSP

SEQ ID NO: 524 - protein, 447 aa, Homo sapiens
QVQLQESGPGLVRPSQTLSLTCTVSGYSITSDHAWSWVRQPPGRGLEWIGYISYSGITTYNPSLKSRVTMLRDTSKNQFSLRLSSVTAADTAVYYCARSLARTTAMDYWGQGSLVTVSSASTKGPSVFPLAPSSKSTSGGTAALGCLVKDYFPEPVTVSWNSGALTSGVHTFPAVLQSSGLYSLSSVVTVPSSSLGTQTYICNVNHKPSNTKVDKRVEPKSCDKTHTCPPCPAPELLGGPSVFLFPPKPKDTLMISRTPEVTCVVVDVSHEDPEVKFNWYVDGVEVHNAKTKPREEQYNSTYRVVSVLTVLHQDWLNGKEYKCKVSNKALPAPIEKTISKAKGQPREPQVYTLPPSREEMTKNQVSLFCCVKGFYPSDIAVEWESNGQPENNYKTTPPVLDSDGSFFLTSKLTVDKSRWQQGNVFSCSVMHEALHNHYTQKSLSLSP

SEQ ID NO: 525 - protein, 447 aa, Homo sapiens
QVQLQESGPGLVRPSQTLSLTCTVSGYSITSDHAWSWVRQPPGRGLEWIGYISYSGITTYNPSLKSRVTMLRDTSKNQFSLRLSSVTAADTAVYYCARSLARTTAMDYWGQGSLVTVSSASTKGPSVFPLAPSSKSTSGGTAALGCLVKDYFPEPVTVSWNSGALTSGVHTFPAVLQSSGLYSLSSVVTVPSSSLGTQTYICNVNHKPSNTKVDKRVEPKSCDKTHTCPPCPAPELLGGPSVFLFPPKPKDTLMISRTPEVTCVVVDVSHEDPEVKFNWYVDGVEVHNAKTKPREEQYNSTYRVVSVLTVLHQDWLNGKEYKCKVSNKALPAPIEKTISKAKGQPREPQVYTLPPSREEMTKNQVSLFCVVKGFYPSDIAVEWESNGQPENNYKTTPPVLDSDGSFFLTSKLTVDKSRWQQGNVFSCSVMHEALHNHYTQKSLSLSP

SEQ ID NO: 526 - protein, 447 aa, Homo sapiens
QVQLQESGPGLVRPSQTLSLTCTVSGYSITSDHAWSWVRQPPGRGLEWIGYISYSGITTYNPSLKSRVTMLRDTSKNQFSLRLSSVTAADTAVYYCARSLARTTAMDYWGQGSLVTVSSASTKGPSVFPLAPSSKSTSGGTAALGCLVKDYFPEPVTVSWNSGALTSGVHTFPAVLQSSGLYSLSSVVTVPSSSLGTQTYICNVNHKPSNTKVDKRVEPKSCDKTHTCPPCPAPELLGGPSVFLFPPKPKDTLMISRTPEVTCVVVDVSHEDPEVKFNWYVDGVEVHNAKTKPREEQYNSTYRVVSVLTVLHQDWLNGKEYKCKVSNKALPAPIEKTISKAKGQPREPQVYTLPPSREEMTKNQVSLFCGVKGFYPSDIAVEWESNGQPENNYKTTPPVLDSDGSFFLTSKLTVDKSRWQQGNVFSCSVMHEALHNHYTQKSLSLSP

SEQ ID NO: 527 - protein, 447 aa, Homo sapiens
QVQLQESGPGLVRPSQTLSLTCTVSGYSITSDHAWSWVRQPPGRGLEWIGYISYSGITTYNPSLKSRVTMLRDTSKNQFSLRLSSVTAADTAVYYCARSLARTTAMDYWGQGSLVTVSSASTKGPSVFPLAPSSKSTSGGTAALGCLVKDYFPEPVTVSWNSGALTSGVHTFPAVLQSSGLYSLSSVVTVPSSSLGTQTYICNVNHKPSNTKVDKRVEPKSCDKTHTCPPCPAPELLGGPSVFLFPPKPKDTLMISRTPEVTCVVVDVSHEDPEVKFNWYVDGVEVHNAKTKPREEQYNSTYRVVSVLTVLHQDWLNGKEYKCKVSNKALPAPIEKTISKAKGQPREPQVYTLPPSREEMTKNQVSLFCSVKGFYPSDIAVEWESNGQPENNYKTTPPVLDSDGSFFLCSKLTVDKSRWQQGNVFSCSVMHEALHNHYTQKSLSLSP

SEQ ID NO: 528 - protein, 447 aa, Homo sapiens
QVQLQESGPGLVRPSQTLSLTCTVSGYSITSDHAWSWVRQPPGRGLEWIGYISYSGITTYNPSLKSRVTMLRDTSKNQFSLRLSSVTAADTAVYYCARSLARTTAMDYWGQGSLVTVSSASTKGPSVFPLAPSSKSTSGGTAALGCLVKDYFPEPVTVSWNSGALTSGVHTFPAVLQSSGLYSLSSVVTVPSSSLGTQTYICNVNHKPSNTKVDKRVEPKSCDKTHTCPPCPAPELLGGPSVFLFPPKPKDTLMISRTPEVTCVVVDVSHEDPEVKFNWYVDGVEVHNAKTKPREEQYNSTYRVVSVLTVLHQDWLNGKEYKCKVSNKALPAPIEKTISKAKGQPREPQVYTLPPSREEMTKNQVSLFCTVKGFYPSDIAVEWESNGQPENNYKTTPPVLDSDGSFFLCSKLTVDKSRWQQGNVFSCSVMHEALHNHYTQKSLSLSP

SEQ ID NO: 529 - protein, 447 aa, Homo sapiens
QVQLQESGPGLVRPSQTLSLTCTVSGYSITSDHAWSWVRQPPGRGLEWIGYISYSGITTYNPSLKSRVTMLRDTSKNQFSLRLSSVTAADTAVYYCARSLARTTAMDYWGQGSLVTVSSASTKGPSVFPLAPSSKSTSGGTAALGCLVKDYFPEPVTVSWNSGALTSGVHTFPAVLQSSGLYSLSSVVTVPSSSLGTQTYICNVNHKPSNTKVDKRVEPKSCDKTHTCPPCPAPELLGGPSVFLFPPKPKDTLMISRTPEVTCVVVDVSHEDPEVKFNWYVDGVEVHNAKTKPREEQYNSTYRVVSVLTVLHQDWLNGKEYKCKVSNKALPAPIEKTISKAKGQPREPQVYTLPPSREEMTKNQVSLFCVVKGFYPSDIAVEWESNGQPENNYKTTPPVLDSDGSFFLCSKLTVDKSRWQQGNVFSCSVMHEALHNHYTQKSLSLSP

SEQ ID NO: 530 - protein, 447 aa, Homo sapiens
QVQLQESGPGLVRPSQTLSLTCTVSGYSITSDHAWSWVRQPPGRGLEWIGYISYSGITTYNPSLKSRVTMLRDTSKNQFSLRLSSVTAADTAVYYCARSLARTTAMDYWGQGSLVTVSSASTKGPSVFPLAPSSKSTSGGTAALGCLVKDYFPEPVTVSWNSGALTSGVHTFPAVLQSSGLYSLSSVVTVPSSSLGTQTYICNVNHKPSNTKVDKRVEPKSCDKTHTCPPCPAPELLGGPSVFLFPPKPKDTLMISRTPEVTCVVVDVSHEDPEVKFNWYVDGVEVHNAKTKPREEQYNSTYRVVSVLTVLHQDWLNGKEYKCKVSNKALPAPIEKTISKAKGQPREPQVYTLPPSREEMTKNQVSLFCGVKGFYPSDIAVEWESNGQPENNYKTTPPVLDSDGSFFLCSKLTVDKSRWQQGNVFSCSVMHEALHNHYTQKSLSLSP

SEQ ID NO: 531 - protein, 447 aa, Homo sapiens
QVQLQESGPGLVRPSQTLSLTCTVSGYSITSDHAWSWVRQPPGRGLEWIGYISYSGITTYNPSLKSRVTMLRDTSKNQFSLRLSSVTAADTAVYYCARSLARTTAMDYWGQGSLVTVSSASTKGPSVFPLAPSSKSTSGGTAALGCLVKDYFPEPVTVSWNSGALTSGVHTFPAVLQSSGLYSLSSVVTVPSSSLGTQTYICNVNHKPSNTKVDKRVEPKSCDKTHTCPPCPAPELLGGPSVFLFPPKPKDTLMISRTPEVTCVVVDVSHEDPEVKFNWYVDGVEVHNAKTKPREEQYNSTYRVVSVLTVLHQDWLNGKEYKCKVSNKALPAPIEKTISKAKGQPREPQVYTLPPSREEMTKNQVSLFCSVKGFYPSDIAVEWESNGQPENNYKTTPPVLDSDGSFFLHSKLTVDKSRWQQGNVFSCSVMHEALHNHYTQKSLSLSP

SEQ ID NO: 532 - protein, 447 aa, Homo sapiens
QVQLQESGPGLVRPSQTLSLTCTVSGYSITSDHAWSWVRQPPGRGLEWIGYISYSGITTYNPSLKSRVTMLRDTSKNQFSLRLSSVTAADTAVYYCARSLARTTAMDYWGQGSLVTVSSASTKGPSVFPLAPSSKSTSGGTAALGCLVKDYFPEPVTVSWNSGALTSGVHTFPAVLQSSGLYSLSSVVTVPSSSLGTQTYICNVNHKPSNTKVDKRVEPKSCDKTHTCPPCPAPELLGGPSVFLFPPKPKDTLMISRTPEVTCVVVDVSHEDPEVKFNWYVDGVEVHNAKTKPREEQYNSTYRVVSVLTVLHQDWLNGKEYKCKVSNKALPAPIEKTISKAKGQPREPQVYTLPPSREEMTKNQVSLFCTVKGFYPSDIAVEWESNGQPENNYKTTPPVLDSDGSFFLHSKLTVDKSRWQQGNVFSCSVMHEALHNHYTQKSLSLSP

SEQ ID NO: 533 - protein, 447 aa, Homo sapiens
QVQLQESGPGLVRPSQTLSLTCTVSGYSITSDHAWSWVRQPPGRGLEWIGYISYSGITTYNPSLKSRVTMLRDTSKNQFSLRLSSVTAADTAVYYCARSLARTTAMDYWGQGSLVTVSSASTKGPSVFPLAPSSKSTSGGTAALGCLVKDYFPEPVTVSWNSGALTSGVHTFPAVLQSSGLYSLSSVVTVPSSSLGTQTYICNVNHKPSNTKVDKRVEPKSCDKTHTCPPCPAPELLGGPSVFLFPPKPKDTLMISRTPEVTCVVVDVSHEDPEVKFNWYVDGVEVHNAKTKPREEQYNSTYRVVSVLTVLHQDWLNGKEYKCKVSNKALPAPIEKTISKAKGQPREPQVYTLPPSREEMTKNQVSLFCCVKGFYPSDIAVEWESNGQPENNYKTTPPVLDSDGSFFLHSKLTVDKSRWQQGNVFSCSVMHEALHNHYTQKSLSLSP

SEQ ID NO: 534 - protein, 447 aa, Homo sapiens
QVQLQESGPGLVRPSQTLSLTCTVSGYSITSDHAWSWVRQPPGRGLEWIGYISYSGITTYNPSLKSRVTMLRDTSKNQFSLRLSSVTAADTAVYYCARSLARTTAMDYWGQGSLVTVSSASTKGPSVFPLAPSSKSTSGGTAALGCLVKDYFPEPVTVSWNSGALTSGVHTFPAVLQSSGLYSLSSVVTVPSSSLGTQTYICNVNHKPSNTKVDKRVEPKSCDKTHTCPPCPAPELLGGPSVFLFPPKPKDTLMISRTPEVTCVVVDVSHEDPEVKFNWYVDGVEVHNAKTKPREEQYNSTYRVVSVLTVLHQDWLNGKEYKCKVSNKALPAPIEKTISKAKGQPREPQVYTLPPSREEMTKNQVSLFCGVKGFYPSDIAVEWESNGQPENNYKTTPPVLDSDGSFFLHSKLTVDKSRWQQGNVFSCSVMHEALHNHYTQKSLSLSP

SEQ ID NO: 535 - protein, 447 aa, Homo sapiens
QVQLQESGPGLVRPSQTLSLTCTVSGYSITSDHAWSWVRQPPGRGLEWIGYISYSGITTYNPSLKSRVTMLRDTSKNQFSLRLSSVTAADTAVYYCARSLARTTAMDYWGQGSLVTVSSASTKGPSVFPLAPSSKSTSGGTAALGCLVKDYFPEPVTVSWNSGALTSGVHTFPAVLQSSGLYSLSSVVTVPSSSLGTQTYICNVNHKPSNTKVDKRVEPKSCDKTHTCPPCPAPELLGGPSVFLFPPKPKDTLMISRTPEVTCVVVDVSHEDPEVKFNWYVDGVEVHNAKTKPREEQYNSTYRVVSVLTVLHQDWLNGKEYKCKVSNKALPAPIEKTISKAKGQPREPQVYTLPPSREEMTKNQVSLFCSVKGFYPSDIAVEWESNGQPENNYKTTPPVLDSDGSFFLNSKLTVDKSRWQQGNVFSCSVMHEALHNHYTQKSLSLSP

SEQ ID NO: 536 - protein, 447 aa, Homo sapiens
QVQLQESGPGLVRPSQTLSLTCTVSGYSITSDHAWSWVRQPPGRGLEWIGYISYSGITTYNPSLKSRVTMLRDTSKNQFSLRLSSVTAADTAVYYCARSLARTTAMDYWGQGSLVTVSSASTKGPSVFPLAPSSKSTSGGTAALGCLVKDYFPEPVTVSWNSGALTSGVHTFPAVLQSSGLYSLSSVVTVPSSSLGTQTYICNVNHKPSNTKVDKRVEPKSCDKTHTCPPCPAPELLGGPSVFLFPPKPKDTLMISRTPEVTCVVVDVSHEDPEVKFNWYVDGVEVHNAKTKPREEQYNSTYRVVSVLTVLHQDWLNGKEYKCKVSNKALPAPIEKTISKAKGQPREPQVYTLPPSREEMTKNQVSLFCCVKGFYPSDIAVEWESNGQPENNYKTTPPVLDSDGSFFLNSKLTVDKSRWQQGNVFSCSVMHEALHNHYTQKSLSLSP

SEQ ID NO: 537 - protein, 447 aa, Homo sapiens
QVQLQESGPGLVRPSQTLSLTCTVSGYSITSDHAWSWVRQPPGRGLEWIGYISYSGITTYNPSLKSRVTMLRDTSKNQFSLRLSSVTAADTAVYYCARSLARTTAMDYWGQGSLVTVSSASTKGPSVFPLAPSSKSTSGGTAALGCLVKDYFPEPVTVSWNSGALTSGVHTFPAVLQSSGLYSLSSVVTVPSSSLGTQTYICNVNHKPSNTKVDKRVEPKSCDKTHTCPPCPAPELLGGPSVFLFPPKPKDTLMISRTPEVTCVVVDVSHEDPEVKFNWYVDGVEVHNAKTKPREEQYNSTYRVVSVLTVLHQDWLNGKEYKCKVSNKALPAPIEKTISKAKGQPREPQVYTLPPSREEMTKNQVSLFCVVKGFYPSDIAVEWESNGQPENNYKTTPPVLDSDGSFFLNSKLTVDKSRWQQGNVFSCSVMHEALHNHYTQKSLSLSP

SEQ ID NO: 538 - protein, 447 aa, Homo sapiens
QVQLQESGPGLVRPSQTLSLTCTVSGYSITSDHAWSWVRQPPGRGLEWIGYISYSGITTYNPSLKSRVTMLRDTSKNQFSLRLSSVTAADTAVYYCARSLARTTAMDYWGQGSLVTVSSASTKGPSVFPLAPSSKSTSGGTAALGCLVKDYFPEPVTVSWNSGALTSGVHTFPAVLQSSGLYSLSSVVTVPSSSLGTQTYICNVNHKPSNTKVDKRVEPKSCDKTHTCPPCPAPELLGGPSVFLFPPKPKDTLMISRTPEVTCVVVDVSHEDPEVKFNWYVDGVEVHNAKTKPREEQYNSTYRVVSVLTVLHQDWLNGKEYKCKVSNKALPAPIEKTISKAKGQPREPQVYTLPPSREEMTKNQVSLFCGVKGFYPSDIAVEWESNGQPENNYKTTPPVLDSDGSFFLNSKLTVDKSRWQQGNVFSCSVMHEALHNHYTQKSLSLSP

SEQ ID NO: 539 - protein, 447 aa, Homo sapiens
QVQLQESGPGLVRPSQTLSLTCTVSGYSITSDHAWSWVRQPPGRGLEWIGYISYSGITTYNPSLKSRVTMLRDTSKNQFSLRLSSVTAADTAVYYCARSLARTTAMDYWGQGSLVTVSSASTKGPSVFPLAPSSKSTSGGTAALGCLVKDYFPEPVTVSWNSGALTSGVHTFPAVLQSSGLYSLSSVVTVPSSSLGTQTYICNVNHKPSNTKVDKRVEPKSCDKTHTCPPCPAPELLGGPSVFLFPPKPKDTLMISRTPEVTCVVVDVSHEDPEVKFNWYVDGVEVHNAKTKPREEQYNSTYRVVSVLTVLHQDWLNGKEYKCKVSNKALPAPIEKTISKAKGQPREPQVYTLPPSREEMTKNQVSLFCSVKGFYPSDIAVEWESNGQPENNYKTTPPVLDSDGSFFLQSKLTVDKSRWQQGNVFSCSVMHEALHNHYTQKSLSLSP

SEQ ID NO: 540 - protein, 447 aa, Homo sapiens
QVQLQESGPGLVRPSQTLSLTCTVSGYSITSDHAWSWVRQPPGRGLEWIGYISYSGITTYNPSLKSRVTMLRDTSKNQFSLRLSSVTAADTAVYYCARSLARTTAMDYWGQGSLVTVSSASTKGPSVFPLAPSSKSTSGGTAALGCLVKDYFPEPVTVSWNSGALTSGVHTFPAVLQSSGLYSLSSVVTVPSSSLGTQTYICNVNHKPSNTKVDKRVEPKSCDKTHTCPPCPAPELLGGPSVFLFPPKPKDTLMISRTPEVTCVVVDVSHEDPEVKFNWYVDGVEVHNAKTKPREEQYNSTYRVVSVLTVLHQDWLNGKEYKCKVSNKALPAPIEKTISKAKGQPREPQVYTLPPSREEMTKNQVSLFCTVKGFYPSDIAVEWESNGQPENNYKTTPPVLDSDGSFFLQSKLTVDKSRWQQGNVFSCSVMHEALHNHYTQKSLSLSP

SEQ ID NO: 541 - protein, 447 aa, Homo sapiens
QVQLQESGPGLVRPSQTLSLTCTVSGYSITSDHAWSWVRQPPGRGLEWIGYISYSGITTYNPSLKSRVTMLRDTSKNQFSLRLSSVTAADTAVYYCARSLARTTAMDYWGQGSLVTVSSASTKGPSVFPLAPSSKSTSGGTAALGCLVKDYFPEPVTVSWNSGALTSGVHTFPAVLQSSGLYSLSSVVTVPSSSLGTQTYICNVNHKPSNTKVDKRVEPKSCDKTHTCPPCPAPELLGGPSVFLFPPKPKDTLMISRTPEVTCVVVDVSHEDPEVKFNWYVDGVEVHNAKTKPREEQYNSTYRVVSVLTVLHQDWLNGKEYKCKVSNKALPAPIEKTISKAKGQPREPQVYTLPPSREEMTKNQVSLFCCVKGFYPSDIAVEWESNGQPENNYKTTPPVLDSDGSFFLQSKLTVDKSRWQQGNVFSCSVMHEALHNHYTQKSLSLSP

SEQ ID NO: 542 - protein, 447 aa, Homo sapiens
QVQLQESGPGLVRPSQTLSLTCTVSGYSITSDHAWSWVRQPPGRGLEWIGYISYSGITTYNPSLKSRVTMLRDTSKNQFSLRLSSVTAADTAVYYCARSLARTTAMDYWGQGSLVTVSSASTKGPSVFPLAPSSKSTSGGTAALGCLVKDYFPEPVTVSWNSGALTSGVHTFPAVLQSSGLYSLSSVVTVPSSSLGTQTYICNVNHKPSNTKVDKRVEPKSCDKTHTCPPCPAPELLGGPSVFLFPPKPKDTLMISRTPEVTCVVVDVSHEDPEVKFNWYVDGVEVHNAKTKPREEQYNSTYRVVSVLTVLHQDWLNGKEYKCKVSNKALPAPIEKTISKAKGQPREPQVYTLPPSREEMTKNQVSLFCVVKGFYPSDIAVEWESNGQPENNYKTTPPVLDSDGSFFLQSKLTVDKSRWQQGNVFSCSVMHEALHNHYTQKSLSLSP

SEQ ID NO: 543 - protein, 447 aa, Homo sapiens
QVQLQESGPGLVRPSQTLSLTCTVSGYSITSDHAWSWVRQPPGRGLEWIGYISYSGITTYNPSLKSRVTMLRDTSKNQFSLRLSSVTAADTAVYYCARSLARTTAMDYWGQGSLVTVSSASTKGPSVFPLAPSSKSTSGGTAALGCLVKDYFPEPVTVSWNSGALTSGVHTFPAVLQSSGLYSLSSVVTVPSSSLGTQTYICNVNHKPSNTKVDKRVEPKSCDKTHTCPPCPAPELLGGPSVFLFPPKPKDTLMISRTPEVTCVVVDVSHEDPEVKFNWYVDGVEVHNAKTKPREEQYNSTYRVVSVLTVLHQDWLNGKEYKCKVSNKALPAPIEKTISKAKGQPREPQVYTLPPSREEMTKNQVSLFCGVKGFYPSDIAVEWESNGQPENNYKTTPPVLDSDGSFFLQSKLTVDKSRWQQGNVFSCSVMHEALHNHYTQKSLSLSP

SEQ ID NO: 544 - protein, 447 aa, Homo sapiens
QVQLQESGPGLVRPSQTLSLTCTVSGYSITSDHAWSWVRQPPGRGLEWIGYISYSGITTYNPSLKSRVTMLRDTSKNQFSLRLSSVTAADTAVYYCARSLARTTAMDYWGQGSLVTVSSASTKGPSVFPLAPSSKSTSGGTAALGCLVKDYFPEPVTVSWNSGALTSGVHTFPAVLQSSGLYSLSSVVTVPSSSLGTQTYICNVNHKPSNTKVDKRVEPKSCDKTHTCPPCPAPELLGGPSVFLFPPKPKDTLMISRTPEVTCVVVDVSHEDPEVKFNWYVDGVEVHNAKTKPREEQYNSTYRVVSVLTVLHQDWLNGKEYKCKVSNKALPAPIEKTISKAKGQPREPQVYTLPPSREEMTKNQVSLFCCVKGFYPSDIAVEWESNGQPENNYKTTPPVLDSDGSFFLCSKLTVDKSRWQQGNVFSCSVMHEALHNHYTQKSLSLSP

SEQ ID NO: 545 - protein, 447 aa, Homo sapiens
QVQLQESGPGLVRPSQTLSLTCTVSGYSITSDHAWSWVRQPPGRGLEWIGYISYSGITTYNPSLKSRVTMLRDTSKNQFSLRLSSVTAADTAVYYCARSLARTTAMDYWGQGSLVTVSSASTKGPSVFPLAPSSKSTSGGTAALGCLVKDYFPEPVTVSWNSGALTSGVHTFPAVLQSSGLYSLSSVVTVPSSSLGTQTYICNVNHKPSNTKVDKRVEPKSCDKTHTCPPCPAPELLGGPSVFLFPPKPKDTLMISRTPEVTCVVVDVSHEDPEVKFNWYVDGVEVHNAKTKPREEQYNSTYRVVSVLTVLHQDWLNGKEYKCKVSNKALPAPIEKTISKAKGQPREPQVYTLPPSREEMTKNQVSLYCTVKGFYPSDIAVEWESNGQPENNYKTTPPVLDSDGSFFLISKLTVDKSRWQQGNVFSCSVMHEALHNHYTQKSLSLSP

SEQ ID NO: 546 - protein, 447 aa, Homo sapiens
QVQLQESGPGLVRPSQTLSLTCTVSGYSITSDHAWSWVRQPPGRGLEWIGYISYSGITTYNPSLKSRVTMLRDTSKNQFSLRLSSVTAADTAVYYCARSLARTTAMDYWGQGSLVTVSSASTKGPSVFPLAPSSKSTSGGTAALGCLVKDYFPEPVTVSWNSGALTSGVHTFPAVLQSSGLYSLSSVVTVPSSSLGTQTYICNVNHKPSNTKVDKRVEPKSCDKTHTCPPCPAPELLGGPSVFLFPPKPKDTLMISRTPEVTCVVVDVSHEDPEVKFNWYVDGVEVHNAKTKPREEQYNSTYRVVSVLTVLHQDWLNGKEYKCKVSNKALPAPIEKTISKAKGQPREPQVYTLPPSREEMTKNQVSLFCVVKGFYPSDIAVEWESNGQPENNYKTTPPVLDSDGSFFLHSKLTVDKSRWQQGNVFSCSVMHEALHNHYTQKSLSLSP

SEQ ID NO: 547 - protein, 447 aa, Homo sapiens
QVQLQESGPGLVRPSQTLSLTCTVSGYSITSDHAWSWVRQPPGRGLEWIGYISYSGITTYNPSLKSRVTMLRDTSKNQFSLRLSSVTAADTAVYYCARSLARTTAMDYWGQGSLVTVSSASTKGPSVFPLAPSSKSTSGGTAALGCLVKDYFPEPVTVSWNSGALTSGVHTFPAVLQSSGLYSLSSVVTVPSSSLGTQTYICNVNHKPSNTKVDKRVEPKSCDKTHTCPPCPAPELLGGPSVFLFPPKPKDTLMISRTPEVTCVVVDVSHEDPEVKFNWYVDGVEVHNAKTKPREEQYNSTYRVVSVLTVLHQDWLNGKEYKCKVSNKALPAPIEKTISKAKGQPREPQVYTLPPSREEMTKNQVSLFCTVKGFYPSDIAVEWESNGQPENNYKTTPPVLDSDGSFFLNSKLTVDKSRWQQGNVFSCSVMHEALHNHYTQKSLSLSP

SEQ ID NO: 548 - protein, 447 aa, Homo sapiens
QVQLQESGPGLVRPSQTLSLTCTVSGYSITSDHAWSWVRQPPGRGLEWIGYISYSGITTYNPSLKSRVTMLRDTSKNQFSLRLSSVTAADTAVYYCARSLARTTAMDYWGQGSLVTVSSASTKGPSVFPLAPSSKSTSGGTAALGCLVKDYFPEPVTVSWNSGALTSGVHTFPAVLQSSGLYSLSSVVTVPSSSLGTQTYICNVNHKPSNTKVDKRVEPKSCDKTHTCPPCPAPELLGGPSVFLFPPKPKDTLMISRTPEVTCVVVDVSHEDPEVKFNWYVDGVEVHNAKTKPREEQYNSTYRVVSVLTVLHQDWLNGKEYKCKVSNKALPAPIEKTISKAKGQPREPQVYTLPPSREEMTKNQVSLYCSVKGFYPSDIAVEWESNGQPENNYKTTPPVLDSDGSFFLCSKLTVDKSRWQQGNVFSCSVMHEALHNHYTQKSLSLSP

SEQ ID NO: 549 - protein, 447 aa, Homo sapiens
QVQLQESGPGLVRPSQTLSLTCTVSGYSITSDHAWSWVRQPPGRGLEWIGYISYSGITTYNPSLKSRVTMLRDTSKNQFSLRLSSVTAADTAVYYCARSLARTTAMDYWGQGSLVTVSSASTKGPSVFPLAPSSKSTSGGTAALGCLVKDYFPEPVTVSWNSGALTSGVHTFPAVLQSSGLYSLSSVVTVPSSSLGTQTYICNVNHKPSNTKVDKRVEPKSCDKTHTCPPCPAPELLGGPSVFLFPPKPKDTLMISRTPEVTCVVVDVSHEDPEVKFNWYVDGVEVHNAKTKPREEQYNSTYRVVSVLTVLHQDWLNGKEYKCKVSNKALPAPIEKTISKAKGQPREPQVYTLPPSREEMTKNQVSLYCVVKGFYPSDIAVEWESNGQPENNYKTTPPVLDSDGSFFLQSKLTVDKSRWQQGNVFSCSVMHEALHNHYTQKSLSLSP

SEQ ID NO: 550 - protein, 447 aa, Homo sapiens
QVQLQESGPGLVRPSQTLSLTCTVSGYSITSDHAWSWVRQPPGRGLEWIGYISYSGITTYNPSLKSRVTMLRDTSKNQFSLRLSSVTAADTAVYYCARSLARTTAMDYWGQGSLVTVSSASTKGPSVFPLAPSSKSTSGGTAALGCLVKDYFPEPVTVSWNSGALTSGVHTFPAVLQSSGLYSLSSVVTVPSSSLGTQTYICNVNHKPSNTKVDKRVEPKSCDKTHTCPPCPAPELLGGPSVFLFPPKPKDTLMISRTPEVTCVVVDVSHEDPEVKFNWYVDGVEVHNAKTKPREEQYNSTYRVVSVLTVLHQDWLNGKEYKCKVSNKALPAPIEKTISKAKGQPREPQVYTLPPSREEMTKNQVSLYCSVKGFYPSDIAVEWESNGQPENNYKTTPPVLDSDGSFFLMSKLTVDKSRWQQGNVFSCSVMHEALHNHYTQKSLSLSP

SEQ ID NO: 551 - protein, 447 aa, Homo sapiens
QVQLQESGPGLVRPSQTLSLTCTVSGYSITSDHAWSWVRQPPGRGLEWIGYISYSGITTYNPSLKSRVTMLRDTSKNQFSLRLSSVTAADTAVYYCARSLARTTAMDYWGQGSLVTVSSASTKGPSVFPLAPSSKSTSGGTAALGCLVKDYFPEPVTVSWNSGALTSGVHTFPAVLQSSGLYSLSSVVTVPSSSLGTQTYICNVNHKPSNTKVDKRVEPKSCDKTHTCPPCPAPELLGGPSVFLFPPKPKDTLMISRTPEVTCVVVDVSHEDPEVKFNWYVDGVEVHNAKTKPREEQYNSTYRVVSVLTVLHQDWLNGKEYKCKVSNKALPAPIEKTISKAKGQPREPQVYTLPPSREEMTKNQVSLYCTVKGFYPSDIAVEWESNGQPENNYKTTPPVLDSDGSFFLMSKLTVDKSRWQQGNVFSCSVMHEALHNHYTQKSLSLSP

SEQ ID NO: 552 - protein, 447 aa, Homo sapiens
QVQLQESGPGLVRPSQTLSLTCTVSGYSITSDHAWSWVRQPPGRGLEWIGYISYSGITTYNPSLKSRVTMLRDTSKNQFSLRLSSVTAADTAVYYCARSLARTTAMDYWGQGSLVTVSSASTKGPSVFPLAPSSKSTSGGTAALGCLVKDYFPEPVTVSWNSGALTSGVHTFPAVLQSSGLYSLSSVVTVPSSSLGTQTYICNVNHKPSNTKVDKRVEPKSCDKTHTCPPCPAPELLGGPSVFLFPPKPKDTLMISRTPEVTCVVVDVSHEDPEVKFNWYVDGVEVHNAKTKPREEQYNSTYRVVSVLTVLHQDWLNGKEYKCKVSNKALPAPIEKTISKAKGQPREPQVYTLPPSREEMTKNQVSLYCCVKGFYPSDIAVEWESNGQPENNYKTTPPVLDSDGSFFLMSKLTVDKSRWQQGNVFSCSVMHEALHNHYTQKSLSLSP

SEQ ID NO: 553 - protein, 447 aa, Homo sapiens
QVQLQESGPGLVRPSQTLSLTCTVSGYSITSDHAWSWVRQPPGRGLEWIGYISYSGITTYNPSLKSRVTMLRDTSKNQFSLRLSSVTAADTAVYYCARSLARTTAMDYWGQGSLVTVSSASTKGPSVFPLAPSSKSTSGGTAALGCLVKDYFPEPVTVSWNSGALTSGVHTFPAVLQSSGLYSLSSVVTVPSSSLGTQTYICNVNHKPSNTKVDKRVEPKSCDKTHTCPPCPAPELLGGPSVFLFPPKPKDTLMISRTPEVTCVVVDVSHEDPEVKFNWYVDGVEVHNAKTKPREEQYNSTYRVVSVLTVLHQDWLNGKEYKCKVSNKALPAPIEKTISKAKGQPREPQVYTLPPSREEMTKNQVSLYCVVKGFYPSDIAVEWESNGQPENNYKTTPPVLDSDGSFFLMSKLTVDKSRWQQGNVFSCSVMHEALHNHYTQKSLSLSP

SEQ ID NO: 554 - protein, 447 aa, Homo sapiens
QVQLQESGPGLVRPSQTLSLTCTVSGYSITSDHAWSWVRQPPGRGLEWIGYISYSGITTYNPSLKSRVTMLRDTSKNQFSLRLSSVTAADTAVYYCARSLARTTAMDYWGQGSLVTVSSASTKGPSVFPLAPSSKSTSGGTAALGCLVKDYFPEPVTVSWNSGALTSGVHTFPAVLQSSGLYSLSSVVTVPSSSLGTQTYICNVNHKPSNTKVDKRVEPKSCDKTHTCPPCPAPELLGGPSVFLFPPKPKDTLMISRTPEVTCVVVDVSHEDPEVKFNWYVDGVEVHNAKTKPREEQYNSTYRVVSVLTVLHQDWLNGKEYKCKVSNKALPAPIEKTISKAKGQPREPQVYTLPPSREEMTKNQVSLYCSVKGFYPSDIAVEWESNGQPENNYKTTPPVLDSDGSFFLASKLTVDKSRWQQGNVFSCSVMHEALHNHYTQKSLSLSP

SEQ ID NO: 555 - protein, 447 aa, Homo sapiens
QVQLQESGPGLVRPSQTLSLTCTVSGYSITSDHAWSWVRQPPGRGLEWIGYISYSGITTYNPSLKSRVTMLRDTSKNQFSLRLSSVTAADTAVYYCARSLARTTAMDYWGQGSLVTVSSASTKGPSVFPLAPSSKSTSGGTAALGCLVKDYFPEPVTVSWNSGALTSGVHTFPAVLQSSGLYSLSSVVTVPSSSLGTQTYICNVNHKPSNTKVDKRVEPKSCDKTHTCPPCPAPELLGGPSVFLFPPKPKDTLMISRTPEVTCVVVDVSHEDPEVKFNWYVDGVEVHNAKTKPREEQYNSTYRVVSVLTVLHQDWLNGKEYKCKVSNKALPAPIEKTISKAKGQPREPQVYTLPPSREEMTKNQVSLYCTVKGFYPSDIAVEWESNGQPENNYKTTPPVLDSDGSFFLASKLTVDKSRWQQGNVFSCSVMHEALHNHYTQKSLSLSP

SEQ ID NO: 556 - protein, 447 aa, Homo sapiens
QVQLQESGPGLVRPSQTLSLTCTVSGYSITSDHAWSWVRQPPGRGLEWIGYISYSGITTYNPSLKSRVTMLRDTSKNQFSLRLSSVTAADTAVYYCARSLARTTAMDYWGQGSLVTVSSASTKGPSVFPLAPSSKSTSGGTAALGCLVKDYFPEPVTVSWNSGALTSGVHTFPAVLQSSGLYSLSSVVTVPSSSLGTQTYICNVNHKPSNTKVDKRVEPKSCDKTHTCPPCPAPELLGGPSVFLFPPKPKDTLMISRTPEVTCVVVDVSHEDPEVKFNWYVDGVEVHNAKTKPREEQYNSTYRVVSVLTVLHQDWLNGKEYKCKVSNKALPAPIEKTISKAKGQPREPQVYTLPPSREEMTKNQVSLYCCVKGFYPSDIAVEWESNGQPENNYKTTPPVLDSDGSFFLASKLTVDKSRWQQGNVFSCSVMHEALHNHYTQKSLSLSP

SEQ ID NO: 557 - protein, 447 aa, Homo sapiens
QVQLQESGPGLVRPSQTLSLTCTVSGYSITSDHAWSWVRQPPGRGLEWIGYISYSGITTYNPSLKSRVTMLRDTSKNQFSLRLSSVTAADTAVYYCARSLARTTAMDYWGQGSLVTVSSASTKGPSVFPLAPSSKSTSGGTAALGCLVKDYFPEPVTVSWNSGALTSGVHTFPAVLQSSGLYSLSSVVTVPSSSLGTQTYICNVNHKPSNTKVDKRVEPKSCDKTHTCPPCPAPELLGGPSVFLFPPKPKDTLMISRTPEVTCVVVDVSHEDPEVKFNWYVDGVEVHNAKTKPREEQYNSTYRVVSVLTVLHQDWLNGKEYKCKVSNKALPAPIEKTISKAKGQPREPQVYTLPPSREEMTKNQVSLYCGVKGFYPSDIAVEWESNGQPENNYKTTPPVLDSDGSFFLQSKLTVDKSRWQQGNVFSCSVMHEALHNHYTQKSLSLSP

SEQ ID NO: 558 - protein, 447 aa, Homo sapiens
QVQLQESGPGLVRPSQTLSLTCTVSGYSITSDHAWSWVRQPPGRGLEWIGYISYSGITTYNPSLKSRVTMLRDTSKNQFSLRLSSVTAADTAVYYCARSLARTTAMDYWGQGSLVTVSSASTKGPSVFPLAPSSKSTSGGTAALGCLVKDYFPEPVTVSWNSGALTSGVHTFPAVLQSSGLYSLSSVVTVPSSSLGTQTYICNVNHKPSNTKVDKRVEPKSCDKTHTCPPCPAPELLGGPSVFLFPPKPKDTLMISRTPEVTCVVVDVSHEDPEVKFNWYVDGVEVHNAKTKPREEQYNSTYRVVSVLTVLHQDWLNGKEYKCKVSNKALPAPIEKTISKAKGQPREPRVYTLPPSREEMTENQVSLTCLVKGFYPSDIAVEWESNGQPENNYKTTPPVLISDGSFTLYSYLTVDKSRWQQGNVFSCSVMHEALHNHYTQKSLSLSP

SEQ ID NO: 559 - protein, 447 aa, Homo sapiens
QVQLQESGPGLVRPSQTLSLTCTVSGYSITSDHAWSWVRQPPGRGLEWIGYISYSGITTYNPSLKSRVTMLRDTSKNQFSLRLSSVTAADTAVYYCARSLARTTAMDYWGQGSLVTVSSASTKGPSVFPLAPSSKSTSGGTAALGCLVKDYFPEPVTVSWNSGALTSGVHTFPAVLQSSGLYSLSSVVTVPSSSLGTQTYICNVNHKPSNTKVDKRVEPKSCDKTHTCPPCPAPELLGGPSVFLFPPKPKDTLMISRTPEVTCVVVDVSHEDPEVKFNWYVDGVEVHNAKTKPREEQYNSTYRVVSVLTVLHQDWLNGKEYKCKVSNKALPAPIEKTISKAKGQPRRPRVYTLPPSREEMTDNQVSLVCLVKGFYPSDIAVEWESNGQPENNYKTTPPVLLSDGSFFLASLLTVDKSRWQQGNVFSCSVMHEALHNHYTQKSLSLSP

SEQ ID NO: 560 - protein, 447 aa, Homo sapiens
QVQLQESGPGLVRPSQTLSLTCTVSGYSITSDHAWSWVRQPPGRGLEWIGYISYSGITTYNPSLKSRVTMLRDTSKNQFSLRLSSVTAADTAVYYCARSLARTTAMDYWGQGSLVTVSSASTKGPSVFPLAPSSKSTSGGTAALGCLVKDYFPEPVTVSWNSGALTSGVHTFPAVLQSSGLYSLSSVVTVPSSSLGTQTYICNVNHKPSNTKVDKRVEPKSCDKTHTCPPCPAPELLGGPSVFLFPPKPKDTLMISRTPEVTCVVVDVSHEDPEVKFNWYVDGVEVHNAKTKPREEQYNSTYRVVSVLTVLHQDWLNGKEYKCKVSNKALPAPIEKTISKAKGQPRRPRVYTLPPSREEMTDNQVSLVCLVKGFYPSDIAVEWESNGQPENNYKTTPPVLISDGSFFLASILTVDKSRWQQGNVFSCSVMHEALHNHYTQKSLSLSP

SEQ ID NO: 561 - protein, 447 aa, Homo sapiens
QVQLQESGPGLVRPSQTLSLTCTVSGYSITSDHAWSWVRQPPGRGLEWIGYISYSGITTYNPSLKSRVTMLRDTSKNQFSLRLSSVTAADTAVYYCARSLARTTAMDYWGQGSLVTVSSASTKGPSVFPLAPSSKSTSGGTAALGCLVKDYFPEPVTVSWNSGALTSGVHTFPAVLQSSGLYSLSSVVTVPSSSLGTQTYICNVNHKPSNTKVDKRVEPKSCDKTHTCPPCPAPELLGGPSVFLFPPKPKDTLMISRTPEVTCVVVDVSHEDPEVKFNWYVDGVEVHNAKTKPREEQYNSTYRVVSVLTVLHQDWLNGKEYKCKVSNKALPAPIEKTISKAKGQPREPQVYTLPPSREEMTKNQVSLWCLVKGFYPSDIAVEWESNGQPENNYKTTPPVLDSDGSFFLYSKLTVDKSRWQQGNVFSCSVMHEALHNHYTQKSLSLSP

SEQ ID NO: 562 - protein, 447 aa, Homo sapiens
QVQLQESGPGLVKPSGTLSLTCAVSGGSISSSNWWSWVRQPPGKGLEWIGEIYHSGSTNYNPSLKSRVTISVDKSKNQFSLKLSSVTAADTAVYYCARWTGRTDAFDIWGQGTMVTVSSASTKGPSVFPLAPSSKSTSGGTAALGCLVKDYFPEPVTVSWNSGALTSGVHTFPAVLQSSGLYSLSSVVTVPSSSLGTQTYICNVNHKPSNTKVDKRVEPKSCDKTHTCPPCPAPELLGGPSVFLFPPKPKDTLMISRTPEVTCVVVDVSHEDPEVKFNWYVDGVEVHNAKTKPREEQYNSTYRVVSVLTVLHQDWLNGKEYKCKVSNKALPAPIEKTISKAKGQPREPQVYTLPPSREEMTKNQVSLSCAVKGFYPSDIAVEWESNGQPENNYKTTPPVLDSDGSFFLVSKLTVDKSRWQQGNVFSCSVMHEALHNHYTQKSLSLSP

SEQ ID NO: 563 - protein, 447 aa, Homo sapiens; identical to SEQ ID NO: 79

SEQ ID NO: 564 - protein, 447 aa, Homo sapiens
QVQLVQSGSELKKPGASVKVSCKASGYTFTDNNMDWVRQAPGQGLEWMGDINTRSGGSIYNEEFQDRVIMTVDKSTDTAYMELSSLRSEDTATYHCARRKSYGYYLDEWGEGTLVTVSSASTKGPSVFPLAPSSKSTSGGTAALGCLVKDYFPEPVTVSWNSGALTSGVHTFPAVLQSSGLYSLSSVVTVPSSSLGTQTYICNVNHKPSNTKVDKRVEPKSCDKTHTCPPCPAPELLGGPSVFLFPPKPKDTLMISRTPEVTCVVVDVSHEDPEVKFNWYVDGVEVHNAKTKPREEQYNSTYRVVSVLTVLHQDWLNGKEYKCKVSNKALPAPIEKTISKAKGQPREPQVYTLPPSREEMTKNQVSLTCLVKGFYPSDIAVEWESNGQPENNYKTWPPVLDSDGSFALYSKLTVDKSRWQQGNVFSCSVMHEALHNHYTQKSLSLSP

SEQ ID NO: 565 - protein, 447 aa, Homo sapiens
QVQLVQSGSELKKPGASVKVSCKASGYTFTDNNMDWVRQAPGQGLEWMGDINTRSGGSIYNEEFQDRVIMTVDKSTDTAYMELSSLRSEDTATYHCARRKSYGYYLDEWGEGTLVTVSSASTKGPSVFPLAPSSKSTSGGTAALGCLVKDYFPEPVTVSWNSGALTSGVHTFPAVLQSSGLYSLSSVVTVPSSSLGTQTYICNVNHKPSNTKVDKRVEPKSCDKTHTCPPCPAPELLGGPSVFLFPPKPKDTLMISRTPEVTCVVVDVSHEDPEVKFNWYVDGVEVHNAKTKPREEQYNSTYRVVSVLTVLHQDWLNGKEYKCKVSNKALPAPIEKTISKAKGQPREPQVYTLPPSRKEMTKNQVSLTCLVKGFYPSDIAVEWESNGQPENNYDTTPPVLKSDGSFFLYSKLTVDKSRWQQGNVFSCSVMHEALHNHYTQESLSLSP

SEQ ID NO: 566 - protein, 447 aa, Homo sapiens; identical to SEQ ID NO: 82

SEQ ID NO: 567 - protein, 450 aa, Homo sapiens
QVQLVESGGGLVQPGGSLRLSCAASGFTFSYYDIQWVRQAPGKGLEWVSSISPSGQSTYYRREVKGRFTISRDNSKNTLYLQMNSLRAEDTAVYYCARRTGREEGGWIFDYWGQGTLVTVSSASTKGPSVFPLAPSSKSTSGGTAALGCLVKDYFPEPVTVSWNSGALTSGVHTFPAVLQSSGLYSLSSVVTVPSSSLGTQTYICNVNHKPSNTKVDKRVEPKSCDKTHTCPPCPAPELLGGPSVFLFPPKPKDTLMISRTPEVTCVVVDVSHEDPEVKFNWYVDGVEVHNAKTKPREEQYNSTYRVVSVLTVLHQDWLNGKEYKCKVSNKALPAPIEKTISKAKGQPREPQVCTLPPSREEMTKNQVSLWCLVKGFYPSDIAVEWESNGQPENNYKTTPPVLDSDGSFFLYSKLTVDKSRWQQGNVFSCSVMHEALHNHYTQKSLSLSP

SEQ ID NO: 568 - protein, 447 aa, Homo sapiens
QVQLVQSGSELKKPGASVKVSCKASGYTFTQNNMDWVRQAPGQGLEWMGDINTRSGGVIYNEEFQDRLIMTVDKSTDTAYMELSSLRSEDTATYHCARRKSYGYYLDVWGEGTLVTVSSASTKGPSVFPLAPSSKSTSGGTAALGCLVKDYFPEPVTVSWNSGALTSGVHTFPAVLQSSGLYSLSSVVTVPSSSLGTQTYICNVNHKPSNTKVDKRVEPKSCDKTHTCPPCPAPELLGGPSVFLFPPKPKDTLMISRTPEVTCVVVDVSHEDPEVKFNWYVDGVEVHNAKTKPREEQYNSTYRVVSVLTVLHQDWLNGKEYKCKVSNKALPAPIEKTISKAKGQPREPQVYTLPPSRCEMTKNQVSLSCAVKGFYPSDIAVEWESNGQPENNYKTTPPVLDSDGSFFLVSKLTVDKSRWQQGNVFSCSVMHEALHNHYTQKSLSLSP

SEQ ID NO: 569 - protein, 447 aa, Homo sapiens; identical to SEQ ID NO: 78

SEQ ID NO: 570 - protein, 447 aa, Homo sapiens
QVQLQESGPGLVKPSETLSLTCAVSGHSISHDHAWSWVRQPPGEGLEWIGFISYSGITNYNPSLQGRVTISRDNSKNTLYLQMNSLRAEDTAVYYCARSLARTTAMDYWGEGTLVTVSSASTKGPSVFPLAPSSKSTSGGTAALGCLVKDYFPEPVTVSWNSGALTSGVHTFPAVLQSSGLYSLSSVVTVPSSSLGTQTYICNVNHKPSNTKVDKRVEPKSCDKTHTCPPCPAPELLGGPSVFLFPPKPKDTLMISRTPEVTCVVVDVSHEDPEVKFNWYVDGVEVHNAKTKPREEQYNSTYRVVSVLTVLHQDWLNGKEYKCKVSNKALPAPIEKTISKAKGQPREPQVYTLPPSREEMTKNQVSLTCLVKGFYPSDIAVEWESNGQPENNYKTWPPVLDSDGSFALYSKLTVDKSRWQQGNVFSCSVMHEALHNHYTQKSLSLSP

SEQ ID NO: 571 - protein, 447 aa, Homo sapiens
QVQLQESGPGLVKPSETLSLTCAVSGHSISHDHAWSWVRQPPGEGLEWIGFISYSGITNYNPSLQGRVTISRDNSKNTLYLQMNSLRAEDTAVYYCARSLARTTAMDYWGEGTLVTVSSASTKGPSVFPLAPSSKSTSGGTAALGCLVKDYFPEPVTVSWNSGALTSGVHTFPAVLQSSGLYSLSSVVTVPSSSLGTQTYICNVNHKPSNTKVDKRVEPKSCDKTHTCPPCPAPELLGGPSVFLFPPKPKDTLMISRTPEVTCVVVDVSHEDPEVKFNWYVDGVEVHNAKTKPREEQYNSTYRVVSVLTVLHQDWLNGKEYKCKVSNKALPAPIEKTISKAKGQPREPQVYTLPPSRKEMTKNQVSLTCLVKGFYPSDIAVEWESNGQPENNYDTTPPVLKSDGSFFLYSKLTVDKSRWQQGNVFSCSVMHEALHNHYTQESLSLSP

SEQ ID NO: 572 - protein, 447 aa, Homo sapiens
QVQLQESGPGLVKPSETLSLTCAVSGHSISHDHAWSWVRQPPGEGLEWIGFISYSGITNYNPSLQGRVTISRDNSKNTLYLQMNSLRAEDTAVYYCARSLARTTAMDYWGEGTLVTVSSASTKGPSVFPLAPSSKSTSGGTAALGCLVKDYFPEPVTVSWNSGALTSGVHTFPAVLQSSGLYSLSSVVTVPSSSLGTQTYICNVNHKPSNTKVDKRVEPKSCDKTHTCPPCPAPELLGGPSVFLFPPKPKDTLMISRTPEVTCVVVDVSHEDPEVKFNWYVDGVEVHNAKTKPREEQYNSTYRVVSVLTVLHQDWLNGKEYKCKVSNKALPAPIEKTISKAKGQPREPRVYTLPPSREEMTENQVSLTCLVKGFYPSDIAVEWESNGQPENNYKTTPPVLVSDGSFTLYSWLTVDKSRWQQGNVFSCSVMHEALHNHYTQKSLSLSP

SEQ ID NO: 573 - protein, 450 aa, Homo sapiens
QVQLVESGGGVVQPGGSLRLSCAASGFTFSNAWMHWVRQAPGKGLEWVAQIKDKSQNYATYVAESVKGRFTISRADSKNSIYLQMNSLKTEDTAVYYCRYVHYAAGYGVDIWGQGTTVTVSSASTKGPSVFPLAPSSKSTSGGTAALGCLVKDYFPEPVTVSWNSGALTSGVHTFPAVLQSSGLYSLSSVVTVPSSSLGTQTYICNVNHKPSNTKVDKRVEPKSCDKTHTCPPCPAPELLGGPSVFLFPPKPKDTLMISRTPEVTCVVVDVSHEDPEVKFNWYVDGVEVHNAKTKPREEQYNSTYRVVSVLTVLHQDWLNGKEYKCKVSNKALPAPIEKTISKAKGQPREPQVYTLPPSREEMTKNQVSLTCLVKGFYPSDIAVEWESNGQPENNYKTTPPVLDSDGSFFLYSKLTVDKSRWQQGNVFSCSVMHEALHNHYTQKSLSLSP

SEQ ID NO: 574 - protein, 450 aa, Homo sapiens
QVQLVESGGGVVQPGGSLRLSCAASGFTFSNAWMHWVRQAPGKGLEWVAQIKDKSQNYATYVAESVKGRFTISRADSKNSIYLQMNSLKTEDTAVYYCRYVHYAAGYGVDIWGQGTTVTVSSASTKGPSVFPLAPSSKSTSGGTAALGCLVKDYFPEPVTVSWNSGALTSGVHTFPAVLQSSGLYSLSSVVTVPSSSLGTQTYICNVNHKPSNTKVDKRVEPKSCDKTHTCPPCPAPELLGGPSVFLFPPKPKDTLMISRTPEVTCVVVDVSHEDPEVKFNWYVDGVEVHNAKTKPREEQYNSTYRVVSVLTVLHQDWLNGKEYKCKVSNKALPAPIEKTISKAKGQPREPRVYTLPPSREEMTENQVSLTCLVKGFYPSDIAVEWESNGQPENNYKTTPPVLVSDGSFTLYSWLTVDKSRWQQGNVFSCSVMHEALHNHYTQKSLSLSP

SEQ ID NO: 575 - protein, 448 aa, Homo sapiens
QVQLVESGGGLVQPGGSLRLSCAASGFTFSYYDIQWVRQAPGKGLEWVSSISPSGQSTYYRREVKGRFTISRDNSKNTLYLQMNSLRAEDTAVYYCARRTGREYGGGWYFDYWGQGTLVTVSSASTKGPSVFPLAPCSRSTSESTAALGCLVKDYFPEPVTVSWNSGALTSGVHTFPAVLQSSGLYSLSSVVTVPSSSLGTKTYTCNVDHKPSNTKVDKRVESKYGPPCPPCPAPEFLGGPSVFLFPPKPKDTLMISRTPEVTCVVVDVSQEDPEVQFNWYVDGVEVHNAKTKPREEQFNSTYRVVSVLTVLHQDWLNGKEYKCKVSNKGLPSSIEKTISKAKGQPREPQVYTLPPSQEEMTKNQVSLTCLVKGFYPSDIAVEWESNGQPENNYKTTPPVLDSDGSFFLYSRLTVDKSRWQEGNVFSCSVMHEALHNHYTQKSLSLSL

SEQ ID NO: 576 - protein, 448 aa, Homo sapiens
QVQLVESGGGLVQPGGSLRLSCAASGFTFSYYDIQWVRQAPGKGLEWVSSISPSGQSTYYRREVKGRFTISRDNSKNTLYLQMNSLRAEDTAVYYCARRTGREYGGGWYFDYWGQGTLVTVSSASTKGPSVFPLAPCSRSTSESTAALGCLVKDYFPEPVTVSWNSGALTSGVHTFPAVLQSSGLYSLSSVVTVPSSSLGTKTYTCNVDHKPSNTKVDKRVESKYGPPCPPCPAPEFLGGPSVFLFPPKPKDTLMISRTPEVTCVVVDVSQEDPEVQFNWYVDGVEVHNAKTKPREEQFNSTYRVVSVLTVLHQDWLNGKEYKCKVSNKGLPSSIEKTISKAKGQPREPQVYTLPPSQEEMTKNQVSLTCLVKGFYPSDIAVEWESNGQPENNYKTWPPVLDSDGSFALYSRLTVDKSRWQEGNVFSCSVMHEALHNHYTQKSLSLSL

SEQ ID NO: 577 - protein, 219 aa, Homo sapiens
DIVMTQSPLSLPVTPGEPASISCRSSQPLVHSNRNTYLHWYQQKPGQAPRLLIYKVSNRFSGVPDRFSGSGSGTDFTLKISRVEAEDVGVYYCGQGTQVPYTFGQGTKLEIKRTVAAPSVFIFPPSDEQLKSGTASVVCLLNNFYPREAKVQWKVDNALQSGNSQESVTEQDSKDSTYSLSSTLTLSKADYEKHKVYACEVTHQGLSSPVTKSFNRGEC

SEQ ID NO: 578 - protein, 214 aa, Homo sapiens
DIQMTQSPSSLSASVGDRVTITCKASRNIERQLAWYQQKPGQAPELLIYQASRKESGVPDRFSGSRYGTDFTLTISSLQPEDIATYYCQQYSDPPLTFGGGTKVEIKRTVAAPSVFIFPPSDEQLKSGTASVVCLLNNFYPREAKVQWKVDNALQSGNSQESVTEQDSKDSTYSLSSTLTLSKADYEKHKVYACEVTHQGLSSPVTKSFNRGEC

SEQ ID NO: 579 - protein, 347 aa, Homo sapiens
EVQLVESGGGLVQPGGSLRLSCAASGSISSVDVMSWYRQAPGKQRELVAFITDRGRTNYKVSVKGRFTISRDNSKNMVYLQMNSLKPEDTADYLCRAESRTSWSSPSPLDVWGRGTQVTVSSDKTHTCPPCPAPELLGGPSVFLFPPKPKDTLMISRTPEVTCVVVDVSHEDPEVKFNWYVDGVEVHNAKTKPREEQYNSTYRVVSVLTVLHQDWLNGKEYKCKVSNKALPAPIEKTISKAKGQPREPQVYTLPPSREEMTKNQVSLTCLVKGFYPSDIAVEWESNGQPENNYKTTPPVLDSDGSFFLYSKLTVDKSRWQQGNVFSCSVMHEALHNHYTQKSLSLSP

SEQ ID NO: 580 - protein, 347 aa, Homo sapiens
EVQLVESGGGLVQPGGSLRLSCAASGSISSVDVMSWYRQAPGKQRELVAFITDRGRTNYKVSVKGRFTISRDNSKNMVYLQMNSLKPEDTADYLCRAESRTSWSSPSPLDVWGRGTQVTVSSDKTHTCPPCPAPELLGGPSVFLFPPKPKDTLMISRTPEVTCVVVDVSHEDPEVKFNWYVDGVEVHNAKTKPREEQYNSTYRVVSVLTVLHQDWLNGKEYKCKVSNKALPAPIEKTISKAKGQPREPQVYTLPPSREEMTKNQVSLTCLVKGFYPSDIAVEWESNGQPENNYKTWPPVLDSDGSFALYSKLTVDKSRWQQGNVFSCSVMHEALHNHYTQKSLSLSP

SEQ ID NO: 581 - protein, 347 aa, Homo sapiens
EVQLVESGGGLVQPGGSLRLSCAASGSISSVDVMSWYRQAPGKQRELVAFITDRGRTNYKVSVKGRFTISRDNSKNMVYLQMNSLKPEDTADYLCRAESRTSWSSPSPLDVWGRGTQVTVSSDKTHTCPPCPAPELLGGPSVFLFPPKPKDTLMISRTPEVTCVVVDVSHEDPEVKFNWYVDGVEVHNAKTKPREEQYNSTYRVVSVLTVLHQDWLNGKEYKCKVSNKALPAPIEKTISKAKGQPREPQVYTLPPSREEMTKNQVSLWCAVKGFYPSDIAVEWESNGQPENNYKTTPPVLDSDGSFFLVSKLTVDKSRWQQGNVFSCSVMHEALHNHYTQKSLSLSP

SEQ ID NO: 582 - protein, 347 aa, Homo sapiens
EVQLVESGGGLVQPGGSLRLSCAASGSISSVDVMSWYRQAPGKQRELVAFITDRGRTNYKVSVKGRFTISRDNSKNMVYLQMNSLKPEDTADYLCRAESRTSWSSPSPLDVWGRGTQVTVSSDKTHTCPPCPAPELLGGPSVFLFPPKPKDTLMISRTPEVTCVVVDVSHEDPEVKFNWYVDGVEVHNAKTKPREEQYNSTYRVVSVLTVLHQDWLNGKEYKCKVSNKALPAPIEKTISKAKGQPREPRVYTLPPSREEMTENQVSLTCLVKGFYPSDIAVEWESNGQPENNYKTTPPVLVSDGSFTLYSWLTVDKSRWQQGNVFSCSVMHEALHNHYTQKSLSLSP

SEQ ID NO: 583 - protein, 347 aa, Homo sapiens
EVQLVESGGGLVQPGGSLRLSCAASGSISSVDVMSWYRQAPGKQRELVAFITDRGRTNYKVSVKGRFTISRDNSKNMVYLQMNSLKPEDTADYLCRAESRTSWSSPSPLDVWGRGTQVTVSSDKTHTCPPCPAPELLGGPSVFLFPPKPKDTLMISRTPEVTCVVVDVSHEDPEVKFNWYVDGVEVHNAKTKPREEQYNSTYRVVSVLTVLHQDWLNGKEYKCKVSNKALPAPIEKTISKAKGQPREPQVYTLPPSREEMTKNQVSLTCLVKGFYPSDIAVEWESNGQPENNYKTFPPVLDSDGSFALYSKLTVDKSRWQQGNVFSCSVMHEALHNHYTQKSLSLSP

SEQ ID NO: 584 - protein, 347 aa, Homo sapiens
EVQLVESGGGLVQPGGSLRLSCAASGSISSVDVMSWYRQAPGKQRELVAFITDRGRTNYKVSVKGRFTISRDNSKNMVYLQMNSLKPEDTADYLCRAESRTSWSSPSPLDVWGRGTQVTVSSDKTHTCPPCPAPELLGGPSVFLFPPKPKDTLMISRTPEVTCVVVDVSHEDPEVKFNWYVDGVEVHNAKTKPREEQYNSTYRVVSVLTVLHQDWLNGKEYKCKVSNKALPAPIEKTISKAKGQPREPQVYTLPPSRKEMTKNQVSLTCLVKGFYPSDIAVEWESNGQPENNYKTTPPVLKSDGSFFLYSELTVDKSRWQQGNVFSCSVMHEALHNHYTQESLSLSP

SEQ ID NO: 585 - protein, 347 aa, Homo sapiens
EVQLVESGGGLVQPGGSLRLSCAASGSISSVDVMSWYRQAPGKQRELVAFITDRGRTNYKVSVKGRFTISRDNSKNMVYLQMNSLKPEDTADYLCRAESRTSWSSPSPLDVWGRGTQVTVSSDKTHTCPPCPAPELLGGPSVFLFPPKPKDTLMISRTPEVTCVVVDVSHEDPEVKFNWYVDGVEVHNAKTKPREEQYNSTYRVVSVLTVLHQDWLNGKEYKCKVSNKALPAPIEKTISKAKGQPREPEVYTLPPYREEMTKNQVSLYCLVKGFYPSDIAVEWESNGQPENNYKTTPPVLDSDGSFFLTSKLTVDKSRWQQGNVFSCSVMHEALHNHYTQKSLSLSP

SEQ ID NO: 586 - protein, 347 aa, Homo sapiens
EVQLVESGGGLVQPGGSLRLSCAASGSISSVDVMSWYRQAPGKQRELVAFITDRGRTNYKVSVKGRFTISRDNSKNMVYLQMNSLKPEDTADYLCRAESRTSWSSPSPLDVWGRGTQVTVSSDKTHTCPPCPAPELLGGPSVFLFPPKPKDTLMISRTPEVTCVVVDVSHEDPEVKFNWYVDGVEVHNAKTKPREEQYNSTYRVVSVLTVLHQDWLNGKEYKCKVSNKALPAPIEKTISKAKGQPREPQVYTLPPSREEMTKNQVSLTCLVKGFYPSDIAVEWESNGQPENNYLTWPPVLDSDGSFALVSKLTVDKSRWQQGNVFSCSVMHEALHNHYTQKSLSLSP

SEQ ID NO: 587 - protein, 347 aa, Homo sapiens
EVQLVESGGGLVQPGGSLRLSCAASGSISSVDVMSWYRQAPGKQRELVAFITDRGRTNYKVSVKGRFTISRDNSKNMVYLQMNSLKPEDTADYLCRAESRTSWSSPSPLDVWGRGTQVTVSSDKTHTCPPCPAPELLGGPSVFLFPPKPKDTLMISRTPEVTCVVVDVSHEDPEVKFNWYVDGVEVHNAKTKPREEQYNSTYRVVSVLTVLHQDWLNGKEYKCKVSNKALPAPIEKTISKAKGQPREPQVYTLPPSRKEMTKNQVSLTCLVKGFYPSDIAVEWESNGQPENNYDTTPPVLKSDGSFFLYSKLTVDKSRWQQGNVFSCSVMHEALHNHYTQESLSLSP

SEQ ID NO: 588 - protein, 347 aa, Homo sapiens
EVQLVESGGGLVQPGGSLRLSCAASGSISSVDVMSWYRQAPGKQRELVAFITDRGRTNYKVSVKGRFTISRDNSKNMVYLQMNSLKPEDTADYLCRAESRTSWSSPSPLDVWGRGTQVTVSSDKTHTCPPCPAPELLGGPSVFLFPPKPKDTLMISRTPEVTCVVVDVSHEDPEVKFNWYVDGVEVHNAKTKPREEQYNSTYRVVSVLTVLHQDWLNGKEYKCKVSNKALPAPIEKTISKAKGQPREPQVYTLPPSREEMTKNQVSLTCLVKGFYPSDIAVEWESNGQPENNYDTTPPVLKSDGSFFLYSDLTVDKSRWQQGNVFSCSVMHEALHNHYTQKSLSLSP

SEQ ID NO: 589 - protein, 347 aa, Homo sapiens
EVQLVESGGGLVQPGGSLRLSCAASGSISSVDVMSWYRQAPGKQRELVAFITDRGRTNYKVSVKGRFTISRDNSKNMVYLQMNSLKPEDTADYLCRAESRTSWSSPSPLDVWGRGTQVTVSSDKTHTCPPCPAPELLGGPSVFLFPPKPKDTLMISRTPEVTCVVVDVSHEDPEVKFNWYVDGVEVHNAKTKPREEQYNSTYRVVSVLTVLHQDWLNGKEYKCKVSNKALPAPIEKTISKAKGQPREPQVCTLPPSRECMTKNQVSLTCLVKGFYPSDIAVEWESNGQPENNYDTTPPVLKSDGSFFLYSKLTVDKSRWQQGNVFSCSVMHEALHNHYTQKSLSLSP

SEQ ID NO: 590 - protein, 347 aa, Homo sapiens
EVQLVESGGGLVQPGGSLRLSCAASGSISSVDVMSWYRQAPGKQRELVAFITDRGRTNYKVSVKGRFTISRDNSKNMVYLQMNSLKPEDTADYLCRAESRTSWSSPSPLDVWGRGTQVTVSSDKTHTCPPCPAPELLGGPSVFLFPPKPKDTLMISRTPEVTCVVVDVSHEDPEVKFNWYVDGVEVHNAKTKPREEQYNSTYRVVSVLTVLHQDWLNGKEYKCKVSNKALPAPIEKTISKAKGQPRRPRVYTLPPSREEMTDNQVSLVCLVKGFYPSDIAVEWESNGQPENNYKTTPPVLMSDGSFFLASVLTVDKSRWQQGNVFSCSVMHEALHNHYTQKSLSLSP

SEQ ID NO: 591 - protein, 347 aa, Homo sapiens
EVQLVESGGGLVQPGGSLRLSCAASGSISSVDVMSWYRQAPGKQRELVAFITDRGRTNYKVSVKGRFTISRDNSKNMVYLQMNSLKPEDTADYLCRAESRTSWSSPSPLDVWGRGTQVTVSSDKTHTCPPCPAPELLGGPSVFLFPPKPKDTLMISRTPEVTCVVVDVSHEDPEVKFNWYVDGVEVHNAKTKPREEQYNSTYRVVSVLTVLHQDWLNGKEYKCKVSNKALPAPIEKTISKAKGQPREPQVYTLPPSRKEMTKNQVSLTCLVKGFYPSDIAVEWESNGQPENNYDTTPPVLKSDGSFFLYSDLTVDKSRWQQGNVFSCSVMHEALHNHYTQKSLSLSP

SEQ ID NO: 592 - protein, 347 aa, Homo sapiens
EVQLVESGGGLVQPGGSLRLSCAASGSISSVDVMSWYRQAPGKQRELVAFITDRGRTNYKVSVKGRFTISRDNSKNMVYLQMNSLKPEDTADYLCRAESRTSWSSPSPLDVWGRGTQVTVSSDKTHTCPPCPAPELLGGPSVFLFPPKPKDTLMISRTPEVTCVVVDVSHEDPEVKFNWYVDGVEVHNAKTKPREEQYNSTYRVVSVLTVLHQDWLNGKEYKCKVSNKALPAPIEKTISKAKGQPRRPQVYTLPPSREEMTENQVSLTCLVKGFYPSDIAVEWESNGQPENNYKTTPPVLMSDGSFFLASVLTVDKSRWQQGNVFSCSVMHEALHNHYTQKSLSLSP

SEQ ID NO: 593 - protein, 347 aa, Homo sapiens
EVQLVESGGGLVQPGGSLRLSCAASGSISSVDVMSWYRQAPGKQRELVAFITDRGRTNYKVSVKGRFTISRDNSKNMVYLQMNSLKPEDTADYLCRAESRTSWSSPSPLDVWGRGTQVTVSSDKTHTCPPCPAPELLGGPSVFLFPPKPKDTLMISRTPEVTCVVVDVSHEDPEVKFNWYVDGVEVHNAKTKPREEQYNSTYRVVSVLTVLHQDWLNGKEYKCKVSNKALPAPIEKTISKAKGQPREPQVYVYPPSREEMTKNQVSLLCLVKGFYPSDIAVEWESNGQPENNYLTWPPVLDSDGSFALVSKLTVDKSRWQQGNVFSCSVMHEALHNHYTQKSLSLSP

SEQ ID NO: 594 - protein, 225 aa, Homo sapiens
DKTHTCPPCPAPELRRGPSVFLFPPKPKDTLMISRTPEVTCVVVDVSHEDPEVKFNWYVDGVEVHNAKTKPREEQYNSTYRVVSVLTVLHQDWLNGKEYKCKVSNKALPAPIEKTISKAKGQPREPQVYTLPPSREEMTKNQVSLTCLVKGFYPSDIAVEWESNGQPENNYKTTPPVLDSDGSFFLYSKLTVDKSRWQQGNVFSCSVMHEALHNHYTQKSLSLSP

SEQ ID NO: 595 - protein, 225 aa, Homo sapiens
DKTHTCPPCPAPEAAGGPSVFLFPPKPKDTLMISRTPEVTCVVVDVSHEDPEVKFNWYVDGVEVHNAKTKPREEQYNSTYRVVSVLTVLHQDWLNGKEYKCKVSNKALPAPIEKTISKAKGQPREPQVYTLPPSREEMTKNQVSLTCLVKGFYPSDIAVEWESNGQPENNYKTTPPVLDSDGSFFLYSKLTVDKSRWQQGNVFSCSVMHEALHNHYTQKSLSLSP

SEQ ID NO: 596 - protein, 225 aa, Homo sapiens
DKTHTCPPCPAPELLGGPSVFLFPPKPKDTLYITREPEVTCVVVDVSHEDPEVKFNWYVDGVEVHNAKTKPREEQYNSTYRVVSVLTVLHQDWLNGKEYKCKVSNKALPAPIEKTISKAKGQPREPQVYTLPPSREEMTKNQVSLTCLVKGFYPSDIAVEWESNGQPENNYKTTPPVLDSDGSFFLYSKLTVDKSRWQQGNVFSCSVMHEALHNHYTQKSLSLSP

SEQ ID NO: 597 - protein, 225 aa, Homo sapiens
DKTHTCPPCPAPELLGGPSVFLFPPKPKDTLMISRTPEVTCVVVDVSHEDPEVKFNWYVDGVEVHNAKTKPREEQYNSTYRVVSVLTVLHQDWLNGKEYKCKVSNKALPAPIEKTISKAKGQPREPQVYTLPPSREEMTKNQVSLTCLVKGFYPSDIAVEWESNGQPENNYKTTPPVLDSDGSFFLYSKLTVDKSRWQQGNVFSCSVLHEALHSHYTQKSLSLSP

SEQ ID NO: 598 - protein, 225 aa, Homo sapiens
DKTHTCPPCPAPEAAGGPSVFLFPPKPKDTLMISRTPEVTCVVVDVSHEDPEVKFNWYVDGVEVHNAKTKPREEQYNSTYRVVSVLTVLHQDWLNGKEYKCKVSNKALGAPIEKTISKAKGQPREPQVYTLPPSREEMTKNQVSLTCLVKGFYPSDIAVEWESNGQPENNYKTTPPVLDSDGSFFLYSKLTVDKSRWQQGNVFSCSVMHEALHNHYTQKSLSLSP

SEQ ID NO: 599 - protein, 225 aa, Homo sapiens
DKTHTCPPCPAPEFEGGPSVFLFPPKPKDTLMISRTPEVTCVVVDVSHEDPEVKFNWYVDGVEVHNAKTKPREEQYNSTYRVVSVLTVLHQDWLNGKEYKCKVSNKALPASIEKTISKAKGQPREPQVYTLPPSREEMTKNQVSLTCLVKGFYPSDIAVEWESNGQPENNYKTTPPVLDSDGSFFLYSKLTVDKSRWQQGNVFSCSVMHEALHNHYTQKSLSLSP

SEQ ID NO: 600 - protein, 225 aa, Homo sapiens
DKTHTCPPCPAPEFEGGPSVFLFPPKPKDTLMISRTPEVTCVVVDVSHEDPEVKFNWYVDGVEVHNAKTKPREEQYNSTYRVVSVLTVLHQDWLNGKEYKCKVSNKALPASIEKTISKAKGQPREPQVYTLPPSREEMTKNQVSLTCLVKGFYPSDIAVEWESNGQPENNYKTWPPVLDSDGSFALYSKLTVDKSRWQQGNVFSCSVMHEALHNHYTQKSLSLSP

SEQ ID NO: 601 - protein, 225 aa, Homo sapiens
DKTHTCPPCPAPEFEGGPSVFLFPPKPKDTLMISRTPEVTCVVVDVSHEDPEVKFNWYVDGVEVHNAKTKPREEQYNSTYRVVSVLTVLHQDWLNGKEYKCKVSNKALPASIEKTISKAKGQPREPQVYTLPPSREEMTKNQVSLWCAVKGFYPSDIAVEWESNGQPENNYKTTPPVLDSDGSFFLVSKLTVDKSRWQQGNVFSCSVMHEALHNHYTQKSLSLSP

SEQ ID NO: 602 - protein, 225 aa, Homo sapiens
DKTHTCPPCPAPEFEGGPSVFLFPPKPKDTLMISRTPEVTCVVVDVSHEDPEVKFNWYVDGVEVHNAKTKPREEQYNSTYRVVSVLTVLHQDWLNGKEYKCKVSNKALPASIEKTISKAKGQPREPRVYTLPPSREEMTENQVSLTCLVKGFYPSDIAVEWESNGQPENNYKTTPPVLVSDGSFTLYSWLTVDKSRWQQGNVFSCSVMHEALHNHYTQKSLSLSP

SEQ ID NO: 603 - protein, 225 aa, Homo sapiens
DKTHTCPPCPAPEFEGGPSVFLFPPKPKDTLMISRTPEVTCVVVDVSHEDPEVKFNWYVDGVEVHNAKTKPREEQYNSTYRVVSVLTVLHQDWLNGKEYKCKVSNKALPASIEKTISKAKGQPREPQVYTLPPSRKEMTKNQVSLTCLVKGFYPSDIAVEWESNGQPENNYDTTPPVLKSDGSFFLYSKLTVDKSRWQQGNVFSCSVMHEALHNHYTQESLSLSP

SEQ ID NO: 604 - protein, 225 aa, Homo sapiens
DKTHTCPPCPAPELLGGPSVFLFPPKPKDTLMISRTPEVTCVVVDVSHEDPEVKFNWYVDGVEVHNAKTKPREEQYNSTYRVVSVLTVLHQDWLNGKEYKCKVSNKALPAPIEKTISKAKGQPRRPQVYTLPPSREEMTKNQVSLTCLVKGFYPSDIAVEWESNGQPENNYKTWPPVLDSDGSFALYSKLTVDKSRWQQGNVFSCSVMHGALHNHYTQKYLSLSP

SEQ ID NO: 605 - protein, 225 aa, Homo sapiens
DKTHTCPPCPAPELLGGPSVFLFPPKPKDTLMISRTPEVTCVVVDVSHEDPEVKFNWYVDGVEVHNAKTKPREEQYNSTYRVVSVLTVLHQDWLNGKEYKCKVSNKALPAPIEKTISKAKGQPRRPQVYTLPPSREEMTKNQVSLWCAVKGFYPSDIAVEWESNGQPENNYKTTPPVLDSDGSFFLVSKLTVDKSRWQQGNVFSCSVMHGALHNHYTQKYLSLSP

SEQ ID NO: 606 - protein, 225 aa, Homo sapiens
DKTHTCPPCPAPELLGGPSVFLFPPKPKDTLMISRTPEVTCVVVDVSHEDPEVKFNWYVDGVEVHNAKTKPREEQYNSTYRVVSVLTVLHQDWLNGKEYKCKVSNKALPAPIEKTISKAKGQPRRPRVYTLPPSREEMTENQVSLTCLVKGFYPSDIAVEWESNGQPENNYKTTPPVLVSDGSFTLYSWLTVDKSRWQQGNVFSCSVMHGALHNHYTQKYLSLSP

SEQ ID NO: 607 - protein, 443 aa, Homo sapiens
QVQLVQSGAEVKKPGASVTVSCKASGYTFTDYEMHWIRQPPGEGLEWIGAIDGPTPDTAYSEKFKGRVTLTADKSTSTAYMELSSLTSEDTAVYYCTRFYSYTYWGQGTLVTVSSASTKGPSVFPLAPSSKSTSGGTAALGCLVKDYFPEPVTVSWNSGALTSGVHTFPAVLQSSGLYSLSSVVTVPSSSLGTQTYICNVNHKPSNTKVDKRVEPKSCDKTHTCPPCPAPELLGGPSVFLFPPKPKDTLMISRTPEVTCVVVDVSHEDPEVKFNWYVDGVEVHNAKTKPREEQYNSTYRVVSVLTVLHQDWLNGKEYKCKVSNKALPAPIEKTISKAKGQPREPQVYTLPPSREEMTKNQVSLTCLVKGFYPSDIAVEWESNGQPENNYKTTPPVLDSDGSFFLYSKLTVDKSRWQQGNVFSCSVMHEALHNHYTQKSLSLSP

SEQ ID NO: 608 - protein, 443 aa, Homo sapiens
QVQLVQSGAEVKKPGASVTVSCKASGYTFTDYEMHWIRQPPGEGLEWIGAIDGPTPDTAYSEKFKGRVTLTADKSTSTAYMELSSLTSEDTAVYYCTRFYSYTYWGQGTLVTVSSASTKGPSVFPLAPSSKSTSGGTAALGCLVKDYFPEPVTVSWNSGALTSGVHTFPAVLQSSGLYSLSSVVTVPSSSLGTQTYICNVNHKPSNTKVDKRVEPKSCDKTHTCPPCPAPELLGGPSVFLFPPKPKDTLMISRTPEVTCVVVDVSHEDPEVKFNWYVDGVEVHNAKTKPREEQYNSTYRVVSVLTVLHQDWLNGKEYKCKVSNKALPAPIEKTISKAKGQPREPQVYTLPPSRKEMTKNQVSLTCLVKGFYPSDIAVEWESNGQPENNYDTTPPVLKSDGSFFLYSKLTVDKSRWQQGNVFSCSVMHEALHNHYTQESLSLSP

SEQ ID NO: 609 - protein, 444 aa, Homo sapiens
QVQLVQSGSELKKPGASVKVSCKASGYTFTDNNMDWVRQAPGQGLEWMGDINTRSGGSIYNEEFQDRVIMTVDKSTDTAYMELSSLRSEDTATYHCARRKSYGYYLDEWGEGTLVTVSSASTKGPSVFPLAPCSRSTSESTAALGCLVKDYFPEPVTVSWNSGALTSGVHTFPAVLQSSGLYSLSSVVTVPSSSLGTKTYTCNVDHKPSNTKVDKRVESKYGPPCPPCPAPEFLGGPSVFLFPPKPKDTLMISRTPEVTCVVVDVSQEDPEVQFNWYVDGVEVHNAKTKPREEQFNSTYRVVSVLTVLHQDWLNGKEYKCKVSNKGLPSSIEKTISKAKGQPREPQVYTLPPSQEEMTKNQVSLTCLVKGFYPSDIAVEWESNGQPENNYKTTPPVLDSDGSFFLYSRLTVDKSRWQEGNVFSCSVMHEALHNHYTQKSLSLSL

SEQ ID NO: 610 - protein, 444 aa, Homo sapiens
QVQLVQSGSELKKPGASVKVSCKASGYTFTDNNMDWVRQAPGQGLEWMGDINTRSGGSIYNEEFQDRVIMTVDKSTDTAYMELSSLRSEDTATYHCARRKSYGYYLDEWGEGTLVTVSSASTKGPSVFPLAPCSRSTSESTAALGCLVKDYFPEPVTVSWNSGALTSGVHTFPAVLQSSGLYSLSSVVTVPSSSLGTKTYTCNVDHKPSNTKVDKRVESKYGPPCPPCPAPEFLGGPSVFLFPPKPKDTLMISRTPEVTCVVVDVSQEDPEVQFNWYVDGVEVHNAKTKPREEQFNSTYRVVSVLTVLHQDWLNGKEYKCKVSNKGLPSSIEKTISKAKGQPREPQVYTLPPSQEEMTKNQVSLWCAVKGFYPSDIAVEWESNGQPENNYKTTPPVLDSDGSFFLVSRLTVDKSRWQEGNVFSCSVMHEALHNHYTQKSLSLSL

SEQ ID NO: 611 - RNA, 1407 nt, Homo sapiens
  source 1..1407: mol_type = mRNA
atggagtttgggctgtcatgggtctttctggtcgctctgctgcggggagtgcagtgtcaggtccagctggtcgaatcaggcggaggcgtggtccagcccggagggtctctgagactgagttgcgccgcttcaggcttcacattttctaacgcctggatgcactgggtgcgacaggctcctggcaaagggctggagtgggtcgcacagatcaaggacaaatcccagaattacgctacttacgttgcagaatccgtgaaggggaggttcaccatttcccgcgccgattccaaaaactccatctacctgcagatgaatagtctgaagaccgaggacacagccgtgtactattgtagatatgtccattacgcagccggctacggagtggacatctggggacagggaactacagtcacagtctcatccgcttccaccaagggcccatcggtcttccccctggcaccctcctccaagtccacctctgggggcacagcggccctgggctgcctggtcaaggactacttccccgaaccggtgacggtgtcgtggaactcaggcgccctgacctccggcgtgcacaccttcccggctgtcctacagtcctcaggactctactccctctcctccgtggtgaccgtgccctcctcgtccttgggcacccagacctacatctgcaacgtgaatcacaagccctccaacaccaaggtggacaagagagttgagcccaaatcttgtgacaaaactcacacatgcccaccgtgcccagcacctgaactcctggggggaccgtcagtcttcctcttccccccaaaacccaaggacaccctcatgatctcccggacccctgaggtcacatgcgtggtggtggacgtgtcccacgaagaccctgaggtcaagttcaactggtacgtggacggcgtggaggtgcataatgccaagacaaagccgcgggaggagcagtacaactccacgtaccgtgtggtctccgtcctcaccgtcctgcaccaggactggctgaatggcaaggagtacaagtgcaaggtctccaacaaagccctcccagcccccatcgagaaaaccatctccaaagccaaagggcagccccgagaaccacaggtgtacaccctgcccccatcccgggaggaaatgaccaagaaccaggtctccctgacctgcctggtcaaaggcttctatccctccgacatcgccgtggagtgggagtccaatgggcagccggagaacaactacaagaccacgcctcccgtgctggactccgacggctccttcttcctctactccaagctcaccgtggacaagtccaggtggcagcaggggaacgtcttctcatgctccgtgatgcatgaggctctgcacaaccactacacgcagaagtcgctctccctgtctccg

SEQ ID NO: 612 - RNA, 1386 nt, Homo sapiens
  source 1..1386: mol_type = mRNA
atgggctggtcctgcatcatcctgtttctggtggccaccgctaccggcgtccatagccaggtgcagctggtgcagtctggagctgaggtgaagaagcctggggcctcagtgaccgtctcctgcaaggcttctggatacaccttcaccgactatgaaatgcactggatacgacagccccctggagaagggcttgagtggatcggagctattgatggtccaactcctgatactgcctacagtgagaagttcaagggcagagtcacgctgaccgcggacaaatccacgagcacagcctacatggagctgagcagcctgacatctgaggacacggccgtgtattactgtacaagattctactcctatacttactggggccagggaaccctggtcaccgtctcctcagcttccaccaagggcccatcggtcttccccctggcaccctcctccaagtccacctctgggggcacagcggccctgggctgcctggtcaaggactacttccccgaaccggtgacggtgtcgtggaactcaggcgccctgacctccggcgtgcacaccttcccggctgtcctacagtcctcaggactctactccctctcctccgtggtgaccgtgccctcctcgtccttgggcacccagacctacatctgcaacgtgaatcacaagccctccaacaccaaggtggacaagagagttgagcccaaatcttgtgacaaaactcacacatgcccaccgtgcccagcacctgaactcctggggggaccgtcagtcttcctcttccccccaaaacccaaggacaccctcatgatctcccggacccctgaggtcacatgcgtggtggtggacgtgtcccacgaagaccctgaggtcaagttcaactggtacgtggacggcgtggaggtgcataatgccaagacaaagccgcgggaggagcagtacaactccacgtaccgtgtggtctccgtcctcaccgtcctgcaccaggactggctgaatggcaaggagtacaagtgcaaggtctccaacaaagccctcccagcccccatcgagaaaaccatctccaaagccaaagggcagccccgagaaccacaggtgtacaccctgcccccatcccgggaggaaatgaccaagaaccaggtctccctgacctgcctggtcaaaggcttctatccctccgacatcgccgtggagtgggagtccaatgggcagccggagaacaactacaagaccacgcctcccgtgctggactccgacggctccttcttcctctactccaagctcaccgtggacaagtccaggtggcagcaggggaacgtcttctcatgctccgtgatgcatgaggctctgcacaaccactacacgcagaagtcgctctccctgtctccg

SEQ ID NO: 613 - RNA, 1407 nt, Homo sapiens
  source 1..1407: mol_type = mRNA
atggagtttgggctgtcatgggtctttctggtcgctctgctgcggggagtgcagtgtcaggtccagctggtcgaatcaggcggaggcgtggtccagcccggagggtctctgagactgagttgcgccgcttcaggcttcacattttctaacgcctggatgcactgggtgcgacaggctcctggcaaagggctggagtgggtcgcacagatcaaggacaaatcccagaattacgctacttacgttgcagaatccgtgaaggggaggttcaccatttcccgcgccgattccaaaaactccatctacctgcagatgaatagtctgaagaccgaggacacagccgtgtactattgtagatatgtccattacgcagccggctacggagtggacatctggggacagggaactacagtcacagtctcatccgcttccaccaagggcccatcggtcttccccctggcaccctcctccaagtccacctctgggggcacagcggccctgggctgcctggtcaaggactacttccccgaaccggtgacggtgtcgtggaactcaggcgccctgacctccggcgtgcacaccttcccggctgtcctacagtcctcaggactctactccctctcctccgtggtgaccgtgccctcctcgtccttgggcacccagacctacatctgcaacgtgaatcacaagccctccaacaccaaggtggacaagagagttgagcccaaatcttgtgacaaaactcacacatgcccaccgtgcccagcacctgaactcctggggggaccgtcagtcttcctcttccccccaaaacccaaggacaccctcatgatctcccggacccctgaggtcacatgcgtggtggtggacgtgtcccacgaagaccctgaggtcaagttcaactggtacgtggacggcgtggaggtgcataatgccaagacaaagccgcgggaggagcagtacaactccacgtaccgtgtggtctccgtcctcaccgtcctgcaccaggactggctgaatggcaaggagtacaagtgcaaggtctccaacaaagccctcccagcccccatcgagaaaaccatctccaaagccaaagggcagccccgagaaccaagagtgtacaccctgcccccatcccgggaggaaatgaccgagaaccaggtctccctgacctgcctggtcaaaggcttctatccctccgacatcgccgtggagtgggagtccaatgggcagccggagaacaactacaagaccacgcctcccgtgctggtgtccgacggctccttcaccctctactcctggctcaccgtggacaagtccaggtggcagcaggggaacgtcttctcatgctccgtgatgcatgaggctctgcacaaccactacacgcagaagtcgctctccctgtctccg

SEQ ID NO: 614 - RNA, 1386 nt, Homo sapiens
  source 1..1386: mol_type = mRNA
atgggctggtcctgcatcatcctgtttctggtggccaccgctaccggcgtccatagccaggtgcagctggtgcagtctggagctgaggtgaagaagcctggggcctcagtgaccgtctcctgcaaggcttctggatacaccttcaccgactatgaaatgcactggatacgacagccccctggagaagggcttgagtggatcggagctattgatggtccaactcctgatactgcctacagtgagaagttcaagggcagagtcacgctgaccgcggacaaatccacgagcacagcctacatggagctgagcagcctgacatctgaggacacggccgtgtattactgtacaagattctactcctatacttactggggccagggaaccctggtcaccgtctcctcagcttccaccaagggcccatcggtcttccccctggcaccctcctccaagtccacctctgggggcacagcggccctgggctgcctggtcaaggactacttccccgaaccggtgacggtgtcgtggaactcaggcgccctgacctccggcgtgcacaccttcccggctgtcctacagtcctcaggactctactccctctcctccgtggtgaccgtgccctcctcgtccttgggcacccagacctacatctgcaacgtgaatcacaagccctccaacaccaaggtggacaagagagttgagcccaaatcttgtgacaaaactcacacatgcccaccgtgcccagcacctgaactcctggggggaccgtcagtcttcctcttccccccaaaacccaaggacaccctcatgatctcccggacccctgaggtcacatgcgtggtggtggacgtgtcccacgaagaccctgaggtcaagttcaactggtacgtggacggcgtggaggtgcataatgccaagacaaagccgcgggaggagcagtacaactccacgtaccgtgtggtctccgtcctcaccgtcctgcaccaggactggctgaatggcaaggagtacaagtgcaaggtctccaacaaagccctcccagcccccatcgagaaaaccatctccaaagccaaagggcagccccgagaaccacaggtgtacaccctgcccccatcccggaaagaaatgaccaagaaccaggtctccctgacctgcctggtcaaaggcttctatccctccgacatcgccgtggagtgggagtccaatgggcagccggagaacaactacgacaccacgcctcccgtcctgaagtccgacggctccttcttcctctactccaagctcaccgtggacaagtccaggtggcagcaggggaacgtcttctcatgctccgtgatgcatgaggctctgcacaaccactacacgcaggagtcgctctccctgtctccg

SEQ ID NO: 615 - RNA, 1401 nt, Homo sapiens
  source 1..1401: mol_type = mRNA
atggagtttgggctgagctgggttttcctcgttgctcttttaagaggtgtccagtgtcaggtgcagctggtggagtctgggggaggcttggtccagcctggggggtccctgagactctcctgtgcagcctctggattcaccttcagttactatgacatccagtgggtccgccaggctccaggcaaggggctggagtgggtgtcatccattagtcctagtggtcagtccacttactatcgacgcgaggtaaagggccgattcaccatctccagggacaactccaagaacacactgtatctgcaaatgaactccctgagagccgaggacacggccgtgtattactgtgcgagacggaccgggcgggagtacggaggtggctggtactttgactactggggccaaggaaccctggtcaccgtgtcctcagctagcaccaagggcccatccgtcttccccctggcgccctgctccaggagcacctccgagagcacagccgccctgggctgcctggtcaaggactacttccccgaaccggtgacggtgtcgtggaactcaggcgccctgaccagcggcgtgcacaccttcccggctgtcctacagtcctcaggactctactccctcagcagcgtggtgaccgtgccctccagcagcttgggcacgaagacctacacctgcaacgtagatcacaagcccagcaacaccaaggtggacaagagagttgagtccaaatatggtcccccatgcccaccatgcccagcacctgagttcctggggggaccatcagtcttcctgttccccccaaaacccaaggacactctcatgatctcccggacccctgaggtcacgtgcgtggtggtggacgtgagccaggaagaccccgaggtccagttcaactggtacgtggatggcgtggaggtgcataatgccaagacaaagccgcgggaggagcagttcaacagcacgtaccgtgtggtcagcgtcctcaccgtcctgcaccaggactggctgaacggcaaggagtacaagtgcaaggtctccaacaaaggcctcccgtcctccatcgagaaaaccatctccaaagccaaagggcagccccgagagccacaggtgtacaccctgcccccatcccaggaggagatgaccaagaaccaggtcagcctgacctgcctggtcaaaggcttctaccccagcgacatcgccgtggagtgggagagcaatgggcagccggagaacaactacaagaccacgcctcccgtgctggactccgacggctccttcttcctctacagcaggctaaccgtggacaagagcaggtggcaggaggggaatgtcttctcatgctccgtgatgcatgaggctctgcacaaccactacacacagaagagcctctccctgtctctg

SEQ ID NO: 616 - RNA, 1389 nt, Homo sapiens
  source 1..1389: mol_type = mRNA
atggactggacctggaggatactcttcttggtggcagcagcgacaggtgcccactcccaggtgcagctggtgcagtctgggtctgagttgaagaagcctggggcctcggtgaaggtctcctgcaaggcttctggatacaccttcaccgacaacaacatggactgggtgcgacaggcccctggacaagggcttgagtggatgggagatattaatactagaagtggtggttctatctacaacgaggagtttcaggacagagtcatcatgaccgtggacaagtccacggacacagcctacatggaattgtcctccctgagatctgaggacacggccacttatcactgcgcgagaaggaagtcctacggctactaccttgacgagtggggcgagggaaccctggtcaccgtctcctcagctagcaccaagggcccatccgtcttccccctggcgccctgctccaggagcacctccgagagcacagccgccctgggctgcctggtcaaggactacttccccgaaccggtgacggtgtcgtggaactcaggcgccctgaccagcggcgtgcacaccttcccggctgtcctacagtcctcaggactctactccctcagcagcgtggtgaccgtgccctccagcagcttgggcacgaagacctacacctgcaacgtagatcacaagcccagcaacaccaaggtggacaagagagttgagtccaaatatggtcccccatgcccaccatgcccagcacctgagttcctggggggaccatcagtcttcctgttccccccaaaacccaaggacactctcatgatctcccggacccctgaggtcacgtgcgtggtggtggacgtgagccaggaagaccccgaggtccagttcaactggtacgtggatggcgtggaggtgcataatgccaagacaaagccgcgggaggagcagttcaacagcacgtaccgtgtggtcagcgtcctcaccgtcctgcaccaggactggctgaacggcaaggagtacaagtgcaaggtctccaacaaaggcctcccgtcctccatcgagaaaaccatctccaaagccaaagggcagccccgagagccacaggtgtacaccctgcccccatcccaggaggagatgaccaagaaccaggtcagcctgacctgcctggtcaaaggcttctaccccagcgacatcgccgtggagtgggagagcaatgggcagccggagaacaactacaagaccacgcctcccgtgctggactccgacggctccttcttcctctacagcaggctaaccgtggacaagagcaggtggcaggaggggaatgtcttctcatgctccgtgatgcatgaggctctgcacaaccactacacacagaagagcctctccctgtctctg

SEQ ID NO: 617 - RNA, 1401 nt, Homo sapiens
  source 1..1401: mol_type = mRNA
atggagtttgggctgagctgggttttcctcgttgctcttttaagaggtgtccagtgtcaggtgcagctggtggagtctgggggaggcttggtccagcctggggggtccctgagactctcctgtgcagcctctggattcaccttcagttactatgacatccagtgggtccgccaggctccaggcaaggggctggagtgggtgtcatccattagtcctagtggtcagtccacttactatcgacgcgaggtaaagggccgattcaccatctccagggacaactccaagaacacactgtatctgcaaatgaactccctgagagccgaggacacggccgtgtattactgtgcgagacggaccgggcgggagtacggaggtggctggtactttgactactggggccaaggaaccctggtcaccgtgtcctcagctagcaccaagggcccatccgtcttccccctggcgccctgctccaggagcacctccgagagcacagccgccctgggctgcctggtcaaggactacttccccgaaccggtgacggtgtcgtggaactcaggcgccctgaccagcggcgtgcacaccttcccggctgtcctacagtcctcaggactctactccctcagcagcgtggtgaccgtgccctccagcagcttgggcacgaagacctacacctgcaacgtagatcacaagcccagcaacaccaaggtggacaagagagttgagtccaaatatggtcccccatgcccaccatgcccagcacctgagttcctggggggaccatcagtcttcctgttccccccaaaacccaaggacactctcatgatctcccggacccctgaggtcacgtgcgtggtggtggacgtgagccaggaagaccccgaggtccagttcaactggtacgtggatggcgtggaggtgcataatgccaagacaaagccgcgggaggagcagttcaacagcacgtaccgtgtggtcagcgtcctcaccgtcctgcaccaggactggctgaacggcaaggagtacaagtgcaaggtctccaacaaaggcctcccgtcctccatcgagaaaaccatctccaaagccaaagggcagccccgagagccacaggtgtacaccctgcccccatcccaggaggagatgaccaagaaccaggtcagcctgacctgcctggtcaaaggcttctaccccagcgacatcgccgtggagtgggagagcaatgggcagccggagaacaactacaagacctggcctcccgtgctggactccgacggctccttcgccctctacagcaggctaaccgtggacaagagcaggtggcaggaggggaatgtcttctcatgctccgtgatgcatgaggctctgcacaaccactacacacagaagagcctctccctgtctctg

SEQ ID NO: 618 - RNA, 1389 nt, Homo sapiens
  source 1..1389: mol_type = mRNA
atggactggacctggaggatactcttcttggtggcagcagcgacaggtgcccactcccaggtgcagctggtgcagtctgggtctgagttgaagaagcctggggcctcggtgaaggtctcctgcaaggcttctggatacaccttcaccgacaacaacatggactgggtgcgacaggcccctggacaagggcttgagtggatgggagatattaatactagaagtggtggttctatctacaacgaggagtttcaggacagagtcatcatgaccgtggacaagtccacggacacagcctacatggaattgtcctccctgagatctgaggacacggccacttatcactgcgcgagaaggaagtcctacggctactaccttgacgagtggggcgagggaaccctggtcaccgtctcctcagctagcaccaagggcccatccgtcttccccctggcgccctgctccaggagcacctccgagagcacagccgccctgggctgcctggtcaaggactacttccccgaaccggtgacggtgtcgtggaactcaggcgccctgaccagcggcgtgcacaccttcccggctgtcctacagtcctcaggactctactccctcagcagcgtggtgaccgtgccctccagcagcttgggcacgaagacctacacctgcaacgtagatcacaagcccagcaacaccaaggtggacaagagagttgagtccaaatatggtcccccatgcccaccatgcccagcacctgagttcctggggggaccatcagtcttcctgttccccccaaaacccaaggacactctcatgatctcccggacccctgaggtcacgtgcgtggtggtggacgtgagccaggaagaccccgaggtccagttcaactggtacgtggatggcgtggaggtgcataatgccaagacaaagccgcgggaggagcagttcaacagcacgtaccgtgtggtcagcgtcctcaccgtcctgcaccaggactggctgaacggcaaggagtacaagtgcaaggtctccaacaaaggcctcccgtcctccatcgagaaaaccatctccaaagccaaagggcagccccgagagccacaggtgtacaccctgcccccatcccaggaggagatgaccaagaaccaggtcagcctgtggtgcgcagtcaaaggcttctaccccagcgacatcgccgtggagtgggagagcaatgggcagccggagaacaactacaagaccacgcctcccgtgctggactccgacggctccttcttcctcgtcagcaggctaaccgtggacaagagcaggtggcaggaggggaatgtcttctcatgctccgtgatgcatgaggctctgcacaaccactacacacagaagagcctctccctgtctctg

SEQ ID NO: 619 - RNA, 714 nt, Homo sapiens
  source 1..714: mol_type = mRNA
atgggctggtcctgcatcatcctgtttctggtggccaccgctaccggcgtccatagcgatattgtgatgactcagtctccactctccctgcccgtcacccctggagagccggcctccatctcctgcagatctagtcagccccttgtacacagtaataggaacacctatttacattggtaccagcagaagccagggcaggctccaaggctcctgatctataaagtttccaaccgattttctggggtccctgacaggttcagtggcagtggatcaggcacagattttacactgaaaatcagcagagtggaggctgaggatgttggggtttattactgcggccaaggtacacaggttccttacacgtttggccaggggaccaagctggagatcaaacgtacggtggctgcaccatctgtcttcatcttcccgccatctgatgagcagttgaaatctggaactgcctctgttgtgtgcctgctgaataacttctatcccagagaggccaaagtacagtggaaggtggataacgccctccaatcgggtaactcccaggagagtgtcacagagcaggactccaaggactccacctactccctctcctccaccctgacgctgtccaaagcagactacgagaaacacaaagtctacgcctgcgaagtcacccatcagggcctgtcctcgcccgtcacaaagtccttcaacaggggagagtgt

SEQ ID NO: 620 - RNA, 708 nt, Homo sapiens
  source 1..708: mol_type = mRNA
atggacatgagggtccccgctcagctcctggggctcctgctactctggctccgaggtgccagatgtgacatccagatgacccagtctccatcctcactgtctgcatctgtaggagacagagtcaccatcacttgtaaagcaagtcggaatattgagagacagttagcctggtatcagcagaaacctggccaggctcccgaactcctcatttatcaggcatccagaaaggaatccggcgtcccagacaggttcagtggcagtcggtatgggacagacttcactctcaccatctctagtctgcaacctgaagatatcgcaacttactactgtcagcaatattctgaccctcctctcacgttcggcggagggaccaaggtggagatcaaacgtacggtggctgcaccatctgtcttcatcttcccgccatctgatgagcagttgaaatctggaactgcctctgttgtgtgcctgctgaataacttctatcccagagaggccaaagtacagtggaaggtggataacgccctccaatcgggtaactcccaggagagtgtcacagagcaggactccaaggactccacctactccctctcctccaccctgacgctgtccaaagcagactacgagaaacacaaagtctacgcctgcgaagtcacccatcagggcctgtcctcgcccgtcacaaagtccttcaacaggggagagtgt